European Patent Application EP 4 268 895 A2, published November 1, 2023. Title: USES OF CYP4V2 AND RDCVF IN PREPARATION OF DRUGS. Applicant: Chigenovo Co. Ltd. Application CN 201911255192. The sequence listing filed with the application follows.

SEQUENCE LISTING (155 sequences)

SEQ ID NO: 1 - DNA, 345 bp, synthetic construct
  misc_feature 1..345: note = OPEFS promoter
  source 1..345: mol_type = other DNA
gggcagagcgcacatcgcccacagtccccgagaagttggggggaggggtcggcaattgaaccggtgcctagagaaggtggcgcggggtaaactgggaaagtgatgtcgtgtactggctccgcctttttcccgagggtgggggagaaccgtatataagtgcagtagtcgccgtgaacgttctttttcgcaacgggtttgccgccagaacacaggtaagtatcaaggttacaagacaggtttaaggagaccaatagaaactgggcttgtcgagacagagaagactcttgcgtttctgataggcacctattggtcttactgacatccactttgcctttctctccacag

SEQ ID NO: 2 - DNA, 212 bp, synthetic construct
  misc_feature 1..212: note = EFS promoter
  source 1..212: mol_type = other DNA
gggcagagcgcacatcgcccacagtccccgagaagttggggggaggggtcggcaattgaaccggtgcctagagaaggtggcgcggggtaaactgggaaagtgatgtcgtgtactggctccgcctttttcccgagggtgggggagaaccgtatataagtgcagtagtcgccgtgaacgttctttttcgcaacgggtttgccgccagaacacag

SEQ ID NO: 3 - DNA, 1162 bp, synthetic construct
  misc_feature 1..1162: note = EF1a promoter
  source 1..1162: mol_type = other DNA
gctccggtgcccgtcagtgggcagagcgcacatcgcccacagtccccgagaagttggggggaggggtcggcaattgaaccggtgcctagagaaggtggcgcggggtaaactgggaaagtgatgtcgtgtactggctccgcctttttcccgagggtgggggagaaccgtatataagtgcagtagtcgccgtgaacgttctttttcgcaacgggtttgccgccagaacacaggtaagtgccgtgtgtggttcccgcgggcctggcctctttacgggttatggcccttgcgtgccttgaattacttccacctggctccagtacgtgattcttgatcccgagctggagccaggggcgggccttgcgctttaggagccccttcgcctcgtgcttgagttgaggcctggcctgggcgctggggccgccgcgtgcgaatctggtggcaccttcgcgcctgtctcgctgctttcgataagtctctagccatttaaaatttttgatgacctgctgcgacgctttttttctggcaagatagtcttgtaaatgcgggccaggatctgcacactggtatttcggtttttggggccgcgggcggcgacggggcccgtgcgtcccagcgcacatgttcggcgaggcggggcctgcgagcgcggccaccgagaatcggacgggggtagtctcaagctggccggcctgctctggtgcctggcctcgcgccgccgtgtatcgccccgccctgggcggcaaggctggcccggtcggcaccagttgcgtgagcggaaagatggccgcttcccggccctgctccagggggctcaaaatggaggacgcggcgctcgggagagcgggcgggtgagtcacccacacaaaggaaaggggcctttccgtcctcagccgtcgcttcatgtgactccacggagtaccgggcgccgtccaggcacctcgattagttctggagcttttggagtacgtcgtctttaggttggggggaggggttttatgcgatggagtttccccacactgagtgggtggagactgaagttaggccagcttggcacttgatgtaattctccttggaatttgccctttttgagtttggatcttggttcattctcaagcctcagacagtggttcaaagtttttttcttccatttcaggtgtcgtga

SEQ ID NO: 4 - DNA, 937 bp, synthetic construct
  misc_feature 1..937: note = CAG promoter
  source 1..937: mol_type = other DNA
ccattgacgtcaataatgacgtatgttcccatagtaacgccaatagggactttccattgacgtcaatgggtggagtatttacggtaaactgcccacttggcagtacatcaagtgtatcatatgccaagtacgccccctattgacgtcaatgacggtaaatggcccgcctggcattatgcccagtacatgaccttatgggactttcctacttggcagtacatctacgtattagtcatcgctattaccatggtcgaggtgagccccacgttctgcttcactctccccatctcccccccctccccacccccaattttgtatttatttattttttaattattttgtgcagcgatgggggcggggggggggggggggcgcgcgccaggcggggcggggcggggcgaggggcggggcggggcgaggcggagaggtgcggcggcagccaatcagagcggcgcgctccgaaagtttccttttatggcgaggcggcggcggcggcggccctataaaaagcgaagcgcgcggcgggcgggagtcgctgcgacgctgccttcgccccgtgccccgctccgccgccgcctcgcgccgcccgccccggctctgactgaccgcgttactcccacaggtgagcgggcgggacggcccttctcctccgggctgtaattagcgcttggtttaatgacggcttgtttcttttctgtggctgcgtgaaagccttgaggggctccgggagggccctttgtgcggggggagcggctcggggctgtccgcggggggacggctgccttcgggggggacggggcagggcggggttcggcttctggcgtgtgaccggcggctctagagcctctgctaaccatgttcatgccttcttctttttcctacagctcctgggcaacgtgctggttattgtgctgtctcatcattttggcaaagaatt

SEQ ID NO: 5 - DNA, 1614 bp, synthetic construct
  misc_feature 1..1614: note = RPE65 promoter
  source 1..1614: mol_type = other DNA
tattgtgcaaataagtgctcactccaaattagtggtatatttattgaagtttaatattgtgtttgtgatacagaagtatttgctttaattctaaataaaaattttatgcttttattgctggtttaagaagatttggattatccttgtactttgaggagaagtttcttatttgaaatattttggaaacaggtcttttaatgtggaaagatagatattaatctcctcttctattactctccaagatccaacaaaagtgattataccccccaaaatatgatggtagtatcttatactaccatcattttataggcatagggctcttagctgcaaataatggaactaactctaataaagcagaacgcaaatattgtaaatattagagagctaacaatctctgggatggctaaaggatggagcttggaggctacccagccagtaacaatattccgggctccactgttgaatggagacactacaactgccttggatgggcagagatattatggatgctaagccccaggtgctaccattaggacttctaccactgtccctaacgggtggagcccatcacatgcctatgccctcactgtaaggaaatgaagctactgttgtatatcttgggaagcacttggattaattgttatacagttttgttgaagaagacccctagggtaagtagccataactgcacactaaatttaaaattgttaatgagtttctcaaaaaaaatgttaaggttgttagctggtatagtatatatcttgcctgttttccaaggacttctttgggcagtaccttgtctgtgctggcaagcaactgagacttaatgaaagagtattggagatatgaatgaattgatgctgtatactctcagagtgccaaacatataccaatggacaagaaggtgaggcagagagcagacaggcattagtgacaagcaaagatatgcagaatttcattctcagcaaatcaaaagtcctcaacctggttggaagaatattggcactgaatggtatcaataaggttgctagagagggttagaggtgcacaatgtgcttccataacattttatacttctccaatcttagcactaatcaaacatggttgaatactttgtttactataactcttacagagttataagatctgtgaagacagggacagggacaatacccatctctgtctggttcataggtggtatgtaatagatatttttaaaaataagtgagttaatgaatgagggtgagaatgaaggcacagaggtattagggggaggtgggccccagagaatggtgccaaggtccagtggggtgactgggatcagctcaggcctgacgctggccactcccacctagctcctttctttctaatctgttctcattctccttgggaaggattgaggtctctggaaaacagccaaacaactgttatgggaacagcaagcccaaataaagccaagcatcagggggatctgagagctgaaagcaacttctgttccccctccctcagctgaaggggtggggaagggctcccaaagccataactccttttaagggatttagaaggcataaaaaggcccctggctgagaacttccttcttcattctgcagttgg

SEQ ID NO: 6 - DNA, 2000 bp, synthetic construct
  misc_feature 1..2000: note = CYP4V2-Pf promoter
  source 1..2000: mol_type = other DNA
acccacctcatcctgcacctgtcactgcgtgggaccctgtgctccaggcaggggcacctcactgccccctgagctcattttacccctcctggctctgcagcatttctgaccatttctgcccaggccgagactcactgctgcccagagcaatctcccttctctccttctggaggggaggggttgtatgttacccgcctggttttatccacagaggttagcagagactgatacagacaaaccctttttctttctaattttagattcaagagcacatgtgcaggtttgttaaatttgcctgacgctgaggtttgagtttctattgatcccctcacctgaatagggaacacagtacccaatacacagtttttcaaccattactccccttccttcctccccctattttagaatccccagtatgtagacaaattgtttacttttatagctgtaattaaccttattatagctcagcctcaaccctttagagaggaggaaactaaagcccatgagacttgcttaaagatactaagtgaacatatttattttttaaagtgttaaagtgattaaacaatgtagacgtgaatgaaataaaaagcgtaagttccccatcttcattcccactccatagagctgatcagtatttttacttgcagacattagtggagccgtagagaaagaaaccttttctccaaaagaaggcattactttacacactccgttctgcaacttgttttgttcacttgctatttcacgtcagcccatgcagatgacttaaaacaaattcaaatggagaaaagccttaggcatgtttttctctgcactaaagaggccctgcaggtggctgtggccaacttatgcagtggcttcgagtgaacgaacgtaattagtaattaagcaaagcgggcatccaggacattcagtttcatcttcctggcactttagtgtttaggaagggcctggcctctcggggagcgacactcctcgcccggccactttgtaagaagcatcgagcgtggaaaaggggctggggtcagcactggggccctctgccgggaagagagactggcggccagcacacgcgtctccccaggctgaaatggggcaccctctcgcggcccttccctcccttcccgggctgggtggcaggtcttggctcttctgcgagtaccccgcggctgcggtctcccggcacccgctgagcagcctcgcccgccttcctctcccacccgcccctgcgtgctctccggggctccggcttcctcggtctggtgcctggtgcgtattttggaaaatacctggctcataaccacctcattgagctcccagtgtcccagtgggccagcggacacacacgggtagctgacttccctaacgtgtccccaaagcctccctggattacagcgcccgctgctccatgtgaccccgcgggagccaggacgcgccccgcctcccggggctgcaagttgcgcagggagcgagcgatgcgcagcagagctgggctccgagccggatgcgccttcctttcctctccagagcaggctgcccgcccgcggaatcccgcacgtagagcaacctcgcagcaccctcagaacagccccgctggggcgcgccgggctgccgcggtgacctttccgacgcccctgaccccgcatccggaggcggccggaagtgtcgccggcctcctcccggcgcagcctccgggcctccagtgcaatcactacgccctggggcccggaaaccgttttccggtctttcgctttcggctggggcgtggaggccgcggtgctgcgtaggccgggccgggcgcaggaacagccccgtggcgccctctctggccgccgcccgggcgggaaacgtcgttccggggaccgggcgaccccgcagcggggagcgcgccaggtccgcgcggggaagtgggcggtgtgcggccggcaccgcctcgcaccacgcccccgcgggcccgcactttcccggagtgcaccccgcggccgccagccggggcg

SEQ ID NO: 7 - DNA, 1700 bp, synthetic construct
  misc_feature 1..1700: note = CYP4V2-P1 promoter
  source 1..1700: mol_type = other DNA
gctgaggtttgagtttctattgatcccctcacctgaatagggaacacagtacccaatacacagtttttcaaccattactccccttccttcctccccctattttagaatccccagtatgtagacaaattgtttacttttatagctgtaattaaccttattatagctcagcctcaaccctttagagaggaggaaactaaagcccatgagacttgcttaaagatactaagtgaacatatttattttttaaagtgttaaagtgattaaacaatgtagacgtgaatgaaataaaaagcgtaagttccccatcttcattcccactccatagagctgatcagtatttttacttgcagacattagtggagccgtagagaaagaaaccttttctccaaaagaaggcattactttacacactccgttctgcaacttgttttgttcacttgctatttcacgtcagcccatgcagatgacttaaaacaaattcaaatggagaaaagccttaggcatgtttttctctgcactaaagaggccctgcaggtggctgtggccaacttatgcagtggcttcgagtgaacgaacgtaattagtaattaagcaaagcgggcatccaggacattcagtttcatcttcctggcactttagtgtttaggaagggcctggcctctcggggagcgacactcctcgcccggccactttgtaagaagcatcgagcgtggaaaaggggctggggtcagcactggggccctctgccgggaagagagactggcggccagcacacgcgtctccccaggctgaaatggggcaccctctcgcggcccttccctcccttcccgggctgggtggcaggtcttggctcttctgcgagtaccccgcggctgcggtctcccggcacccgctgagcagcctcgcccgccttcctctcccacccgcccctgcgtgctctccggggctccggcttcctcggtctggtgcctggtgcgtattttggaaaatacctggctcataaccacctcattgagctcccagtgtcccagtgggccagcggacacacacgggtagctgacttccctaacgtgtccccaaagcctccctggattacagcgcccgctgctccatgtgaccccgcgggagccaggacgcgccccgcctcccggggctgcaagttgcgcagggagcgagcgatgcgcagcagagctgggctccgagccggatgcgccttcctttcctctccagagcaggctgcccgcccgcggaatcccgcacgtagagcaacctcgcagcaccctcagaacagccccgctggggcgcgccgggctgccgcggtgacctttccgacgcccctgaccccgcatccggaggcggccggaagtgtcgccggcctcctcccggcgcagcctccgggcctccagtgcaatcactacgccctggggcccggaaaccgttttccggtctttcgctttcggctggggcgtggaggccgcggtgctgcgtaggccgggccgggcgcaggaacagccccgtggcgccctctctggccgccgcccgggcgggaaacgtcgttccggggaccgggcgaccccgcagcggggagcgcgccaggtccgcgcggggaagtgggcggtgtgcggccggcaccgcctcgcaccacgcccccgcgggcccgcactttcccggagtgcaccccgcggccgccagccggggcg

SEQ ID NO: 8 - DNA, 1400 bp, synthetic construct
  misc_feature 1..1400: note = CYP4V2-P2 promoter
  source 1..1400: mol_type = other DNA
ccccatcttcattcccactccatagagctgatcagtatttttacttgcagacattagtggagccgtagagaaagaaaccttttctccaaaagaaggcattactttacacactccgttctgcaacttgttttgttcacttgctatttcacgtcagcccatgcagatgacttaaaacaaattcaaatggagaaaagccttaggcatgtttttctctgcactaaagaggccctgcaggtggctgtggccaacttatgcagtggcttcgagtgaacgaacgtaattagtaattaagcaaagcgggcatccaggacattcagtttcatcttcctggcactttagtgtttaggaagggcctggcctctcggggagcgacactcctcgcccggccactttgtaagaagcatcgagcgtggaaaaggggctggggtcagcactggggccctctgccgggaagagagactggcggccagcacacgcgtctccccaggctgaaatggggcaccctctcgcggcccttccctcccttcccgggctgggtggcaggtcttggctcttctgcgagtaccccgcggctgcggtctcccggcacccgctgagcagcctcgcccgccttcctctcccacccgcccctgcgtgctctccggggctccggcttcctcggtctggtgcctggtgcgtattttggaaaatacctggctcataaccacctcattgagctcccagtgtcccagtgggccagcggacacacacgggtagctgacttccctaacgtgtccccaaagcctccctggattacagcgcccgctgctccatgtgaccccgcgggagccaggacgcgccccgcctcccggggctgcaagttgcgcagggagcgagcgatgcgcagcagagctgggctccgagccggatgcgccttcctttcctctccagagcaggctgcccgcccgcggaatcccgcacgtagagcaacctcgcagcaccctcagaacagccccgctggggcgcgccgggctgccgcggtgacctttccgacgcccctgaccccgcatccggaggcggccggaagtgtcgccggcctcctcccggcgcagcctccgggcctccagtgcaatcactacgccctggggcccggaaaccgttttccggtctttcgctttcggctggggcgtggaggccgcggtgctgcgtaggccgggccgggcgcaggaacagccccgtggcgccctctctggccgccgcccgggcgggaaacgtcgttccggggaccgggcgaccccgcagcggggagcgcgccaggtccgcgcggggaagtgggcggtgtgcggccggcaccgcctcgcaccacgcccccgcgggcccgcactttcccggagtgcaccccgcggccgccagccggggcg

SEQ ID NO: 9 - DNA, 1100 bp, synthetic construct
  misc_feature 1..1100: note = CYP4V2-P3 promoter
  source 1..1100: mol_type = other DNA
gcatccaggacattcagtttcatcttcctggcactttagtgtttaggaagggcctggcctctcggggagcgacactcctcgcccggccactttgtaagaagcatcgagcgtggaaaaggggctggggtcagcactggggccctctgccgggaagagagactggcggccagcacacgcgtctccccaggctgaaatggggcaccctctcgcggcccttccctcccttcccgggctgggtggcaggtcttggctcttctgcgagtaccccgcggctgcggtctcccggcacccgctgagcagcctcgcccgccttcctctcccacccgcccctgcgtgctctccggggctccggcttcctcggtctggtgcctggtgcgtattttggaaaatacctggctcataaccacctcattgagctcccagtgtcccagtgggccagcggacacacacgggtagctgacttccctaacgtgtccccaaagcctccctggattacagcgcccgctgctccatgtgaccccgcgggagccaggacgcgccccgcctcccggggctgcaagttgcgcagggagcgagcgatgcgcagcagagctgggctccgagccggatgcgccttcctttcctctccagagcaggctgcccgcccgcggaatcccgcacgtagagcaacctcgcagcaccctcagaacagccccgctggggcgcgccgggctgccgcggtgacctttccgacgcccctgaccccgcatccggaggcggccggaagtgtcgccggcctcctcccggcgcagcctccgggcctccagtgcaatcactacgccctggggcccggaaaccgttttccggtctttcgctttcggctggggcgtggaggccgcggtgctgcgtaggccgggccgggcgcaggaacagccccgtggcgccctctctggccgccgcccgggcgggaaacgtcgttccggggaccgggcgaccccgcagcggggagcgcgccaggtccgcgcggggaagtgggcggtgtgcggccggcaccgcctcgcaccacgcccccgcgggcccgcactttcccggagtgcaccccgcggccgccagccggggcg

SEQ ID NO: 10 - DNA, 800 bp, synthetic construct
  misc_feature 1..800: note = CYP4V2-P4 promoter
  source 1..800: mol_type = other DNA
cctcgcccgccttcctctcccacccgcccctgcgtgctctccggggctccggcttcctcggtctggtgcctggtgcgtattttggaaaatacctggctcataaccacctcattgagctcccagtgtcccagtgggccagcggacacacacgggtagctgacttccctaacgtgtccccaaagcctccctggattacagcgcccgctgctccatgtgaccccgcgggagccaggacgcgccccgcctcccggggctgcaagttgcgcagggagcgagcgatgcgcagcagagctgggctccgagccggatgcgccttcctttcctctccagagcaggctgcccgcccgcggaatcccgcacgtagagcaacctcgcagcaccctcagaacagccccgctggggcgcgccgggctgccgcggtgacctttccgacgcccctgaccccgcatccggaggcggccggaagtgtcgccggcctcctcccggcgcagcctccgggcctccagtgcaatcactacgccctggggcccggaaaccgttttccggtctttcgctttcggctggggcgtggaggccgcggtgctgcgtaggccgggccgggcgcaggaacagccccgtggcgccctctctggccgccgcccgggcgggaaacgtcgttccggggaccgggcgaccccgcagcggggagcgcgccaggtccgcgcggggaagtgggcggtgtgcggccggcaccgcctcgcaccacgcccccgcgggcccgcactttcccggagtgcaccccgcggccgccagccggggcg

SEQ ID NO: 11 - DNA, 500 bp, synthetic construct
  misc_feature 1..500: note = CYP4V2-P5 promoter
  source 1..500: mol_type = other DNA
gagccggatgcgccttcctttcctctccagagcaggctgcccgcccgcggaatcccgcacgtagagcaacctcgcagcaccctcagaacagccccgctggggcgcgccgggctgccgcggtgacctttccgacgcccctgaccccgcatccggaggcggccggaagtgtcgccggcctcctcccggcgcagcctccgggcctccagtgcaatcactacgccctggggcccggaaaccgttttccggtctttcgctttcggctggggcgtggaggccgcggtgctgcgtaggccgggccgggcgcaggaacagccccgtggcgccctctctggccgccgcccgggcgggaaacgtcgttccggggaccgggcgaccccgcagcggggagcgcgccaggtccgcgcggggaagtgggcggtgtgcggccggcaccgcctcgcaccacgcccccgcgggcccgcactttcccggagtgcaccccgcggccgccagccggggcg

SEQ ID NO: 12 - DNA, 200 bp, synthetic construct
  misc_feature 1..200: note = CYP4V2-P6 promoter
  source 1..200: mol_type = other DNA
gcgcaggaacagccccgtggcgccctctctggccgccgcccgggcgggaaacgtcgttccggggaccgggcgaccccgcagcggggagcgcgccaggtccgcgcggggaagtgggcggtgtgcggccggcaccgcctcgcaccacgcccccgcgggcccgcactttcccggagtgcaccccgcggccgccagccggggcg

SEQ ID NO: 13 - DNA, 133 bp, synthetic construct
  misc_feature 1..133: note = human -globin intron
  source 1..133: mol_type = other DNA
gtaagtatcaaggttacaagacaggtttaaggagaccaatagaaactgggcttgtcgagacagagaagactcttgcgtttctgataggcacctattggtcttactgacatccactttgcctttctctccacag

SEQ ID NO: 14 - DNA, 99 bp, synthetic construct
  misc_feature 1..99: note = SV40 intron
  source 1..99: mol_type = other DNA
gtaagtttagtctttttgtcttttatttcaggtcccggatccggtggtggtgcaaatcaaagaactgctcctcagtggatgttgcctttacttctaggc

SEQ ID NO: 15 - DNA, 296 bp, synthetic construct
  misc_feature 1..296: note = artificial intron
  source 1..296: mol_type = other DNA
gaattaattcgctgtctgcgagggccagctgttggggtgagtactccctctcaaaagcgggcatgacttctgcgctaagattgtcagtttccaaaaacgaggaggatttgatattcacctggcccgcggtgatgcctttgagggtggccgcgtccatctggtcagaaaagacaatctttttgttgtcaagcttgaggtgtggcaggcttgagatctggccatacacttgagtgacaatgacatccactttgcctttctctccacaggtgtccactcccaggtccaactgcaggtcg

SEQ ID NO: 16 - DNA, 409 bp, synthetic construct
  misc_feature 1..409: note = hybrid CBA/MVM intron
  source 1..409: mol_type = other DNA
ggagtcgctgcgacgctgccttcgccccgtgccccgctccgccgccgcctcgcgccgcccgccccggctctgactgaccgcgttactcccacaggtgagcgggcgggacggcccttctcctccgggctgtaattagcgcttggtttaatgacggcttgtttcttttctgtggctgcgtgaaagccttgaggggctccgggagggccctttgtgcggggggagcggctcggggctgtccgcggggggacggctgccttcgggggggacggggcagggcggggttcggcttctggcgtgtgaccggcggctctagagcctctgctaaccatgttcatgccttcttctttttcctacagctcctgggcaacgtgctggttattgtgctgtctcatcattttggcaaagaatt

SEQ ID NO: 17 - DNA, 122 bp, synthetic construct
  misc_feature 1..122: note = SV40 signal site
  source 1..122: mol_type = other DNA
aacttgtttattgcagcttataatggttacaaataaagcaatagcatcacaaatttcacaaataaagcatttttttcactgcattctagttgtggtttgtccaaactcatcaatgtatctta

SEQ ID NO: 18 - DNA, 225 bp, synthetic construct
  misc_feature 1..225: note = BGH signal site
  source 1..225: mol_type = other DNA
ctgtgccttctagttgccagccatctgttgtttgcccctcccccgtgccttccttgaccctggaaggtgccactcccactgtcctttcctaataaaatgaggaaattgcatcgcattgtctgagtaggtgtcattctattctggggggtggggtggggcaggacagcaagggggaggattgggaagacaatagcaggcatgctggggatgcggtgggctctatgg

SEQ ID NO: 19 - DNA, 589 bp, synthetic construct
  misc_feature 1..589: note = WPRE signal site
  source 1..589: mol_type = other DNA
aatcaacctctggattacaaaatttgtgaaagattgactggtattcttaactatgttgctccttttacgctatgtggatacgctgctttaatgcctttgtatcatgctattgcttcccgtatggctttcattttctcctccttgtataaatcctggttgctgtctctttatgaggagttgtggcccgttgtcaggcaacgtggcgtggtgtgcactgtgtttgctgacgcaacccccactggttggggcattgccaccacctgtcagctcctttccgggactttcgctttccccctccctattgccacggcggaactcatcgccgcctgccttgcccgctgctggacaggggctcggctgttgggcactgacaattccgtggtgttgtcggggaaatcatcgtcctttccttggctgctcgcctgtgttgccacctggattctgcgcgggacgtccttctgctacgtcccttcggccctcaatccagcggaccttccttcccgcggcctgctgccggctctgcggcctcttccgcgtcttcgccttcgccctcagacgagtcggatctccctttgggccgcctccccgc

SEQ ID NO: 20 - DNA, 717 bp, synthetic construct
  misc_feature 1..717: note = WPRE-SV40 signal site
  source 1..717: mol_type = other DNA
aatcaacctctggattacaaaatttgtgaaagattgactggtattcttaactatgttgctccttttacgctatgtggatacgctgctttaatgcctttgtatcatgctattgcttcccgtatggctttcattttctcctccttgtataaatcctggttgctgtctctttatgaggagttgtggcccgttgtcaggcaacgtggcgtggtgtgcactgtgtttgctgacgcaacccccactggttggggcattgccaccacctgtcagctcctttccgggactttcgctttccccctccctattgccacggcggaactcatcgccgcctgccttgcccgctgctggacaggggctcggctgttgggcactgacaattccgtggtgttgtcggggaaatcatcgtcctttccttggctgctcgcctgtgttgccacctggattctgcgcgggacgtccttctgctacgtcccttcggccctcaatccagcggaccttccttcccgcggcctgctgccggctctgcggcctcttccgcgtcttcgccttcgccctcagacgagtcggatctccctttgggccgcctccccgcggtaacaacttgtttattgcagcttataatggttacaaataaagcaatagcatcacaaatttcacaaataaagcatttttttcactgcattctagttgtggtttgtccaaactcatcaatgtatctta

SEQ ID NO: 21 - DNA, 820 bp, synthetic construct
  misc_feature 1..820: note = WPRE-BGH signal site
  source 1..820: mol_type = other DNA
aatcaacctctggattacaaaatttgtgaaagattgactggtattcttaactatgttgctccttttacgctatgtggatacgctgctttaatgcctttgtatcatgctattgcttcccgtatggctttcattttctcctccttgtataaatcctggttgctgtctctttatgaggagttgtggcccgttgtcaggcaacgtggcgtggtgtgcactgtgtttgctgacgcaacccccactggttggggcattgccaccacctgtcagctcctttccgggactttcgctttccccctccctattgccacggcggaactcatcgccgcctgccttgcccgctgctggacaggggctcggctgttgggcactgacaattccgtggtgttgtcggggaaatcatcgtcctttccttggctgctcgcctgtgttgccacctggattctgcgcgggacgtccttctgctacgtcccttcggccctcaatccagcggaccttccttcccgcggcctgctgccggctctgcggcctcttccgcgtcttcgccttcgccctcagacgagtcggatctccctttgggccgcctccccgcctcgagctgtgccttctagttgccagccatctgttgtttgcccctcccccgtgccttccttgaccctggaaggtgccactcccactgtcctttcctaataaaatgaggaaattgcatcgcattgtctgagtaggtgtcattctattctggggggtggggtggggcaggacagcaagggggaggattgggaagacaatagcaggcatgctggggatgcggtgggctctatgg

SEQ ID NO: 22 - DNA, 66 bp, synthetic construct
  misc_feature 1..66: note = P2A cleaving peptide
  source 1..66: mol_type = other DNA
ggaagcggagctactaacttcagcctgctgaagcaggctggagacgtggaggagaaccctggacct

SEQ ID NO: 23 - DNA, 63 bp, synthetic construct
  misc_feature 1..63: note = T2A cleaving peptide
  source 1..63: mol_type = other DNA
ggaagcggagagggcagaggaagtctgctaacatgcggtgacgtcgaggagaatcctggacct

SEQ ID NO: 24 - DNA, 69 bp, synthetic construct
  misc_feature 1..69: note = E2A cleaving peptide
  source 1..69: mol_type = other DNA
ggaagcggacagtgtactaattatgctctcttgaaattggctggagatgttgagagcaaccctggacct

SEQ ID NO: 25 - DNA, 75 bp, synthetic construct
  misc_feature 1..75: note = F2A cleaving peptide
  source 1..75: mol_type = other DNA
ggaagcggagtgaaacagactttgaattttgaccttctcaagttggcgggagacgtggagtccaaccctggacct

SEQ ID NO: 26 - protein, 22 aa, synthetic construct
  REGION 1..22: note = P2A cleaving peptide
GSGATNFSLLKQAGDVEENPGP

SEQ ID NO: 27 - protein, 22 aa, synthetic construct
  REGION 1..22: note = T2A cleaving peptide
GSGATNFSLLKQAGDVEENPGP

SEQ ID NO: 28 - protein, 23 aa, synthetic construct
  REGION 1..23: note = E2A cleaving peptide
GSGQCTNYALLKLAGDVESNPGP

SEQ ID NO: 29 - protein, 25 aa, synthetic construct
  REGION 1..25: note = F2A cleaving peptide
GSGVKQTLNFDLLKLAGDVESNPGP

SEQ ID NO: 30 - DNA, 46 bp, synthetic construct
  misc_feature 1..46: note = CYP4V2-Pf promoter forward primer
  source 1..46: mol_type = other DNA
cgtctagtactagtcgcgtaggatccggatccacccacctcatcct

SEQ ID NO: 31 - DNA, 46 bp, synthetic construct
  misc_feature 1..46: note = CYP4V2-P1 promoter forward primer
  source 1..46: mol_type = other DNA
cgtctagtactagtcgcgtaggatccgctgaggtttgagtttctat

SEQ ID NO: 32 - DNA, 46 bp, synthetic construct
  misc_feature 1..46: note = CYP4V2-P2 promoter forward primer
  source 1..46: mol_type = other DNA
cgtctagtactagtcgcgtaggatccccccatcttcattcccactc

SEQ ID NO: 33 - DNA, 46 bp, synthetic construct
  misc_feature 1..46: note = CYP4V2-P3 promoter forward primer
  source 1..46: mol_type = other DNA
cgtctagtactagtcgcgtaggatccgcatccaggacattcagttt

SEQ ID NO: 34 - DNA, 46 bp, synthetic construct
  misc_feature 1..46: note = CYP4V2-P4 promoter forward primer
  source 1..46: mol_type = other DNA
cgtctagtactagtcgcgtaggatcccctcgcccgccttcctctcc

SEQ ID NO: 35 - DNA, 46 bp, synthetic construct
  misc_feature 1..46: note = CYP4V2-P5 promoter forward primer
  source 1..46: mol_type = other DNA
cgtctagtactagtcgcgtaggatccgagccggatgcgccttcctt

SEQ ID NO: 36 - DNA, 46 bp, synthetic construct
  misc_feature 1..46: note = CYP4V2-P6 promoter forward primer
  source 1..46: mol_type = other DNA
cgtctagtactagtcgcgtaggatccgcgcaggaacagccccgtgg

SEQ ID NO: 37 - DNA, 46 bp, synthetic construct
  misc_feature 1..46: note = CYP4V2-Pf/P1/P2/P3/P4/P5/P6 promoter reverse primer
  source 1..46: mol_type = other DNA
agagccccgccatggtggcggaattccgccccggctggcggccgcg

SEQ ID NO: 38 - DNA, 18 bp, synthetic construct
  misc_feature 1..18: note = pAV-CAG-CYP4V2-P2A-EGFP vector linearized forward primer
  source 1..18: mol_type = other DNA
gaattccgccaccatggc

SEQ ID NO: 39 - DNA, 20 bp, synthetic construct
  misc_feature 1..20: note = pAV-CAG-CYP4V2-P2A-EGFP vector linearized reverse primer
  source 1..20: mol_type = other DNA
tacgcgactagtactagacg

SEQ ID NO: 40 - DNA, 28 bp, synthetic construct
  misc_feature 1..28: note = EF1a forward primer
  source 1..28: mol_type = other DNA
cgtaggatccgctccggtgcccgtcagt

SEQ ID NO: 41 - DNA, 30 bp, synthetic construct
  misc_feature 1..30: note = EF1a reverse primer
  source 1..30: mol_type = other DNA
cgtagaattctcacgacacctgaaatggaa

SEQ ID NO: 42 - DNA, 31 bp, synthetic construct
  misc_feature 1..31: note = EFS forward primer
  source 1..31: mol_type = other DNA
cgtaggatccgggcagagcgcacatcgccca

SEQ ID NO: 43 - DNA, 30 bp, synthetic construct
  misc_feature 1..30: note = EFS reverse primer
  source 1..30: mol_type = other DNA
cgtagaattcctgtgttctggcggcaaacc

SEQ ID NO: 44 - DNA, 89 bp, synthetic construct
  misc_feature 1..89: note = OPEFS-overlapR1 primer
  source 1..89: mol_type = other DNA
gagtcttctctgtctcgacaagcccagtttctattggtctccttaaacctgtcttgtaaccttgatacttacctgtgttctggcggcaa

SEQ ID NO: 45 - DNA, 89 bp, synthetic construct
  misc_feature 1..89: note = OPEFS-overlapR2 primer
  source 1..89: mol_type = other DNA
cagtgaattcctgtggagagaaaggcaaagtggatgtcagtaagaccaataggtgcctatcagaaacgcaagagtcttctctgtctcga

SEQ ID NO: 46 - DNA, 46 bp, synthetic construct; identical to SEQ ID NO: 35
  misc_feature 1..46: note = CYP4V2-P5F primer
  source 1..46: mol_type = other DNA

SEQ ID NO: 47 - DNA, 31 bp, synthetic construct
  misc_feature 1..31: note = CYP4V2-P5(in) reverse primer
  source 1..31: mol_type = other DNA
ttgatacttaccgccccggctggcggccgcg

SEQ ID NO: 48 - DNA, 35 bp, synthetic construct
  misc_feature 1..35: note = -globin intron (c) forward primer
  source 1..35: mol_type = other DNA
agccggggcggtaagtatcaaggttacaagacagg

SEQ ID NO: 49 - DNA, 50 bp, synthetic construct
  misc_feature 1..50: note = -globin intron reverse primer
  source 1..50: mol_type = other DNA
agccagagccccgccatggtggcggaattcctgtggagagaaaggcaaag

SEQ ID NO: 50 - DNA, 33 bp, synthetic construct
  misc_feature 1..33: note = CYP4V2-Fpr primer sequence
  source 1..33: mol_type = other DNA
cgccagccggggcggaattccgccaccatggcg

SEQ ID NO: 51 - DNA, 34 bp, synthetic construct
  misc_feature 1..34: note = CYP4V2-E1-R primer sequence
  source 1..34: mol_type = other DNA
aaccttgatacttacctcgcccgtccggcttcat

SEQ ID NO: 52 - DNA, 48 bp, synthetic construct
  misc_feature 1..48: note = CYP4V2-E2-F primer sequence
  source 1..48: mol_type = other DNA
cctttctctccacagaattttttcagcagatcattgagtacacagagg

SEQ ID NO: 53 - DNA, 45 bp, synthetic construct
  misc_feature 1..45: note = CYP4V2-R
  source 1..45: mol_type = other DNA
gtagctccgcttccacgcgttttatcgtcgtcatccttataatcg

SEQ ID NO: 54 - DNA, 40 bp, synthetic construct
  misc_feature 1..40: note = Intron-F
  source 1..40: mol_type = other DNA
agccggacgggcgaggtaagtatcaaggttacaagacagg

SEQ ID NO: 55 - DNA, 33 bp, synthetic construct
  misc_feature 1..33: note = Intron-R
  source 1..33: mol_type = other DNA
tctgctgaaaaaattctgtggagagaaaggcaa

SEQ ID NO: 56 - DNA, 20 bp, synthetic construct
  misc_feature 1..20: note = RC5-F
  source 1..20: mol_type = other DNA
ctgtcagaccaagtttactc

SEQ ID NO: 57 - DNA, 20 bp, synthetic construct
  misc_feature 1..20: note = RC5-R
  source 1..20: mol_type = other DNA
cacatttccccgaaaagtgc

SEQ ID NO: 58 - DNA, 40 bp, synthetic construct
  misc_feature 1..40: note = Kana-F
  source 1..40: mol_type = other DNA
gcacttttcggggaaatgtgcgcggaacccctatttgttt

SEQ ID NO: 59 - DNA, 41 bp, synthetic construct
  misc_feature 1..41: note = Kana-R
  source 1..41: mol_type = other DNA
gagtaaacttggtctgacagtcagaagaactcgtcaagaag

SEQ ID NO: 60 - DNA, 20 bp, synthetic construct
  misc_feature 1..20: note = RC5-Kana-F
  source 1..20: mol_type = other DNA
ttgcttgttaatcaataaac

SEQ ID NO: 61 - DNA, 20 bp, synthetic construct
  misc_feature 1..20: note = RC5-Kana-R
  source 1..20: mol_type = other DNA
acctgatttaaatcatttat

SEQ ID NO: 62 - DNA, 1575 bp, synthetic construct
  misc_feature 1..1575: note = CYP4V2 coding sequence
  source 1..1575: mol_type = other DNA
atggcggggctctggctggggctcgtgtggcagaagctgctgctgtggggcgcggcgagtgccctttccctggccggcgccagtctggtcctgagtctgctgcagagggtggcgagctacgcgcggaaatggcagcagatgcggcccatccccacggtggcccgcgcctacccactggtgggccacgcgctgctgatgaagccggacgggcgagaattttttcagcagatcattgagtacacagaggaataccgccacatgccgctgctgaagctctgggtcgggccagtgcccatggtggccctttataatgcagaaaatgtggaggtaattttaactagttcaaagcaaattgacaaatcctctatgtacaagtttttagaaccatggcttggcctaggacttcttacaagtactggaaacaaatggcgctccaggagaaagatgttaacacccactttccattttaccattctggaagatttcttagatatcatgaatgaacaagcaaatatattggttaagaaacttgaaaaacacattaaccaagaagcatttaactgctttttttacatcactctttgtgccttagatatcatctgtgaaacagctatggggaagaatattggtgctcaaagtaatgatgattccgagtatgtccgtgcagtttatagaatgagtgagatgatatttcgaagaataaagatgccctggctttggcttgatctctggtaccttatgtttaaagaaggatgggaacacaaaaagagccttcagatcctacatacttttaccaacagtgtcatcgcggaacgggccaatgaaatgaacgccaatgaagactgtagaggtgatggcaggggctctgccccctccaaaaataaacgcagggcctttcttgacttgcttttaagtgtgactgatgacgaagggaacaggctaagtcatgaagatattcgagaagaagttgacaccttcatgtttgaggggcacgatacaactgcagctgcaataaactggtccttatacctgttgggttctaacccagaagtccagaaaaaagtggatcatgaattggatgacgtgtttgggaagtctgaccgtcccgctacagtagaagacctgaagaaacttcggtatctggaatgtgttattaaggagacccttcgcctttttccttctgttcctttatttgcccgtagtgttagtgaagattgtgaagtggcaggttacagagttctaaaaggcactgaagccgtcatcattccctatgcattgcacagagatccgagatacttccccaaccccgaggagttccagcctgagcggttcttccccgagaatgcacaagggcgccatccatatgcctacgtgcccttctctgctggccccaggaactgtataggtcaaaagtttgctgtgatggaagaaaagaccattctttcgtgcatcctgaggcacttttggatagaatccaaccagaaaagagaagagcttggtctagaaggacagttgattcttcgtccaagtaatggcatctggatcaagttgaagaggagaaatgcagatgaacgc

SEQ ID NO: 63 - DNA, 1578 bp, synthetic construct
  misc_feature 1..1578: note = chimpanzee CYP4V2 coding sequence
  source 1..1578: mol_type = other DNA
atggcggggctctggctggggctcgtgtggcagaagctgctgctgtggggcgcggcgagtgccgtttccctggcgggcgccagtctggtcctgagcctgctgcagagggtagcgacctacgcgcggaaatggcagcagatgcggcccatccccacggtggcccgcgcctacccactggtgggccacgcgctgctgatgaagccggacgggcgagaattttttcagcagatcattgagtacacagaggagtaccgccacatgccgctgctgaagctctgggtcgggccggtgcccatggtggccctttataatgcagaaaatgtggaggtaattttaactagttcaaagcaaattgacaaatcctctatgtacaagtttttagaaccatggcttggcctaggacttcttacaagtactggaaacaaatggcgctccaggagaaagatgttaacacccactttccattttaccattctggaagatttcttagatatcatgaatgaacaagcaaatacattggttaagaaacttgaaaaacacattaaccaagaagcatttaactgctttttttacatcactctttgtgccttagatatcatctgtgaaacagctatggggaagaatattggtgctcaaagtaatgatgattccgagtatgtccgtgcagtttatagaatgagtgagatgatatttcgaagaataaagatgccctggctttggcttgatctctggtaccttatgtttaaagaaggatgggaacacaaaaagagccttaagatcctacatacttttaccaacagtgtcatcgctgaacgggccaatgaaatgaacgccaatgaagactgtagaggtgatggcaggggctctgccccctccaaaaataaacgcagggcctttcttgacttgcttttaagtgtgactgatgacgaagggaacaggctaagtcatgaagatattcgagaagaagttgacaccttcatgtttgaggggcacgacacaactgcagctgcaataaactggtccttatacctgttgggttctaacccagaagtccagaaaaaagtggatcatgaattggatgacgtgtttgggaagtctgaccgtcccgctacggtagaagacctgaagaaacttcggtatttggaatgtgttattaaggagacccttcgcctttttccttctgttcctttatttgcccgtagtgttagtgaagattgtgaagtggcaggttacagagttctaaaaggcactgaagccgtcatcattccctatgcattgcacagagatccgagatacttccccaaccccgaggagttccagcctgagcggttcttccccaagaatgcacaagggcgccatccatatgcctatgtgcccttctctgctggccccaggaactgtataggtcaaaagtttgctgtgatggaggaaaagaccattctttcatgcatcctgaggcacttttggatagaatccaaccagaaaagagaagagcttggtctagaaggacagttgattcttcgtccaagtaatggcatctggatcaagttgaagaggagaaatgcagatgaacgctaa

SEQ ID NO: 64 - DNA, 1578 bp, synthetic construct
  misc_feature 1..1578: note = gorilla CYP4V2 coding sequence
  source 1..1578: mol_type = other DNA
atggcggggctctggctggggctcgtgtggcagaagctgctgctgtggggcgcggcgagtgccgtttccctggccggcgccagtctggtcctgagcctgctgcagagggtggcgagctacgcgcggaaatggcagcagatgcgacccatccccacggtggcccgcgcctacccactggtgggccacgcgctgctgatgaagccggacgggcgagaattttttcagcagatcattgagtacacagaggagtaccgccacatgccgctgctgaagctctgggtcgggccggtgcccatggtggccctttataatgcagaaaatgtggaggtaattttaactagttcaaagcaaattgacaaatcctctatgtacaagtttttagaaccatggcttggcctaggacttcttacaagtactggaaacaaatggcgctccaggagaaagatgttaacacccactttccattttaccattctggaagatttcttagatatcatgaatgaacaagcaaatatattggttaagaaacttgaaaaacacattaaccaagaagcatttaactgctttttttacatcactctttgtgccttagatatcatctgtgaaacagctatggggaagaatattggtgctcaaagtaatgatgattccgagtatgtccgtgcagtttatagaatgagtgagatgatatttcgaagaataaagatgccctggctttggcttgatctctggtaccttatgtttaaagaaggatgggaacacaaaaagagccttaagatcctacatacttttaccaacagtgtcatcgctgaacgggccaatgaaatgaacgccaatgaagactgtagaggtgatggcaggggctctgccccctccaaaaataaacgcagggcctttcttgacttgcttttaagtgtgactgatgacgaagggaacaggctaagtcatgaagatattcgagaagaagttgacaccttcatgtttgaggggcacgacacaactgcagctgcaataaactggtccttatacctgttgggttctaacccagaagtccagaaaaaagtggatcatgaattggatgacgtgtttgggaagtctgaccgtcccgctacggtagaagacctgaagaaacttcggtatctggaatgtgttattaaggagacccttcgcctttttccttctgttcctttatttgcccgtagtgttagtgaagattgtgaagtggcaggttacagagttctaaaaggcactgaagccgtcatcattccctatgcattgcacagagatccaagatacttccccaaccccgaggagttccagcctgagcgtttcttccccgagaatgcacaagggcgccatccgtatgcctacgtgcccttctctgctggccccaggaactgtataggtcaaaagtttgctgtgatggaagaaaagaccattctttcgtgcatcctgagacacttttggatagaatccaaccagaaaagagaagagcttggtctagaaggacagttgattcttcgtccaagtaatggcatctggatcaagttgaagaggagaaatgcagatgaacgctaa

SEQ ID NO: 65 - DNA, 1578 bp, synthetic construct
  misc_feature 1..1578: note = cynomolgus monkey CYP4V2 coding sequence
  source 1..1578: mol_type = other DNA
atggcgggcatctggctggggctcgtgtggcagaagctgctgctgtggggcgcggcgagtgccgtgtccctggccggcgccagtctggtcctgagcctgctgcagagggtggcgagctacgtgaggaaatggcagcagatgcggcccatccccacggtggcccgcgcctacccactggtgggccacgcgctgctgatgaagcgggacgggcgagaattttttcagcagatcattgagtacacagaggaataccgccacatgccactcctgaagctctgggtcgggccggtgcccatggtggccctttataatgcagaaaatgtggaggtaattttaactagttcaaagcaaattgacaaatcctctatgtacaagtttttagaaccatggcttggcctaggacttcttacaagtactggaaacaaatggcgctccaggagaaagatgttaacacccactttccattttaccattctggaagatttcttagatatcatgaatgaacaagcaaatatattggttaagaaacttgaaaaacatgttaaccaagaagcatttaactgctttgtttacatcactctttgtgccttagatatcatctgtgaaacagctatggggaagaatattggtgctcaaagtaacgatgattccgagtatgtccgtgcagtttatagaatgagtgagatgatatttcgaagaataaagatgccgtggctttggcttgacctctggtaccttatgtttaaagagggatgggaacacaaaaagagccttaagatcctacatgcttttaccaacaatgttatcgctgaacgggccaatgaaatgaacgtggatgaagactgtagaggtgatggcagggactccgccccctccaaaaataaacgcagggcctttcttgacttgcttttaagtgtgactgacgacgaagggaacaggctaagtcatgaagatattcgagaagaagttgacaccttcatgtttgagggccacgacacaactgcagctgcaatgaactggtccttatacctgttggggtctaacccagaagtccagaaaaaagtggaccatgaactggatgacgtgtttgggaggtctgaccgtcccgctactgtagaagacctgaagaaacttcggtatctggaatgtgttattaaggagacccttcgcctttttccttctgttcctttatttgcccgcagtgttagtgaagattgtgaagtggcaggttacagagttctgaaaggcactgaagccgtcatcattccctatgcattgcatagagatccaagatacttccccaaccctgaggagttccggcctgagcggttcttccccgagaatgcacaagggcgccatccatatgcctacgtgcccttctctgctggccccaggaactgtataggtcaaaagtttgctgtgatggaagaaaagaccattctttcatgcatcctaaggcacttttggatagaatccaaccagaaaagagaagaacttggtctagaaggacagttgattcttcgtccaactaatggcatctggatcaagttgaagaggagaaatgcagatgaaccctaa

SEQ ID NO: 66 - DNA, 1578 bp, synthetic construct
  misc_feature 1..1578: note = mouse CYP4V3 coding sequence
  source 1..1578: mol_type = other DNA
atgttgtggctgtggttagggctcagtgggcagaaactattgctttggggcgcagcgagcgcggtctccctggccggcgccactatcctgatcagcatctttccgatgctggtaagctacgcgcggaaatggcagcagatgcggtcaatcccgtcggtggcccgcgcctaccccttggtgggacacgcgctttatatgaagcccaacaacgcagaattttttcagcagctaatttattacacagaagaatttcgacacctgccgatcattaaactttggattggacccgtgcccctggtggcactttataaggcagagaatgtggaggtgattttgaccagttctaagcaaattgataaatcgtttttgtacaagttcctacagccatggctgggactaggacttcttacaagtacggggagcaaatggcgcaccaggaggaagatgctaacgcccactttccattttaccattctggagaacttcttggatgtcatgaatgagcaagcaaatatattggttaataagcttgaaaaacacgtcaaccaagaagcctttaattgttttttttacatcactctttgtgctctggatataatctgtgaaacggctatggggaagaacatcggagctcaaagcaataatgattccgagtatgtccgtacagtgtataggatgagtgatatgatatatagaagaatgaagatgccctggctttggtttgacctttggtaccttgtgtttaaagaaggacgggaccacaaaaggggactcaaatgcctacatactttcaccaacaatgtcattgctgaacgagtcaaagaaaggaaggcagaggaagactggacgggtgctggcaggggtcctatcccctccaaaaataagcgcaaggctttccttgacttgcttttgagtgtgactgatgaggaaggaaacagattaagccaggaagacatccgagaggaagttgacaccttcatgtttgagggtcacgatacaactgctgctgcaatcaactggtccttatacctattgggcacgaatccagaagtccagaggaaagtggatcaggagctggatgaagtgtttggaagatcccatcgtcctgtcaccttggaagacctgaagaaacttaaatatttggattgcgtcattaaggagactctccgagttttcccatctgtccctttatttgcccggagtcttagcgaggactgtgaagtgggcggttacaaagtcacaaaaggaacggaagcaatcatcattccctacgcactacaccgagaccccagatacttcccagatccagaggaattccgaccagagcggttctttcctgaaaattcccaaggacgccatccctatgcctatgtgccattttctgctggacctcgaaactgtattggtcaaaagtttgctgtcatggaggagaagaccattcttgcctgtatcctgaggcagttttgggtagaatccaaccagaagagagaagaactcggcctggctggagatttgattcttaggccaaataatggcatctggatcaagctgaagaggagacatgaagatgacccctaa

SEQ ID NO: 67 - DNA, 1578 bp, synthetic construct
  misc_feature 1..1578: note = rat CYP4V3 coding sequence
  source 1..1578: mol_type = other DNA
atgttgtggctgtggttagggctcagcgggcagaagctattgctttggggcgcagcgagcgcggtctccgtggccggcgccactgtcttgctcaacatcctgcagatgttggtaagctatgcacgaaagtggcagcagatgcggccaatcccgtcggtggctcgcgcttaccccttggtgggacatgcgctgtttatgaagcccaacaacacagaattttttcagcagataattcagtacacagaagaattccgacacctgcccatcattaaactctggattggaccagtgcccctggtggcactttataaggcagagaatgtggaggtgattttgaccagttcgaagcaaattgataaatcctttatgtacaagttcctacagccatggctgggactaggacttcttacaagtactgggagcaaatggcgtgccaggaggaagatgttaacacccagtttccattttacaattctggaggatttcttagatgtcatgaatgagcaagcaaatatattggttaacaagcttgaaaaacatgtcaatcaagaggcctttaactgctttttccccatcactctttgtgctctggatataatctgtgaaacggctatggggaagaacattggagctcaaagtaatggtgattctgagtatgtccgtacagtgtataggatgagcgatatgatatacagaagaatgaagatgccctggttttggtttgacctttggtaccttatgtttaaagaaggaagggaccacaaaaagggactaaagagtctacatacttttaccaacaatgtcattgctgaacgggttaatgcaaggaaggcagagcaagactgcataggtgctgggaggggtcctctcccctcgaaaactaagcgcaaggcctttcttgacttgcttttgagtgtgactgatgaggaaggaaacaaattaagccatgaagacatccgagaggaagttgacaccttcatgtttgagggtcacgatacaactgctgctgccataaactggtccttatacctcctgggctctaatccagaagtccagaggaaagtggacaaggagctggatgatgtgtttggaagatcccatcgccctgtcaccttggaagacctgaagaaacttaaatatctggattgtgtcattaaggagaccctccgtgttttcccatctgtccctttatttgcccggagtcttagcgaagactgtgaagtggcgggttacaaaatctcaaaaggaacggaagcagtcatcattccctatgcactacatcgagaccctagatacttcccagaccctgaggaattccagccagagcggttctttcctgaaaactcccaaggacgccacccctatgcctatgtgccattctctgctggacctagaaactgcattggtcaaaagtttgcggtcatggaggaaaagaccattcttgcctgtatcctgagggagttttggatagaatccaaccagaagagagaagaactcggcctggctggagatttgattcttaggccaaataatggcatctggatcaagctgaagaggaggcatgaagatgacccctaa

SEQ ID NO: 68 - DNA, 1572 bp, synthetic construct
  misc_feature 1..1572: note = dog CYP4V2 coding sequence
  source 1..1572: mol_type = other DNA
cccctgtggctggtgccccttgggcagaaactgcttttgtggggcgccttgggccccccctccttggggggcccccccctagtggtaaggttcctccaaatgctggcaagttacgcccaaaaatgccaccaaatgagggccttccccagtttaccgggggcttacccgttggtggaacactcccttttaataaacccccccggaaaagaattttttcagcaggtcattctttacagcgaagaatcccgacacctgccactcctgaaactctggcttgggcccataccaatagtggccatttatagtgctgaaaatgtagaggtaattttaactagttcaaggcaaatcgacaaatcctatgtatacaagttcctagaaccatggcttggcctaggacttcttacaagtactggaaacaaatggcgatctaggagaaaaatgttaacacccactttccattttacgattctggaagatttcttagatgtcatgaatgaacacgcaaatatattggttaataagcttgaaaaacatgttaaccaagaagcatttaactgctttttttacatcactctttgtgcattagatataatttgtgaaacagctatggggaagaatattggggctcaaaataatgaggattctgagtatgttcgtgccatctacagaatgagtgatacgatacatcgaagaatgaagatgccctggctctggcttgactttttgtttcttatgtttaaagaaggccgggaacacaaaaggaacctagagatcctacataattttaccaataatgtcatcactgaacgggccagtgaactgaagagagacgaagaacatggaagtgctgacaaggactgctccccctccaaaaataaacgcagagcttttcttgacttgcttttaaatgtgactgatgatgaagggaacaagctacgtcatgaagatgttcgagaagaagttgacaccttcatgtttgagggccatgatacgacagcagcggcgataaactggtccttatatctcttgggttcttacccagaagtccagaaacaagtggacagtgaactggaggacgtgtttgggaagtctgatcgtcctgctaccttagaagacctgaagaaactcaaatacctggagtgtgtcattaaggagagccttcgcctttttccttcagttcccttatttgcccgtaatcttaacgaagattgtgtagttgcgggttacaaggttgtgaaaggctcccaagcgatcatcattccctacgcacttcatagagatccaagatatttcccaaatcccgaggagttccagccagagcggttctttcctgaaaatttgcaaggacgccacccatatgcatacattcccttttctgctggacccagaaactgtataggtcaaaggtttgccataatggaagaaaagactgttctttcctgtgtcctgaggcatttttgggtagaatccaaccagaaaagagaagaacttggtctggcaggagagttgattcttcgtccaactaatggcatctggatcaagttgaagaggagaaatgcagatgaatcttaa

SEQ ID NO: 69 - DNA, 327 bp, synthetic construct
  misc_feature 1..327: note = human truncated RdCVF coding sequence
  source 1..327: mol_type = other DNA
atggcctccctgttctctggccgcatcctgatccgcaacaatagcgaccaggacgagctggatacggaggctgaggtcagtcgcaggctggagaaccggctggtgctgctgttctttggtgctggggcttgtccacagtgccaggccttcgtgcccatcctcaaggacttcttcgtgcggctcacagatgagttctatgtactgcgggcggctcagctggccctggtgtacgtgtcccaggactccacggaggagcagcaggacctgttcctcaaggacatgccaaagaaatggcttttcctgccctttgaggatgatctgaggagg

SEQ ID NO: 70 - DNA, 327 bp, synthetic construct
  misc_feature 1..327: note = chimpanzee truncated RdCVF coding sequence
  source 1..327: mol_type = other DNA
atggcctccctgttctctggccgcatcctgatccgcaacaatagcgaccaggacgaactggatacggaggctgaggtcagtcgcaggctggagaaccggctggtgctgctgttctttggtgccggggcttgtccacagtgccaggccttcgtgcccatcctcaaggacttcttcgtgcggctcacagatgagttctatgtactgcgggcggctcagctggccctggtgtacgtgtcccaggactccacggaggagcagcaggacctgttcctcaaggacatgccaaagaagtggcttttcctgccctttgaggatgatctgaggagg

SEQ ID NO: 71 - DNA, 327 bp, synthetic construct; identical to SEQ ID NO: 69
  misc_feature 1..327: note = gorilla truncated RdCVF coding sequence
  source 1..327: mol_type = other DNA

SEQ ID NO: 72 - DNA, 327 bp, synthetic construct; identical to SEQ ID NO: 69
  misc_feature 1..327: note = cynomolgus monkey truncated RdCVF coding sequence
  source 1..327: mol_type = other DNA

SEQ ID NO: 73 - DNA, 327 bp, synthetic construct
  misc_feature 1..327: note = mouse truncated RdCVF coding sequence
  source 1..327: mol_type = other DNA
atggcatctctcttctctggacgcatcttgatcaggaacaacagcgaccaggatgaagtggagacagaggcagagctgagccgtaggttagagaatcgtctggtgttgctgttcttcggcgccggcgcctgtccccagtgccaggcctttgccccagtcctcaaagacttcttcgtgcggctcactgacgagttctacgtgctgcgggcagcacagctggccctggtctatgtgtcccaggaccctacagaggagcaacaggacctcttcctcagggacatgcctgaaaaatggctcttcctgccgttccatgatgaactgaggagg

SEQ ID NO: 74 - DNA, 327 bp, synthetic construct
  misc_feature 1..327: note = rat truncated RdCVF coding sequence
  source 1..327: mol_type = other DNA
atggtgtctctcttctctggccgcatcttgatcaggaacaacagcgaccaggatgaagtggagacagaggcagagctgagccgccggttagagaatcgtcttgtgctactgttcttcggtgctggggcctgtccccagtgccaggccttcgccccagtcctcaaagacttcttcgtgcggctcactgatgagttctacgtgctacgggcagcacagctggccctggtctatgtgtcccaggaccctacagaggagcaacaggacctgttcctccgggacatgcctgaaaagtggctcttcctgccgttccatgatgacctgaggaga

SEQ ID NO: 75 - DNA, 327 bp, synthetic construct
  misc_feature 1..327: note = dog truncated RdCVF coding sequence
  source 1..327: mol_type = other DNA
atggcctccttgttctctggccgcgtcctgattcgcaacaacagtgaccaggacgagctggacacggaggccgagctcagccgcaggctggagaaccggctggtgctgctgttctttggcgccgggtcgtgcccgcagtgccaagccttcgcgcctatcctcagggatttctttgtgaggctcacagatgagttctatgtgctgcgggcagcccaactggctctggtgtacgtgtcccaggaccccacagaggagcagcaggatctgtttctcagggacatgccgaagaagtggctcttcctgccctttgaggatgacctgaggagg

SEQ ID NO: 76 - protein, 525 aa, synthetic construct
  REGION 1..525: note = human CYP4V2 polypeptide sequence
MAGLWLGLVWQKLLLWGAASALSLAGASLVLSLLQRVASYARKWQQMRPIPTVARAYPLVGHALLMKPDGREFFQQIIEYTEEYRHMPLLKLWVGPVPMVALYNAENVEVILTSSKQIDKSSMYKFLEPWLGLGLLTSTGNKWRSRRKMLTPTFHFTILEDFLDIMNEQANILVKKLEKHINQEAFNCFFYITLCALDIICETAMGKNIGAQSNDDSEYVRAVYRMSEMIFRRIKMPWLWLDLWYLMFKEGWEHKKSLQILHTFTNSVIAERANEMNANEDCRGDGRGSAPSKNKRRAFLDLLLSVTDDEGNRLSHEDIREEVDTFMFEGHDTTAAAINWSLYLLGSNPEVQKKVDHELDDVFGKSDRPATVEDLKKLRYLECVIKETLRLFPSVPLFARSVSEDCEVAGYRVLKGTEAVIIPYALHRDPRYFPNPEEFQPERFFPENAQGRHPYAYVPFSAGPRNCIGQKFAVMEEKTILSCILRHFWIESNQKREELGLEGQLILRPSNGIWIKLKRRNADER

SEQ ID NO: 77 - protein, 525 aa, synthetic construct
  REGION 1..525: note = chimpanzee CYP4V2 polypeptide sequence
MAGLWLGLVWQKLLLWGAASAVSLAGASLVLSLLQRVATYARKWQQMRPIPTVARAYPLVGHALLMKPDGREFFQQIIEYTEEYRHMPLLKLWVGPVPMVALYNAENVEVILTSSKQIDKSSMYKFLEPWLGLGLLTSTGNKWRSRRKMLTPTFHFTILEDFLDIMNEQANTLVKKLEKHINQEAFNCFFYITLCALDIICETAMGKNIGAQSNDDSEYVRAVYRMSEMIFRRIKMPWLWLDLWYLMFKEGWEHKKSLKILHTFTNSVIAERANEMNANEDCRGDGRGSAPSKNKRRAFLDLLLSVTDDEGNRLSHEDIREEVDTFMFEGHDTTAAAINWSLYLLGSNPEVQKKVDHELDDVFGKSDRPATVEDLKKLRYLECVIKETLRLFPSVPLFARSVSEDCEVAGYRVLKGTEAVIIPYALHRDPRYFPNPEEFQPERFFPKNAQGRHPYAYVPFSAGPRNCIGQKFAVMEEKTILSCILRHFWIESNQKREELGLEGQLILRPSNGIWIKLKRRNADER

SEQ ID NO: 78 - protein, 525 aa, synthetic construct [sequence omitted]

SEQ ID NO: 79 - protein, 525 aa, synthetic construct
  REGION 1..525: note = cynomolgus monkey CYP4V2 polypeptide sequence
MAGIWLGLVWQKLLLWGAASAVSLAGASLVLSLLQRVASYVRKWQQMRPIPTVARAYPLVGHALLMKRDGREFFQQIIEYTEEYRHMPLLKLWVGPVPMVALYNAENVEVILTSSKQIDKSSMYKFLEPWLGLGLLTSTGNKWRSRRKMLTPTFHFTILEDFLDIMNEQANILVKKLEKHVNQEAFNCFVYITLCALDIICETAMGKNIGAQSNDDSEYVRAVYRMSEMIFRRIKMPWLWLDLWYLMFKEGWEHKKSLKILHAFTNNVIAERANEMNVDEDCRGDGRDSAPSKNKRRAFLDLLLSVTDDEGNRLSHEDIREEVDTFMFEGHDTTAAAMNWSLYLLGSNPEVQKKVDHELDDVFGRSDRPATVEDLKKLRYLECVIKETLRLFPSVPLFARSVSEDCEVAGYRVLKGTEAVIIPYALHRDPRYFPNPEEFRPERFFPENAQGRHPYAYVPFSAGPRNCIGQKFAVMEEKTILSCILRHFWIESNQKREELGLEGQLILRPTNGIWIKLKRRNADEP

SEQ ID NO: 80 - protein, 525 aa, synthetic construct
  REGION 1..525: note = mouse CYP4V3 polypeptide sequence
MLWLWLGLSGQKLLLWGAASAVSLAGATILISIFPMLVSYARKWQQMRSIPSVARAYPLVGHALYMKPNNAEFFQQLIYYTEEFRHLPIIKLWIGPVPLVALYKAENVEVILTSSKQIDKSFLYKFLQPWLGLGLLTSTGSKWRTRRKMLTPTFHFTILENFLDVMNEQANILVNKLEKHVNQEAFNCFFYITLCALDIICETAMGKNIGAQSNNDSEYVRTVYRMSDMIYRRMKMPWLWFDLWYLVFKEGRDHKRGLKCLHTFTNNVIAERVKERKAEEDWTGAGRGPIPSKNKRKAFLDLLLSVTDEEGNRLSQEDIREEVDTFMFEGHDTTAAAINWSLYLLGTNPEVQRKVDQELDEVFGRSHRPVTLEDLKKLKYLDCVIKETLRVFPSVPLFARSLSEDCEVGGYKVTKGTEAIIIPYALHRDPRYFPDPEEFRPERFFPENSQGRHPYAYVPFSAGPRNCIGQKFAVMEEKTILACILRQFWVESNQKREELGLAGDLILRPNNGIWIKLKRRHEDDP

SEQ ID NO: 81 - protein, 525 aa, synthetic construct
  REGION 1..525: note = rat CYP4V2 polypeptide sequence
MLWLWLGLSGQKLLLWGAASAVSVAGATVLLNILQMLVSYARKWQQMRPIPSVARAYPLVGHALFMKPNNTEFFQQIIQYTEEFRHLPIIKLWIGPVPLVALYKAENVEVILTSSKQIDKSFMYKFLQPWLGLGLLTSTGSKWRARRKMLTPSFHFTILEDFLDVMNEQANILVNKLEKHVNQEAFNCFFPITLCALDIICETAMGKNIGAQSNGDSEYVRTVYRMSDMIYRRMKMPWFWFDLWYLMFKEGRDHKKGLKSLHTFTNNVIAERVNARKAEQDCIGAGRGPLPSKTKRKAFLDLLLSVTDEEGNKLSHEDIREEVDTFMFEGHDTTAAAINWSLYLLGSNPEVQRKVDKELDDVFGRSHRPVTLEDLKKLKYLDCVIKETLRVFPSVPLFARSLSEDCEVAGYKISKGTEAVIIPYALHRDPRYFPDPEEFQPERFFPENSQGRHPYAYVPFSAGPRNCIGQKFAVMEEKTILACILREFWIESNQKREELGLAGDLILRPNNGIWIKLKRRHEDDP

SEQ ID NO: 82 - protein, 523 aa, synthetic construct
  REGION 1..523: note = dog CYP4V2 polypeptide sequence
PLWLVPLGQKLLLWGALGPPSLGGPPLVVRFLQMLASYAQKCHQMRAFPSLPGAYPLVEHSLLINPPGKEFFQQVILYSEESRHLPLLKLWLGPIPIVAIYSAENVEVILTSSRQIDKSYVYKFLEPWLGLGLLTSTGNKWRSRRKMLTPTFHFTILEDFLDVMNEHANILVNKLEKHVNQEAFNCFFYITLCALDIICETAMGKNIGAQNNEDSEYVRAIYRMSDTIHRRMKMPWLWLDFLFLMFKEGREHKRNLEILHNFTNNVITERASELKRDEEHGSADKDCSPSKNKRRAFLDLLLNVTDDEGNKLRHEDVREEVDTFMFEGHDTTAAAINWSLYLLGSYPEVQKQVDSELEDVFGKSDRPATLEDLKKLKYLECVIKESLRLFPSVPLFARNLNEDCVVAGYKVVKGSQAIIIPYALHRDPRYFPNPEEFQPERFFPENLQGRHPYAYIPFSAGPRNCIGQRFAIMEEKTVLSCVLRHFWVESNQKREELGLAGELILRPTNGIWIKLKRRNADES

SEQ ID NO: 83 - protein, 109 aa, synthetic construct
  REGION 1..109: note = human truncated RdCVF polypeptide sequence
MASLFSGRILIRNNSDQDELDTEAEVSRRLENRLVLLFFGAGACPQCQAFVPILKDFFVRLTDEFYVLRAAQLALVYVSQDSTEEQQDLFLKDMPKKWLFLPFEDDLRR

SEQ ID NO: 84 - protein, 109 aa, synthetic construct; identical to SEQ ID NO: 83
  REGION 1..109: note = chimpanzee truncated RdCVF polypeptide sequence

SEQ ID NO: 85 - protein, 109 aa, synthetic construct
  REGION 1..109: note = gorilla truncated RdCVF polypeptide sequence
MASLFSGRILICNNSDQDELDTEAEVSRRLENRLVLLFFGAGACPQCQAFVPILKDFFVRLTDEFYVLRAAQLALVYVSQDSTEEQQDLFLKDMPKKWLFLPFEDDLRR

SEQ ID NO: 86 - protein, 109 aa, synthetic construct
  REGION 1..109: note = cynomolgus monkey truncated RdCVF polypeptide sequence
MASLFSGRILICNNNDQDELDTEAEVSRRLENRLVLLFFGAGACPQCQAFVPILKDFFVRLTDEFYVLRAAQLALVYVSQDSTEEQQDLFLKDMPKKWLFLPFEDELRR

SEQ ID NO: 87 - protein, 109 aa, synthetic construct
  REGION 1..109: note = mouse truncated RdCVF polypeptide sequence
MASLFSGRILIRNNSDQDEVETEAELSRRLENRLVLLFFGAGACPQCQAFAPVLKDFFVRLTDEFYVLRAAQLALVYVSQDPTEEQQDLFLRDMPEKWLFLPFHDELRR

SEQ ID NO: 88 - protein, 109 aa, synthetic construct
  REGION 1..109: note = rat truncated RdCVF polypeptide sequence
MVSLFSGRILIRNNSDQDEVETEAELSRRLENRLVLLFFGAGACPQCQAFAPVLKDFFVRLTDEFYVLRAAQLALVYVSQDPTEEQQDLFLRDMPEKWLFLPFHDDLRR

SEQ ID NO: 89 - protein, 109 aa, synthetic construct
  REGION 1..109: note = dog truncated RdCVF polypeptide sequence
MASLFSGRVLIRNNSDQDELDTEAELSRRLENRLVLLFFGAGSCPQCQAFAPILRDFFVRLTDEFYVLRAAQLALVYVSQDPTEEQQDLFLRDMPKKWLFLPFEDDLRR

SEQ ID NO: 90 - DNA, 2337 bp, synthetic construct
  misc_feature 1..2337: note = OPEFS-CYP4V2-BGH
  source 1..2337: mol_type = other DNA
gggcagagcgcacatcgcccacagtccccgagaagttggggggaggggtcggcaattgaaccggtgcctagagaaggtggcgcggggtaaactgggaaagtgatgtcgtgtactggctccgcctttttcccgagggtgggggagaaccgtatataagtgcagtagtcgccgtgaacgttctttttcgcaacgggtttgccgccagaacacaggtaagtatcaaggttacaagacaggtttaaggagaccaatagaaactgggcttgtcgagacagagaagactcttgcgtttctgataggcacctattggtcttactgacatccactttgcctttctctccacaggaattccgccaccatggcggggctctggctggggctcgtgtggcagaagctgctgctgtggggcgcggcgagtgccctttccctggccggcgccagtctggtcctgagtctgctgcagagggtggcgagctacgcgcggaaatggcagcagatgcggcccatccccacggtggcccgcgcctacccactggtgggccacgcgctgctgatgaagccggacgggcgagaattttttcagcagatcattgagtacacagaggaataccgccacatgccgctgctgaagctctgggtcgggccagtgcccatggtggccctttataatgcagaaaatgtggaggtaattttaactagttcaaagcaaattgacaaatcctctatgtacaagtttttagaaccatggcttggcctaggacttcttacaagtactggaaacaaatggcgctccaggagaaagatgttaacacccactttccattttaccattctggaagatttcttagatatcatgaatgaacaagcaaatatattggttaagaaacttgaaaaacacattaaccaagaagcatttaactgctttttttacatcactctttgtgccttagatatcatctgtgaaacagctatggggaagaatattggtgctcaaagtaatgatgattccgagtatgtccgtgcagtttatagaatgagtgagatgatatttcgaagaataaagatgccctggctttggcttgatctctggtaccttatgtttaaagaaggatgggaacacaaaaagagccttcagatcctacatacttttaccaacagtgtcatcgcggaacgggccaatgaaatgaacgccaatgaagactgtagaggtgatggcaggggctctgccccctccaaaaataaacgcagggcctttcttgacttgcttttaagtgtgactgatgacgaagggaacaggctaagtcatgaagatattcgagaagaagttgacaccttcatgtttgaggggcacgatacaactgcagctgcaataaactggtccttatacctgttgggttctaacccagaagtccagaaaaaagtggatcatgaattggatgacgtgtttgggaagtctgaccgtcccgctacagtagaagacctgaagaaacttcggtatctggaatgtgttattaaggagacccttcgcctttttccttctgttcctttatttgcccgtagtgttagtgaagattgtgaagtggcaggttacagagttctaaaaggcactgaagccgtcatcattccctatgcattgcacagagatccgagatacttccccaaccccgaggagttccagcctgagcggttcttccccgagaatgcacaagggcgccatccatatgcctacgtgcccttctctgctggccccaggaactgtataggtcaaaagtttgctgtgatggaagaaaagaccattctttcgtgcatcctgaggcacttttggatagaatccaaccagaaaagagaagagcttggtctagaaggacagttgattcttcgtccaagtaatggcatctggatcaagttgaagaggagaaatgcagatgaacgctaaacgcgtggtttatccgatccaccggatctagataagatatccgatccaccggatctagataactgatcataatcagccataccacatttgtagaggttttacttgctttaaaaaacctcccacacctccccctgaacctgaaacataaaatgaatgcaattggcggccgcctcgagctgtgccttctagttgccagccatctgttgtttgcccctcccccgtgccttccttgaccctggaaggtgccactcccactgtcctttcctaataaaatgaggaaattgcatcgcattgtctgagtaggtgtcattctattctggggggtggggtggggcaggacagcaagggggaggattgggaagacaatagcaggcatgctggggatgcggtgggctctatgg

SEQ ID NO: 91 - DNA, 2492 bp, synthetic construct
  misc_feature 1..2492: note = P5-CYP4V2-BGH
  source 1..2492: mol_type = other DNA
gagccggatgcgccttcctttcctctccagagcaggctgcccgcccgcggaatcccgcacgtagagcaacctcgcagcaccctcagaacagccccgctggggcgcgccgggctgccgcggtgacctttccgacgcccctgaccccgcatccggaggcggccggaagtgtcgccggcctcctcccggcgcagcctccgggcctccagtgcaatcactacgccctggggcccggaaaccgttttccggtctttcgctttcggctggggcgtggaggccgcggtgctgcgtaggccgggccgggcgcaggaacagccccgtggcgccctctctggccgccgcccgggcgggaaacgtcgttccggggaccgggcgaccccgcagcggggagcgcgccaggtccgcgcggggaagtgggcggtgtgcggccggcaccgcctcgcaccacgcccccgcgggcccgcactttcccggagtgcaccccgcggccgccagccggggcggaattccgccaccatggcggggctctggctggggctcgtgtggcagaagctgctgctgtggggcgcggcgagtgccctttccctggccggcgccagtctggtcctgagtctgctgcagagggtggcgagctacgcgcggaaatggcagcagatgcggcccatccccacggtggcccgcgcctacccactggtgggccacgcgctgctgatgaagccggacgggcgagaattttttcagcagatcattgagtacacagaggaataccgccacatgccgctgctgaagctctgggtcgggccagtgcccatggtggccctttataatgcagaaaatgtggaggtaattttaactagttcaaagcaaattgacaaatcctctatgtacaagtttttagaaccatggcttggcctaggacttcttacaagtactggaaacaaatggcgctccaggagaaagatgttaacacccactttccattttaccattctggaagatttcttagatatcatgaatgaacaagcaaatatattggttaagaaacttgaaaaacacattaaccaagaagcatttaactgctttttttacatcactctttgtgccttagatatcatctgtgaaacagctatggggaagaatattggtgctcaaagtaatgatgattccgagtatgtccgtgcagtttatagaatgagtgagatgatatttcgaagaataaagatgccctggctttggcttgatctctggtaccttatgtttaaagaaggatgggaacacaaaaagagccttcagatcctacatacttttaccaacagtgtcatcgcggaacgggccaatgaaatgaacgccaatgaagactgtagaggtgatggcaggggctctgccccctccaaaaataaacgcagggcctttcttgacttgcttttaagtgtgactgatgacgaagggaacaggctaagtcatgaagatattcgagaagaagttgacaccttcatgtttgaggggcacgatacaactgcagctgcaataaactggtccttatacctgttgggttctaacccagaagtccagaaaaaagtggatcatgaattggatgacgtgtttgggaagtctgaccgtcccgctacagtagaagacctgaagaaacttcggtatctggaatgtgttattaaggagacccttcgcctttttccttctgttcctttatttgcccgtagtgttagtgaagattgtgaagtggcaggttacagagttctaaaaggcactgaagccgtcatcattccctatgcattgcacagagatccgagatacttccccaaccccgaggagttccagcctgagcggttcttccccgagaatgcacaagggcgccatccatatgcctacgtgcccttctctgctggccccaggaactgtataggtcaaaagtttgctgtgatggaagaaaagaccattctttcgtgcatcctgaggcacttttggatagaatccaaccagaaaagagaagagcttggtctagaaggacagttgattcttcgtccaagtaatggcatctggatcaagttgaagaggagaaatgcagatgaacgctaaacgcgtggtttatccgatccaccggatctagataagatatccgatccaccggatctagataactgatcataatcagccataccacatttgtagaggttttacttgctttaaaaaacctcccacacctccccctgaacctgaaacataaaatgaatgcaattggcggccgcctcgagctgtgccttctagttgccagccatctgttgtttgcccctcccccgtgccttccttgaccctggaaggtgccactcccactgtcctttcctaataaaatgaggaaattgcatcgcattgtctgagtaggtgtcattctattctggggggtggggtggggcaggacagcaagggggaggattgggaagacaatagcaggcatgctggggatgcggtgggctctatgg

SEQ ID NO: 92 - DNA, 3692 bp, synthetic construct
  misc_feature 1..3692: note = P1-CYP4V2-BGH
  source 1..3692: mol_type = other DNA
gctgaggtttgagtttctattgatcccctcacctgaatagggaacacagtacccaatacacagtttttcaaccattactccccttccttcctccccctattttagaatccccagtatgtagacaaattgtttacttttatagctgtaattaaccttattatagctcagcctcaaccctttagagaggaggaaactaaagcccatgagacttgcttaaagatactaagtgaacatatttattttttaaagtgttaaagtgattaaacaatgtagacgtgaatgaaataaaaagcgtaagttccccatcttcattcccactccatagagctgatcagtatttttacttgcagacattagtggagccgtagagaaagaaaccttttctccaaaagaaggcattactttacacactccgttctgcaacttgttttgttcacttgctatttcacgtcagcccatgcagatgacttaaaacaaattcaaatggagaaaagccttaggcatgtttttctctgcactaaagaggccctgcaggtggctgtggccaacttatgcagtggcttcgagtgaacgaacgtaattagtaattaagcaaagcgggcatccaggacattcagtttcatcttcctggcactttagtgtttaggaagggcctggcctctcggggagcgacactcctcgcccggccactttgtaagaagcatcgagcgtggaaaaggggctggggtcagcactggggccctctgccgggaagagagactggcggccagcacacgcgtctccccaggctgaaatggggcaccctctcgcggcccttccctcccttcccgggctgggtggcaggtcttggctcttctgcgagtaccccgcggctgcggtctcccggcacccgctgagcagcctcgcccgccttcctctcccacccgcccctgcgtgctctccggggctccggcttcctcggtctggtgcctggtgcgtattttggaaaatacctggctcataaccacctcattgagctcccagtgtcccagtgggccagcggacacacacgggtagctgacttccctaacgtgtccccaaagcctccctggattacagcgcccgctgctccatgtgaccccgcgggagccaggacgcgccccgcctcccggggctgcaagttgcgcagggagcgagcgatgcgcagcagagctgggctccgagccggatgcgccttcctttcctctccagagcaggctgcccgcccgcggaatcccgcacgtagagcaacctcgcagcaccctcagaacagccccgctggggcgcgccgggctgccgcggtgacctttccgacgcccctgaccccgcatccggaggcggccggaagtgtcgccggcctcctcccggcgcagcctccgggcctccagtgcaatcactacgccctggggcccggaaaccgttttccggtctttcgctttcggctggggcgtggaggccgcggtgctgcgtaggccgggccgggcgcaggaacagccccgtggcgccctctctggccgccgcccgggcgggaaacgtcgttccggggaccgggcgaccccgcagcggggagcgcgccaggtccgcgcggggaagtgggcggtgtgcggccggcaccgcctcgcaccacgcccccgcgggcccgcactttcccggagtgcaccccgcggccgccagccggggcggaattccgccaccatggcggggctctggctggggctcgtgtggcagaagctgctgctgtggggcgcggcgagtgccctttccctggccggcgccagtctggtcctgagtctgctgcagagggtggcgagctacgcgcggaaatggcagcagatgcggcccatccccacggtggcccgcgcctacccactggtgggccacgcgctgctgatgaagccggacgggcgagaattttttcagcagatcattgagtacacagaggaataccgccacatgccgctgctgaagctctgggtcgggccagtgcccatggtggccctttataatgcagaaaatgtggaggtaattttaactagttcaaagcaaattgacaaatcctctatgtacaagtttttagaaccatggcttggcctaggacttcttacaagtactggaaacaaatggcgctccaggagaaagatgttaacacccactttccattttaccattctggaagatttcttagatatcatgaatgaacaagcaaatatattggttaagaaacttgaaaaacacattaaccaagaagcatttaactgctttttttacatcactctttgtgccttagatatcatctgtgaaacagctatggggaagaatattggtgctcaaagtaatgatgattccgagtatgtccgtgcagtttatagaatgagtgagatgatatttcgaagaataaagatgccctggctttggcttgatctctggtaccttatgtttaaagaaggatgggaacacaaaaagagccttcagatcctacatacttttaccaacagtgtcatcgcggaacgggccaatgaaatgaacgccaatgaagactgtagaggtgatggcaggggctctgccccctccaaaaataaacgcagggcctttcttgacttgcttttaagtgtgactgatgacgaagggaacaggctaagtcatgaagatattcgagaagaagttgacaccttcatgtttgaggggcacgatacaactgcagctgcaataaactggtccttatacctgttgggttctaacccagaagtccagaaaaaagtggatcatgaattggatgacgtgtttgggaagtctgaccgtcccgctacagtagaagacctgaagaaacttcggtatctggaatgtgttattaaggagacccttcgcctttttccttctgttcctttatttgcccgtagtgttagtgaagattgtgaagtggcaggttacagagttctaaaaggcactgaagccgtcatcattccctatgcattgcacagagatccgagatacttccccaaccccgaggagttccagcctgagcggttcttccccgagaatgcacaagggcgccatccatatgcctacgtgcccttctctgctggccccaggaactgtataggtcaaaagtttgctgtgatggaagaaaagaccattctttcgtgcatcctgaggcacttttggatagaatccaaccagaaaagagaagagcttggtctagaaggacagttgattcttcgtccaagtaatggcatctggatcaagttgaagaggagaaatgcagatgaacgctaaacgcgtggtttatccgatccaccggatctagataagatatccgatccaccggatctagataactgatcataatcagccataccacatttgtagaggttttacttgctttaaaaaacctcccacacctccccctgaacctgaaacataaaatgaatgcaattggcggccgcctcgagctgtgccttctagttgccagccatctgttgtttgcccctcccccgtgccttccttgaccctggaaggtgccactcccactgtcctttcctaataaaatgaggaaattgcatcgcattgtctgagtaggtgtcattctattctggggggtggggtggggcaggacagcaagggggaggattgggaagacaatagcaggcatgctggggatgcggtgggctctatgg

SEQ ID NO: 93 - DNA, 2625 bp, synthetic construct
  misc_feature 1..2625: note = P5-intron-CYP4V2-BGH
  source 1..2625: mol_type = other DNA
gagccggatgcgccttcctttcctctccagagcaggctgcccgcccgcggaatcccgcacgtagagcaacctcgcagcaccctcagaacagccccgctggggcgcgccgggctgccgcggtgacctttccgacgcccctgaccccgcatccggaggcggccggaagtgtcgccggcctcctcccggcgcagcctccgggcctccagtgcaatcactacgccctggggcccggaaaccgttttccggtctttcgctttcggctggggcgtggaggccgcggtgctgcgtaggccgggccgggcgcaggaacagccccgtggcgccctctctggccgccgcccgggcgggaaacgtcgttccggggaccgggcgaccccgcagcggggagcgcgccaggtccgcgcggggaagtgggcggtgtgcggccggcaccgcctcgcaccacgcccccgcgggcccgcactttcccggagtgcaccccgcggccgccagccggggcggtaagtatcaaggttacaagacaggtttaaggagaccaatagaaactgggcttgtcgagacagagaagactcttgcgtttctgataggcacctattggtcttactgacatccactttgcctttctctccacaggaattccgccaccatggcggggctctggctggggctcgtgtggcagaagctgctgctgtggggcgcggcgagtgccctttccctggccggcgccagtctggtcctgagtctgctgcagagggtggcgagctacgcgcggaaatggcagcagatgcggcccatccccacggtggcccgcgcctacccactggtgggccacgcgctgctgatgaagccggacgggcgagaattttttcagcagatcattgagtacacagaggaataccgccacatgccgctgctgaagctctgggtcgggccagtgcccatggtggccctttataatgcagaaaatgtggaggtaattttaactagttcaaagcaaattgacaaatcctctatgtacaagtttttagaaccatggcttggcctaggacttcttacaagtactggaaacaaatggcgctccaggagaaagatgttaacacccactttccattttaccattctggaagatttcttagatatcatgaatgaacaagcaaatatattggttaagaaacttgaaaaacacattaaccaagaagcatttaactgctttttttacatcactctttgtgccttagatatcatctgtgaaacagctatggggaagaatattggtgctcaaagtaatgatgattccgagtatgtccgtgcagtttatagaatgagtgagatgatatttcgaagaataaagatgccctggctttggcttgatctctggtaccttatgtttaaagaaggatgggaacacaaaaagagccttcagatcctacatacttttaccaacagtgtcatcgcggaacgggccaatgaaatgaacgccaatgaagactgtagaggtgatggcaggggctctgccccctccaaaaataaacgcagggcctttcttgacttgcttttaagtgtgactgatgacgaagggaacaggctaagtcatgaagatattcgagaagaagttgacaccttcatgtttgaggggcacgatacaactgcagctgcaataaactggtccttatacctgttgggttctaacccagaagtccagaaaaaagtggatcatgaattggatgacgtgtttgggaagtctgaccgtcccgctacagtagaagacctgaagaaacttcggtatctggaatgtgttattaaggagacccttcgcctttttccttctgttcctttatttgcccgtagtgttagtgaagattgtgaagtggcaggttacagagttctaaaaggcactgaagccgtcatcattccctatgcattgcacagagatccgagatacttccccaaccccgaggagttccagcctgagcggttcttccccgagaatgcacaagggcgccatccatatgcctacgtgcccttctctgctggccccaggaactgtataggtcaaaagtttgctgtgatggaagaaaagaccattctttcgtgcatcctgaggcacttttggatagaatccaaccagaaaagagaagagcttggtctagaaggacagttgattcttcgtccaagtaatggcatctggatcaagttgaagaggagaaatgcagatgaacgctaaacgcgtggtttatccgatccaccggatctagataagatatccgatccaccggatctagataactgatcataatcagccataccacatttgtagaggttttacttgctttaaaaaacctcccacacctccccctgaacctgaaacataaaatgaatgcaattggcggccgcctcgagctgtgccttctagttgccagccatctgttgtttgcccctcccccgtgccttccttgaccctggaaggtgccactcccactgtcctttcctaataaaatgaggaaattgcatcgcattgtctgagtaggtgtcattctattctggggggtggggtggggcaggacagcaagggggaggattgggaagacaatagcaggcatgctggggatgcggtgggctctatgg

SEQ ID NO: 94 - DNA, 3117 bp, synthetic construct
  misc_feature 1..3117: note = P5-intron-CYP4V2-WPRE-SV40
  source 1..3117: mol_type = other DNA
gagccggatgcgccttcctttcctctccagagcaggctgcccgcccgcggaatcccgcacgtagagcaacctcgcagcaccctcagaacagccccgctggggcgcgccgggctgccgcggtgacctttccgacgcccctgaccccgcatccggaggcggccggaagtgtcgccggcctcctcccggcgcagcctccgggcctccagtgcaatcactacgccctggggcccggaaaccgttttccggtctttcgctttcggctggggcgtggaggccgcggtgctgcgtaggccgggccgggcgcaggaacagccccgtggcgccctctctggccgccgcccgggcgggaaacgtcgttccggggaccgggcgaccccgcagcggggagcgcgccaggtccgcgcggggaagtgggcggtgtgcggccggcaccgcctcgcaccacgcccccgcgggcccgcactttcccggagtgcaccccgcggccgccagccggggcggtaagtatcaaggttacaagacaggtttaaggagaccaatagaaactgggcttgtcgagacagagaagactcttgcgtttctgataggcacctattggtcttactgacatccactttgcctttctctccacaggaattccgccaccatggcggggctctggctggggctcgtgtggcagaagctgctgctgtggggcgcggcgagtgccctttccctggccggcgccagtctggtcctgagtctgctgcagagggtggcgagctacgcgcggaaatggcagcagatgcggcccatccccacggtggcccgcgcctacccactggtgggccacgcgctgctgatgaagccggacgggcgagaattttttcagcagatcattgagtacacagaggaataccgccacatgccgctgctgaagctctgggtcgggccagtgcccatggtggccctttataatgcagaaaatgtggaggtaattttaactagttcaaagcaaattgacaaatcctctatgtacaagtttttagaaccatggcttggcctaggacttcttacaagtactggaaacaaatggcgctccaggagaaagatgttaacacccactttccattttaccattctggaagatttcttagatatcatgaatgaacaagcaaatatattggttaagaaacttgaaaaacacattaaccaagaagcatttaactgctttttttacatcactctttgtgccttagatatcatctgtgaaacagctatggggaagaatattggtgctcaaagtaatgatgattccgagtatgtccgtgcagtttatagaatgagtgagatgatatttcgaagaataaagatgccctggctttggcttgatctctggtaccttatgtttaaagaaggatgggaacacaaaaagagccttcagatcctacatacttttaccaacagtgtcatcgcggaacgggccaatgaaatgaacgccaatgaagactgtagaggtgatggcaggggctctgccccctccaaaaataaacgcagggcctttcttgacttgcttttaagtgtgactgatgacgaagggaacaggctaagtcatgaagatattcgagaagaagttgacaccttcatgtttgaggggcacgatacaactgcagctgcaataaactggtccttatacctgttgggttctaacccagaagtccagaaaaaagtggatcatgaattggatgacgtgtttgggaagtctgaccgtcccgctacagtagaagacctgaagaaacttcggtatctggaatgtgttattaaggagacccttcgcctttttccttctgttcctttatttgcccgtagtgttagtgaagattgtgaagtggcaggttacagagttctaaaaggcactgaagccgtcatcattccctatgcattgcacagagatccgagatacttccccaaccccgaggagttccagcctgagcggttcttccccgagaatgcacaagggcgccatccatatgcctacgtgcccttctctgctggccccaggaactgtataggtcaaaagtttgctgtgatggaagaaaagaccattctttcgtgcatcctgaggcacttttggatagaatccaaccagaaaagagaagagcttggtctagaaggacagttgattcttcgtccaagtaatggcatctggatcaagttgaagaggagaaatgcagatgaacgctaaacgcgtggtttatccgatccaccggatctagataagatatccgatccaccggatctagataactgatcataatcagccataccacatttgtagaggttttacttgctttaaaaaacctcccacacctccccctgaacctgaaacataaaatgaatgcaattggcggccgcctcgagaatcaacctctggattacaaaatttgtgaaagattgactggtattcttaactatgttgctccttttacgctatgtggatacgctgctttaatgcctttgtatcatgctattgcttcccgtatggctttcattttctcctccttgtataaatcctggttgctgtctctttatgaggagttgtggcccgttgtcaggcaacgtggcgtggtgtgcactgtgtttgctgacgcaacccccactggttggggcattgccaccacctgtcagctcctttccgggactttcgctttccccctccctattgccacggcggaactcatcgccgcctgccttgcccgctgctggacaggggctcggctgttgggcactgacaattccgtggtgttgtcggggaaatcatcgtcctttccttggctgctcgcctgtgttgccacctggattctgcgcgggacgtccttctgctacgtcccttcggccctcaatccagcggaccttccttcccgcggcctgctgccggctctgcggcctcttccgcgtcttcgccttcgccctcagacgagtcggatctccctttgggccgcctccccgcggtaacaacttgtttattgcagcttataatggttacaaataaagcaatagcatcacaaatttcacaaataaagcatttttttcactgcattctagttgtggtttgtccaaactcatcaatgtatctta

SEQ ID NO: 95 - DNA, 2624 bp, synthetic construct
  misc_feature 1..2624: note = P5-CDS intron-CYP4V2-BGH
  source 1..2624: mol_type = other DNA
gagccggatgcgccttcctttcctctccagagcaggctgcccgcccgcggaatcccgcacgtagagcaacctcgcagcaccctcagaacagccccgctggggcgcgccgggctgccgcggtgacctttccgacgcccctgaccccgcatccggaggcggccggaagtgtcgccggcctcctcccggcgcagcctccgggcctccagtgcaatcactacgccctggggcccggaaaccgttttccggtctttcgctttcggctggggcgtggaggccgcggtgctgcgtaggccgggccgggcgcaggaacagccccgtggcgccctctctggccgccgcccgggcgggaaacgtcgttccggggaccgggcgaccccgcagcggggagcgcgccaggtccgcgcggggaagtgggcggtgtgcggccggcaccgcctcgcaccacgcccccgcgggcccgcactttcccggagtgcaccccgcggccgccagccggggcggaattcgccaccatggcggggctctggctggggctcgtgtggcagaagctgctgctgtggggcgcggcgagtgccctttccctggccggcgccagtctggtcctgagtctgctgcagagggtggcgagctacgcgcggaaatggcagcagatgcggcccatccccacggtggcccgcgcctacccactggtgggccacgcgctgctgatgaagccggacgggcgaggtaagtatcaaggttacaagacaggtttaaggagaccaatagaaactgggcttgtcgagacagagaagactcttgcgtttctgataggcacctattggtcttactgacatccactttgcctttctctccacagaattttttcagcagatcattgagtacacagaggaataccgccacatgccgctgctgaagctctgggtcgggccagtgcccatggtggccctttataatgcagaaaatgtggaggtaattttaactagttcaaagcaaattgacaaatcctctatgtacaagtttttagaaccatggcttggcctaggacttcttacaagtactggaaacaaatggcgctccaggagaaagatgttaacacccactttccattttaccattctggaagatttcttagatatcatgaatgaacaagcaaatatattggttaagaaacttgaaaaacacattaaccaagaagcatttaactgctttttttacatcactctttgtgccttagatatcatctgtgaaacagctatggggaagaatattggtgctcaaagtaatgatgattccgagtatgtccgtgcagtttatagaatgagtgagatgatatttcgaagaataaagatgccctggctttggcttgatctctggtaccttatgtttaaagaaggatgggaacacaaaaagagccttcagatcctacatacttttaccaacagtgtcatcgcggaacgggccaatgaaatgaacgccaatgaagactgtagaggtgatggcaggggctctgccccctccaaaaataaacgcagggcctttcttgacttgcttttaagtgtgactgatgacgaagggaacaggctaagtcatgaagatattcgagaagaagttgacaccttcatgtttgaggggcacgatacaactgcagctgcaataaactggtccttatacctgttgggttctaacccagaagtccagaaaaaagtggatcatgaattggatgacgtgtttgggaagtctgaccgtcccgctacagtagaagacctgaagaaacttcggtatctggaatgtgttattaaggagacccttcgcctttttccttctgttcctttatttgcccgtagtgttagtgaagattgtgaagtggcaggttacagagttctaaaaggcactgaagccgtcatcattccctatgcattgcacagagatccgagatacttccccaaccccgaggagttccagcctgagcggttcttccccgagaatgcacaagggcgccatccatatgcctacgtgcccttctctgctggccccaggaactgtataggtcaaaagtttgctgtgatggaagaaaagaccattctttcgtgcatcctgaggcacttttggatagaatccaaccagaaaagagaagagcttggtctagaaggacagttgattcttcgtccaagtaatggcatctggatcaagttgaagaggagaaatgcagatgaacgctaaacgcgtggtttatccgatccaccggatctagataagatatccgatccaccggatctagataactgatcataatcagccataccacatttgtagaggttttacttgctttaaaaaacctcccacacctccccctgaacctgaaacataaaatgaatgcaattggcggccgcctcgagctgtgccttctagttgccagccatctgttgtttgcccctcccccgtgccttccttgaccctggaaggtgccactcccactgtcctttcctaataaaatgaggaaattgcatcgcattgtctgagtaggtgtcattctattctggggggtggggtggggcaggacagcaagggggaggattgggaagacaatagcaggcatgctggggatgcggtgggctctatgg

SEQ ID NO: 96 - DNA, 1092 bp, synthetic construct
  misc_feature 1..1092: note = OPEFS-RdCVF-BGH
  source 1..1092: mol_type = other DNA
gggcagagcgcacatcgcccacagtccccgagaagttggggggaggggtcggcaattgaaccggtgcctagagaaggtggcgcggggtaaactgggaaagtgatgtcgtgtactggctccgcctttttcccgagggtgggggagaaccgtatataagtgcagtagtcgccgtgaacgttctttttcgcaacgggtttgccgccagaacacaggtaagtatcaaggttacaagacaggtttaaggagaccaatagaaactgggcttgtcgagacagagaagactcttgcgtttctgataggcacctattggtcttactgacatccactttgcctttctctccacaggaattccgccaccatggcctccctgttctctggccgcatcctgatccgcaacaatagcgaccaggacgagctggatacggaggctgaggtcagtcgcaggctggagaaccggctggtgctgctgttctttggtgctggggcttgtccacagtgccaggccttcgtgcccatcctcaaggacttcttcgtgcggctcacagatgagttctatgtactgcgggcggctcagctggccctggtgtacgtgtcccaggactccacggaggagcagcaggacctgttcctcaaggacatgccaaagaaatggcttttcctgccctttgaggatgatctgaggaggtgataaacgcgtggtttatccgatccaccggatctagataagatatccgatccaccggatctagataactgatcataatcagccataccacatttgtagaggttttacttgctttaaaaaacctcccacacctccccctgaacctgaaacataaaatgaatgcaattggcggccgcctcgagctgtgccttctagttgccagccatctgttgtttgcccctcccccgtgccttccttgaccctggaaggtgccactcccactgtcctttcctaataaaatgaggaaattgcatcgcattgtctgagtaggtgtcattctattctggggggtggggtggggcaggacagcaagggggaggattgggaagacaatagcaggcatgctggggatgcggtgggctctatgg

SEQ ID NO: 97 - DNA, 1247 bp, synthetic construct
  misc_feature 1..1247: note = P5-RdCVF-BGH
  source 1..1247: mol_type = other DNA
gagccggatgcgccttcctttcctctccagagcaggctgcccgcccgcggaatcccgcacgtagagcaacctcgcagcaccctcagaacagccccgctggggcgcgccgggctgccgcggtgacctttccgacgcccctgaccccgcatccggaggcggccggaagtgtcgccggcctcctcccggcgcagcctccgggcctccagtgcaatcactacgccctggggcccggaaaccgttttccggtctttcgctttcggctggggcgtggaggccgcggtgctgcgtaggccgggccgggcgcaggaacagccccgtggcgccctctctggccgccgcccgggcgggaaacgtcgttccggggaccgggcgaccccgcagcggggagcgcgccaggtccgcgcggggaagtgggcggtgtgcggccggcaccgcctcgcaccacgcccccgcgggcccgcactttcccggagtgcaccccgcggccgccagccggggcggaattccgccaccatggcctccctgttctctggccgcatcctgatccgcaacaatagcgaccaggacgagctggatacggaggctgaggtcagtcgcaggctggagaaccggctggtgctgctgttctttggtgctggggcttgtccacagtgccaggccttcgtgcccatcctcaaggacttcttcgtgcggctcacagatgagttctatgtactgcgggcggctcagctggccctggtgtacgtgtcccaggactccacggaggagcagcaggacctgttcctcaaggacatgccaaagaaatggcttttcctgccctttgaggatgatctgaggaggtgataaacgcgtggtttatccgatccaccggatctagataagatatccgatccaccggatctagataactgatcataatcagccataccacatttgtagaggttttacttgctttaaaaaacctcccacacctccccctgaacctgaaacataaaatgaatgcaattggcggccgcctcgagctgtgccttctagttgccagccatctgttgtttgcccctcccccgtgccttccttgaccctggaaggtgccactcccactgtcctttcctaataaaatgaggaaattgcatcgcattgtctgagtaggtgtcattctattctggggggtggggtggggcaggacagcaagggggaggattgggaagacaatagcaggcatgctggggatgcggtgggctctatgg

SEQ ID NO: 98 - DNA, 2447 bp, synthetic construct
  misc_feature 1..2447: note = P1-RdCVF-BGH
  source 1..2447: mol_type = other DNA
gctgaggtttgagtttctattgatcccctcacctgaatagggaacacagtacccaatacacagtttttcaaccattactccccttccttcctccccctattttagaatccccagtatgtagacaaattgtttacttttatagctgtaattaaccttattatagctcagcctcaaccctttagagaggaggaaactaaagcccatgagacttgcttaaagatactaagtgaacatatttattttttaaagtgttaaagtgattaaacaatgtagacgtgaatgaaataaaaagcgtaagttccccatcttcattcccactccatagagctgatcagtatttttacttgcagacattagtggagccgtagagaaagaaaccttttctccaaaagaaggcattactttacacactccgttctgcaacttgttttgttcacttgctatttcacgtcagcccatgcagatgacttaaaacaaattcaaatggagaaaagccttaggcatgtttttctctgcactaaagaggccctgcaggtggctgtggccaacttatgcagtggcttcgagtgaacgaacgtaattagtaattaagcaaagcgggcatccaggacattcagtttcatcttcctggcactttagtgtttaggaagggcctggcctctcggggagcgacactcctcgcccggccactttgtaagaagcatcgagcgtggaaaaggggctggggtcagcactggggccctctgccgggaagagagactggcggccagcacacgcgtctccccaggctgaaatggggcaccctctcgcggcccttccctcccttcccgggctgggtggcaggtcttggctcttctgcgagtaccccgcggctgcggtctcccggcacccgctgagcagcctcgcccgccttcctctcccacccgcccctgcgtgctctccggggctccggcttcctcggtctggtgcctggtgcgtattttggaaaatacctggctcataaccacctcattgagctcccagtgtcccagtgggccagcggacacacacgggtagctgacttccctaacgtgtccccaaagcctccctggattacagcgcccgctgctccatgtgaccccgcgggagccaggacgcgccccgcctcccggggctgcaagttgcgcagggagcgagcgatgcgcagcagagctgggctccgagccggatgcgccttcctttcctctccagagcaggctgcccgcccgcggaatcccgcacgtagagcaacctcgcagcaccctcagaacagccccgctggggcgcgccgggctgccgcggtgacctttccgacgcccctgaccccgcatccggaggcggccggaagtgtcgccggcctcctcccggcgcagcctccgggcctccagtgcaatcactacgccctggggcccggaaaccgttttccggtctttcgctttcggctggggcgtggaggccgcggtgctgcgtaggccgggccgggcgcaggaacagccccgtggcgccctctctggccgccgcccgggcgggaaacgtcgttccggggaccgggcgaccccgcagcggggagcgcgccaggtccgcgcggggaagtgggcggtgtgcggccggcaccgcctcgcaccacgcccccgcgggcccgcactttcccggagtgcaccccgcggccgccagccggggcggaattccgccaccatggcctccctgttctctggccgcatcctgatccgcaacaatagcgaccaggacgagctggatacggaggctgaggtcagtcgcaggctggagaaccggctggtgctgctgttctttggtgctggggcttgtccacagtgccaggccttcgtgcccatcctcaaggacttcttcgtgcggctcacagatgagttctatgtactgcgggcggctcagctggccctggtgtacgtgtcccaggactccacggaggagcagcaggacctgttcctcaaggacatgccaaagaaatggcttttcctgccctttgaggatgatctgaggaggtgataaacgcgtggtttatccgatccaccggatctagataagatatccgatccaccggatctagataactgatcataatcagccataccacatttgtagaggttttacttgctttaaaaaacctcccacacctccccctgaacctgaaacataaaatgaatgcaattggcggccgcctcgagctgtgccttctagttgccagccatctgttgtttgcccctcccccgtgccttccttgaccctggaaggtgccactcccactgtcctttcctaataaaatgaggaaattgcatcgcattgtctgagtaggtgtcattctattctggggggtggggtggggcaggacagcaagggggaggattgggaagacaatagcaggcatgctggggatgcggtgggctctatgg

SEQ ID NO: 99 - DNA, 1380 bp, synthetic construct
  misc_feature 1..1380: note = P5-intron-RdCVF-BGH
  source 1..1380: mol_type = other DNA
gagccggatgcgccttcctttcctctccagagcaggctgcccgcccgcggaatcccgcacgtagagcaacctcgcagcaccctcagaacagccccgctggggcgcgccgggctgccgcggtgacctttccgacgcccctgaccccgcatccggaggcggccggaagtgtcgccggcctcctcccggcgcagcctccgggcctccagtgcaatcactacgccctggggcccggaaaccgttttccggtctttcgctttcggctggggcgtggaggccgcggtgctgcgtaggccgggccgggcgcaggaacagccccgtggcgccctctctggccgccgcccgggcgggaaacgtcgttccggggaccgggcgaccccgcagcggggagcgcgccaggtccgcgcggggaagtgggcggtgtgcggccggcaccgcctcgcaccacgcccccgcgggcccgcactttcccggagtgcaccccgcggccgccagccggggcggtaagtatcaaggttacaagacaggtttaaggagaccaatagaaactgggcttgtcgagacagagaagactcttgcgtttctgataggcacctattggtcttactgacatccactttgcctttctctccacaggaattccgccaccatggcctccctgttctctggccgcatcctgatccgcaacaatagcgaccaggacgagctggatacggaggctgaggtcagtcgcaggctggagaaccggctggtgctgctgttctttggtgctggggcttgtccacagtgccaggccttcgtgcccatcctcaaggacttcttcgtgcggctcacagatgagttctatgtactgcgggcggctcagctggccctggtgtacgtgtcccaggactccacggaggagcagcaggacctgttcctcaaggacatgccaaagaaatggcttttcctgccctttgaggatgatctgaggaggtgataaacgcgtggtttatccgatccaccggatctagataagatatccgatccaccggatctagataactgatcataatcagccataccacatttgtagaggttttacttgctttaaaaaacctcccacacctccccctgaacctgaaacataaaatgaatgcaattggcggccgcctcgagctgtgccttctagttgccagccatctgttgtttgcccctcccccgtgccttccttgaccctggaaggtgccactcccactgtcctttcctaataaaatgaggaaattgcatcgcattgtctgagtaggtgtcattctattctggggggtggggtggggcaggacagcaagggggaggattgggaagacaatagcaggcatgctggggatgcggtgggctctatgg

SEQ ID NO: 100 - DNA, 1869 bp, synthetic construct
  misc_feature 1..1869: note = P5-intron-RdCVF-WPRE-SV40
  source 1..1869: mol_type = other DNA
gagccggatgcgccttcctttcctctccagagcaggctgcccgcccgcggaatcccgcacgtagagcaacctcgcagcaccctcagaacagccccgctggggcgcgccgggctgccgcggtgacctttccgacgcccctgaccccgcatccggaggcggccggaagtgtcgccggcctcctcccggcgcagcctccgggcctccagtgcaatcactacgccctggggcccggaaaccgttttccggtctttcgctttcggctggggcgtggaggccgcggtgctgcgtaggccgggccgggcgcaggaacagccccgtggcgccctctctggccgccgcccgggcgggaaacgtcgttccggggaccgggcgaccccgcagcggggagcgcgccaggtccgcgcggggaagtgggcggtgtgcggccggcaccgcctcgcaccacgcccccgcgggcccgcactttcccggagtgcaccccgcggccgccagccggggcggtaagtatcaaggttacaagacaggtttaaggagaccaatagaaactgggcttgtcgagacagagaagactcttgcgtttctgataggcacctattggtcttactgacatccactttgcctttctctccacaggaattccgccaccatggcctccctgttctctggccgcatcctgatccgcaacaatagcgaccaggacgagctggatacggaggctgaggtcagtcgcaggctggagaaccggctggtgctgctgttctttggtgctggggcttgtccacagtgccaggccttcgtgcccatcctcaaggacttcttcgtgcggctcacagatgagttctatgtactgcgggcggctcagctggccctggtgtacgtgtcccaggactccacggaggagcagcaggacctgttcctcaaggacatgccaaagaaatggcttttcctgccctttgaggatgatctgaggaggtgaacgcgtggtttatccgatccaccggatctagataagatatccgatccaccggatctagataactgatcataatcagccataccacatttgtagaggttttacttgctttaaaaaacctcccacacctccccctgaacctgaaacataaaatgaatgcaattggcggccgcctcgagaatcaacctctggattacaaaatttgtgaaagattgactggtattcttaactatgttgctccttttacgctatgtggatacgctgctttaatgcctttgtatcatgctattgcttcccgtatggctttcattttctcctccttgtataaatcctggttgctgtctctttatgaggagttgtggcccgttgtcaggcaacgtggcgtggtgtgcactgtgtttgctgacgcaacccccactggttggggcattgccaccacctgtcagctcctttccgggactttcgctttccccctccctattgccacggcggaactcatcgccgcctgccttgcccgctgctggacaggggctcggctgttgggcactgacaattccgtggtgttgtcggggaaatcatcgtcctttccttggctgctcgcctgtgttgccacctggattctgcgcgggacgtccttctgctacgtcccttcggccctcaatccagcggaccttccttcccgcggcctgctgccggctctgcggcctcttccgcgtcttcgccttcgccctcagacgagtcggatctccctttgggccgcctccccgcggtaacaacttgtttattgcagcttataatggttacaaataaagcaatagcatcacaaatttcacaaataaagcatttttttcactgcattctagttgtggtttgtccaaactcatcaatgtatctta

SEQ ID NO: 101 - DNA, 2329 bp, synthetic construct
  misc_feature 1..2329: note = OPEFS-CYP4V2-P2A-RdCVF
  source 1..2329: mol_type = other DNA
gggcagagcgcacatcgcccacagtccccgagaagttggggggaggggtcggcaattgaaccggtgcctagagaaggtggcgcggggtaaactgggaaagtgatgtcgtgtactggctccgcctttttcccgagggtgggggagaaccgtatataagtgcagtagtcgccgtgaacgttctttttcgcaacgggtttgccgccagaacacaggtaagtatcaaggttacaagacaggtttaaggagaccaatagaaactgggcttgtcgagacagagaagactcttgcgtttctgataggcacctattggtcttactgacatccactttgcctttctctccacaggaattccgccaccatggcggggctctggctggggctcgtgtggcagaagctgctgctgtggggcgcggcgagtgccctttccctggccggcgccagtctggtcctgagtctgctgcagagggtggcgagctacgcgcggaaatggcagcagatgcggcccatccccacggtggcccgcgcctacccactggtgggccacgcgctgctgatgaagccggacgggcgagaattttttcagcagatcattgagtacacagaggaataccgccacatgccgctgctgaagctctgggtcgggccagtgcccatggtggccctttataatgcagaaaatgtggaggtaattttaactagttcaaagcaaattgacaaatcctctatgtacaagtttttagaaccatggcttggcctaggacttcttacaagtactggaaacaaatggcgctccaggagaaagatgttaacacccactttccattttaccattctggaagatttcttagatatcatgaatgaacaagcaaatatattggttaagaaacttgaaaaacacattaaccaagaagcatttaactgctttttttacatcactctttgtgccttagatatcatctgtgaaacagctatggggaagaatattggtgctcaaagtaatgatgattccgagtatgtccgtgcagtttatagaatgagtgagatgatatttcgaagaataaagatgccctggctttggcttgatctctggtaccttatgtttaaagaaggatgggaacacaaaaagagccttcagatcctacatacttttaccaacagtgtcatcgcggaacgggccaatgaaatgaacgccaatgaagactgtagaggtgatggcaggggctctgccccctccaaaaataaacgcagggcctttcttgacttgcttttaagtgtgactgatgacgaagggaacaggctaagtcatgaagatattcgagaagaagttgacaccttcatgtttgaggggcacgatacaactgcagctgcaataaactggtccttatacctgttgggttctaacccagaagtccagaaaaaagtggatcatgaattggatgacgtgtttgggaagtctgaccgtcccgctacagtagaagacctgaagaaacttcggtatctggaatgtgttattaaggagacccttcgcctttttccttctgttcctttatttgcccgtagtgttagtgaagattgtgaagtggcaggttacagagttctaaaaggcactgaagccgtcatcattccctatgcattgcacagagatccgagatacttccccaaccccgaggagttccagcctgagcggttcttccccgagaatgcacaagggcgccatccatatgcctacgtgcccttctctgctggccccaggaactgtataggtcaaaagtttgctgtgatggaagaaaagaccattctttcgtgcatcctgaggcacttttggatagaatccaaccagaaaagagaagagcttggtctagaaggacagttgattcttcgtccaagtaatggcatctggatcaagttgaagaggagaaatgcagatgaacgcggaagcggagctactaacttcagcctgctgaagcaggctggagacgtggaggagaaccctggacctatggcctccctgttctctggccgcatcctgatccgcaacaatagcgaccaggacgagctggatacggaggctgaggtcagtcgcaggctggagaaccggctggtgctgctgttctttggtgctggggcttgtccacagtgccaggccttcgtgcccatcctcaaggacttcttcgtgcggctcacagatgagttctatgtactgcgggcggctcagctggccctggtgtacgtgtcccaggactccacggaggagcagcaggacctgttcctcaaggacatgccaaagaaatggcttttcctgccctttgaggatgatctgaggaggtga

SEQ ID NO: 102 - DNA, 2484 bp, synthetic construct
  misc_feature 1..2484: note = P5-CYP4V2-P2A-RdCVF
  source 1..2484: mol_type = other DNA
gagccggatgcgccttcctttcctctccagagcaggctgcccgcccgcggaatcccgcacgtagagcaacctcgcagcaccctcagaacagccccgctggggcgcgccgggctgccgcggtgacctttccgacgcccctgaccccgcatccggaggcggccggaagtgtcgccggcctcctcccggcgcagcctccgggcctccagtgcaatcactacgccctggggcccggaaaccgttttccggtctttcgctttcggctggggcgtggaggccgcggtgctgcgtaggccgggccgggcgcaggaacagccccgtggcgccctctctggccgccgcccgggcgggaaacgtcgttccggggaccgggcgaccccgcagcggggagcgcgccaggtccgcgcggggaagtgggcggtgtgcggccggcaccgcctcgcaccacgcccccgcgggcccgcactttcccggagtgcaccccgcggccgccagccggggcggaattccgccaccatggcggggctctggctggggctcgtgtggcagaagctgctgctgtggggcgcggcgagtgccctttccctggccggcgccagtctggtcctgagtctgctgcagagggtggcgagctacgcgcggaaatggcagcagatgcggcccatccccacggtggcccgcgcctacccactggtgggccacgcgctgctgatgaagccggacgggcgagaattttttcagcagatcattgagtacacagaggaataccgccacatgccgctgctgaagctctgggtcgggccagtgcccatggtggccctttataatgcagaaaatgtggaggtaattttaactagttcaaagcaaattgacaaatcctctatgtacaagtttttagaaccatggcttggcctaggacttcttacaagtactggaaacaaatggcgctccaggagaaagatgttaacacccactttccattttaccattctggaagatttcttagatatcatgaatgaacaagcaaatatattggttaagaaacttgaaaaacacattaaccaagaagcatttaactgctttttttacatcactctttgtgccttagatatcatctgtgaaacagctatggggaagaatattggtgctcaaagtaatgatgattccgagtatgtccgtgcagtttatagaatgagtgagatgatatttcgaagaataaagatgccctggctttggcttgatctctggtaccttatgtttaaagaaggatgggaacacaaaaagagccttcagatcctacatacttttaccaacagtgtcatcgcggaacgggccaatgaaatgaacgccaatgaagactgtagaggtgatggcaggggctctgccccctccaaaaataaacgcagggcctttcttgacttgcttttaagtgtgactgatgacgaagggaacaggctaagtcatgaagatattcgagaagaagttgacaccttcatgtttgaggggcacgatacaactgcagctgcaataaactggtccttatacctgttgggttctaacccagaagtccagaaaaaagtggatcatgaattggatgacgtgtttgggaagtctgaccgtcccgctacagtagaagacctgaagaaacttcggtatctggaatgtgttattaaggagacccttcgcctttttccttctgttcctttatttgcccgtagtgttagtgaagattgtgaagtggcaggttacagagttctaaaaggcactgaagccgtcatcattccctatgcattgcacagagatccgagatacttccccaaccccgaggagttccagcctgagcggttcttccccgagaatgcacaagggcgccatccatatgcctacgtgcccttctctgctggccccaggaactgtataggtcaaaagtttgctgtgatggaagaaaagaccattctttcgtgcatcctgaggcacttttggatagaatccaaccagaaaagagaagagcttggtctagaaggacagttgattcttcgtccaagtaatggcatctggatcaagttgaagaggagaaatgcagatgaacgcggaagcggagctactaacttcagcctgctgaagcaggctggagacgtggaggagaaccctggacctatggcctccctgttctctggccgcatcctgatccgcaacaatagcgaccaggacgagctggatacggaggctgaggtcagtcgcaggctggagaaccggctggtgctgctgttctttggtgctggggcttgtccacagtgccaggccttcgtgcccatcctcaaggacttcttcgtgcggctcacagatgagttctatgtactgcgggcggctcagctggccctggtgtacgtgtcccaggactccacggaggagcagcaggacctgttcctcaaggacatgccaaagaaatggcttttcctgccctttgaggatgatctgaggaggtga

SEQ ID NO: 103 - DNA, 3984 bp, synthetic construct
  misc_feature 1..3984: note = Pf-CYP4V2-P2A-RdCVF
  source 1..3984: mol_type = other DNA
acccacctcatcctgcacctgtcactgcgtgggaccctgtgctccaggcaggggcacctcactgccccctgagctcattttacccctcctggctctgcagcatttctgaccatttctgcccaggccgagactcactgctgcccagagcaatctcccttctctccttctggaggggaggggttgtatgttacccgcctggttttatccacagaggttagcagagactgatacagacaaaccctttttctttctaattttagattcaagagcacatgtgcaggtttgttaaatttgcctgacgctgaggtttgagtttctattgatcccctcacctgaatagggaacacagtacccaatacacagtttttcaaccattactccccttccttcctccccctattttagaatccccagtatgtagacaaattgtttacttttatagctgtaattaaccttattatagctcagcctcaaccctttagagaggaggaaactaaagcccatgagacttgcttaaagatactaagtgaacatatttattttttaaagtgttaaagtgattaaacaatgtagacgtgaatgaaataaaaagcgtaagttccccatcttcattcccactccatagagctgatcagtatttttacttgcagacattagtggagccgtagagaaagaaaccttttctccaaaagaaggcattactttacacactccgttctgcaacttgttttgttcacttgctatttcacgtcagcccatgcagatgacttaaaacaaattcaaatggagaaaagccttaggcatgtttttctctgcactaaagaggccctgcaggtggctgtggccaacttatgcagtggcttcgagtgaacgaacgtaattagtaattaagcaaagcgggcatccaggacattcagtttcatcttcctggcactttagtgtttaggaagggcctggcctctcggggagcgacactcctcgcccggccactttgtaagaagcatcgagcgtggaaaaggggctggggtcagcactggggccctctgccgggaagagagactggcggccagcacacgcgtctccccaggctgaaatggggcaccctctcgcggcccttccctcccttcccgggctgggtggcaggtcttggctcttctgcgagtaccccgcggctgcggtctcccggcacccgctgagcagcctcgcccgccttcctctcccacccgcccctgcgtgctctccggggctccggcttcctcggtctggtgcctggtgcgtattttggaaaatacctggctcataaccacctcattgagctcccagtgtcccagtgggccagcggacacacacgggtagctgacttccctaacgtgtccccaaagcctccctggattacagcgcccgctgctccatgtgaccccgcgggagccaggacgcgccccgcctcccggggctgcaagttgcgcagggagcgagcgatgcgcagcagagctgggctccgagccggatgcgccttcctttcctctccagagcaggctgcccgcccgcggaatcccgcacgtagagcaacctcgcagcaccctcagaacagccccgctggggcgcgccgggctgccgcggtgacctttccgacgcccctgaccccgcatccggaggcggccggaagtgtcgccggcctcctcccggcgcagcctccgggcctccagtgcaatcactacgccctggggcccggaaaccgttttccggtctttcgctttcggctggggcgtggaggccgcggtgctgcgtaggccgggccgggcgcaggaacagccccgtggcgccctctctggccgccgcccgggcgggaaacgtcgttccggggaccgggcgaccccgcagcggggagcgcgccaggtccgcgcggggaagtgggcggtgtgcggccggcaccgcctcgcaccacgcccccgcgggcccgcactttcccggagtgcaccccgcggccgccagccggggcggaattccgccaccatggcggggctctggctggggctcgtgtggcagaagctgctgctgtggggcgcggcgagtgccctttccctggccggcgccagtctggtcctgagtctgctgcagagggtggcgagctacgcgcggaaatggcagcagatgcggcccatccccacggtggcccgcgcctacccactggtgggccacgcgctgctgatgaagccggacgggcgagaattttttcagcagatcattgagtacacagaggaataccgccacatgccgctgctgaagctctgggtcgggccagtgcccatggtggccctttataatgcagaaaatgtggaggtaattttaactagttcaaagcaaattgacaaatcctctatgtacaagtttttagaaccatggcttggcctaggacttcttacaagtactggaaacaaatggcgctccaggagaaagatgttaacacccactttccattttaccattctggaagatttcttagatatcatgaatgaacaagcaaatatattggttaagaaacttgaaaaacacattaaccaagaagcatttaactgctttttttacatcactctttgtgccttagatatcatctgtgaaacagctatggggaagaatattggtgctcaaagtaatgatgattccgagtatgtccgtgcagtttatagaatgagtgagatgatatttcgaagaataaagatgccctggctttggcttgatctctggtaccttatgtttaaagaaggatgggaacacaaaaagagccttcagatcctacatacttttaccaacagtgtcatcgcggaacgggccaatgaaatgaacgccaatgaagactgtagaggtgatggcaggggctctgccccctccaaaaataaacgcagggcctttcttgacttgcttttaagtgtgactgatgacgaagggaacaggctaagtcatgaagatattcgagaagaagttgacaccttcatgtttgaggggcacgatacaactgcagctgcaataaactggtccttatacctgttgggttctaacccagaagtccagaaaaaagtggatcatgaattggatgacgtgtttgggaagtctgaccgtcccgctacagtagaagacctgaagaaacttcggtatctggaatgtgttattaaggagacccttcgcctttttccttctgttcctttatttgcccgtagtgttagtgaagattgtgaagtggcaggttacagagttctaaaaggcactgaagccgtcatcattccctatgcattgcacagagatccgagatacttccccaaccccgaggagttccagcctgagcggttcttccccgagaatgcacaagggcgccatccatatgcctacgtgcccttctctgctggccccaggaactgtataggtcaaaagtttgctgtgatggaagaaaagaccattctttcgtgcatcctgaggcacttttggatagaatccaaccagaaaagagaagagcttggtctagaaggacagttgattcttcgtccaagtaatggcatctggatcaagttgaagaggagaaatgcagatgaacgcggaagcggagctactaacttcagcctgctgaagcaggctggagacgtggaggagaaccctggacctatggcctccctgttctctggccgcatcctgatccgcaacaatagcgaccaggacgagctggatacggaggctgaggtcagtcgcaggctggagaaccggctggtgctgctgttctttggtgctggggcttgtccacagtgccaggccttcgtgcccatcctcaaggacttcttcgtgcggctcacagatgagttctatgtactgcgggcggctcagctggccctggtgtacgtgtcccaggactccacggaggagcagcaggacctgttcctcaaggacatgccaaagaaatggcttttcctgccctttgaggatgatctgaggaggtga

SEQ ID NO: 104 - DNA, 3146 bp, synthetic construct
  misc_feature 1..3146: note = EF1a-CYP4V2-P2A-RdCVF
  source 1..3146: mol_type = other DNA
gctccggtgcccgtcagtgggcagagcgcacatcgcccacagtccccgagaagttggggggaggggtcggcaattgaaccggtgcctagagaaggtggcgcggggtaaactgggaaagtgatgtcgtgtactggctccgcctttttcccgagggtgggggagaaccgtatataagtgcagtagtcgccgtgaacgttctttttcgcaacgggtttgccgccagaacacaggtaagtgccgtgtgtggttcccgcgggcctggcctctttacgggttatggcccttgcgtgccttgaattacttccacctggctccagtacgtgattcttgatcccgagctggagccaggggcgggccttgcgctttaggagccccttcgcctcgtgcttgagttgaggcctggcctgggcgctggggccgccgcgtgcgaatctggtggcaccttcgcgcctgtctcgctgctttcgataagtctctagccatttaaaatttttgatgacctgctgcgacgctttttttctggcaagatagtcttgtaaatgcgggccaggatctgcacactggtatttcggtttttgggcccgcggccggcgacggggcccgtgcgtcccagcgcacatgttcggcgaggcggggcctgcgagcgcggccaccgagaatcggacgggggtagtctcaagctggccggcctgctctggtgcctggcctcgcgccgccgtgtatcgccccgccctgggcggcaaggctggcccggtcggcaccagttgcgtgagcggaaagatggccgcttcccggccctgctccagggggctcaaaatggaggacgcggcgctcgggagagcgggcgggtgagtcacccacacaaaggaaaagggcctttccgtcctcagccgtcgcttcatgtgactccacggagtaccgggcgccgtccaggcacctcgattagttctggagcttttggagtacgtcgtctttaggttggggggaggggttttatgcgatggagtttccccacactgagtgggtggagactgaagttaggccagcttggcacttgatgtaattctccttggaatttggcctttttgagtttggatcttggttcattctcaagcctcagacagtggttcaaagtttttttcttccatttcaggtgtcgtgagaattccgccaccatggcggggctctggctggggctcgtgtggcagaagctgctgctgtggggcgcggcgagtgccctttccctggccggcgccagtctggtcctgagtctgctgcagagggtggcgagctacgcgcggaaatggcagcagatgcggcccatccccacggtggcccgcgcctacccactggtgggccacgcgctgctgatgaagccggacgggcgagaattttttcagcagatcattgagtacacagaggaataccgccacatgccgctgctgaagctctgggtcgggccagtgcccatggtggccctttataatgcagaaaatgtggaggtaattttaactagttcaaagcaaattgacaaatcctctatgtacaagtttttagaaccatggcttggcctaggacttcttacaagtactggaaacaaatggcgctccaggagaaagatgttaacacccactttccattttaccattctggaagatttcttagatatcatgaatgaacaagcaaatatattggttaagaaacttgaaaaacacattaaccaagaagcatttaactgctttttttacatcactctttgtgccttagatatcatctgtgaaacagctatggggaagaatattggtgctcaaagtaatgatgattccgagtatgtccgtgcagtttatagaatgagtgagatgatatttcgaagaataaagatgccctggctttggcttgatctctggtaccttatgtttaaagaaggatgggaacacaaaaagagccttcagatcctacatacttttaccaacagtgtcatcgcggaacgggccaatgaaatgaacgccaatgaagactgtagaggtgatggcaggggctctgccccctccaaaaataaacgcagggcctttcttgacttgcttttaagtgtgactgatgacgaagggaacaggctaagtcatgaagatattcgagaagaagttgacaccttcatgtttgaggggcacgatacaactgcagctgcaataaactggtccttatacctgttgggttctaacccagaagtccagaaaaaagtggatcatgaattggatgacgtgtttgggaagtctgaccgtcccgctacagtagaagacctgaagaaacttcggtatctggaatgtgttattaaggagacccttcgcctttttccttctgttcctttatttgcccgtagtgttagtgaagattgtgaagtggcaggttacagagttctaaaaggcactgaagccgtcatcattccctatgcattgcacagagatccgagatacttccccaaccccgaggagttccagcctgagcggttcttccccgagaatgcacaagggcgccatccatatgcctacgtgcccttctctgctggccccaggaactgtataggtcaaaagtttgctgtgatggaagaaaagaccattctttcgtgcatcctgaggcacttttggatagaatccaaccagaaaagagaagagcttggtctagaaggacagttgattcttcgtccaagtaatggcatctggatcaagttgaagaggagaaatgcagatgaacgcggaagcggagctactaacttcagcctgctgaagcaggctggagacgtggaggagaaccctggacctatggcctccctgttctctggccgcatcctgatccgcaacaatagcgaccaggacgagctggatacggaggctgaggtcagtcgcaggctggagaaccggctggtgctgctgttctttggtgctggggcttgtccacagtgccaggccttcgtgcccatcctcaaggacttcttcgtgcggctcacagatgagttctatgtactgcgggcggctcagctggccctggtgtacgtgtcccaggactccacggaggagcagcaggacctgttcctcaaggacatgccaaagaaatggcttttcctgccctttgaggatgatctgaggaggtga

SEQ ID NO: 105 - DNA, 2941 bp, synthetic construct
  misc_feature 1..2941: note = CAG-CYP4V2-T2A-RdCVF
  source 1..2941: mol_type = other DNA
ccattgacgtcaataatgacgtatgttcccatagtaacgccaatagggactttccattgacgtcaatgggtggagtatttacggtaaactgcccacttggcagtacatcaagtgtatcatatgccaagtacgccccctattgacgtcaatgacggtaaatggcccgcctggcattatgcccagtacatgaccttatgggactttcctacttggcagtacatctacgtattagtcatcgctattaccatggtcgaggtgagccccacgttctgcttcactctccccatctcccccccctccccacccccaattttgtatttatttattttttaattattttgtgcagcgatgggggcggggggggggggggggcgcgcgccaggcggggcggggcggggcgaggggcggggcggggcgaggcggagaggtgcggcggcagccaatcagagcggcgcgctccgaaagtttccttttatggcgaggcggcggcggcggcggccctataaaaagcgaagcgcgcggcgggcgggagtcgctgcgacgctgccttcgccccgtgccccgctccgccgccgcctcgcgccgcccgccccggctctgactgaccgcgttactcccacaggtgagcgggcgggacggcccttctcctccgggctgtaattagcgcttggtttaatgacggcttgtttcttttctgtggctgcgtgaaagccttgaggggctccgggagggccctttgtgcggggggagcggctcggggctgtccgcggggggacggctgccttcgggggggacggggcagggcggggttcggcttctggcgtgtgaccggcggctctagagcctctgctaaccatgttcatgccttcttctttttcctacagctcctgggcaacgtgctggttattgtgctgtctcatcattttggcaaagaattggatcggtaccgaggagatctgccgccgcgatcgccatggcggggctctggctggggctcgtgtggcagaagctgctgctgtggggcgcggcgagtgccctttccctggccggcgccagtctggtcctgagtctgctgcagagggtggcgagctacgcgcggaaatggcagcagatgcggcccatccccacggtggcccgcgcctacccactggtgggccacgcgctgctgatgaagccggacgggcgagaattttttcagcagatcattgagtacacagaggaataccgccacatgccgctgctgaagctctgggtcgggccagtgcccatggtggccctttataatgcagaaaatgtggaggtaattttaactagttcaaagcaaattgacaaatcctctatgtacaagtttttagaaccatggcttggcctaggacttcttacaagtactggaaacaaatggcgctccaggagaaagatgttaacacccactttccattttaccattctggaagatttcttagatatcatgaatgaacaagcaaatatattggttaagaaacttgaaaaacacattaaccaagaagcatttaactgctttttttacatcactctttgtgccttagatatcatctgtgaaacagctatggggaagaatattggtgctcaaagtaatgatgattccgagtatgtccgtgcagtttatagaatgagtgagatgatatttcgaagaataaagatgccctggctttggcttgatctctggtaccttatgtttaaagaaggatgggaacacaaaaagagccttcagatcctacatacttttaccaacagtgtcatcgcggaacgggccaatgaaatgaacgccaatgaagactgtagaggtgatggcaggggctctgccccctccaaaaataaacgcagggcctttcttgacttgcttttaagtgtgactgatgacgaagggaacaggctaagtcatgaagatattcgagaagaagttgacaccttcatgtttgaggggcacgatacaactgcagctgcaataaactggtccttatacctgttgggttctaacccagaagtccagaaaaaagtggatcatgaattggatgacgtgtttgggaagtctgaccgtcccgctacagtagaagacctgaagaaacttcggtatctggaatgtgttattaaggagacccttcgcctttttccttctgttcctttatttgcccgtagtgttagtgaagattgtgaagtggcaggttacagagttctaaaaggcactgaagccgtcatcattccctatgcattgcacagagatccgagatacttccccaaccccgaggagttccagcctgagcggttcttccccgagaatgcacaagggcgccatccatatgcctacgtgcccttctctgctggccccaggaactgtataggtcaaaagtttgctgtgatggaagaaaagaccattctttcgtgcatcctgaggcacttttggatagaatccaaccagaaaagagaagagcttggtctagaaggacagttgattcttcgtccaagtaatggcatctggatcaagttgaagaggagaaatgcagatgaacgcggaagcggagagggcagaggaagtctgctaacatgcggtgacgtcgaggagaatcctggacctatggcctccctgttctctggccgcatcctgatccgcaacaatagcgaccaggacgagctggatacggaggctgaggtcagtcgcaggctggagaaccggctggtgctgctgttctttggtgctggggcttgtccacagtgccaggccttcgtgcccatcctcaaggacttcttcgtgcggctcacagatgagttctatgtactgcgggcggctcagctggccctggtgtacgtgtcccaggactccacggaggagcagcaggacctgttcctcaaggacatgccaaagaaatggcttttcctgccctttgaggatgatctgaggaggtga

SEQ ID NO: 106 - DNA, 2733 bp, synthetic construct
  misc_feature 1..2733: note = OPEFS-CYP4V2-P2A-RdCVF-BGH
  source 1..2733: mol_type = other DNA
gggcagagcgcacatcgcccacagtccccgagaagttggggggaggggtcggcaattgaaccggtgcctagagaaggtggcgcggggtaaactgggaaagtgatgtcgtgtactggctccgcctttttcccgagggtgggggagaaccgtatataagtgcagtagtcgccgtgaacgttctttttcgcaacgggtttgccgccagaacacaggtaagtatcaaggttacaagacaggtttaaggagaccaatagaaactgggcttgtcgagacagagaagactcttgcgtttctgataggcacctattggtcttactgacatccactttgcctttctctccacaggaattccgccaccatggcggggctctggctggggctcgtgtggcagaagctgctgctgtggggcgcggcgagtgccctttccctggccggcgccagtctggtcctgagtctgctgcagagggtggcgagctacgcgcggaaatggcagcagatgcggcccatccccacggtggcccgcgcctacccactggtgggccacgcgctgctgatgaagccggacgggcgagaattttttcagcagatcattgagtacacagaggaataccgccacatgccgctgctgaagctctgggtcgggccagtgcccatggtggccctttataatgcagaaaatgtggaggtaattttaactagttcaaagcaaattgacaaatcctctatgtacaagtttttagaaccatggcttggcctaggacttcttacaagtactggaaacaaatggcgctccaggagaaagatgttaacacccactttccattttaccattctggaagatttcttagatatcatgaatgaacaagcaaatatattggttaagaaacttgaaaaacacattaaccaagaagcatttaactgctttttttacatcactctttgtgccttagatatcatctgtgaaacagctatggggaagaatattggtgctcaaagtaatgatgattccgagtatgtccgtgcagtttatagaatgagtgagatgatatttcgaagaataaagatgccctggctttggcttgatctctggtaccttatgtttaaagaaggatgggaacacaaaaagagccttcagatcctacatacttttaccaacagtgtcatcgcggaacgggccaatgaaatgaacgccaatgaagactgtagaggtgatggcaggggctctgccccctccaaaaataaacgcagggcctttcttgacttgcttttaagtgtgactgatgacgaagggaacaggctaagtcatgaagatattcgagaagaagttgacaccttcatgtttgaggggcacgatacaactgcagctgcaataaactggtccttatacctgttgggttctaacccagaagtccagaaaaaagtggatcatgaattggatgacgtgtttgggaagtctgaccgtcccgctacagtagaagacctgaagaaacttcggtatctggaatgtgttattaaggagacccttcgcctttttccttctgttcctttatttgcccgtagtgttagtgaagattgtgaagtggcaggttacagagttctaaaaggcactgaagccgtcatcattccctatgcattgcacagagatccgagatacttccccaaccccgaggagttccagcctgagcggttcttccccgagaatgcacaagggcgccatccatatgcctacgtgcccttctctgctggccccaggaactgtataggtcaaaagtttgctgtgatggaagaaaagaccattctttcgtgcatcctgaggcacttttggatagaatccaaccagaaaagagaagagcttggtctagaaggacagttgattcttcgtccaagtaatggcatctggatcaagttgaagaggagaaatgcagatgaacgcggaagcggagctactaacttcagcctgctgaagcaggctggagacgtggaggagaaccctggacctatggcctccctgttctctggccgcatcctgatccgcaacaatagcgaccaggacgagctggatacggaggctgaggtcagtcgcaggctggagaaccggctggtgctgctgttctttggtgctggggcttgtccacagtgccaggccttcgtgcccatcctcaaggacttcttcgtgcggctcacagatgagttctatgtactgcgggcggctcagctggccctggtgtacgtgtcccaggactccacggaggagcagcaggacctgttcctcaaggacatgccaaagaaatggcttttcctgccctttgaggatgatctgaggaggtgataaacgcgtggtttatccgatccaccggatctagataagatatccgatccaccggatctagataactgatcataatcagccataccacatttgtagaggttttacttgctttaaaaaacctcccacacctccccctgaacctgaaacataaaatgaatgcaattggcggccgcctcgagctgtgccttctagttgccagccatctgttgtttgcccctcccccgtgccttccttgaccctggaaggtgccactcccactgtcctttcctaataaaatgaggaaattgcatcgcattgtctgagtaggtgtcattctattctggggggtggggtggggcaggacagcaagggggaggattgggaagacaatagcaggcatgctggggatgcggtgggctctatgg

SEQ ID NO: 107 - DNA, 2888 bp, synthetic construct
  misc_feature 1..2888: note = P5-CYP4V2-P2A-RdCVF-BGH
  source 1..2888: mol_type = other DNA
gagccggatgcgccttcctttcctctccagagcaggctgcccgcccgcggaatcccgcacgtagagcaacctcgcagcaccctcagaacagccccgctggggcgcgccgggctgccgcggtgacctttccgacgcccctgaccccgcatccggaggcggccggaagtgtcgccggcctcctcccggcgcagcctccgggcctccagtgcaatcactacgccctggggcccggaaaccgttttccggtctttcgctttcggctggggcgtggaggccgcggtgctgcgtaggccgggccgggcgcaggaacagccccgtggcgccctctctggccgccgcccgggcgggaaacgtcgttccggggaccgggcgaccccgcagcggggagcgcgccaggtccgcgcggggaagtgggcggtgtgcggccggcaccgcctcgcaccacgcccccgcgggcccgcactttcccggagtgcaccccgcggccgccagccggggcggaattccgccaccatggcggggctctggctggggctcgtgtggcagaagctgctgctgtggggcgcggcgagtgccctttccctggccggcgccagtctggtcctgagtctgctgcagagggtggcgagctacgcgcggaaatggcagcagatgcggcccatccccacggtggcccgcgcctacccactggtgggccacgcgctgctgatgaagccggacgggcgagaattttttcagcagatcattgagtacacagaggaataccgccacatgccgctgctgaagctctgggtcgggccagtgcccatggtggccctttataatgcagaaaatgtggaggtaattttaactagttcaaagcaaattgacaaatcctctatgtacaagtttttagaaccatggcttggcctaggacttcttacaagtactggaaacaaatggcgctccaggagaaagatgttaacacccactttccattttaccattctggaagatttcttagatatcatgaatgaacaagcaaatatattggttaagaaacttgaaaaacacattaaccaagaagcatttaactgctttttttacatcactctttgtgccttagatatcatctgtgaaacagctatggggaagaatattggtgctcaaagtaatgatgattccgagtatgtccgtgcagtttatagaatgagtgagatgatatttcgaagaataaagatgccctggctttggcttgatctctggtaccttatgtttaaagaaggatgggaacacaaaaagagccttcagatcctacatacttttaccaacagtgtcatcgcggaacgggccaatgaaatgaacgccaatgaagactgtagaggtgatggcaggggctctgccccctccaaaaataaacgcagggcctttcttgacttgcttttaagtgtgactgatgacgaagggaacaggctaagtcatgaagatattcgagaagaagttgacaccttcatgtttgaggggcacgatacaactgcagctgcaataaactggtccttatacctgttgggttctaacccagaagtccagaaaaaagtggatcatgaattggatgacgtgtttgggaagtctgaccgtcccgctacagtagaagacctgaagaaacttcggtatctggaatgtgttattaaggagacccttcgcctttttccttctgttcctttatttgcccgtagtgttagtgaagattgtgaagtggcaggttacagagttctaaaaggcactgaagccgtcatcattccctatgcattgcacagagatccgagatacttccccaaccccgaggagttccagcctgagcggttcttccccgagaatgcacaagggcgccatccatatgcctacgtgcccttctctgctggccccaggaactgtataggtcaaaagtttgctgtgatggaagaaaagaccattctttcgtgcatcctgaggcacttttggatagaatccaaccagaaaagagaagagcttggtctagaaggacagttgattcttcgtccaagtaatggcatctggatcaagttgaagaggagaaatgcagatgaacgcggaagcggagctactaacttcagcctgctgaagcaggctggagacgtggaggagaaccctggacctatggcctccctgttctctggccgcatcctgatccgcaacaatagcgaccaggacgagctggatacggaggctgaggtcagtcgcaggctggagaaccggctggtgctgctgttctttggtgctggggcttgtccacagtgccaggccttcgtgcccatcctcaaggacttcttcgtgcggctcacagatgagttctatgtactgcgggcggctcagctggccctggtgtacgtgtcccaggactccacggaggagcagcaggacctgttcctcaaggacatgccaaagaaatggcttttcctgccctttgaggatgatctgaggaggtgataaacgcgtggtttatccgatccaccggatctagataagatatccgatccaccggatctagataactgatcataatcagccataccacatttgtagaggttttacttgctttaaaaaacctcccacacctccccctgaacctgaaacataaaatgaatgcaattggcggccgcctcgagctgtgccttctagttgccagccatctgttgtttgcccctcccccgtgccttccttgaccctggaaggtgccactcccactgtcctttcctaataaaatgaggaaattgcatcgcattgtctgagtaggtgtcattctattctggggggtggggtggggcaggacagcaagggggaggattgggaagacaatagcaggcatgctggggatgcggtgggctctatgg

SEQ ID NO: 108 - DNA, 4088 bp, synthetic construct
  misc_feature 1..4088: note = P1-CYP4V2-P2A-RdCVF-BGH
  source 1..4088: mol_type = other DNA
gctgaggtttgagtttctattgatcccctcacctgaatagggaacacagtacccaatacacagtttttcaaccattactccccttccttcctccccctattttagaatccccagtatgtagacaaattgtttacttttatagctgtaattaaccttattatagctcagcctcaaccctttagagaggaggaaactaaagcccatgagacttgcttaaagatactaagtgaacatatttattttttaaagtgttaaagtgattaaacaatgtagacgtgaatgaaataaaaagcgtaagttccccatcttcattcccactccatagagctgatcagtatttttacttgcagacattagtggagccgtagagaaagaaaccttttctccaaaagaaggcattactttacacactccgttctgcaacttgttttgttcacttgctatttcacgtcagcccatgcagatgacttaaaacaaattcaaatggagaaaagccttaggcatgtttttctctgcactaaagaggccctgcaggtggctgtggccaacttatgcagtggcttcgagtgaacgaacgtaattagtaattaagcaaagcgggcatccaggacattcagtttcatcttcctggcactttagtgtttaggaagggcctggcctctcggggagcgacactcctcgcccggccactttgtaagaagcatcgagcgtggaaaaggggctggggtcagcactggggccctctgccgggaagagagactggcggccagcacacgcgtctccccaggctgaaatggggcaccctctcgcggcccttccctcccttcccgggctgggtggcaggtcttggctcttctgcgagtaccccgcggctgcggtctcccggcacccgctgagcagcctcgcccgccttcctctcccacccgcccctgcgtgctctccggggctccggcttcctcggtctggtgcctggtgcgtattttggaaaatacctggctcataaccacctcattgagctcccagtgtcccagtgggccagcggacacacacgggtagctgacttccctaacgtgtccccaaagcctccctggattacagcgcccgctgctccatgtgaccccgcgggagccaggacgcgccccgcctcccggggctgcaagttgcgcagggagcgagcgatgcgcagcagagctgggctccgagccggatgcgccttcctttcctctccagagcaggctgcccgcccgcggaatcccgcacgtagagcaacctcgcagcaccctcagaacagccccgctggggcgcgccgggctgccgcggtgacctttccgacgcccctgaccccgcatccggaggcggccggaagtgtcgccggcctcctcccggcgcagcctccgggcctccagtgcaatcactacgccctggggcccggaaaccgttttccggtctttcgctttcggctggggcgtggaggccgcggtgctgcgtaggccgggccgggcgcaggaacagccccgtggcgccctctctggccgccgcccgggcgggaaacgtcgttccggggaccgggcgaccccgcagcggggagcgcgccaggtccgcgcggggaagtgggcggtgtgcggccggcaccgcctcgcaccacgcccccgcgggcccgcactttcccggagtgcaccccgcggccgccagccggggcggaattccgccaccatggcggggctctggctggggctcgtgtggcagaagctgctgctgtggggcgcggcgagtgccctttccctggccggcgccagtctggtcctgagtctgctgcagagggtggcgagctacgcgcggaaatggcagcagatgcggcccatccccacggtggcccgcgcctacccactggtgggccacgcgctgctgatgaagccggacgggcgagaattttttcagcagatcattgagtacacagaggaataccgccacatgccgctgctgaagctctgggtcgggccagtgcccatggtggccctttataatgcagaaaatgtggaggtaattttaactagttcaaagcaaattgacaaatcctctatgtacaagtttttagaaccatggcttggcctaggacttcttacaagtactggaaacaaatggcgctccaggagaaagatgttaacacccactttccattttaccattctggaagatttcttagatatcatgaatgaacaagcaaatatattggttaagaaacttgaaaaacacattaaccaagaagcatttaactgctttttttacatcactctttgtgccttagatatcatctgtgaaacagctatggggaagaatattggtgctcaaagtaatgatgattccgagtatgtccgtgcagtttatagaatgagtgagatgatatttcgaagaataaagatgccctggctttggcttgatctctggtaccttatgtttaaagaaggatgggaacacaaaaagagccttcagatcctacatacttttaccaacagtgtcatcgcggaacgggccaatgaaatgaacgccaatgaagactgtagaggtgatggcaggggctctgccccctccaaaaataaacgcagggcctttcttgacttgcttttaagtgtgactgatgacgaagggaacaggctaagtcatgaagatattcgagaagaagttgacaccttcatgtttgaggggcacgatacaactgcagctgcaataaactggtccttatacctgttgggttctaacccagaagtccagaaaaaagtggatcatgaattggatgacgtgtttgggaagtctgaccgtcccgctacagtagaagacctgaagaaacttcggtatctggaatgtgttattaaggagacccttcgcctttttccttctgttcctttatttgcccgtagtgttagtgaagattgtgaagtggcaggttacagagttctaaaaggcactgaagccgtcatcattccctatgcattgcacagagatccgagatacttccccaaccccgaggagttccagcctgagcggttcttccccgagaatgcacaagggcgccatccatatgcctacgtgcccttctctgctggccccaggaactgtataggtcaaaagtttgctgtgatggaagaaaagaccattctttcgtgcatcctgaggcacttttggatagaatccaaccagaaaagagaagagcttggtctagaaggacagttgattcttcgtccaagtaatggcatctggatcaagttgaagaggagaaatgcagatgaacgcggaagcggagctactaacttcagcctgctgaagcaggctggagacgtggaggagaaccctggacctatggcctccctgttctctggccgcatcctgatccgcaacaatagcgaccaggacgagctggatacggaggctgaggtcagtcgcaggctggagaaccggctggtgctgctgttctttggtgctggggcttgtccacagtgccaggccttcgtgcccatcctcaaggacttcttcgtgcggctcacagatgagttctatgtactgcgggcggctcagctggccctggtgtacgtgtcccaggactccacggaggagcagcaggacctgttcctcaaggacatgccaaagaaatggcttttcctgccctttgaggatgatctgaggaggtgataaacgcgtggtttatccgatccaccggatctagataagatatccgatccaccggatctagataactgatcataatcagccataccacatttgtagaggttttacttgctttaaaaaacctcccacacctccccctgaacctgaaacataaaatgaatgcaattggcggccgcctcgagctgtgccttctagttgccagccatctgttgtttgcccctcccccgtgccttccttgaccctggaaggtgccactcccactgtcctttcctaataaaatgaggaaattgcatcgcattgtctgagtaggtgtcattctattctggggggtggggtggggcaggacagcaagggggaggattgggaagacaatagcaggcatgctggggatgcggtgggctctatgg

SEQ ID NO: 109 - DNA, 2617 bp, synthetic construct
  misc_feature 1..2617: note = P5-intron-CYP4V2-P2A-RdCVF
  source 1..2617: mol_type = other DNA
gagccggatgcgccttcctttcctctccagagcaggctgcccgcccgcggaatcccgcacgtagagcaacctcgcagcaccctcagaacagccccgctggggcgcgccgggctgccgcggtgacctttccgacgcccctgaccccgcatccggaggcggccggaagtgtcgccggcctcctcccggcgcagcctccgggcctccagtgcaatcactacgccctggggcccggaaaccgttttccggtctttcgctttcggctggggcgtggaggccgcggtgctgcgtaggccgggccgggcgcaggaacagccccgtggcgccctctctggccgccgcccgggcgggaaacgtcgttccggggaccgggcgaccccgcagcggggagcgcgccaggtccgcgcggggaagtgggcggtgtgcggccggcaccgcctcgcaccacgcccccgcgggcccgcactttcccggagtgcaccccgcggccgccagccggggcggtaagtatcaaggttacaagacaggtttaaggagaccaatagaaactgggcttgtcgagacagagaagactcttgcgtttctgataggcacctattggtcttactgacatccactttgcctttctctccacaggaattccgccaccatggcggggctctggctggggctcgtgtggcagaagctgctgctgtggggcgcggcgagtgccctttccctggccggcgccagtctggtcctgagtctgctgcagagggtggcgagctacgcgcggaaatggcagcagatgcggcccatccccacggtggcccgcgcctacccactggtgggccacgcgctgctgatgaagccggacgggcgagaattttttcagcagatcattgagtacacagaggaataccgccacatgccgctgctgaagctctgggtcgggccagtgcccatggtggccctttataatgcagaaaatgtggaggtaattttaactagttcaaagcaaattgacaaatcctctatgtacaagtttttagaaccatggcttggcctaggacttcttacaagtactggaaacaaatggcgctccaggagaaagatgttaacacccactttccattttaccattctggaagatttcttagatatcatgaatgaacaagcaaatatattggttaagaaacttgaaaaacacattaaccaagaagcatttaactgctttttttacatcactctttgtgccttagatatcatctgtgaaacagctatggggaagaatattggtgctcaaagtaatgatgattccgagtatgtccgtgcagtttatagaatgagtgagatgatatttcgaagaataaagatgccctggctttggcttgatctctggtaccttatgtttaaagaaggatgggaacacaaaaagagccttcagatcctacatacttttaccaacagtgtcatcgcggaacgggccaatgaaatgaacgccaatgaagactgtagaggtgatggcaggggctctgccccctccaaaaataaacgcagggcctttcttgacttgcttttaagtgtgactgatgacgaagggaacaggctaagtcatgaagatattcgagaagaagttgacaccttcatgtttgaggggcacgatacaactgcagctgcaataaactggtccttatacctgttgggttctaacccagaagtccagaaaaaagtggatcatgaattggatgacgtgtttgggaagtctgaccgtcccgctacagtagaagacctgaagaaacttcggtatctggaatgtgttattaaggagacccttcgcctttttccttctgttcctttatttgcccgtagtgttagtgaagattgtgaagtggcaggttacagagttctaaaaggcactgaagccgtcatcattccctatgcattgcacagagatccgagatacttccccaaccccgaggagttccagcctgagcggttcttccccgagaatgcacaagggcgccatccatatgcctacgtgcccttctctgctggccccaggaactgtataggtcaaaagtttgctgtgatggaagaaaagaccattctttcgtgcatcctgaggcacttttggatagaatccaaccagaaaagagaagagcttggtctagaaggacagttgattcttcgtccaagtaatggcatctggatcaagttgaagaggagaaatgcagatgaacgcggaagcggagctactaacttcagcctgctgaagcaggctggagacgtggaggagaaccctggacctatggcctccctgttctctggccgcatcctgatccgcaacaatagcgaccaggacgagctggatacggaggctgaggtcagtcgcaggctggagaaccggctggtgctgctgttctttggtgctggggcttgtccacagtgccaggccttcgtgcccatcctcaaggacttcttcgtgcggctcacagatgagttctatgtactgcgggcggctcagctggccctggtgtacgtgtcccaggactccacggaggagcagcaggacctgttcctcaaggacatgccaaagaaatggcttttcctgccctttgaggatgatctgaggaggtga

SEQ ID NO: 110 - DNA, 3183 bp, synthetic construct
  misc_feature 1..3183: note = P3-SV40 intron-CYP4V2-P2A-RdCVF
  source 1..3183: mol_type = other DNA
gcatccaggacattcagtttcatcttcctggcactttagtgtttaggaagggcctggcctctcggggagcgacactcctcgcccggccactttgtaagaagcatcgagcgtggaaaaggggctggggtcagcactggggccctctgccgggaagagagactggcggccagcacacgcgtctccccaggctgaaatggggcaccctctcgcggcccttccctcccttcccgggctgggtggcaggtcttggctcttctgcgagtaccccgcggctgcggtctcccggcacccgctgagcagcctcgcccgccttcctctcccacccgcccctgcgtgctctccggggctccggcttcctcggtctggtgcctggtgcgtattttggaaaatacctggctcataaccacctcattgagctcccagtgtcccagtgggccagcggacacacacgggtagctgacttccctaacgtgtccccaaagcctccctggattacagcgcccgctgctccatgtgaccccgcgggagccaggacgcgccccgcctcccggggctgcaagttgcgcagggagcgagcgatgcgcagcagagctgggctccgagccggatgcgccttcctttcctctccagagcaggctgcccgcccgcggaatcccgcacgtagagcaacctcgcagcaccctcagaacagccccgctggggcgcgccgggctgccgcggtgacctttccgacgcccctgaccccgcatccggaggcggccggaagtgtcgccggcctcctcccggcgcagcctccgggcctccagtgcaatcactacgccctggggcccggaaaccgttttccggtctttcgctttcggctggggcgtggaggccgcggtgctgcgtaggccgggccgggcgcaggaacagccccgtggcgccctctctggccgccgcccgggcgggaaacgtcgttccggggaccgggcgaccccgcagcggggagcgcgccaggtccgcgcggggaagtgggcggtgtgcggccggcaccgcctcgcaccacgcccccgcgggcccgcactttcccggagtgcaccccgcggccgccagccggggcggtaagtttagtctttttgtcttttatttcaggtcccggatccggtggtggtgcaaatcaaagaactgctcctcagtggatgttgcctttacttctaggcgaattccgccaccatggcggggctctggctggggctcgtgtggcagaagctgctgctgtggggcgcggcgagtgccctttccctggccggcgccagtctggtcctgagtctgctgcagagggtggcgagctacgcgcggaaatggcagcagatgcggcccatccccacggtggcccgcgcctacccactggtgggccacgcgctgctgatgaagccggacgggcgagaattttttcagcagatcattgagtacacagaggaataccgccacatgccgctgctgaagctctgggtcgggccagtgcccatggtggccctttataatgcagaaaatgtggaggtaattttaactagttcaaagcaaattgacaaatcctctatgtacaagtttttagaaccatggcttggcctaggacttcttacaagtactggaaacaaatggcgctccaggagaaagatgttaacacccactttccattttaccattctggaagatttcttagatatcatgaatgaacaagcaaatatattggttaagaaacttgaaaaacacattaaccaagaagcatttaactgctttttttacatcactctttgtgccttagatatcatctgtgaaacagctatggggaagaatattggtgctcaaagtaatgatgattccgagtatgtccgtgcagtttatagaatgagtgagatgatatttcgaagaataaagatgccctggctttggcttgatctctggtaccttatgtttaaagaaggatgggaacacaaaaagagccttcagatcctacatacttttaccaacagtgtcatcgcggaacgggccaatgaaatgaacgccaatgaagactgtagaggtgatggcaggggctctgccccctccaaaaataaacgcagggcctttcttgacttgcttttaagtgtgactgatgacgaagggaacaggctaagtcatgaagatattcgagaagaagttgacaccttcatgtttgaggggcacgatacaactgcagctgcaataaactggtccttatacctgttgggttctaacccagaagtccagaaaaaagtggatcatgaattggatgacgtgtttgggaagtctgaccgtcccgctacagtagaagacctgaagaaacttcggtatctggaatgtgttattaaggagacccttcgcctttttccttctgttcctttatttgcccgtagtgttagtgaagattgtgaagtggcaggttacagagttctaaaaggcactgaagccgtcatcattccctatgcattgcacagagatccgagatacttccccaaccccgaggagttccagcctgagcggttcttccccgagaatgcacaagggcgccatccatatgcctacgtgcccttctctgctggccccaggaactgtataggtcaaaagtttgctgtgatggaagaaaagaccattctttcgtgcatcctgaggcacttttggatagaatccaaccagaaaagagaagagcttggtctagaaggacagttgattcttcgtccaagtaatggcatctggatcaagttgaagaggagaaatgcagatgaacgcggaagcggagctactaacttcagcctgctgaagcaggctggagacgtggaggagaaccctggacctatggcctccctgttctctggccgcatcctgatccgcaacaatagcgaccaggacgagctggatacggaggctgaggtcagtcgcaggctggagaaccggctggtgctgctgttctttggtgctggggcttgtccacagtgccaggccttcgtgcccatcctcaaggacttcttcgtgcggctcacagatgagttctatgtactgcgggcggctcagctggccctggtgtacgtgtcccaggactccacggaggagcagcaggacctgttcctcaaggacatgccaaagaaatggcttttcctgccctttgaggatgatctgaggaggtga

SEQ ID NO: 111 - DNA, 4083 bp, synthetic construct
  misc_feature 1..4083: note = Pf-SV40 intron-CYP4V2-P2A-RdCVF
  source 1..4083: mol_type = other DNA
acccacctcatcctgcacctgtcactgcgtgggaccctgtgctccaggcaggggcacctcactgccccctgagctcattttacccctcctggctctgcagcatttctgaccatttctgcccaggccgagactcactgctgcccagagcaatctcccttctctccttctggaggggaggggttgtatgttacccgcctggttttatccacagaggttagcagagactgatacagacaaaccctttttctttctaattttagattcaagagcacatgtgcaggtttgttaaatttgcctgacgctgaggtttgagtttctattgatcccctcacctgaatagggaacacagtacccaatacacagtttttcaaccattactccccttccttcctccccctattttagaatccccagtatgtagacaaattgtttacttttatagctgtaattaaccttattatagctcagcctcaaccctttagagaggaggaaactaaagcccatgagacttgcttaaagatactaagtgaacatatttattttttaaagtgttaaagtgattaaacaatgtagacgtgaatgaaataaaaagcgtaagttccccatcttcattcccactccatagagctgatcagtatttttacttgcagacattagtggagccgtagagaaagaaaccttttctccaaaagaaggcattactttacacactccgttctgcaacttgttttgttcacttgctatttcacgtcagcccatgcagatgacttaaaacaaattcaaatggagaaaagccttaggcatgtttttctctgcactaaagaggccctgcaggtggctgtggccaacttatgcagtggcttcgagtgaacgaacgtaattagtaattaagcaaagcgggcatccaggacattcagtttcatcttcctggcactttagtgtttaggaagggcctggcctctcggggagcgacactcctcgcccggccactttgtaagaagcatcgagcgtggaaaaggggctggggtcagcactggggccctctgccgggaagagagactggcggccagcacacgcgtctccccaggctgaaatggggcaccctctcgcggcccttccctcccttcccgggctgggtggcaggtcttggctcttctgcgagtaccccgcggctgcggtctcccggcacccgctgagcagcctcgcccgccttcctctcccacccgcccctgcgtgctctccggggctccggcttcctcggtctggtgcctggtgcgtattttggaaaatacctggctcataaccacctcattgagctcccagtgtcccagtgggccagcggacacacacgggtagctgacttccctaacgtgtccccaaagcctccctggattacagcgcccgctgctccatgtgaccccgcgggagccaggacgcgccccgcctcccggggctgcaagttgcgcagggagcgagcgatgcgcagcagagctgggctccgagccggatgcgccttcctttcctctccagagcaggctgcccgcccgcggaatcccgcacgtagagcaacctcgcagcaccctcagaacagccccgctggggcgcgccgggctgccgcggtgacctttccgacgcccctgaccccgcatccggaggcggccggaagtgtcgccggcctcctcccggcgcagcctccgggcctccagtgcaatcactacgccctggggcccggaaaccgttttccggtctttcgctttcggctggggcgtggaggccgcggtgctgcgtaggccgggccgggcgcaggaacagccccgtggcgccctctctggccgccgcccgggcgggaaacgtcgttccggggaccgggcgaccccgcagcggggagcgcgccaggtccgcgcggggaagtgggcggtgtgcggccggcaccgcctcgcaccacgcccccgcgggcccgcactttcccggagtgcaccccgcggccgccagccggggcggtaagtttagtctttttgtcttttatttcaggtcccggatccggtggtggtgcaaatcaaagaactgctcctcagtggatgttgcctttacttctaggcgaattccgccaccatggcggggctctggctggggctcgtgtggcagaagctgctgctgtggggcgcggcgagtgccctttccctggccggcgccagtctggtcctgagtctgctgcagagggtggcgagctacgcgcggaaatggcagcagatgcggcccatccccacggtggcccgcgcctacccactggtgggccacgcgctgctgatgaagccggacgggcgagaattttttcagcagatcattgagtacacagaggaataccgccacatgccgctgctgaagctctgggtcgggccagtgcccatggtggccctttataatgcagaaaatgtggaggtaattttaactagttcaaagcaaattgacaaatcctctatgtacaagtttttagaaccatggcttggcctaggacttcttacaagtactggaaacaaatggcgctccaggagaaagatgttaacacccactttccattttaccattctggaagatttcttagatatcatgaatgaacaagcaaatatattggttaagaaacttgaaaaacacattaaccaagaagcatttaactgctttttttacatcactctttgtgccttagatatcatctgtgaaacagctatggggaagaatattggtgctcaaagtaatgatgattccgagtatgtccgtgcagtttatagaatgagtgagatgatatttcgaagaataaagatgccctggctttggcttgatctctggtaccttatgtttaaagaaggatgggaacacaaaaagagccttcagatcctacatacttttaccaacagtgtcatcgcggaacgggccaatgaaatgaacgccaatgaagactgtagaggtgatggcaggggctctgccccctccaaaaataaacgcagggcctttcttgacttgcttttaagtgtgactgatgacgaagggaacaggctaagtcatgaagatattcgagaagaagttgacaccttcatgtttgaggggcacgatacaactgcagctgcaataaactggtccttatacctgttgggttctaacccagaagtccagaaaaaagtggatcatgaattggatgacgtgtttgggaagtctgaccgtcccgctacagtagaagacctgaagaaacttcggtatctggaatgtgttattaaggagacccttcgcctttttccttctgttcctttatttgcccgtagtgttagtgaagattgtgaagtggcaggttacagagttctaaaaggcactgaagccgtcatcattccctatgcattgcacagagatccgagatacttccccaaccccgaggagttccagcctgagcggttcttccccgagaatgcacaagggcgccatccatatgcctacgtgcccttctctgctggccccaggaactgtataggtcaaaagtttgctgtgatggaagaaaagaccattctttcgtgcatcctgaggcacttttggatagaatccaaccagaaaagagaagagcttggtctagaaggacagttgattcttcgtccaagtaatggcatctggatcaagttgaagaggagaaatgcagatgaacgcggaagcggagctactaacttcagcctgctgaagcaggctggagacgtggaggagaaccctggacctatggcctccctgttctctggccgcatcctgatccgcaacaatagcgaccaggacgagctggatacggaggctgaggtcagtcgcaggctggagaaccggctggtgctgctgttctttggtgctggggcttgtccacagtgccaggccttcgtgcccatcctcaaggacttcttcgtgcggctcacagatgagttctatgtactgcgggcggctcagctggccctggtgtacgtgtcccaggactccacggaggagcagcaggacctgttcctcaaggacatgccaaagaaatggcttttcctgccctttgaggatgatctgaggaggtga

SEQ ID NO: 112 - DNA, 3728 bp, synthetic construct
  misc_feature 1..3728: note = RPE65-intron-CYP4V2-T2A-RdCVF
  source 1..3728: mol_type = other DNA
tattgtgcaaataagtgctcactccaaattagtggtatatttattgaagtttaatattgtgtttgtgatacagaagtatttgctttaattctaaataaaaattttatgcttttattgctggtttaagaagatttggattatccttgtactttgaggagaagtttcttatttgaaatattttggaaacaggtcttttaatgtggaaagatagatattaatctcctcttctattactctccaagatccaacaaaagtgattataccccccaaaatatgatggtagtatcttatactaccatcattttataggcatagggctcttagctgcaaataatggaactaactctaataaagcagaacgcaaatattgtaaatattagagagctaacaatctctgggatggctaaaggatggagcttggaggctacccagccagtaacaatattccgggctccactgttgaatggagacactacaactgccttggatgggcagagatattatggatgctaagccccaggtgctaccattaggacttctaccactgtccctaacgggtggagcccatcacatgcctatgccctcactgtaaggaaatgaagctactgttgtatatcttgggaagcacttggattaattgttatacagttttgttgaagaagacccctagggtaagtagccataactgcacactaaatttaaaattgttaatgagtttctcaaaaaaaatgttaaggttgttagctggtatagtatatatcttgcctgttttccaaggacttctttgggcagtaccttgtctgtgctggcaagcaactgagacttaatgaaagagtattggagatatgaatgaattgatgctgtatactctcagagtgccaaacatataccaatggacaagaaggtgaggcagagagcagacaggcattagtgacaagcaaagatatgcagaatttcattctcagcaaatcaaaagtcctcaacctggttggaagaatattggcactgaatggtatcaataaggttgctagagagggttagaggtgcacaatgtgcttccataacattttatacttctccaatcttagcactaatcaaacatggttgaatactttgtttactataactcttacagagttataagatctgtgaagacagggacagggacaatacccatctctgtctggttcataggtggtatgtaatagatatttttaaaaataagtgagttaatgaatgagggtgagaatgaaggcacagaggtattagggggaggtgggccccagagaatggtgccaaggtccagtggggtgactgggatcagctcaggcctgacgctggccactcccacctagctcctttctttctaatctgttctcattctccttgggaaggattgaggtctctggaaaacagccaaacaactgttatgggaacagcaagcccaaataaagccaagcatcagggggatctgagagctgaaagcaacttctgttccccctccctcagctgaaggggtggggaagggctcccaaagccataactccttttaagggatttagaaggcataaaaaggcccctggctgagaacttccttcttcattctgcagttgggtaagtatcaaggttacaagacaggtttaaggagaccaatagaaactgggcttgtcgagacagagaagactcttgcgtttctgataggcacctattggtcttactgacatccactttgcctttctctccacaggaattccgccaccatggcggggctctggctggggctcgtgtggcagaagctgctgctgtggggcgcggcgagtgccctttccctggccggcgccagtctggtcctgagtctgctgcagagggtggcgagctacgcgcggaaatggcagcagatgcggcccatccccacggtggcccgcgcctacccactggtgggccacgcgctgctgatgaagccggacgggcgagaattttttcagcagatcattgagtacacagaggaataccgccacatgccgctgctgaagctctgggtcgggccagtgcccatggtggccctttataatgcagaaaatgtggaggtaattttaactagttcaaagcaaattgacaaatcctctatgtacaagtttttagaaccatggcttggcctaggacttcttacaagtactggaaacaaatggcgctccaggagaaagatgttaacacccactttccattttaccattctggaagatttcttagatatcatgaatgaacaagcaaatatattggttaagaaacttgaaaaacacattaaccaagaagcatttaactgctttttttacatcactctttgtgccttagatatcatctgtgaaacagctatggggaagaatattggtgctcaaagtaatgatgattccgagtatgtccgtgcagtttatagaatgagtgagatgatatttcgaagaataaagatgccctggctttggcttgatctctggtaccttatgtttaaagaaggatgggaacacaaaaagagccttcagatcctacatacttttaccaacagtgtcatcgcggaacgggccaatgaaatgaacgccaatgaagactgtagaggtgatggcaggggctctgccccctccaaaaataaacgcagggcctttcttgacttgcttttaagtgtgactgatgacgaagggaacaggctaagtcatgaagatattcgagaagaagttgacaccttcatgtttgaggggcacgatacaactgcagctgcaataaactggtccttatacctgttgggttctaacccagaagtccagaaaaaagtggatcatgaattggatgacgtgtttgggaagtctgaccgtcccgctacagtagaagacctgaagaaacttcggtatctggaatgtgttattaaggagacccttcgcctttttccttctgttcctttatttgcccgtagtgttagtgaagattgtgaagtggcaggttacagagttctaaaaggcactgaagccgtcatcattccctatgcattgcacagagatccgagatacttccccaaccccgaggagttccagcctgagcggttcttccccgagaatgcacaagggcgccatccatatgcctacgtgcccttctctgctggccccaggaactgtataggtcaaaagtttgctgtgatggaagaaaagaccattctttcgtgcatcctgaggcacttttggatagaatccaaccagaaaagagaagagcttggtctagaaggacagttgattcttcgtccaagtaatggcatctggatcaagttgaagaggagaaatgcagatgaacgcggaagcggagagggcagaggaagtctgctaacatgcggtgacgtcgaggagaatcctggacctatggcctccctgttctctggccgcatcctgatccgcaacaatagcgaccaggacgagctggatacggaggctgaggtcagtcgcaggctggagaaccggctggtgctgctgttctttggtgctggggcttgtccacagtgccaggccttcgtgcccatcctcaaggacttcttcgtgcggctcacagatgagttctatgtactgcgggcggctcagctggccctggtgtacgtgtcccaggactccacggaggagcagcaggacctgttcctcaaggacatgccaaagaaatggcttttcctgccctttgaggatgatctgaggaggtga

SEQ ID NO: 113 - DNA, 3021 bp, synthetic construct
  misc_feature 1..3021: note = P5-intron-CYP4V2-P2A-RdCVF-BGH
  source 1..3021: mol_type = other DNA
gagccggatgcgccttcctttcctctccagagcaggctgcccgcccgcggaatcccgcacgtagagcaacctcgcagcaccctcagaacagccccgctggggcgcgccgggctgccgcggtgacctttccgacgcccctgaccccgcatccggaggcggccggaagtgtcgccggcctcctcccggcgcagcctccgggcctccagtgcaatcactacgccctggggcccggaaaccgttttccggtctttcgctttcggctggggcgtggaggccgcggtgctgcgtaggccgggccgggcgcaggaacagccccgtggcgccctctctggccgccgcccgggcgggaaacgtcgttccggggaccgggcgaccccgcagcggggagcgcgccaggtccgcgcggggaagtgggcggtgtgcggccggcaccgcctcgcaccacgcccccgcgggcccgcactttcccggagtgcaccccgcggccgccagccggggcggtaagtatcaaggttacaagacaggtttaaggagaccaatagaaactgggcttgtcgagacagagaagactcttgcgtttctgataggcacctattggtcttactgacatccactttgcctttctctccacaggaattccgccaccatggcggggctctggctggggctcgtgtggcagaagctgctgctgtggggcgcggcgagtgccctttccctggccggcgccagtctggtcctgagtctgctgcagagggtggcgagctacgcgcggaaatggcagcagatgcggcccatccccacggtggcccgcgcctacccactggtgggccacgcgctgctgatgaagccggacgggcgagaattttttcagcagatcattgagtacacagaggaataccgccacatgccgctgctgaagctctgggtcgggccagtgcccatggtggccctttataatgcagaaaatgtggaggtaattttaactagttcaaagcaaattgacaaatcctctatgtacaagtttttagaaccatggcttggcctaggacttcttacaagtactggaaacaaatggcgctccaggagaaagatgttaacacccactttccattttaccattctggaagatttcttagatatcatgaatgaacaagcaaatatattggttaagaaacttgaaaaacacattaaccaagaagcatttaactgctttttttacatcactctttgtgccttagatatcatctgtgaaacagctatggggaagaatattggtgctcaaagtaatgatgattccgagtatgtccgtgcagtttatagaatgagtgagatgatatttcgaagaataaagatgccctggctttggcttgatctctggtaccttatgtttaaagaaggatgggaacacaaaaagagccttcagatcctacatacttttaccaacagtgtcatcgcggaacgggccaatgaaatgaacgccaatgaagactgtagaggtgatggcaggggctctgccccctccaaaaataaacgcagggcctttcttgacttgcttttaagtgtgactgatgacgaagggaacaggctaagtcatgaagatattcgagaagaagttgacaccttcatgtttgaggggcacgatacaactgcagctgcaataaactggtccttatacctgttgggttctaacccagaagtccagaaaaaagtggatcatgaattggatgacgtgtttgggaagtctgaccgtcccgctacagtagaagacctgaagaaacttcggtatctggaatgtgttattaaggagacccttcgcctttttccttctgttcctttatttgcccgtagtgttagtgaagattgtgaagtggcaggttacagagttctaaaaggcactgaagccgtcatcattccctatgcattgcacagagatccgagatacttccccaaccccgaggagttccagcctgagcggttcttccccgagaatgcacaagggcgccatccatatgcctacgtgcccttctctgctggccccaggaactgtataggtcaaaagtttgctgtgatggaagaaaagaccattctttcgtgcatcctgaggcacttttggatagaatccaaccagaaaagagaagagcttggtctagaaggacagttgattcttcgtccaagtaatggcatctggatcaagttgaagaggagaaatgcagatgaacgcggaagcggagctactaacttcagcctgctgaagcaggctggagacgtggaggagaaccctggacctatggcctccctgttctctggccgcatcctgatccgcaacaatagcgaccaggacgagctggatacggaggctgaggtcagtcgcaggctggagaaccggctggtgctgctgttctttggtgctggggcttgtccacagtgccaggccttcgtgcccatcctcaaggacttcttcgtgcggctcacagatgagttctatgtactgcgggcggctcagctggccctggtgtacgtgtcccaggactccacggaggagcagcaggacctgttcctcaaggacatgccaaagaaatggcttttcctgccctttgaggatgatctgaggaggtgataaacgcgtggtttatccgatccaccggatctagataagatatccgatccaccggatctagataactgatcataatcagccataccacatttgtagaggttttacttgctttaaaaaacctcccacacctccccctgaacctgaaacataaaatgaatgcaattggcggccgcctcgagctgtgccttctagttgccagccatctgttgtttgcccctcccccgtgccttccttgaccctggaaggtgccactcccactgtcctttcctaataaaatgaggaaattgcatcgcattgtctgagtaggtgtcattctattctggggggtggggtggggcaggacagcaagggggaggattgggaagacaatagcaggcatgctggggatgcggtgggctctatgg

SEQ ID NO: 114 - DNA, 3510 bp, synthetic construct
  misc_feature 1..3510: note = P5-intron-CYP4V2-P2A-RdCVF-WPRE-SV40
  source 1..3510: mol_type = other DNA
gagccggatgcgccttcctttcctctccagagcaggctgcccgcccgcggaatcccgcacgtagagcaacctcgcagcaccctcagaacagccccgctggggcgcgccgggctgccgcggtgacctttccgacgcccctgaccccgcatccggaggcggccggaagtgtcgccggcctcctcccggcgcagcctccgggcctccagtgcaatcactacgccctggggcccggaaaccgttttccggtctttcgctttcggctggggcgtggaggccgcggtgctgcgtaggccgggccgggcgcaggaacagccccgtggcgccctctctggccgccgcccgggcgggaaacgtcgttccggggaccgggcgaccccgcagcggggagcgcgccaggtccgcgcggggaagtgggcggtgtgcggccggcaccgcctcgcaccacgcccccgcgggcccgcactttcccggagtgcaccccgcggccgccagccggggcggtaagtatcaaggttacaagacaggtttaaggagaccaatagaaactgggcttgtcgagacagagaagactcttgcgtttctgataggcacctattggtcttactgacatccactttgcctttctctccacaggaattccgccaccatggcggggctctggctggggctcgtgtggcagaagctgctgctgtggggcgcggcgagtgccctttccctggccggcgccagtctggtcctgagtctgctgcagagggtggcgagctacgcgcggaaatggcagcagatgcggcccatccccacggtggcccgcgcctacccactggtgggccacgcgctgctgatgaagccggacgggcgagaattttttcagcagatcattgagtacacagaggaataccgccacatgccgctgctgaagctctgggtcgggccagtgcccatggtggccctttataatgcagaaaatgtggaggtaattttaactagttcaaagcaaattgacaaatcctctatgtacaagtttttagaaccatggcttggcctaggacttcttacaagtactggaaacaaatggcgctccaggagaaagatgttaacacccactttccattttaccattctggaagatttcttagatatcatgaatgaacaagcaaatatattggttaagaaacttgaaaaacacattaaccaagaagcatttaactgctttttttacatcactctttgtgccttagatatcatctgtgaaacagctatggggaagaatattggtgctcaaagtaatgatgattccgagtatgtccgtgcagtttatagaatgagtgagatgatatttcgaagaataaagatgccctggctttggcttgatctctggtaccttatgtttaaagaaggatgggaacacaaaaagagccttcagatcctacatacttttaccaacagtgtcatcgcggaacgggccaatgaaatgaacgccaatgaagactgtagaggtgatggcaggggctctgccccctccaaaaataaacgcagggcctttcttgacttgcttttaagtgtgactgatgacgaagggaacaggctaagtcatgaagatattcgagaagaagttgacaccttcatgtttgaggggcacgatacaactgcagctgcaataaactggtccttatacctgttgggttctaacccagaagtccagaaaaaagtggatcatgaattggatgacgtgtttgggaagtctgaccgtcccgctacagtagaagacctgaagaaacttcggtatctggaatgtgttattaaggagacccttcgcctttttccttctgttcctttatttgcccgtagtgttagtgaagattgtgaagtggcaggttacagagttctaaaaggcactgaagccgtcatcattccctatgcattgcacagagatccgagatacttccccaaccccgaggagttccagcctgagcggttcttccccgagaatgcacaagggcgccatccatatgcctacgtgcccttctctgctggccccaggaactgtataggtcaaaagtttgctgtgatggaagaaaagaccattctttcgtgcatcctgaggcacttttggatagaatccaaccagaaaagagaagagcttggtctagaaggacagttgattcttcgtccaagtaatggcatctggatcaagttgaagaggagaaatgcagatgaacgcggaagcggagctactaacttcagcctgctgaagcaggctggagacgtggaggagaaccctggacctatggcctccctgttctctggccgcatcctgatccgcaacaatagcgaccaggacgagctggatacggaggctgaggtcagtcgcaggctggagaaccggctggtgctgctgttctttggtgctggggcttgtccacagtgccaggccttcgtgcccatcctcaaggacttcttcgtgcggctcacagatgagttctatgtactgcgggcggctcagctggccctggtgtacgtgtcccaggactccacggaggagcagcaggacctgttcctcaaggacatgccaaagaaatggcttttcctgccctttgaggatgatctgaggaggtgaacgcgtggtttatccgatccaccggatctagataagatatccgatccaccggatctagataactgatcataatcagccataccacatttgtagaggttttacttgctttaaaaaacctcccacacctccccctgaacctgaaacataaaatgaatgcaattggcggccgcctcgagaatcaacctctggattacaaaatttgtgaaagattgactggtattcttaactatgttgctccttttacgctatgtggatacgctgctttaatgcctttgtatcatgctattgcttcccgtatggctttcattttctcctccttgtataaatcctggttgctgtctctttatgaggagttgtggcccgttgtcaggcaacgtggcgtggtgtgcactgtgtttgctgacgcaacccccactggttggggcattgccaccacctgtcagctcctttccgggactttcgctttccccctccctattgccacggcggaactcatcgccgcctgccttgcccgctgctggacaggggctcggctgttgggcactgacaattccgtggtgttgtcggggaaatcatcgtcctttccttggctgctcgcctgtgttgccacctggattctgcgcgggacgtccttctgctacgtcccttcggccctcaatccagcggaccttccttcccgcggcctgctgccggctctgcggcctcttccgcgtcttcgccttcgccctcagacgagtcggatctccctttgggccgcctccccgcggtaacaacttgtttattgcagcttataatggttacaaataaagcaatagcatcacaaatttcacaaataaagcatttttttcactgcattctagttgtggtttgtccaaactcatcaatgtatctta

SEQ ID NO: 115 - DNA, 3020 bp, synthetic construct
  misc_feature 1..3020: note = P5-CDS intron-CYP4V2-P2A-RdCVF-BGH
  source 1..3020: mol_type = other DNA
gagccggatgcgccttcctttcctctccagagcaggctgcccgcccgcggaatcccgcacgtagagcaacctcgcagcaccctcagaacagccccgctggggcgcgccgggctgccgcggtgacctttccgacgcccctgaccccgcatccggaggcggccggaagtgtcgccggcctcctcccggcgcagcctccgggcctccagtgcaatcactacgccctggggcccggaaaccgttttccggtctttcgctttcggctggggcgtggaggccgcggtgctgcgtaggccgggccgggcgcaggaacagccccgtggcgccctctctggccgccgcccgggcgggaaacgtcgttccggggaccgggcgaccccgcagcggggagcgcgccaggtccgcgcggggaagtgggcggtgtgcggccggcaccgcctcgcaccacgcccccgcgggcccgcactttcccggagtgcaccccgcggccgccagccggggcggaattcgccaccatggcggggctctggctggggctcgtgtggcagaagctgctgctgtggggcgcggcgagtgccctttccctggccggcgccagtctggtcctgagtctgctgcagagggtggcgagctacgcgcggaaatggcagcagatgcggcccatccccacggtggcccgcgcctacccactggtgggccacgcgctgctgatgaagccggacgggcgaggtaagtatcaaggttacaagacaggtttaaggagaccaatagaaactgggcttgtcgagacagagaagactcttgcgtttctgataggcacctattggtcttactgacatccactttgcctttctctccacagaattttttcagcagatcattgagtacacagaggaataccgccacatgccgctgctgaagctctgggtcgggccagtgcccatggtggccctttataatgcagaaaatgtggaggtaattttaactagttcaaagcaaattgacaaatcctctatgtacaagtttttagaaccatggcttggcctaggacttcttacaagtactggaaacaaatggcgctccaggagaaagatgttaacacccactttccattttaccattctggaagatttcttagatatcatgaatgaacaagcaaatatattggttaagaaacttgaaaaacacattaaccaagaagcatttaactgctttttttacatcactctttgtgccttagatatcatctgtgaaacagctatggggaagaatattggtgctcaaagtaatgatgattccgagtatgtccgtgcagtttatagaatgagtgagatgatatttcgaagaataaagatgccctggctttggcttgatctctggtaccttatgtttaaagaaggatgggaacacaaaaagagccttcagatcctacatacttttaccaacagtgtcatcgcggaacgggccaatgaaatgaacgccaatgaagactgtagaggtgatggcaggggctctgccccctccaaaaataaacgcagggcctttcttgacttgcttttaagtgtgactgatgacgaagggaacaggctaagtcatgaagatattcgagaagaagttgacaccttcatgtttgaggggcacgatacaactgcagctgcaataaactggtccttatacctgttgggttctaacccagaagtccagaaaaaagtggatcatgaattggatgacgtgtttgggaagtctgaccgtcccgctacagtagaagacctgaagaaacttcggtatctggaatgtgttattaaggagacccttcgcctttttccttctgttcctttatttgcccgtagtgttagtgaagattgtgaagtggcaggttacagagttctaaaaggcactgaagccgtcatcattccctatgcattgcacagagatccgagatacttccccaaccccgaggagttccagcctgagcggttcttccccgagaatgcacaagggcgccatccatatgcctacgtgcccttctctgctggccccaggaactgtataggtcaaaagtttgctgtgatggaagaaaagaccattctttcgtgcatcctgaggcacttttggatagaatccaaccagaaaagagaagagcttggtctagaaggacagttgattcttcgtccaagtaatggcatctggatcaagttgaagaggagaaatgcagatgaacgcggaagcggagctactaacttcagcctgctgaagcaggctggagacgtggaggagaaccctggacctatggcctccctgttctctggccgcatcctgatccgcaacaatagcgaccaggacgagctggatacggaggctgaggtcagtcgcaggctggagaaccggctggtgctgctgttctttggtgctggggcttgtccacagtgccaggccttcgtgcccatcctcaaggacttcttcgtgcggctcacagatgagttctatgtactgcgggcggctcagctggccctggtgtacgtgtcccaggactccacggaggagcagcaggacctgttcctcaaggacatgccaaagaaatggcttttcctgccctttgaggatgatctgaggaggtgataaacgcgtggtttatccgatccaccggatctagataagatatccgatccaccggatctagataactgatcataatcagccataccacatttgtagaggttttacttgctttaaaaaacctcccacacctccccctgaacctgaaacataaaatgaatgcaattggcggccgcctcgagctgtgccttctagttgccagccatctgttgtttgcccctcccccgtgccttccttgaccctggaaggtgccactcccactgtcctttcctaataaaatgaggaaattgcatcgcattgtctgagtaggtgtcattctattctggggggtggggtggggcaggacagcaagggggaggattgggaagacaatagcaggcatgctggggatgcggtgggctctatgg

SEQ ID NO: 116 - DNA, 1711 bp, synthetic construct
  misc_feature 1..1711: note = CDS intron-CYP4V2
  source 1..1711: mol_type = other DNA
atggcggggctctggctggggctcgtgtggcagaagctgctgctgtggggcgcggcgagtgccctttccctggccggcgccagtctggtcctgagtctgctgcagagggtggcgagctacgcgcggaaatggcagcagatgcggcccatccccacggtggcccgcgcctacccactggtgggccacgcgctgctgatgaagccggacgggcgaggtaagtatcaaggttacaagacaggtttaaggagaccaatagaaactgggcttgtcgagacagagaagactcttgcgtttctgataggcacctattggtcttactgacatccactttgcctttctctccacagaattttttcagcagatcattgagtacacagaggaataccgccacatgccgctgctgaagctctgggtcgggccagtgcccatggtggccctttataatgcagaaaatgtggaggtaattttaactagttcaaagcaaattgacaaatcctctatgtacaagtttttagaaccatggcttggcctaggacttcttacaagtactggaaacaaatggcgctccaggagaaagatgttaacacccactttccattttaccattctggaagatttcttagatatcatgaatgaacaagcaaatatattggttaagaaacttgaaaaacacattaaccaagaagcatttaactgctttttttacatcactctttgtgccttagatatcatctgtgaaacagctatggggaagaatattggtgctcaaagtaatgatgattccgagtatgtccgtgcagtttatagaatgagtgagatgatatttcgaagaataaagatgccctggctttggcttgatctctggtaccttatgtttaaagaaggatgggaacacaaaaagagccttcagatcctacatacttttaccaacagtgtcatcgcggaacgggccaatgaaatgaacgccaatgaagactgtagaggtgatggcaggggctctgccccctccaaaaataaacgcagggcctttcttgacttgcttttaagtgtgactgatgacgaagggaacaggctaagtcatgaagatattcgagaagaagttgacaccttcatgtttgaggggcacgatacaactgcagctgcaataaactggtccttatacctgttgggttctaacccagaagtccagaaaaaagtggatcatgaattggatgacgtgtttgggaagtctgaccgtcccgctacagtagaagacctgaagaaacttcggtatctggaatgtgttattaaggagacccttcgcctttttccttctgttcctttatttgcccgtagtgttagtgaagattgtgaagtggcaggttacagagttctaaaaggcactgaagccgtcatcattccctatgcattgcacagagatccgagatacttccccaaccccgaggagttccagcctgagcggttcttccccgagaatgcacaagggcgccatccatatgcctacgtgcccttctctgctggccccaggaactgtataggtcaaaagtttgctgtgatggaagaaaagaccattctttcgtgcatcctgaggcacttttggatagaatccaaccagaaaagagaagagcttggtctagaaggacagttgattcttcgtccaagtaatggcatctggatcaagttgaagaggagaaatgcagatgaacgctaa

SEQ ID NO: 117 - DNA, 5521 bp, synthetic construct
  misc_feature 1..5521: note = pAV-p5-CYP4V2
  source 1..5521: mol_type = other DNA
cctgcaggcagctgcgcgctcgctcgctcactgaggccgcccgggcgtcgggcgacctttggtcgcccggcctcagtgagcgagcgagcgcgcagagagggagtggccaactccatcactaggggttcctgcggccggtcgcgtctagtactagtcgcgtaggatccgagccggatgcgccttcctttcctctccagagcaggctgcccgcccgcggaatcccgcacgtagagcaacctcgcagcaccctcagaacagccccgctggggcgcgccgggctgccgcggtgacctttccgacgcccctgaccccgcatccggaggcggccggaagtgtcgccggcctcctcccggcgcagcctccgggcctccagtgcaatcactacgccctggggcccggaaaccgttttccggtctttcgctttcggctggggcgtggaggccgcggtgctgcgtaggccgggccgggcgcaggaacagccccgtggcgccctctctggccgccgcccgggcgggaaacgtcgttccggggaccgggcgaccccgcagcggggagcgcgccaggtccgcgcggggaagtgggcggtgtgcggccggcaccgcctcgcaccacgcccccgcgggcccgcactttcccggagtgcaccccgcggccgccagccggggcggaattccgccaccatggcggggctctggctggggctcgtgtggcagaagctgctgctgtggggcgcggcgagtgccctttccctggccggcgccagtctggtcctgagtctgctgcagagggtggcgagctacgcgcggaaatggcagcagatgcggcccatccccacggtggcccgcgcctacccactggtgggccacgcgctgctgatgaagccggacgggcgagaattttttcagcagatcattgagtacacagaggaataccgccacatgccgctgctgaagctctgggtcgggccagtgcccatggtggccctttataatgcagaaaatgtggaggtaattttaactagttcaaagcaaattgacaaatcctctatgtacaagtttttagaaccatggcttggcctaggacttcttacaagtactggaaacaaatggcgctccaggagaaagatgttaacacccactttccattttaccattctggaagatttcttagatatcatgaatgaacaagcaaatatattggttaagaaacttgaaaaacacattaaccaagaagcatttaactgctttttttacatcactctttgtgccttagatatcatctgtgaaacagctatggggaagaatattggtgctcaaagtaatgatgattccgagtatgtccgtgcagtttatagaatgagtgagatgatatttcgaagaataaagatgccctggctttggcttgatctctggtaccttatgtttaaagaaggatgggaacacaaaaagagccttcagatcctacatacttttaccaacagtgtcatcgcggaacgggccaatgaaatgaacgccaatgaagactgtagaggtgatggcaggggctctgccccctccaaaaataaacgcagggcctttcttgacttgcttttaagtgtgactgatgacgaagggaacaggctaagtcatgaagatattcgagaagaagttgacaccttcatgtttgaggggcacgatacaactgcagctgcaataaactggtccttatacctgttgggttctaacccagaagtccagaaaaaagtggatcatgaattggatgacgtgtttgggaagtctgaccgtcccgctacagtagaagacctgaagaaacttcggtatctggaatgtgttattaaggagacccttcgcctttttccttctgttcctttatttgcccgtagtgttagtgaagattgtgaagtggcaggttacagagttctaaaaggcactgaagccgtcatcattccctatgcattgcacagagatccgagatacttccccaaccccgaggagttccagcctgagcggttcttccccgagaatgcacaagggcgccatccatatgcctacgtgcccttctctgctggccccaggaactgtataggtcaaaagtttgctgtgatggaagaaaagaccattctttcgtgcatcctgaggcacttttggatagaatccaaccagaaaagagaagagcttggtctagaaggacagttgattcttcgtccaagtaatggcatctggatcaagttgaagaggagaaatgcagatgaacgctaaacgcgtggtttatccgatccaccggatctagataagatatccgatccaccggatctagataactgatcataatcagccataccacatttgtagaggttttacttgctttaaaaaacctcccacacctccccctgaacctgaaacataaaatgaatgcaattggcggccgcctcgagcacgtgcggacccaacggccgcaggaacccctagtgatggagttggccactccctctctgcgcgctcgctcgctcactgaggccgggcgaccaaaggtcgcccgacgcccgggctttgcccgggcggcctcagtgagcgagcgagcgcgcagctgcctgcaggggcgcctgatgcggtattttctccttacgcatctgtgcggtatttcacaccgcatacgtcaaagcaaccatagtacgcgccctgtagcggcacattaagcgcggcgggtgtggtggttacgcgcagcgtgaccgctacacttgccagcgccttagcgcccgctcctttcgctttcttcccttcctttctcgccacgttcgccggctttccccgtcaagctctaaatcgggggctccctttagggttccgatttagtgctttacggcacctcgaccccaaaaaacttgatttgggtgatggttcacgtagtgggccatcgccctgatagacggtttttcgccctttgacgttggagtccacgttctttaatagtggactcttgttccaaactggaacaacactcaactctatctcgggctattcttttgatttataagggattttgccgatttcggtctattggttaaaaaatgagctgatttaacaaaaatttaacgcgaattttaacaaaatattaacgtttacaattttatggtgcactctcagtacaatctgctctgatgccgcatagttaagccagccccgacacccgccaacacccgctgacgcgccctgacgggcttgtctgctcccggcatccgcttacagacaagctgtgaccgtctccgggagctgcatgtgtcagaggttttcaccgtcatcaccgaaacgcgcgagacgaaagggcctcgtgatacgcctatttttataggttaatgtcatgataataatggtttcttagacgtcaggtggcacttttcggggaaatgtgcgcggaacccctatttgtttatttttctaaatacattcaaatatgtatccgctcatgagacaataaccctgataaatgcttcaataatattgaaaaaggaagagtcctgaggcggaaagaaccagctgtggaatgtgtgtcagttagggtgtggaaagtccccaggctccccagcaggcagaagtatgcaaagcatgcatctcaattagtcagcaaccaggtgtggaaagtccccaggctccccagcaggcagaagtatgcaaagcatgcatctcaattagtcagcaaccatagtcccgcccctaactccgcccatcccgcccctaactccgcccagttccgcccattctccgccccatggctgactaattttttttatttatgcagaggccgaggccgcctcggcctctgagctattccagaagtagtgaggaggcttttttggaggcctaggcttttgcaaagatcgatcaagagacaggatgaggatcgtttcgcatgattgaacaagatggattgcacgcaggttctccggccgcttgggtggagaggctattcggctatgactgggcacaacagacaatcggctgctctgatgccgccgtgttccggctgtcagcgcaggggcgcccggttctttttgtcaagaccgacctgtccggtgccctgaatgaactgcaagacgaggcagcgcggctatcgtggctggccacgacgggcgttccttgcgcagctgtgctcgacgttgtcactgaagcgggaagggactggctgctattgggcgaagtgccggggcaggatctcctgtcatctcaccttgctcctgccgagaaagtatccatcatggctgatgcaatgcggcggctgcatacgcttgatccggctacctgcccattcgaccaccaagcgaaacatcgcatcgagcgagcacgtactcggatggaagccggtcttgtcgatcaggatgatctggacgaagagcatcaggggctcgcgccagccgaactgttcgccaggctcaaggcgagcatgcccgacggcgaggatctcgtcgtgacccatggcgatgcctgcttgccgaatatcatggtggaaaatggccgcttttctggattcatcgactgtggccggctgggtgtggcggaccgctatcaggacatagcgttggctacccgtgatattgctgaagagcttggcggcgaatgggctgaccgcttcctcgtgctttacggtatcgccgctcccgattcgcagcgcatcgccttctatcgccttcttgacgagttcttctgactgtcagaccaagtttactcatatatactttagattgatttaaaacttcatttttaatttaaaaggatctaggtgaagatcctttttgataatctcatgaccaaaatcccttaacgtgagttttcgttccactgagcgtcagaccccgtagaaaagatcaaaggatcttcttgagatcctttttttctgcgcgtaatctgctgcttgcaaacaaaaaaaccaccgctaccagcggtggtttgtttgccggatcaagagctaccaactctttttccgaaggtaactggcttcagcagagcgcagataccaaatactgttcttctagtgtagccgtagttaggccaccacttcaagaactctgtagcaccgcctacatacctcgctctgctaatcctgttaccagtggctgctgccagtggcgataagtcgtgtcttaccgggttggactcaagacgatagttaccggataaggcgcagcggtcgggctgaacggggggttcgtgcacacagcccagcttggagcgaacgacctacaccgaactgagatacctacagcgtgagctatgagaaagcgccacgcttcccgaagggagaaaggcggacaggtatccggtaagcggcagggtcggaacaggagagcgcacgagggagcttccagggggaaacgcctggtatctttatagtcctgtcgggtttcgccacctctgacttgagcgtcgatttttgtgatgctcgtcaggggggcggagcctatggaaaaacgccagcaacgcggcctttttacggttcctggccttttgctggccttttgctcacatgt

SEQ ID NO: 118 - DNA, 5885 bp, synthetic construct
  misc_feature 1..5885: note = pAV-p5-intron-CYP4V2-BGH
  source 1..5885: mol_type = other DNA
cctgcaggcagctgcgcgctcgctcgctcactgaggccgcccgggcgtcgggcgacctttggtcgcccggcctcagtgagcgagcgagcgcgcagagagggagtggccaactccatcactaggggttcctgcggccggtcgcgtctagtactagtcgcgtaggatccgagccggatgcgccttcctttcctctccagagcaggctgcccgcccgcggaatcccgcacgtagagcaacctcgcagcaccctcagaacagccccgctggggcgcgccgggctgccgcggtgacctttccgacgcccctgaccccgcatccggaggcggccggaagtgtcgccggcctcctcccggcgcagcctccgggcctccagtgcaatcactacgccctggggcccggaaaccgttttccggtctttcgctttcggctggggcgtggaggccgcggtgctgcgtaggccgggccgggcgcaggaacagccccgtggcgccctctctggccgccgcccgggcgggaaacgtcgttccggggaccgggcgaccccgcagcggggagcgcgccaggtccgcgcggggaagtgggcggtgtgcggccggcaccgcctcgcaccacgcccccgcgggcccgcactttcccggagtgcaccccgcggccgccagccggggcggtaagtatcaaggttacaagacaggtttaaggagaccaatagaaactgggcttgtcgagacagagaagactcttgcgtttctgataggcacctattggtcttactgacatccactttgcctttctctccacaggaattccgccaccatggcggggctctggctggggctcgtgtggcagaagctgctgctgtggggcgcggcgagtgccctttccctggccggcgccagtctggtcctgagtctgctgcagagggtggcgagctacgcgcggaaatggcagcagatgcggcccatccccacggtggcccgcgcctacccactggtgggccacgcgctgctgatgaagccggacgggcgagaattttttcagcagatcattgagtacacagaggaataccgccacatgccgctgctgaagctctgggtcgggccagtgcccatggtggccctttataatgcagaaaatgtggaggtaattttaactagttcaaagcaaattgacaaatcctctatgtacaagtttttagaaccatggcttggcctaggacttcttacaagtactggaaacaaatggcgctccaggagaaagatgttaacacccactttccattttaccattctggaagatttcttagatatcatgaatgaacaagcaaatatattggttaagaaacttgaaaaacacattaaccaagaagcatttaactgctttttttacatcactctttgtgccttagatatcatctgtgaaacagctatggggaagaatattggtgctcaaagtaatgatgattccgagtatgtccgtgcagtttatagaatgagtgagatgatatttcgaagaataaagatgccctggctttggcttgatctctggtaccttatgtttaaagaaggatgggaacacaaaaagagccttcagatcctacatacttttaccaacagtgtcatcgcggaacgggccaatgaaatgaacgccaatgaagactgtagaggtgatggcaggggctctgccccctccaaaaataaacgcagggcctttcttgacttgcttttaagtgtgactgatgacgaagggaacaggctaagtcatgaagatattcgagaagaagttgacaccttcatgtttgaggggcacgatacaactgcagctgcaataaactggtccttatacctgttgggttctaacccagaagtccagaaaaaagtggatcatgaattggatgacgtgtttgggaagtctgaccgtcccgctacagtagaagacctgaagaaacttcggtatctggaatgtgttattaaggagacccttcgcctttttccttctgttcctttatttgcccgtagtgttagtgaagattgtgaagtggcaggttacagagttctaaaaggcactgaagccgtcatcattccctatgcattgcacagagatccgagatacttccccaaccccgaggagttccagcctgagcggttcttccccgagaatgcacaagggcgccatccatatgcctacgtgcccttctctgctggccccaggaactgtataggtcaaaagtttgctgtgatggaagaaaagaccattctttcgtgcatcctgaggcacttttggatagaatccaaccagaaaagagaagagcttggtctagaaggacagttgattcttcgtccaagtaatggcatctggatcaagttgaagaggagaaatgcagatgaacgctaaacgcgtggtttatccgatccaccggatctagataagatatccgatccaccggatctagataactgatcataatcagccataccacatttgtagaggttttacttgctttaaaaaacctcccacacctccccctgaacctgaaacataaaatgaatgcaattggcggccgcctcgagctgtgccttctagttgccagccatctgttgtttgcccctcccccgtgccttccttgaccctggaaggtgccactcccactgtcctttcctaataaaatgaggaaattgcatcgcattgtctgagtaggtgtcattctattctggggggtggggtggggcaggacagcaagggggaggattgggaagacaatagcaggcatgctggggatgcggtgggctctatggggtaaccacgtgcggacccaacggccgcaggaacccctagtgatggagttggccactccctctctgcgcgctcgctcgctcactgaggccgggcgaccaaaggtcgcccgacgcccgggctttgcccgggcggcctcagtgagcgagcgagcgcgcagctgcctgcaggggcgcctgatgcggtattttctccttacgcatctgtgcggtatttcacaccgcatacgtcaaagcaaccatagtacgcgccctgtagcggcacattaagcgcggcgggtgtggtggttacgcgcagcgtgaccgctacacttgccagcgccttagcgcccgctcctttcgctttcttcccttcctttctcgccacgttcgccggctttccccgtcaagctctaaatcgggggctccctttagggttccgatttagtgctttacggcacctcgaccccaaaaaacttgatttgggtgatggttcacgtagtgggccatcgccctgatagacggtttttcgccctttgacgttggagtccacgttctttaatagtggactcttgttccaaactggaacaacactcaactctatctcgggctattcttttgatttataagggattttgccgatttcggtctattggttaaaaaatgagctgatttaacaaaaatttaacgcgaattttaacaaaatattaacgtttacaattttatggtgcactctcagtacaatctgctctgatgccgcatagttaagccagccccgacacccgccaacacccgctgacgcgccctgacgggcttgtctgctcccggcatccgcttacagacaagctgtgaccgtctccgggagctgcatgtgtcagaggttttcaccgtcatcaccgaaacgcgcgagacgaaagggcctcgtgatacgcctatttttataggttaatgtcatgataataatggtttcttagacgtcaggtggcacttttcggggaaatgtgcgcggaacccctatttgtttatttttctaaatacattcaaatatgtatccgctcatgagacaataaccctgataaatgcttcaataatattgaaaaaggaagagtcctgaggcggaaagaaccagctgtggaatgtgtgtcagttagggtgtggaaagtccccaggctccccagcaggcagaagtatgcaaagcatgcatctcaattagtcagcaaccaggtgtggaaagtccccaggctccccagcaggcagaagtatgcaaagcatgcatctcaattagtcagcaaccatagtcccgcccctaactccgcccatcccgcccctaactccgcccagttccgcccattctccgccccatggctgactaattttttttatttatgcagaggccgaggccgcctcggcctctgagctattccagaagtagtgaggaggcttttttggaggcctaggcttttgcaaagatcgatcaagagacaggatgaggatcgtttcgcatgattgaacaagatggattgcacgcaggttctccggccgcttgggtggagaggctattcggctatgactgggcacaacagacaatcggctgctctgatgccgccgtgttccggctgtcagcgcaggggcgcccggttctttttgtcaagaccgacctgtccggtgccctgaatgaactgcaagacgaggcagcgcggctatcgtggctggccacgacgggcgttccttgcgcagctgtgctcgacgttgtcactgaagcgggaagggactggctgctattgggcgaagtgccggggcaggatctcctgtcatctcaccttgctcctgccgagaaagtatccatcatggctgatgcaatgcggcggctgcatacgcttgatccggctacctgcccattcgaccaccaagcgaaacatcgcatcgagcgagcacgtactcggatggaagccggtcttgtcgatcaggatgatctggacgaagagcatcaggggctcgcgccagccgaactgttcgccaggctcaaggcgagcatgcccgacggcgaggatctcgtcgtgacccatggcgatgcctgcttgccgaatatcatggtggaaaatggccgcttttctggattcatcgactgtggccggctgggtgtggcggaccgctatcaggacatagcgttggctacccgtgatattgctgaagagcttggcggcgaatgggctgaccgcttcctcgtgctttacggtatcgccgctcccgattcgcagcgcatcgccttctatcgccttcttgacgagttcttctgactgtcagaccaagtttactcatatatactttagattgatttaaaacttcatttttaatttaaaaggatctaggtgaagatcctttttgataatctcatgaccaaaatcccttaacgtgagttttcgttccactgagcgtcagaccccgtagaaaagatcaaaggatcttcttgagatcctttttttctgcgcgtaatctgctgcttgcaaacaaaaaaaccaccgctaccagcggtggtttgtttgccggatcaagagctaccaactctttttccgaaggtaactggcttcagcagagcgcagataccaaatactgttcttctagtgtagccgtagttaggccaccacttcaagaactctgtagcaccgcctacatacctcgctctgctaatcctgttaccagtggctgctgccagtggcgataagtcgtgtcttaccgggttggactcaagacgatagttaccggataaggcgcagcggtcgggctgaacggggggttcgtgcacacagcccagcttggagcgaacgacctacaccgaactgagatacctacagcgtgagctatgagaaagcgccacgcttcccgaagggagaaaggcggacaggtatccggtaagcggcagggtcggaacaggagagcgcacgagggagcttccagggggaaacgcctggtatctttatagtcctgtcgggtttcgccacctctgacttgagcgtcgatttttgtgatgctcgtcaggggggcggagcctatggaaaaacgccagcaacgcggcctttttacggttcctggccttttgctggccttttgctcacatgt

SEQ ID NO: 119 - DNA, 5884 bp, synthetic construct
  misc_feature 1..5884: note = pAV-p5-CDS intron-CYP4V2-BGH
  source 1..5884: mol_type = other DNA
cctgcaggcagctgcgcgctcgctcgctcactgaggccgcccgggcgtcgggcgacctttggtcgcccggcctcagtgagcgagcgagcgcgcagagagggagtggccaactccatcactaggggttcctgcggccggtcgcgtctagtactagtcgcgtaggatccgagccggatgcgccttcctttcctctccagagcaggctgcccgcccgcggaatcccgcacgtagagcaacctcgcagcaccctcagaacagccccgctggggcgcgccgggctgccgcggtgacctttccgacgcccctgaccccgcatccggaggcggccggaagtgtcgccggcctcctcccggcgcagcctccgggcctccagtgcaatcactacgccctggggcccggaaaccgttttccggtctttcgctttcggctggggcgtggaggccgcggtgctgcgtaggccgggccgggcgcaggaacagccccgtggcgccctctctggccgccgcccgggcgggaaacgtcgttccggggaccgggcgaccccgcagcggggagcgcgccaggtccgcgcggggaagtgggcggtgtgcggccggcaccgcctcgcaccacgcccccgcgggcccgcactttcccggagtgcaccccgcggccgccagccggggcggaattcgccaccatggcggggctctggctggggctcgtgtggcagaagctgctgctgtggggcgcggcgagtgccctttccctggccggcgccagtctggtcctgagtctgctgcagagggtggcgagctacgcgcggaaatggcagcagatgcggcccatccccacggtggcccgcgcctacccactggtgggccacgcgctgctgatgaagccggacgggcgaggtaagtatcaaggttacaagacaggtttaaggagaccaatagaaactgggcttgtcgagacagagaagactcttgcgtttctgataggcacctattggtcttactgacatccactttgcctttctctccacagaattttttcagcagatcattgagtacacagaggaataccgccacatgccgctgctgaagctctgggtcgggccagtgcccatggtggccctttataatgcagaaaatgtggaggtaattttaactagttcaaagcaaattgacaaatcctctatgtacaagtttttagaaccatggcttggcctaggacttcttacaagtactggaaacaaatggcgctccaggagaaagatgttaacacccactttccattttaccattctggaagatttcttagatatcatgaatgaacaagcaaatatattggttaagaaacttgaaaaacacattaaccaagaagcatttaactgctttttttacatcactctttgtgccttagatatcatctgtgaaacagctatggggaagaatattggtgctcaaagtaatgatgattccgagtatgtccgtgcagtttatagaatgagtgagatgatatttcgaagaataaagatgccctggctttggcttgatctctggtaccttatgtttaaagaaggatgggaacacaaaaagagccttcagatcctacatacttttaccaacagtgtcatcgcggaacgggccaatgaaatgaacgccaatgaagactgtagaggtgatggcaggggctctgccccctccaaaaataaacgcagggcctttcttgacttgcttttaagtgtgactgatgacgaagggaacaggctaagtcatgaagatattcgagaagaagttgacaccttcatgtttgaggggcacgatacaactgcagctgcaataaactggtccttatacctgttgggttctaacccagaagtccagaaaaaagtggatcatgaattggatgacgtgtttgggaagtctgaccgtcccgctacagtagaagacctgaagaaacttcggtatctggaatgtgttattaaggagacccttcgcctttttccttctgttcctttatttgcccgtagtgttagtgaagattgtgaagtggcaggttacagagttctaaaaggcactgaagccgtcatcattccctatgcattgcacagagatccgagatacttccccaaccccgaggagttccagcctgagcggttcttccccgagaatgcacaagggcgccatccatatgcctacgtgcccttctctgctggccccaggaactgtataggtcaaaagtttgctgtgatggaagaaaagaccattctttcgtgcatcctgaggcacttttggatagaatccaaccagaaaagagaagagcttggtctagaaggacagttgattcttcgtccaagtaatggcatctggatcaagttgaagaggagaaatgcagatgaacgctaaacgcgtggtttatccgatccaccggatctagataagatatccgatccaccggatctagataactgatcataatcagccataccacatttgtagaggttttacttgctttaaaaaacctcccacacctccccctgaacctgaaacataaaatgaatgcaattggcggccgcctcgagctgtgccttctagttgccagccatctgttgtttgcccctcccccgtgccttccttgaccctggaaggtgccactcccactgtcctttcctaataaaatgaggaaattgcatcgcattgtctgagtaggtgtcattctattctggggggtggggtggggcaggacagcaagggggaggattgggaagacaatagcaggcatgctggggatgcggtgggctctatggggtaaccacgtgcggacccaacggccgcaggaacccctagtgatggagttggccactccctctctgcgcgctcgctcgctcactgaggccgggcgaccaaaggtcgcccgacgcccgggctttgcccgggcggcctcagtgagcgagcgagcgcgcagctgcctgcaggggcgcctgatgcggtattttctccttacgcatctgtgcggtatttcacaccgcatacgtcaaagcaaccatagtacgcgccctgtagcggcacattaagcgcggcgggtgtggtggttacgcgcagcgtgaccgctacacttgccagcgccttagcgcccgctcctttcgctttcttcccttcctttctcgccacgttcgccggctttccccgtcaagctctaaatcgggggctccctttagggttccgatttagtgctttacggcacctcgaccccaaaaaacttgatttgggtgatggttcacgtagtgggccatcgccctgatagacggtttttcgccctttgacgttggagtccacgttctttaatagtggactcttgttccaaactggaacaacactcaactctatctcgggctattcttttgatttataagggattttgccgatttcggtctattggttaaaaaatgagctgatttaacaaaaatttaacgcgaattttaacaaaatattaacgtttacaattttatggtgcactctcagtacaatctgctctgatgccgcatagttaagccagccccgacacccgccaacacccgctgacgcgccctgacgggcttgtctgctcccggcatccgcttacagacaagctgtgaccgtctccgggagctgcatgtgtcagaggttttcaccgtcatcaccgaaacgcgcgagacgaaagggcctcgtgatacgcctatttttataggttaatgtcatgataataatggtttcttagacgtcaggtggcacttttcggggaaatgtgcgcggaacccctatttgtttatttttctaaatacattcaaatatgtatccgctcatgagacaataaccctgataaatgcttcaataatattgaaaaaggaagagtcctgaggcggaaagaaccagctgtggaatgtgtgtcagttagggtgtggaaagtccccaggctccccagcaggcagaagtatgcaaagcatgcatctcaattagtcagcaaccaggtgtggaaagtccccaggctccccagcaggcagaagtatgcaaagcatgcatctcaattagtcagcaaccatagtcccgcccctaactccgcccatcccgcccctaactccgcccagttccgcccattctccgccccatggctgactaattttttttatttatgcagaggccgaggccgcctcggcctctgagctattccagaagtagtgaggaggcttttttggaggcctaggcttttgcaaagatcgatcaagagacaggatgaggatcgtttcgcatgattgaacaagatggattgcacgcaggttctccggccgcttgggtggagaggctattcggctatgactgggcacaacagacaatcggctgctctgatgccgccgtgttccggctgtcagcgcaggggcgcccggttctttttgtcaagaccgacctgtccggtgccctgaatgaactgcaagacgaggcagcgcggctatcgtggctggccacgacgggcgttccttgcgcagctgtgctcgacgttgtcactgaagcgggaagggactggctgctattgggcgaagtgccggggcaggatctcctgtcatctcaccttgctcctgccgagaaagtatccatcatggctgatgcaatgcggcggctgcatacgcttgatccggctacctgcccattcgaccaccaagcgaaacatcgcatcgagcgagcacgtactcggatggaagccggtcttgtcgatcaggatgatctggacgaagagcatcaggggctcgcgccagccgaactgttcgccaggctcaaggcgagcatgcccgacggcgaggatctcgtcgtgacccatggcgatgcctgcttgccgaatatcatggtggaaaatggccgcttttctggattcatcgactgtggccggctgggtgtggcggaccgctatcaggacatagcgttggctacccgtgatattgctgaagagcttggcggcgaatgggctgaccgcttcctcgtgctttacggtatcgccgctcccgattcgcagcgcatcgccttctatcgccttcttgacgagttcttctgactgtcagaccaagtttactcatatatactttagattgatttaaaacttcatttttaatttaaaaggatctaggtgaagatcctttttgataatctcatgaccaaaatcccttaacgtgagttttcgttccactgagcgtcagaccccgtagaaaagatcaaaggatcttcttgagatcctttttttctgcgcgtaatctgctgcttgcaaacaaaaaaaccaccgctaccagcggtggtttgtttgccggatcaagagctaccaactctttttccgaaggtaactggcttcagcagagcgcagataccaaatactgttcttctagtgtagccgtagttaggccaccacttcaagaactctgtagcaccgcctacatacctcgctctgctaatcctgttaccagtggctgctgccagtggcgataagtcgtgtcttaccgggttggactcaagacgatagttaccggataaggcgcagcggtcgggctgaacggggggttcgtgcacacagcccagcttggagcgaacgacctacaccgaactgagatacctacagcgtgagctatgagaaagcgccacgcttcccgaagggagaaaggcggacaggtatccggtaagcggcagggtcggaacaggagagcgcacgagggagcttccagggggaaacgcctggtatctttatagtcctgtcgggtttcgccacctctgacttgagcgtcgatttttgtgatgctcgtcaggggggcggagcctatggaaaaacgccagcaacgcggcctttttacggttcctggccttttgctggccttttgctcacatgt

SEQ ID NO: 120 - DNA, 4276 bp, synthetic construct
  misc_feature 1..4276: note = pAV-p5-RdCVF
  source 1..4276: mol_type = other DNA
cctgcaggcagctgcgcgctcgctcgctcactgaggccgcccgggcgtcgggcgacctttggtcgcccggcctcagtgagcgagcgagcgcgcagagagggagtggccaactccatcactaggggttcctgcggccggtcgcgtctagtactagtcgcgtaggatccgagccggatgcgccttcctttcctctccagagcaggctgcccgcccgcggaatcccgcacgtagagcaacctcgcagcaccctcagaacagccccgctggggcgcgccgggctgccgcggtgacctttccgacgcccctgaccccgcatccggaggcggccggaagtgtcgccggcctcctcccggcgcagcctccgggcctccagtgcaatcactacgccctggggcccggaaaccgttttccggtctttcgctttcggctggggcgtggaggccgcggtgctgcgtaggccgggccgggcgcaggaacagccccgtggcgccctctctggccgccgcccgggcgggaaacgtcgttccggggaccgggcgaccccgcagcggggagcgcgccaggtccgcgcggggaagtgggcggtgtgcggccggcaccgcctcgcaccacgcccccgcgggcccgcactttcccggagtgcaccccgcggccgccagccggggcggaattccgccaccatggcctccctgttctctggccgcatcctgatccgcaacaatagcgaccaggacgagctggatacggaggctgaggtcagtcgcaggctggagaaccggctggtgctgctgttctttggtgctggggcttgtccacagtgccaggccttcgtgcccatcctcaaggacttcttcgtgcggctcacagatgagttctatgtactgcgggcggctcagctggccctggtgtacgtgtcccaggactccacggaggagcagcaggacctgttcctcaaggacatgccaaagaaatggcttttcctgccctttgaggatgatctgaggaggtgataaacgcgtggtttatccgatccaccggatctagataagatatccgatccaccggatctagataactgatcataatcagccataccacatttgtagaggttttacttgctttaaaaaacctcccacacctccccctgaacctgaaacataaaatgaatgcaattggcggccgcctcgagcacgtgcggacccaacggccgcaggaacccctagtgatggagttggccactccctctctgcgcgctcgctcgctcactgaggccgggcgaccaaaggtcgcccgacgcccgggctttgcccgggcggcctcagtgagcgagcgagcgcgcagctgcctgcaggggcgcctgatgcggtattttctccttacgcatctgtgcggtatttcacaccgcatacgtcaaagcaaccatagtacgcgccctgtagcggcacattaagcgcggcgggtgtggtggttacgcgcagcgtgaccgctacacttgccagcgccttagcgcccgctcctttcgctttcttcccttcctttctcgccacgttcgccggctttccccgtcaagctctaaatcgggggctccctttagggttccgatttagtgctttacggcacctcgaccccaaaaaacttgatttgggtgatggttcacgtagtgggccatcgccctgatagacggtttttcgccctttgacgttggagtccacgttctttaatagtggactcttgttccaaactggaacaacactcaactctatctcgggctattcttttgatttataagggattttgccgatttcggtctattggttaaaaaatgagctgatttaacaaaaatttaacgcgaattttaacaaaatattaacgtttacaattttatggtgcactctcagtacaatctgctctgatgccgcatagttaagccagccccgacacccgccaacacccgctgacgcgccctgacgggcttgtctgctcccggcatccgcttacagacaagctgtgaccgtctccgggagctgcatgtgtcagaggttttcaccgtcatcaccgaaacgcgcgagacgaaagggcctcgtgatacgcctatttttataggttaatgtcatgataataatggtttcttagacgtcaggtggcacttttcggggaaatgtgcgcggaacccctatttgtttatttttctaaatacattcaaatatgtatccgctcatgagacaataaccctgataaatgcttcaataatattgaaaaaggaagagtcctgaggcggaaagaaccagctgtggaatgtgtgtcagttagggtgtggaaagtccccaggctccccagcaggcagaagtatgcaaagcatgcatctcaattagtcagcaaccaggtgtggaaagtccccaggctccccagcaggcagaagtatgcaaagcatgcatctcaattagtcagcaaccatagtcccgcccctaactccgcccatcccgcccctaactccgcccagttccgcccattctccgccccatggctgactaattttttttatttatgcagaggccgaggccgcctcggcctctgagctattccagaagtagtgaggaggcttttttggaggcctaggcttttgcaaagatcgatcaagagacaggatgaggatcgtttcgcatgattgaacaagatggattgcacgcaggttctccggccgcttgggtggagaggctattcggctatgactgggcacaacagacaatcggctgctctgatgccgccgtgttccggctgtcagcgcaggggcgcccggttctttttgtcaagaccgacctgtccggtgccctgaatgaactgcaagacgaggcagcgcggctatcgtggctggccacgacgggcgttccttgcgcagctgtgctcgacgttgtcactgaagcgggaagggactggctgctattgggcgaagtgccggggcaggatctcctgtcatctcaccttgctcctgccgagaaagtatccatcatggctgatgcaatgcggcggctgcatacgcttgatccggctacctgcccattcgaccaccaagcgaaacatcgcatcgagcgagcacgtactcggatggaagccggtcttgtcgatcaggatgatctggacgaagagcatcaggggctcgcgccagccgaactgttcgccaggctcaaggcgagcatgcccgacggcgaggatctcgtcgtgacccatggcgatgcctgcttgccgaatatcatggtggaaaatggccgcttttctggattcatcgactgtggccggctgggtgtggcggaccgctatcaggacatagcgttggctacccgtgatattgctgaagagcttggcggcgaatgggctgaccgcttcctcgtgctttacggtatcgccgctcccgattcgcagcgcatcgccttctatcgccttcttgacgagttcttctgactgtcagaccaagtttactcatatatactttagattgatttaaaacttcatttttaatttaaaaggatctaggtgaagatcctttttgataatctcatgaccaaaatcccttaacgtgagttttcgttccactgagcgtcagaccccgtagaaaagatcaaaggatcttcttgagatcctttttttctgcgcgtaatctgctgcttgcaaacaaaaaaaccaccgctaccagcggtggtttgtttgccggatcaagagctaccaactctttttccgaaggtaactggcttcagcagagcgcagataccaaatactgttcttctagtgtagccgtagttaggccaccacttcaagaactctgtagcaccgcctacatacctcgctctgctaatcctgttaccagtggctgctgccagtggcgataagtcgtgtcttaccgggttggactcaagacgatagttaccggataaggcgcagcggtcgggctgaacggggggttcgtgcacacagcccagcttggagcgaacgacctacaccgaactgagatacctacagcgtgagctatgagaaagcgccacgcttcccgaagggagaaaggcggacaggtatccggtaagcggcagggtcggaacaggagagcgcacgagggagcttccagggggaaacgcctggtatctttatagtcctgtcgggtttcgccacctctgacttgagcgtcgatttttgtgatgctcgtcaggggggcggagcctatggaaaaacgccagcaacgcggcctttttacggttcctggccttttgctggccttttgctcacatgt

SEQ ID NO: 121 - DNA, 4637 bp, synthetic construct
  misc_feature 1..4637: note = pAV-p5-intron-RdCVF-BGH
  source 1..4637: mol_type = other DNA
cctgcaggcagctgcgcgctcgctcgctcactgaggccgcccgggcgtcgggcgacctttggtcgcccggcctcagtgagcgagcgagcgcgcagagagggagtggccaactccatcactaggggttcctgcggccggtcgcgtctagtactagtcgcgtaggatccgagccggatgcgccttcctttcctctccagagcaggctgcccgcccgcggaatcccgcacgtagagcaacctcgcagcaccctcagaacagccccgctggggcgcgccgggctgccgcggtgacctttccgacgcccctgaccccgcatccggaggcggccggaagtgtcgccggcctcctcccggcgcagcctccgggcctccagtgcaatcactacgccctggggcccggaaaccgttttccggtctttcgctttcggctggggcgtggaggccgcggtgctgcgtaggccgggccgggcgcaggaacagccccgtggcgccctctctggccgccgcccgggcgggaaacgtcgttccggggaccgggcgaccccgcagcggggagcgcgccaggtccgcgcggggaagtgggcggtgtgcggccggcaccgcctcgcaccacgcccccgcgggcccgcactttcccggagtgcaccccgcggccgccagccggggcggtaagtatcaaggttacaagacaggtttaaggagaccaatagaaactgggcttgtcgagacagagaagactcttgcgtttctgataggcacctattggtcttactgacatccactttgcctttctctccacaggaattccgccaccatggcctccctgttctctggccgcatcctgatccgcaacaatagcgaccaggacgagctggatacggaggctgaggtcagtcgcaggctggagaaccggctggtgctgctgttctttggtgctggggcttgtccacagtgccaggccttcgtgcccatcctcaaggacttcttcgtgcggctcacagatgagttctatgtactgcgggcggctcagctggccctggtgtacgtgtcccaggactccacggaggagcagcaggacctgttcctcaaggacatgccaaagaaatggcttttcctgccctttgaggatgatctgaggaggtaaacgcgtggtttatccgatccaccggatctagataagatatccgatccaccggatctagataactgatcataatcagccataccacatttgtagaggttttacttgctttaaaaaacctcccacacctccccctgaacctgaaacataaaatgaatgcaattggcggccgcctcgagctgtgccttctagttgccagccatctgttgtttgcccctcccccgtgccttccttgaccctggaaggtgccactcccactgtcctttcctaataaaatgaggaaattgcatcgcattgtctgagtaggtgtcattctattctggggggtggggtggggcaggacagcaagggggaggattgggaagacaatagcaggcatgctggggatgcggtgggctctatggggtaaccacgtgcggacccaacggccgcaggaacccctagtgatggagttggccactccctctctgcgcgctcgctcgctcactgaggccgggcgaccaaaggtcgcccgacgcccgggctttgcccgggcggcctcagtgagcgagcgagcgcgcagctgcctgcaggggcgcctgatgcggtattttctccttacgcatctgtgcggtatttcacaccgcatacgtcaaagcaaccatagtacgcgccctgtagcggcacattaagcgcggcgggtgtggtggttacgcgcagcgtgaccgctacacttgccagcgccttagcgcccgctcctttcgctttcttcccttcctttctcgccacgttcgccggctttccccgtcaagctctaaatcgggggctccctttagggttccgatttagtgctttacggcacctcgaccccaaaaaacttgatttgggtgatggttcacgtagtgggccatcgccctgatagacggtttttcgccctttgacgttggagtccacgttctttaatagtggactcttgttccaaactggaacaacactcaactctatctcgggctattcttttgatttataagggattttgccgatttcggtctattggttaaaaaatgagctgatttaacaaaaatttaacgcgaattttaacaaaatattaacgtttacaattttatggtgcactctcagtacaatctgctctgatgccgcatagttaagccagccccgacacccgccaacacccgctgacgcgccctgacgggcttgtctgctcccggcatccgcttacagacaagctgtgaccgtctccgggagctgcatgtgtcagaggttttcaccgtcatcaccgaaacgcgcgagacgaaagggcctcgtgatacgcctatttttataggttaatgtcatgataataatggtttcttagacgtcaggtggcacttttcggggaaatgtgcgcggaacccctatttgtttatttttctaaatacattcaaatatgtatccgctcatgagacaataaccctgataaatgcttcaataatattgaaaaaggaagagtcctgaggcggaaagaaccagctgtggaatgtgtgtcagttagggtgtggaaagtccccaggctccccagcaggcagaagtatgcaaagcatgcatctcaattagtcagcaaccaggtgtggaaagtccccaggctccccagcaggcagaagtatgcaaagcatgcatctcaattagtcagcaaccatagtcccgcccctaactccgcccatcccgcccctaactccgcccagttccgcccattctccgccccatggctgactaattttttttatttatgcagaggccgaggccgcctcggcctctgagctattccagaagtagtgaggaggcttttttggaggcctaggcttttgcaaagatcgatcaagagacaggatgaggatcgtttcgcatgattgaacaagatggattgcacgcaggttctccggccgcttgggtggagaggctattcggctatgactgggcacaacagacaatcggctgctctgatgccgccgtgttccggctgtcagcgcaggggcgcccggttctttttgtcaagaccgacctgtccggtgccctgaatgaactgcaagacgaggcagcgcggctatcgtggctggccacgacgggcgttccttgcgcagctgtgctcgacgttgtcactgaagcgggaagggactggctgctattgggcgaagtgccggggcaggatctcctgtcatctcaccttgctcctgccgagaaagtatccatcatggctgatgcaatgcggcggctgcatacgcttgatccggctacctgcccattcgaccaccaagcgaaacatcgcatcgagcgagcacgtactcggatggaagccggtcttgtcgatcaggatgatctggacgaagagcatcaggggctcgcgccagccgaactgttcgccaggctcaaggcgagcatgcccgacggcgaggatctcgtcgtgacccatggcgatgcctgcttgccgaatatcatggtggaaaatggccgcttttctggattcatcgactgtggccggctgggtgtggcggaccgctatcaggacatagcgttggctacccgtgatattgctgaagagcttggcggcgaatgggctgaccgcttcctcgtgctttacggtatcgccgctcccgattcgcagcgcatcgccttctatcgccttcttgacgagttcttctgactgtcagaccaagtttactcatatatactttagattgatttaaaacttcatttttaatttaaaaggatctaggtgaagatcctttttgataatctcatgaccaaaatcccttaacgtgagttttcgttccactgagcgtcagaccccgtagaaaagatcaaaggatcttcttgagatcctttttttctgcgcgtaatctgctgcttgcaaacaaaaaaaccaccgctaccagcggtggtttgtttgccggatcaagagctaccaactctttttccgaaggtaactggcttcagcagagcgcagataccaaatactgttcttctagtgtagccgtagttaggccaccacttcaagaactctgtagcaccgcctacatacctcgctctgctaatcctgttaccagtggctgctgccagtggcgataagtcgtgtcttaccgggttggactcaagacgatagttaccggataaggcgcagcggtcgggctgaacggggggttcgtgcacacagcccagcttggagcgaacgacctacaccgaactgagatacctacagcgtgagctatgagaaagcgccacgcttcccgaagggagaaaggcggacaggtatccggtaagcggcagggtcggaacaggagagcgcacgagggagcttccagggggaaacgcctggtatctttatagtcctgtcgggtttcgccacctctgacttgagcgtcgatttttgtgatgctcgtcaggggggcggagcctatggaaaaacgccagcaacgcggcctttttacggttcctggccttttgctggccttttgctcacatgt

SEQ ID NO: 122 - DNA, 5917 bp, synthetic construct
  misc_feature 1..5917: note = pAV-p5-CYP4V2-P2A-RdCV
  source 1..5917: mol_type = other DNA
cctgcaggcagctgcgcgctcgctcgctcactgaggccgcccgggcgtcgggcgacctttggtcgcccggcctcagtgagcgagcgagcgcgcagagagggagtggccaactccatcactaggggttcctgcggccggtcgcgtctagtactagtcgcgtaggatccgagccggatgcgccttcctttcctctccagagcaggctgcccgcccgcggaatcccgcacgtagagcaacctcgcagcaccctcagaacagccccgctggggcgcgccgggctgccgcggtgacctttccgacgcccctgaccccgcatccggaggcggccggaagtgtcgccggcctcctcccggcgcagcctccgggcctccagtgcaatcactacgccctggggcccggaaaccgttttccggtctttcgctttcggctggggcgtggaggccgcggtgctgcgtaggccgggccgggcgcaggaacagccccgtggcgccctctctggccgccgcccgggcgggaaacgtcgttccggggaccgggcgaccccgcagcggggagcgcgccaggtccgcgcggggaagtgggcggtgtgcggccggcaccgcctcgcaccacgcccccgcgggcccgcactttcccggagtgcaccccgcggccgccagccggggcggaattccgccaccatggcggggctctggctggggctcgtgtggcagaagctgctgctgtggggcgcggcgagtgccctttccctggccggcgccagtctggtcctgagtctgctgcagagggtggcgagctacgcgcggaaatggcagcagatgcggcccatccccacggtggcccgcgcctacccactggtgggccacgcgctgctgatgaagccggacgggcgagaattttttcagcagatcattgagtacacagaggaataccgccacatgccgctgctgaagctctgggtcgggccagtgcccatggtggccctttataatgcagaaaatgtggaggtaattttaactagttcaaagcaaattgacaaatcctctatgtacaagtttttagaaccatggcttggcctaggacttcttacaagtactggaaacaaatggcgctccaggagaaagatgttaacacccactttccattttaccattctggaagatttcttagatatcatgaatgaacaagcaaatatattggttaagaaacttgaaaaacacattaaccaagaagcatttaactgctttttttacatcactctttgtgccttagatatcatctgtgaaacagctatggggaagaatattggtgctcaaagtaatgatgattccgagtatgtccgtgcagtttatagaatgagtgagatgatatttcgaagaataaagatgccctggctttggcttgatctctggtaccttatgtttaaagaaggatgggaacacaaaaagagccttcagatcctacatacttttaccaacagtgtcatcgcggaacgggccaatgaaatgaacgccaatgaagactgtagaggtgatggcaggggctctgccccctccaaaaataaacgcagggcctttcttgacttgcttttaagtgtgactgatgacgaagggaacaggctaagtcatgaagatattcgagaagaagttgacaccttcatgtttgaggggcacgatacaactgcagctgcaataaactggtccttatacctgttgggttctaacccagaagtccagaaaaaagtggatcatgaattggatgacgtgtttgggaagtctgaccgtcccgctacagtagaagacctgaagaaacttcggtatctggaatgtgttattaaggagacccttcgcctttttccttctgttcctttatttgcccgtagtgttagtgaagattgtgaagtggcaggttacagagttctaaaaggcactgaagccgtcatcattccctatgcattgcacagagatccgagatacttccccaaccccgaggagttccagcctgagcggttcttccccgagaatgcacaagggcgccatccatatgcctacgtgcccttctctgctggccccaggaactgtataggtcaaaagtttgctgtgatggaagaaaagaccattctttcgtgcatcctgaggcacttttggatagaatccaaccagaaaagagaagagcttggtctagaaggacagttgattcttcgtccaagtaatggcatctggatcaagttgaagaggagaaatgcagatgaacgcggaagcggagctactaacttcagcctgctgaagcaggctggagacgtggaggagaaccctggacctatggcctccctgttctctggccgcatcctgatccgcaacaatagcgaccaggacgagctggatacggaggctgaggtcagtcgcaggctggagaaccggctggtgctgctgttctttggtgctggggcttgtccacagtgccaggccttcgtgcccatcctcaaggacttcttcgtgcggctcacagatgagttctatgtactgcgggcggctcagctggccctggtgtacgtgtcccaggactccacggaggagcagcaggacctgttcctcaaggacatgccaaagaaatggcttttcctgccctttgaggatgatctgaggaggtgataaacgcgtggtttatccgatccaccggatctagataagatatccgatccaccggatctagataactgatcataatcagccataccacatttgtagaggttttacttgctttaaaaaacctcccacacctccccctgaacctgaaacataaaatgaatgcaattggcggccgcctcgagcacgtgcggacccaacggccgcaggaacccctagtgatggagttggccactccctctctgcgcgctcgctcgctcactgaggccgggcgaccaaaggtcgcccgacgcccgggctttgcccgggcggcctcagtgagcgagcgagcgcgcagctgcctgcaggggcgcctgatgcggtattttctccttacgcatctgtgcggtatttcacaccgcatacgtcaaagcaaccatagtacgcgccctgtagcggcacattaagcgcggcgggtgtggtggttacgcgcagcgtgaccgctacacttgccagcgccttagcgcccgctcctttcgctttcttcccttcctttctcgccacgttcgccggctttccccgtcaagctctaaatcgggggctccctttagggttccgatttagtgctttacggcacctcgaccccaaaaaacttgatttgggtgatggttcacgtagtgggccatcgccctgatagacggtttttcgccctttgacgttggagtccacgttctttaatagtggactcttgttccaaactggaacaacactcaactctatctcgggctattcttttgatttataagggattttgccgatttcggtctattggttaaaaaatgagctgatttaacaaaaatttaacgcgaattttaacaaaatattaacgtttacaattttatggtgcactctcagtacaatctgctctgatgccgcatagttaagccagccccgacacccgccaacacccgctgacgcgccctgacgggcttgtctgctcccggcatccgcttacagacaagctgtgaccgtctccgggagctgcatgtgtcagaggttttcaccgtcatcaccgaaacgcgcgagacgaaagggcctcgtgatacgcctatttttataggttaatgtcatgataataatggtttcttagacgtcaggtggcacttttcggggaaatgtgcgcggaacccctatttgtttatttttctaaatacattcaaatatgtatccgctcatgagacaataaccctgataaatgcttcaataatattgaaaaaggaagagtcctgaggcggaaagaaccagctgtggaatgtgtgtcagttagggtgtggaaagtccccaggctccccagcaggcagaagtatgcaaagcatgcatctcaattagtcagcaaccaggtgtggaaagtccccaggctccccagcaggcagaagtatgcaaagcatgcatctcaattagtcagcaaccatagtcccgcccctaactccgcccatcccgcccctaactccgcccagttccgcccattctccgccccatggctgactaattttttttatttatgcagaggccgaggccgcctcggcctctgagctattccagaagtagtgaggaggcttttttggaggcctaggcttttgcaaagatcgatcaagagacaggatgaggatcgtttcgcatgattgaacaagatggattgcacgcaggttctccggccgcttgggtggagaggctattcggctatgactgggcacaacagacaatcggctgctctgatgccgccgtgttccggctgtcagcgcaggggcgcccggttctttttgtcaagaccgacctgtccggtgccctgaatgaactgcaagacgaggcagcgcggctatcgtggctggccacgacgggcgttccttgcgcagctgtgctcgacgttgtcactgaagcgggaagggactggctgctattgggcgaagtgccggggcaggatctcctgtcatctcaccttgctcctgccgagaaagtatccatcatggctgatgcaatgcggcggctgcatacgcttgatccggctacctgcccattcgaccaccaagcgaaacatcgcatcgagcgagcacgtactcggatggaagccggtcttgtcgatcaggatgatctggacgaagagcatcaggggctcgcgccagccgaactgttcgccaggctcaaggcgagcatgcccgacggcgaggatctcgtcgtgacccatggcgatgcctgcttgccgaatatcatggtggaaaatggccgcttttctggattcatcgactgtggccggctgggtgtggcggaccgctatcaggacatagcgttggctacccgtgatattgctgaagagcttggcggcgaatgggctgaccgcttcctcgtgctttacggtatcgccgctcccgattcgcagcgcatcgccttctatcgccttcttgacgagttcttctgactgtcagaccaagtttactcatatatactttagattgatttaaaacttcatttttaatttaaaaggatctaggtgaagatcctttttgataatctcatgaccaaaatcccttaacgtgagttttcgttccactgagcgtcagaccccgtagaaaagatcaaaggatcttcttgagatcctttttttctgcgcgtaatctgctgcttgcaaacaaaaaaaccaccgctaccagcggtggtttgtttgccggatcaagagctaccaactctttttccgaaggtaactggcttcagcagagcgcagataccaaatactgttcttctagtgtagccgtagttaggccaccacttcaagaactctgtagcaccgcctacatacctcgctctgctaatcctgttaccagtggctgctgccagtggcgataagtcgtgtcttaccgggttggactcaagacgatagttaccggataaggcgcagcggtcgggctgaacggggggttcgtgcacacagcccagcttggagcgaacgacctacaccgaactgagatacctacagcgtgagctatgagaaagcgccacgcttcccgaagggagaaaggcggacaggtatccggtaagcggcagggtcggaacaggagagcgcacgagggagcttccagggggaaacgcctggtatctttatagtcctgtcgggtttcgccacctctgacttgagcgtcgatttttgtgatgctcgtcaggggggcggagcctatggaaaaacgccagcaacgcggcctttttacggttcctggccttttgctggccttttgctcacatgt

SEQ ID NO: 123 - DNA, 7648 bp, synthetic construct
  misc_feature 1..7648: note = pAV-Pf-CYP4V2-P2A-RdCVF
  source 1..7648: mol_type = other DNA
cctgcaggcagctgcgcgctcgctcgctcactgaggccgcccgggcgtcgggcgacctttggtcgcccggcctcagtgagcgagcgagcgcgcagagagggagtggccaactccatcactaggggttcctgcggccggtcgcgtctagtactagtcgcgtaggatccacccacctcatcctgcacctgtcactgcgtgggaccctgtgctccaggcaggggcacctcactgccccctgagctcattttacccctcctggctctgcagcatttctgaccatttctgcccaggccgagactcactgctgcccagagcaatctcccttctctccttctggaggggaggggttgtatgttacccgcctggttttatccacagaggttagcagagactgatacagacaaaccctttttctttctaattttagattcaagagcacatgtgcaggtttgttaaatttgcctgacgctgaggtttgagtttctattgatcccctcacctgaatagggaacacagtacccaatacacagtttttcaaccattactccccttccttcctccccctattttagaatccccagtatgtagacaaattgtttacttttatagctgtaattaaccttattatagctcagcctcaaccctttagagaggaggaaactaaagcccatgagacttgcttaaagatactaagtgaacatatttattttttaaagtgttaaagtgattaaacaatgtagacgtgaatgaaataaaaagcgtaagttccccatcttcattcccactccatagagctgatcagtatttttacttgcagacattagtggagccgtagagaaagaaaccttttctccaaaagaaggcattactttacacactccgttctgcaacttgttttgttcacttgctatttcacgtcagcccatgcagatgacttaaaacaaattcaaatggagaaaagccttaggcatgtttttctctgcactaaagaggccctgcaggtggctgtggccaacttatgcagtggcttcgagtgaacgaacgtaattagtaattaagcaaagcgggcatccaggacattcagtttcatcttcctggcactttagtgtttaggaagggcctggcctctcggggagcgacactcctcgcccggccactttgtaagaagcatcgagcgtggaaaaggggctggggtcagcactggggccctctgccgggaagagagactggcggccagcacacgcgtctccccaggctgaaatggggcaccctctcgcggcccttccctcccttcccgggctgggtggcaggtcttggctcttctgcgagtaccccgcggctgcggtctcccggcacccgctgagcagcctcgcccgccttcctctcccacccgcccctgcgtgctctccggggctccggcttcctcggtctggtgcctggtgcgtattttggaaaatacctggctcataaccacctcattgagctcccagtgtcccagtgggccagcggacacacacgggtagctgacttccctaacgtgtccccaaagcctccctggattacagcgcccgctgctccatgtgaccccgcgggagccaggacgcgccccgcctcccggggctgcaagttgcgcagggagcgagcgatgcgcagcagagctgggctccgagccggatgcgccttcctttcctctccagagcaggctgcccgcccgcggaatcccgcacgtagagcaacctcgcagcaccctcagaacagccccgctggggcgcgccgggctgccgcggtgacctttccgacgcccctgaccccgcatccggaggcggccggaagtgtcgccggcctcctcccggcgcagcctccgggcctccagtgcaatcactacgccctggggcccggaaaccgttttccggtctttcgctttcggctggggcgtggaggccgcggtgctgcgtaggccgggccgggcgcaggaacagccccgtggcgccctctctggccgccgcccgggcgggaaacgtcgttccggggaccgggcgaccccgcagcggggagcgcgccaggtccgcgcggggaagtgggcggtgtgcggccggcaccgcctcgcaccacgcccccgcgggcccgcactttcccggagtgcaccccgcggccgccagccggggcggaattccgccaccatggcggggctctggctggggctcgtgtggcagaagctgctgctgtggggcgcggcgagtgccctttccctggccggcgccagtctggtcctgagtctgctgcagagggtggcgagctacgcgcggaaatggcagcagatgcggcccatccccacggtggcccgcgcctacccactggtgggccacgcgctgctgatgaagccggacgggcgagaattttttcagcagatcattgagtacacagaggaataccgccacatgccgctgctgaagctctgggtcgggccagtgcccatggtggccctttataatgcagaaaatgtggaggtaattttaactagttcaaagcaaattgacaaatcctctatgtacaagtttttagaaccatggcttggcctaggacttcttacaagtactggaaacaaatggcgctccaggagaaagatgttaacacccactttccattttaccattctggaagatttcttagatatcatgaatgaacaagcaaatatattggttaagaaacttgaaaaacacattaaccaagaagcatttaactgctttttttacatcactctttgtgccttagatatcatctgtgaaacagctatggggaagaatattggtgctcaaagtaatgatgattccgagtatgtccgtgcagtttatagaatgagtgagatgatatttcgaagaataaagatgccctggctttggcttgatctctggtaccttatgtttaaagaaggatgggaacacaaaaagagccttcagatcctacatacttttaccaacagtgtcatcgcggaacgggccaatgaaatgaacgccaatgaagactgtagaggtgatggcaggggctctgccccctccaaaaataaacgcagggcctttcttgacttgcttttaagtgtgactgatgacgaagggaacaggctaagtcatgaagatattcgagaagaagttgacaccttcatgtttgaggggcacgatacaactgcagctgcaataaactggtccttatacctgttgggttctaacccagaagtccagaaaaaagtggatcatgaattggatgacgtgtttgggaagtctgaccgtcccgctacagtagaagacctgaagaaacttcggtatctggaatgtgttattaaggagacccttcgcctttttccttctgttcctttatttgcccgtagtgttagtgaagattgtgaagtggcaggttacagagttctaaaaggcactgaagccgtcatcattccctatgcattgcacagagatccgagatacttccccaaccccgaggagttccagcctgagcggttcttccccgagaatgcacaagggcgccatccatatgcctacgtgcccttctctgctggccccaggaactgtataggtcaaaagtttgctgtgatggaagaaaagaccattctttcgtgcatcctgaggcacttttggatagaatccaaccagaaaagagaagagcttggtctagaaggacagttgattcttcgtccaagtaatggcatctggatcaagttgaagaggagaaatgcagatgaacgcggaagcggagctactaacttcagcctgctgaagcaggctggagacgtggaggagaaccctggacctatggcctccctgttctctggccgcatcctgatccgcaacaatagcgaccaggacgagctggatacggaggctgaggtcagtcgcaggctggagaaccggctggtgctgctgttctttggtgctggggcttgtccacagtgccaggccttcgtgcccatcctcaaggacttcttcgtgcggctcacagatgagttctatgtactgcgggcggctcagctggccctggtgtacgtgtcccaggactccacggaggagcagcaggacctgttcctcaaggacatgccaaagaaatggcttttcctgccctttgaggatgatctgaggaggtgataaacgcgtggtttatccgatccaccggatctagataagatatccgatccaccggatctagataactgatcataatcagccataccacatttgtagaggttttacttgctttaaaaaacctcccacacctccccctgaacctgaaacataaaatgaatgcaattggcggccgcctcgagctgtgccttctagttgccagccatctgttgtttgcccctcccccgtgccttccttgaccctggaaggtgccactcccactgtcctttcctaataaaatgaggaaattgcatcgcattgtctgagtaggtgtcattctattctggggggtggggtggggcaggacagcaagggggaggattgggaagacaatagcaggcatgctggggatgcggtgggctctatggggtaaccacgtgcggacccaacggccgcaggaacccctagtgatggagttggccactccctctctgcgcgctcgctcgctcactgaggccgggcgaccaaaggtcgcccgacgcccgggctttgcccgggcggcctcagtgagcgagcgagcgcgcagctgcctgcaggggcgcctgatgcggtattttctccttacgcatctgtgcggtatttcacaccgcatacgtcaaagcaaccatagtacgcgccctgtagcggcacattaagcgcggcgggtgtggtggttacgcgcagcgtgaccgctacacttgccagcgccttagcgcccgctcctttcgctttcttcccttcctttctcgccacgttcgccggctttccccgtcaagctctaaatcgggggctccctttagggttccgatttagtgctttacggcacctcgaccccaaaaaacttgatttgggtgatggttcacgtagtgggccatcgccctgatagacggtttttcgccctttgacgttggagtccacgttctttaatagtggactcttgttccaaactggaacaacactcaactctatctcgggctattcttttgatttataagggattttgccgatttcggtctattggttaaaaaatgagctgatttaacaaaaatttaacgcgaattttaacaaaatattaacgtttacaattttatggtgcactctcagtacaatctgctctgatgccgcatagttaagccagccccgacacccgccaacacccgctgacgcgccctgacgggcttgtctgctcccggcatccgcttacagacaagctgtgaccgtctccgggagctgcatgtgtcagaggttttcaccgtcatcaccgaaacgcgcgagacgaaagggcctcgtgatacgcctatttttataggttaatgtcatgataataatggtttcttagacgtcaggtggcacttttcggggaaatgtgcgcggaacccctatttgtttatttttctaaatacattcaaatatgtatccgctcatgagacaataaccctgataaatgcttcaataatattgaaaaaggaagagtcctgaggcggaaagaaccagctgtggaatgtgtgtcagttagggtgtggaaagtccccaggctccccagcaggcagaagtatgcaaagcatgcatctcaattagtcagcaaccaggtgtggaaagtccccaggctccccagcaggcagaagtatgcaaagcatgcatctcaattagtcagcaaccatagtcccgcccctaactccgcccatcccgcccctaactccgcccagttccgcccattctccgccccatggctgactaattttttttatttatgcagaggccgaggccgcctcggcctctgagctattccagaagtagtgaggaggcttttttggaggcctaggcttttgcaaagatcgatcaagagacaggatgaggatcgtttcgcatgattgaacaagatggattgcacgcaggttctccggccgcttgggtggagaggctattcggctatgactgggcacaacagacaatcggctgctctgatgccgccgtgttccggctgtcagcgcaggggcgcccggttctttttgtcaagaccgacctgtccggtgccctgaatgaactgcaagacgaggcagcgcggctatcgtggctggccacgacgggcgttccttgcgcagctgtgctcgacgttgtcactgaagcgggaagggactggctgctattgggcgaagtgccggggcaggatctcctgtcatctcaccttgctcctgccgagaaagtatccatcatggctgatgcaatgcggcggctgcatacgcttgatccggctacctgcccattcgaccaccaagcgaaacatcgcatcgagcgagcacgtactcggatggaagccggtcttgtcgatcaggatgatctggacgaagagcatcaggggctcgcgccagccgaactgttcgccaggctcaaggcgagcatgcccgacggcgaggatctcgtcgtgacccatggcgatgcctgcttgccgaatatcatggtggaaaatggccgcttttctggattcatcgactgtggccggctgggtgtggcggaccgctatcaggacatagcgttggctacccgtgatattgctgaagagcttggcggcgaatgggctgaccgcttcctcgtgctttacggtatcgccgctcccgattcgcagcgcatcgccttctatcgccttcttgacgagttcttctgactgtcagaccaagtttactcatatatactttagattgatttaaaacttcatttttaatttaaaaggatctaggtgaagatcctttttgataatctcatgaccaaaatcccttaacgtgagttttcgttccactgagcgtcagaccccgtagaaaagatcaaaggatcttcttgagatcctttttttctgcgcgtaatctgctgcttgcaaacaaaaaaaccaccgctaccagcggtggtttgtttgccggatcaagagctaccaactctttttccgaaggtaactggcttcagcagagcgcagataccaaatactgttcttctagtgtagccgtagttaggccaccacttcaagaactctgtagcaccgcctacatacctcgctctgctaatcctgttaccagtggctgctgccagtggcgataagtcgtgtcttaccgggttggactcaagacgatagttaccggataaggcgcagcggtcgggctgaacggggggttcgtgcacacagcccagcttggagcgaacgacctacaccgaactgagatacctacagcgtgagctatgagaaagcgccacgcttcccgaagggagaaaggcggacaggtatccggtaagcggcagggtcggaacaggagagcgcacgagggagcttccagggggaaacgcctggtatctttatagtcctgtcgggtttcgccacctctgacttgagcgtcgatttttgtgatgctcgtcaggggggcggagcctatggaaaaacgccagcaacgcggcctttttacggttcctggccttttgctggccttttgctcacatgt

SEQ ID NO: 124 - DNA, 5993 bp, synthetic construct
  misc_feature 1..5993: note = pAV-OPEFS-CYP4V2-P2A-RdCVF
  source 1..5993: mol_type = other DNA
cctgcaggcagctgcgcgctcgctcgctcactgaggccgcccgggcgtcgggcgacctttggtcgcccggcctcagtgagcgagcgagcgcgcagagagggagtggccaactccatcactaggggttcctgcggccggtcgcgtctagtactagtcgcgtaggatccgggcagagcgcacatcgcccacagtccccgagaagttggggggaggggtcggcaattgaaccggtgcctagagaaggtggcgcggggtaaactgggaaagtgatgtcgtgtactggctccgcctttttcccgagggtgggggagaaccgtatataagtgcagtagtcgccgtgaacgttctttttcgcaacgggtttgccgccagaacacaggtaagtatcaaggttacaagacaggtttaaggagaccaatagaaactgggcttgtcgagacagagaagactcttgcgtttctgataggcacctattggtcttactgacatccactttgcctttctctccacaggaattccgccaccatggcggggctctggctggggctcgtgtggcagaagctgctgctgtggggcgcggcgagtgccctttccctggccggcgccagtctggtcctgagtctgctgcagagggtggcgagctacgcgcggaaatggcagcagatgcggcccatccccacggtggcccgcgcctacccactggtgggccacgcgctgctgatgaagccggacgggcgagaattttttcagcagatcattgagtacacagaggaataccgccacatgccgctgctgaagctctgggtcgggccagtgcccatggtggccctttataatgcagaaaatgtggaggtaattttaactagttcaaagcaaattgacaaatcctctatgtacaagtttttagaaccatggcttggcctaggacttcttacaagtactggaaacaaatggcgctccaggagaaagatgttaacacccactttccattttaccattctggaagatttcttagatatcatgaatgaacaagcaaatatattggttaagaaacttgaaaaacacattaaccaagaagcatttaactgctttttttacatcactctttgtgccttagatatcatctgtgaaacagctatggggaagaatattggtgctcaaagtaatgatgattccgagtatgtccgtgcagtttatagaatgagtgagatgatatttcgaagaataaagatgccctggctttggcttgatctctggtaccttatgtttaaagaaggatgggaacacaaaaagagccttcagatcctacatacttttaccaacagtgtcatcgcggaacgggccaatgaaatgaacgccaatgaagactgtagaggtgatggcaggggctctgccccctccaaaaataaacgcagggcctttcttgacttgcttttaagtgtgactgatgacgaagggaacaggctaagtcatgaagatattcgagaagaagttgacaccttcatgtttgaggggcacgatacaactgcagctgcaataaactggtccttatacctgttgggttctaacccagaagtccagaaaaaagtggatcatgaattggatgacgtgtttgggaagtctgaccgtcccgctacagtagaagacctgaagaaacttcggtatctggaatgtgttattaaggagacccttcgcctttttccttctgttcctttatttgcccgtagtgttagtgaagattgtgaagtggcaggttacagagttctaaaaggcactgaagccgtcatcattccctatgcattgcacagagatccgagatacttccccaaccccgaggagttccagcctgagcggttcttccccgagaatgcacaagggcgccatccatatgcctacgtgcccttctctgctggccccaggaactgtataggtcaaaagtttgctgtgatggaagaaaagaccattctttcgtgcatcctgaggcacttttggatagaatccaaccagaaaagagaagagcttggtctagaaggacagttgattcttcgtccaagtaatggcatctggatcaagttgaagaggagaaatgcagatgaacgcggaagcggagctactaacttcagcctgctgaagcaggctggagacgtggaggagaaccctggacctatggcctccctgttctctggccgcatcctgatccgcaacaatagcgaccaggacgagctggatacggaggctgaggtcagtcgcaggctggagaaccggctggtgctgctgttctttggtgctggggcttgtccacagtgccaggccttcgtgcccatcctcaaggacttcttcgtgcggctcacagatgagttctatgtactgcgggcggctcagctggccctggtgtacgtgtcccaggactccacggaggagcagcaggacctgttcctcaaggacatgccaaagaaatggcttttcctgccctttgaggatgatctgaggaggtgataaacgcgtggtttatccgatccaccggatctagataagatatccgatccaccggatctagataactgatcataatcagccataccacatttgtagaggttttacttgctttaaaaaacctcccacacctccccctgaacctgaaacataaaatgaatgcaattggcggccgcctcgagctgtgccttctagttgccagccatctgttgtttgcccctcccccgtgccttccttgaccctggaaggtgccactcccactgtcctttcctaataaaatgaggaaattgcatcgcattgtctgagtaggtgtcattctattctggggggtggggtggggcaggacagcaagggggaggattgggaagacaatagcaggcatgctggggatgcggtgggctctatggggtaaccacgtgcggacccaacggccgcaggaacccctagtgatggagttggccactccctctctgcgcgctcgctcgctcactgaggccgggcgaccaaaggtcgcccgacgcccgggctttgcccgggcggcctcagtgagcgagcgagcgcgcagctgcctgcaggggcgcctgatgcggtattttctccttacgcatctgtgcggtatttcacaccgcatacgtcaaagcaaccatagtacgcgccctgtagcggcacattaagcgcggcgggtgtggtggttacgcgcagcgtgaccgctacacttgccagcgccttagcgcccgctcctttcgctttcttcccttcctttctcgccacgttcgccggctttccccgtcaagctctaaatcgggggctccctttagggttccgatttagtgctttacggcacctcgaccccaaaaaacttgatttgggtgatggttcacgtagtgggccatcgccctgatagacggtttttcgccctttgacgttggagtccacgttctttaatagtggactcttgttccaaactggaacaacactcaactctatctcgggctattcttttgatttataagggattttgccgatttcggtctattggttaaaaaatgagctgatttaacaaaaatttaacgcgaattttaacaaaatattaacgtttacaattttatggtgcactctcagtacaatctgctctgatgccgcatagttaagccagccccgacacccgccaacacccgctgacgcgccctgacgggcttgtctgctcccggcatccgcttacagacaagctgtgaccgtctccgggagctgcatgtgtcagaggttttcaccgtcatcaccgaaacgcgcgagacgaaagggcctcgtgatacgcctatttttataggttaatgtcatgataataatggtttcttagacgtcaggtggcacttttcggggaaatgtgcgcggaacccctatttgtttatttttctaaatacattcaaatatgtatccgctcatgagacaataaccctgataaatgcttcaataatattgaaaaaggaagagtcctgaggcggaaagaaccagctgtggaatgtgtgtcagttagggtgtggaaagtccccaggctccccagcaggcagaagtatgcaaagcatgcatctcaattagtcagcaaccaggtgtggaaagtccccaggctccccagcaggcagaagtatgcaaagcatgcatctcaattagtcagcaaccatagtcccgcccctaactccgcccatcccgcccctaactccgcccagttccgcccattctccgccccatggctgactaattttttttatttatgcagaggccgaggccgcctcggcctctgagctattccagaagtagtgaggaggcttttttggaggcctaggcttttgcaaagatcgatcaagagacaggatgaggatcgtttcgcatgattgaacaagatggattgcacgcaggttctccggccgcttgggtggagaggctattcggctatgactgggcacaacagacaatcggctgctctgatgccgccgtgttccggctgtcagcgcaggggcgcccggttctttttgtcaagaccgacctgtccggtgccctgaatgaactgcaagacgaggcagcgcggctatcgtggctggccacgacgggcgttccttgcgcagctgtgctcgacgttgtcactgaagcgggaagggactggctgctattgggcgaagtgccggggcaggatctcctgtcatctcaccttgctcctgccgagaaagtatccatcatggctgatgcaatgcggcggctgcatacgcttgatccggctacctgcccattcgaccaccaagcgaaacatcgcatcgagcgagcacgtactcggatggaagccggtcttgtcgatcaggatgatctggacgaagagcatcaggggctcgcgccagccgaactgttcgccaggctcaaggcgagcatgcccgacggcgaggatctcgtcgtgacccatggcgatgcctgcttgccgaatatcatggtggaaaatggccgcttttctggattcatcgactgtggccggctgggtgtggcggaccgctatcaggacatagcgttggctacccgtgatattgctgaagagcttggcggcgaatgggctgaccgcttcctcgtgctttacggtatcgccgctcccgattcgcagcgcatcgccttctatcgccttcttgacgagttcttctgactgtcagaccaagtttactcatatatactttagattgatttaaaacttcatttttaatttaaaaggatctaggtgaagatcctttttgataatctcatgaccaaaatcccttaacgtgagttttcgttccactgagcgtcagaccccgtagaaaagatcaaaggatcttcttgagatcctttttttctgcgcgtaatctgctgcttgcaaacaaaaaaaccaccgctaccagcggtggtttgtttgccggatcaagagctaccaactctttttccgaaggtaactggcttcagcagagcgcagataccaaatactgttcttctagtgtagccgtagttaggccaccacttcaagaactctgtagcaccgcctacatacctcgctctgctaatcctgttaccagtggctgctgccagtggcgataagtcgtgtcttaccgggttggactcaagacgatagttaccggataaggcgcagcggtcgggctgaacggggggttcgtgcacacagcccagcttggagcgaacgacctacaccgaactgagatacctacagcgtgagctatgagaaagcgccacgcttcccgaagggagaaaggcggacaggtatccggtaagcggcagggtcggaacaggagagcgcacgagggagcttccagggggaaacgcctggtatctttatagtcctgtcgggtttcgccacctctgacttgagcgtcgatttttgtgatgctcgtcaggggggcggagcctatggaaaaacgccagcaacgcggcctttttacggttcctggccttttgctggccttttgctcacatgt

SEQ ID NO: 125 - DNA, 6581 bp, synthetic construct
  misc_feature 1..6581: note = pAV-CAG-CYP4V2-T2A-RdCVF
  source 1..6581: mol_type = other DNA
cctgcaggcagctgcgcgctcgctcgctcactgaggccgcccgggcgtcgggcgacctttggtcgcccggcctcagtgagcgagcgagcgcgcagagagggagtggccaactccatcactaggggttcctgcggccggtcgcgtctagtactagtcgcgtaggatccccattgacgtcaataatgacgtatgttcccatagtaacgccaatagggactttccattgacgtcaatgggtggagtsaatttacggtaaactgcccacttggcagtacatcaagtgtatcatatgccaagtacgccccctattgacgtcaatgacggtaaatggcccgcctggcattatgcccagtacatgaccttatgggactttcctacttggcagtacatctacgtattagtcatcgctattaccatggtcgaggtgagccccacgttctgcttcactctccccatctcccccccctccccacccccaattttgtatttatttattttttaattattttgtgcagcgatgggggcggggggggggggggggcgcgcgccaggcggggcggggcggggcgaggggcggggcggggcgaggcggagaggtgcggcggcagccaatcagagcggcgcgctccgaaagtttccttttatggcgaggcggcggcggcggcggccctataaaaagcgaagcgcgcggcgggcgggagtcgctgcgacgctgccttcgccccgtgccccgctccgccgccgcctcgcgccgcccgccccggctctgactgaccgcgttactcccacaggtgagcgggcgggacggcccttctcctccgggctgtaattagcgcttggtttaatgacggcttgtttcttttctgtggctgcgtgaaagccttgaggggctccgggagggccctttgtgcggggggagcggctcggggctgtccgcggggggacggctgccttcgggggggacggggcagggcggggttcggcttctggcgtgtgaccggcggctctagagcctctgctaaccatgttcatgccttcttctttttcctacagctcctgggcaacgtgctggttattgtgctgtctcatcattttggcaaagaattgaattccgccaccatggcggggctctggctggggctcgtgtggcagaagctgctgctgtggggcgcggcgagtgccctttccctggccggcgccagtctggtcctgagtctgctgcagagggtggcgagctacgcgcggaaatggcagcagatgcggcccatccccacggtggcccgcgcctacccactggtgggccacgcgctgctgatgaagccggacgggcgagaattttttcagcagatcattgagtacacagaggaataccgccacatgccgctgctgaagctctgggtcgggccagtgcccatggtggccctttataatgcagaaaatgtggaggtaattttaactagttcaaagcaaattgacaaatcctctatgtacaagtttttagaaccatggcttggcctaggacttcttacaagtactggaaacaaatggcgctccaggagaaagatgttaacacccactttccattttaccattctggaagatttcttagatatcatgaatgaacaagcaaatatattggttaagaaacttgaaaaacacattaaccaagaagcatttaactgctttttttacatcactctttgtgccttagatatcatctgtgaaacagctatggggaagaatattggtgctcaaagtaatgatgattccgagtatgtccgtgcagtttatagaatgagtgagatgatatttcgaagaataaagatgccctggctttggcttgatctctggtaccttatgtttaaagaaggatgggaacacaaaaagagccttcagatcctacatacttttaccaacagtgtcatcgcggaacgggccaatgaaatgaacgccaatgaagactgtagaggtgatggcaggggctctgccccctccaaaaataaacgcagggcctttcttgacttgcttttaagtgtgactgatgacgaagggaacaggctaagtcatgaagatattcgagaagaagttgacaccttcatgtttgaggggcacgatacaactgcagctgcaataaactggtccttatacctgttgggttctaacccagaagtccagaaaaaagtggatcatgaattggatgacgtgtttgggaagtctgaccgtcccgctacagtagaagacctgaagaaacttcggtatctggaatgtgttattaaggagacccttcgcctttttccttctgttcctttatttgcccgtagtgttagtgaagattgtgaagtggcaggttacagagttctaaaaggcactgaagccgtcatcattccctatgcattgcacagagatccgagatacttccccaaccccgaggagttccagcctgagcggttcttccccgagaatgcacaagggcgccatccatatgcctacgtgcccttctctgctggccccaggaactgtataggtcaaaagtttgctgtgatggaagaaaagaccattctttcgtgcatcctgaggcacttttggatagaatccaaccagaaaagagaagagcttggtctagaaggacagttgattcttcgtccaagtaatggcatctggatcaagttgaagaggagaaatgcagatgaacgcggaagcggagagggcagaggaagtctgctaacatgcggtgacgtcgaggagaatcctggacctatggcctccctgttctctggccgcatcctgatccgcaacaatagcgaccaggacgagctggatacggaggctgaggtcagtcgcaggctggagaaccggctggtgctgctgttctttggtgctggggcttgtccacagtgccaggccttcgtgcccatcctcaaggacttcttcgtgcggctcacagatgagttctatgtactgcgggcggctcagctggccctggtgtacgtgtcccaggactccacggaggagcagcaggacctgttcctcaaggacatgccaaagaaatggcttttcctgccctttgaggatgatctgaggaggtaaacgcgtggtttatccgatccaccggatctagataagatatccgatccaccggatctagataactgatcataatcagccataccacatttgtagaggttttacttgctttaaaaaacctcccacacctccccctgaacctgaaacataaaatgaatgcaattggcggccgcctcgagctgtgccttctagttgccagccatctgttgtttgcccctcccccgtgccttccttgaccctggaaggtgccactcccactgtcctttcctaataaaatgaggaaattgcatcgcattgtctgagtaggtgtcattctattctggggggtggggtggggcaggacagcaagggggaggattgggaagacaatagcaggcatgctggggatgcggtgggctctatggggtaaccacgtgcggacccaacggccgcaggaacccctagtgatggagttggccactccctctctgcgcgctcgctcgctcactgaggccgggcgaccaaaggtcgcccgacgcccgggctttgcccgggcggcctcagtgagcgagcgagcgcgcagctgcctgcaggggcgcctgatgcggtattttctccttacgcatctgtgcggtatttcacaccgcatacgtcaaagcaaccatagtacgcgccctgtagcggcacattaagcgcggcgggtgtggtggttacgcgcagcgtgaccgctacacttgccagcgccttagcgcccgctcctttcgctttcttcccttcctttctcgccacgttcgccggctttccccgtcaagctctaaatcgggggctccctttagggttccgatttagtgctttacggcacctcgaccccaaaaaacttgatttgggtgatggttcacgtagtgggccatcgccctgatagacggtttttcgccctttgacgttggagtccacgttctttaatagtggactcttgttccaaactggaacaacactcaactctatctcgggctattcttttgatttataagggattttgccgatttcggtctattggttaaaaaatgagctgatttaacaaaaatttaacgcgaattttaacaaaatattaacgtttacaattttatggtgcactctcagtacaatctgctctgatgccgcatagttaagccagccccgacacccgccaacacccgctgacgcgccctgacgggcttgtctgctcccggcatccgcttacagacaagctgtgaccgtctccgggagctgcatgtgtcagaggttttcaccgtcatcaccgaaacgcgcgagacgaaagggcctcgtgatacgcctatttttataggttaatgtcatgataataatggtttcttagacgtcaggtggcacttttcggggaaatgtgcgcggaacccctatttgtttatttttctaaatacattcaaatatgtatccgctcatgagacaataaccctgataaatgcttcaataatattgaaaaaggaagagtcctgaggcggaaagaaccagctgtggaatgtgtgtcagttagggtgtggaaagtccccaggctccccagcaggcagaagtatgcaaagcatgcatctcaattagtcagcaaccaggtgtggaaagtccccaggctccccagcaggcagaagtatgcaaagcatgcatctcaattagtcagcaaccatagtcccgcccctaactccgcccatcccgcccctaactccgcccagttccgcccattctccgccccatggctgactaattttttttatttatgcagaggccgaggccgcctcggcctctgagctattccagaagtagtgaggaggcttttttggaggcctaggcttttgcaaagatcgatcaagagacaggatgaggatcgtttcgcatgattgaacaagatggattgcacgcaggttctccggccgcttgggtggagaggctattcggctatgactgggcacaacagacaatcggctgctctgatgccgccgtgttccggctgtcagcgcaggggcgcccggttctttttgtcaagaccgacctgtccggtgccctgaatgaactgcaagacgaggcagcgcggctatcgtggctggccacgacgggcgttccttgcgcagctgtgctcgacgttgtcactgaagcgggaagggactggctgctattgggcgaagtgccggggcaggatctcctgtcatctcaccttgctcctgccgagaaagtatccatcatggctgatgcaatgcggcggctgcatacgcttgatccggctacctgcccattcgaccaccaagcgaaacatcgcatcgagcgagcacgtactcggatggaagccggtcttgtcgatcaggatgatctggacgaagagcatcaggggctcgcgccagccgaactgttcgccaggctcaaggcgagcatgcccgacggcgaggatctcgtcgtgacccatggcgatgcctgcttgccgaatatcatggtggaaaatggccgcttttctggattcatcgactgtggccggctgggtgtggcggaccgctatcaggacatagcgttggctacccgtgatattgctgaagagcttggcggcgaatgggctgaccgcttcctcgtgctttacggtatcgccgctcccgattcgcagcgcatcgccttctatcgccttcttgacgagttcttctgactgtcagaccaagtttactcatatatactttagattgatttaaaacttcatttttaatttaaaaggatctaggtgaagatcctttttgataatctcatgaccaaaatcccttaacgtgagttttcgttccactgagcgtcagaccccgtagaaaagatcaaaggatcttcttgagatcctttttttctgcgcgtaatctgctgcttgcaaacaaaaaaaccaccgctaccagcggtggtttgtttgccggatcaagagctaccaactctttttccgaaggtaactggcttcagcagagcgcagataccaaatactgttcttctagtgtagccgtagttaggccaccacttcaagaactctgtagcaccgcctacatacctcgctctgctaatcctgttaccagtggctgctgccagtggcgataagtcgtgtcttaccgggttggactcaagacgatagttaccggataaggcgcagcggtcgggctgaacggggggttcgtgcacacagcccagcttggagcgaacgacctacaccgaactgagatacctacagcgtgagctatgagaaagcgccacgcttcccgaagggagaaaggcggacaggtatccggtaagcggcagggtcggaacaggagagcgcacgagggagcttccagggggaaacgcctggtatctttatagtcctgtcgggtttcgccacctctgacttgagcgtcgatttttgtgatgctcgtcaggggggcggagcctatggaaaaacgccagcaacgcggcctttttacggttcctggccttttgctggccttttgctcacatgt

SEQ ID NO: 126 - DNA, 6807 bp, synthetic construct
  misc_feature 1..6807: note = pAV-EF1a-CYP4V2-P2A-RdCVF
  source 1..6807: mol_type = other DNA
cctgcaggcagctgcgcgctcgctcgctcactgaggccgcccgggcgtcgggcgacctttggtcgcccggcctcagtgagcgagcgagcgcgcagagagggagtggccaactccatcactaggggttcctgcggccggtcgcgtctagtactagtcgcgtaggatccgctccggtgcccgtcagtgggcagagcgcacatcgcccacagtccccgagaagttggggggaggggtcggcaattgaaccggtgcctagagaaggtggcgcggggtaaactgggaaagtgatgtcgtgtactggctccgcctttttcccgagggtgggggagaaccgtatataagtgcagtagtcgccgtgaacgttctttttcgcaacgggtttgccgccagaacacaggtaagtgccgtgtgtggttcccgcgggcctggcctctttacgggttatggcccttgcgtgccttgaattacttccacctggctccagtacgtgattcttgatcccgagctggagccaggggcgggccttgcgctttaggagccccttcgcctcgtgcttgagttgaggcctggcctgggcgctggggccgccgcgtgcgaatctggtggcaccttcgcgcctgtctcgctgctttcgataagtctctagccatttaaaatttttgatgacctgctgcgacgctttttttctggcaagatagtcttgtaaatgcgggccaggatctgcacactggtatttcggtttttggggccgcgggcggcgacggggcccgtgcgtcccagcgcacatgttcggcgaggcggggcctgcgagcgcggccaccgagaatcggacgggggtagtctcaagctggccggcctgctctggtgcctggcctcgcgccgccgtgtatcgccccgccctgggcggcaaggctggcccggtcggcaccagttgcgtgagcggaaagatggccgcttcccggccctgctccagggggctcaaaatggaggacgcggcgctcgggagagcgggcgggtgagtcacccacacaaaggaaaggggcctttccgtcctcagccgtcgcttcatgtgactccacggagtaccgggcgccgtccaggcacctcgattagttctggagcttttggagtacgtcgtctttaggttggggggaggggttttatgcgatggagtttccccacactgagtgggtggagactgaagttaggccagcttggcacttgatgtaattctccttggaatttgccctttttgagtttggatcttggttcattctcaagcctcagacagtggttcaaagtttttttcttccatttcaggtgtcgtgagaattccgccaccatggcggggctctggctggggctcgtgtggcagaagctgctgctgtggggcgcggcgagtgccctttccctggccggcgccagtctggtcctgagtctgctgcagagggtggcgagctacgcgcggaaatggcagcagatgcggcccatccccacggtggcccgcgcctacccactggtgggccacgcgctgctgatgaagccggacgggcgagaattttttcagcagatcattgagtacacagaggaataccgccacatgccgctgctgaagctctgggtcgggccagtgcccatggtggccctttataatgcagaaaatgtggaggtaattttaactagttcaaagcaaattgacaaatcctctatgtacaagtttttagaaccatggcttggcctaggacttcttacaagtactggaaacaaatggcgctccaggagaaagatgttaacacccactttccattttaccattctggaagatttcttagatatcatgaatgaacaagcaaatatattggttaagaaacttgaaaaacacattaaccaagaagcatttaactgctttttttacatcactctttgtgccttagatatcatctgtgaaacagctatggggaagaatattggtgctcaaagtaatgatgattccgagtatgtccgtgcagtttatagaatgagtgagatgatatttcgaagaataaagatgccctggctttggcttgatctctggtaccttatgtttaaagaaggatgggaacacaaaaagagccttcagatcctacatacttttaccaacagtgtcatcgcggaacgggccaatgaaatgaacgccaatgaagactgtagaggtgatggcaggggctctgccccctccaaaaataaacgcagggcctttcttgacttgcttttaagtgtgactgatgacgaagggaacaggctaagtcatgaagatattcgagaagaagttgacaccttcatgtttgaggggcacgatacaactgcagctgcaataaactggtccttatacctgttgggttctaacccagaagtccagaaaaaagtggatcatgaattggatgacgtgtttgggaagtctgaccgtcccgctacagtagaagacctgaagaaacttcggtatctggaatgtgttattaaggagacccttcgcctttttccttctgttcctttatttgcccgtagtgttagtgaagattgtgaagtggcaggttacagagttctaaaaggcactgaagccgtcatcattccctatgcattgcacagagatccgagatacttccccaaccccgaggagttccagcctgagcggttcttccccgagaatgcacaagggcgccatccatatgcctacgtgcccttctctgctggccccaggaactgtataggtcaaaagtttgctgtgatggaagaaaagaccattctttcgtgcatcctgaggcacttttggatagaatccaaccagaaaagagaagagcttggtctagaaggacagttgattcttcgtccaagtaatggcatctggatcaagttgaagaggagaaatgcagatgaacgcggaagcggagctactaacttcagcctgctgaagcaggctggagacgtggaggagaaccctggacctatggcctccctgttctctggccgcatcctgatccgcaacaatagcgaccaggacgagctggatacggaggctgaggtcagtcgcaggctggagaaccggctggtgctgctgttctttggtgctggggcttgtccacagtgccaggccttcgtgcccatcctcaaggacttcttcgtgcggctcacagatgagttctatgtactgcgggcggctcagctggccctggtgtacgtgtcccaggactccacggaggagcagcaggacctgttcctcaaggacatgccaaagaaatggcttttcctgccctttgaggatgatctgaggaggtaaacgcgtggtttatccgatccaccggatctagataagatatccgatccaccggatctagataactgatcataatcagccataccacatttgtagaggttttacttgctttaaaaaacctcccacacctccccctgaacctgaaacataaaatgaatgcaattggcggccgcctcgagctgtgccttctagttgccagccatctgttgtttgcccctcccccgtgccttccttgaccctggaaggtgccactcccactgtcctttcctaataaaatgaggaaattgcatcgcattgtctgagtaggtgtcattctattctggggggtggggtggggcaggacagcaagggggaggattgggaagacaatagcaggcatgctggggatgcggtgggctctatggggtaaccacgtgcggacccaacggccgcaggaacccctagtgatggagttggccactccctctctgcgcgctcgctcgctcactgaggccgggcgaccaaaggtcgcccgacgcccgggctttgcccgggcggcctcagtgagcgagcgagcgcgcagctgcctgcaggggcgcctgatgcggtattttctccttacgcatctgtgcggtatttcacaccgcatacgtcaaagcaaccatagtacgcgccctgtagcggcacattaagcgcggcgggtgtggtggttacgcgcagcgtgaccgctacacttgccagcgccttagcgcccgctcctttcgctttcttcccttcctttctcgccacgttcgccggctttccccgtcaagctctaaatcgggggctccctttagggttccgatttagtgctttacggcacctcgaccccaaaaaacttgatttgggtgatggttcacgtagtgggccatcgccctgatagacggtttttcgccctttgacgttggagtccacgttctttaatagtggactcttgttccaaactggaacaacactcaactctatctcgggctattcttttgatttataagggattttgccgatttcggtctattggttaaaaaatgagctgatttaacaaaaatttaacgcgaattttaacaaaatattaacgtttacaattttatggtgcactctcagtacaatctgctctgatgccgcatagttaagccagccccgacacccgccaacacccgctgacgcgccctgacgggcttgtctgctcccggcatccgcttacagacaagctgtgaccgtctccgggagctgcatgtgtcagaggttttcaccgtcatcaccgaaacgcgcgagacgaaagggcctcgtgatacgcctatttttataggttaatgtcatgataataatggtttcttagacgtcaggtggcacttttcggggaaatgtgcgcggaacccctatttgtttatttttctaaatacattcaaatatgtatccgctcatgagacaataaccctgataaatgcttcaataatattgaaaaaggaagagtcctgaggcggaaagaaccagctgtggaatgtgtgtcagttagggtgtggaaagtccccaggctccccagcaggcagaagtatgcaaagcatgcatctcaattagtcagcaaccaggtgtggaaagtccccaggctccccagcaggcagaagtatgcaaagcatgcatctcaattagtcagcaaccatagtcccgcccctaactccgcccatcccgcccctaactccgcccagttccgcccattctccgccccatggctgactaattttttttatttatgcagaggccgaggccgcctcggcctctgagctattccagaagtagtgaggaggcttttttggaggcctaggcttttgcaaagatcgatcaagagacaggatgaggatcgtttcgcatgattgaacaagatggattgcacgcaggttctccggccgcttgggtggagaggctattcggctatgactgggcacaacagacaatcggctgctctgatgccgccgtgttccggctgtcagcgcaggggcgcccggttctttttgtcaagaccgacctgtccggtgccctgaatgaactgcaagacgaggcagcgcggctatcgtggctggccacgacgggcgttccttgcgcagctgtgctcgacgttgtcactgaagcgggaagggactggctgctattgggcgaagtgccggggcaggatctcctgtcatctcaccttgctcctgccgagaaagtatccatcatggctgatgcaatgcggcggctgcatacgcttgatccggctacctgcccattcgaccaccaagcgaaacatcgcatcgagcgagcacgtactcggatggaagccggtcttgtcgatcaggatgatctggacgaagagcatcaggggctcgcgccagccgaactgttcgccaggctcaaggcgagcatgcccgacggcgaggatctcgtcgtgacccatggcgatgcctgcttgccgaatatcatggtggaaaatggccgcttttctggattcatcgactgtggccggctgggtgtggcggaccgctatcaggacatagcgttggctacccgtgatattgctgaagagcttggcggcgaatgggctgaccgcttcctcgtgctttacggtatcgccgctcccgattcgcagcgcatcgccttctatcgccttcttgacgagttcttctgactgtcagaccaagtttactcatatatactttagattgatttaaaacttcatttttaatttaaaaggatctaggtgaagatcctttttgataatctcatgaccaaaatcccttaacgtgagttttcgttccactgagcgtcagaccccgtagaaaagatcaaaggatcttcttgagatcctttttttctgcgcgtaatctgctgcttgcaaacaaaaaaaccaccgctaccagcggtggtttgtttgccggatcaagagctaccaactctttttccgaaggtaactggcttcagcagagcgcagataccaaatactgttcttctagtgtagccgtagttaggccaccacttcaagaactctgtagcaccgcctacatacctcgctctgctaatcctgttaccagtggctgctgccagtggcgataagtcgtgtcttaccgggttggactcaagacgatagttaccggataaggcgcagcggtcgggctgaacggggggttcgtgcacacagcccagcttggagcgaacgacctacaccgaactgagatacctacagcgtgagctatgagaaagcgccacgcttcccgaagggagaaaggcggacaggtatccggtaagcggcagggtcggaacaggagagcgcacgagggagcttccagggggaaacgcctggtatctttatagtcctgtcgggtttcgccacctctgacttgagcgtcgatttttgtgatgctcgtcaggggggcggagcctatggaaaaacgccagcaacgcggcctttttacggttcctggccttttgctggccttttgctcacatgt

SEQ ID NO: 127 - DNA, 6281 bp, synthetic construct
  misc_feature 1..6281: note = pAV-P5-intron-CYP4V2-P2A-RdCVF
  source 1..6281: mol_type = other DNA
cctgcaggcagctgcgcgctcgctcgctcactgaggccgcccgggcgtcgggcgacctttggtcgcccggcctcagtgagcgagcgagcgcgcagagagggagtggccaactccatcactaggggttcctgcggccggtcgcgtctagtactagtcgcgtaggatccgagccggatgcgccttcctttcctctccagagcaggctgcccgcccgcggaatcccgcacgtagagcaacctcgcagcaccctcagaacagccccgctggggcgcgccgggctgccgcggtgacctttccgacgcccctgaccccgcatccggaggcggccggaagtgtcgccggcctcctcccggcgcagcctccgggcctccagtgcaatcactacgccctggggcccggaaaccgttttccggtctttcgctttcggctggggcgtggaggccgcggtgctgcgtaggccgggccgggcgcaggaacagccccgtggcgccctctctggccgccgcccgggcgggaaacgtcgttccggggaccgggcgaccccgcagcggggagcgcgccaggtccgcgcggggaagtgggcggtgtgcggccggcaccgcctcgcaccacgcccccgcgggcccgcactttcccggagtgcaccccgcggccgccagccggggcggtaagtatcaaggttacaagacaggtttaaggagaccaatagaaactgggcttgtcgagacagagaagactcttgcgtttctgataggcacctattggtcttactgacatccactttgcctttctctccacaggaattccgccaccatggcggggctctggctggggctcgtgtggcagaagctgctgctgtggggcgcggcgagtgccctttccctggccggcgccagtctggtcctgagtctgctgcagagggtggcgagctacgcgcggaaatggcagcagatgcggcccatccccacggtggcccgcgcctacccactggtgggccacgcgctgctgatgaagccggacgggcgagaattttttcagcagatcattgagtacacagaggaataccgccacatgccgctgctgaagctctgggtcgggccagtgcccatggtggccctttataatgcagaaaatgtggaggtaattttaactagttcaaagcaaattgacaaatcctctatgtacaagtttttagaaccatggcttggcctaggacttcttacaagtactggaaacaaatggcgctccaggagaaagatgttaacacccactttccattttaccattctggaagatttcttagatatcatgaatgaacaagcaaatatattggttaagaaacttgaaaaacacattaaccaagaagcatttaactgctttttttacatcactctttgtgccttagatatcatctgtgaaacagctatggggaagaatattggtgctcaaagtaatgatgattccgagtatgtccgtgcagtttatagaatgagtgagatgatatttcgaagaataaagatgccctggctttggcttgatctctggtaccttatgtttaaagaaggatgggaacacaaaaagagccttcagatcctacatacttttaccaacagtgtcatcgcggaacgggccaatgaaatgaacgccaatgaagactgtagaggtgatggcaggggctctgccccctccaaaaataaacgcagggcctttcttgacttgcttttaagtgtgactgatgacgaagggaacaggctaagtcatgaagatattcgagaagaagttgacaccttcatgtttgaggggcacgatacaactgcagctgcaataaactggtccttatacctgttgggttctaacccagaagtccagaaaaaagtggatcatgaattggatgacgtgtttgggaagtctgaccgtcccgctacagtagaagacctgaagaaacttcggtatctggaatgtgttattaaggagacccttcgcctttttccttctgttcctttatttgcccgtagtgttagtgaagattgtgaagtggcaggttacagagttctaaaaggcactgaagccgtcatcattccctatgcattgcacagagatccgagatacttccccaaccccgaggagttccagcctgagcggttcttccccgagaatgcacaagggcgccatccatatgcctacgtgcccttctctgctggccccaggaactgtataggtcaaaagtttgctgtgatggaagaaaagaccattctttcgtgcatcctgaggcacttttggatagaatccaaccagaaaagagaagagcttggtctagaaggacagttgattcttcgtccaagtaatggcatctggatcaagttgaagaggagaaatgcagatgaacgcggaagcggagctactaacttcagcctgctgaagcaggctggagacgtggaggagaaccctggacctatggcctccctgttctctggccgcatcctgatccgcaacaatagcgaccaggacgagctggatacggaggctgaggtcagtcgcaggctggagaaccggctggtgctgctgttctttggtgctggggcttgtccacagtgccaggccttcgtgcccatcctcaaggacttcttcgtgcggctcacagatgagttctatgtactgcgggcggctcagctggccctggtgtacgtgtcccaggactccacggaggagcagcaggacctgttcctcaaggacatgccaaagaaatggcttttcctgccctttgaggatgatctgaggaggtgataaacgcgtggtttatccgatccaccggatctagataagatatccgatccaccggatctagataactgatcataatcagccataccacatttgtagaggttttacttgctttaaaaaacctcccacacctccccctgaacctgaaacataaaatgaatgcaattggcggccgcctcgagctgtgccttctagttgccagccatctgttgtttgcccctcccccgtgccttccttgaccctggaaggtgccactcccactgtcctttcctaataaaatgaggaaattgcatcgcattgtctgagtaggtgtcattctattctggggggtggggtggggcaggacagcaagggggaggattgggaagacaatagcaggcatgctggggatgcggtgggctctatggggtaaccacgtgcggacccaacggccgcaggaacccctagtgatggagttggccactccctctctgcgcgctcgctcgctcactgaggccgggcgaccaaaggtcgcccgacgcccgggctttgcccgggcggcctcagtgagcgagcgagcgcgcagctgcctgcaggggcgcctgatgcggtattttctccttacgcatctgtgcggtatttcacaccgcatacgtcaaagcaaccatagtacgcgccctgtagcggcacattaagcgcggcgggtgtggtggttacgcgcagcgtgaccgctacacttgccagcgccttagcgcccgctcctttcgctttcttcccttcctttctcgccacgttcgccggctttccccgtcaagctctaaatcgggggctccctttagggttccgatttagtgctttacggcacctcgaccccaaaaaacttgatttgggtgatggttcacgtagtgggccatcgccctgatagacggtttttcgccctttgacgttggagtccacgttctttaatagtggactcttgttccaaactggaacaacactcaactctatctcgggctattcttttgatttataagggattttgccgatttcggtctattggttaaaaaatgagctgatttaacaaaaatttaacgcgaattttaacaaaatattaacgtttacaattttatggtgcactctcagtacaatctgctctgatgccgcatagttaagccagccccgacacccgccaacacccgctgacgcgccctgacgggcttgtctgctcccggcatccgcttacagacaagctgtgaccgtctccgggagctgcatgtgtcagaggttttcaccgtcatcaccgaaacgcgcgagacgaaagggcctcgtgatacgcctatttttataggttaatgtcatgataataatggtttcttagacgtcaggtggcacttttcggggaaatgtgcgcggaacccctatttgtttatttttctaaatacattcaaatatgtatccgctcatgagacaataaccctgataaatgcttcaataatattgaaaaaggaagagtcctgaggcggaaagaaccagctgtggaatgtgtgtcagttagggtgtggaaagtccccaggctccccagcaggcagaagtatgcaaagcatgcatctcaattagtcagcaaccaggtgtggaaagtccccaggctccccagcaggcagaagtatgcaaagcatgcatctcaattagtcagcaaccatagtcccgcccctaactccgcccatcccgcccctaactccgcccagttccgcccattctccgccccatggctgactaattttttttatttatgcagaggccgaggccgcctcggcctctgagctattccagaagtagtgaggaggcttttttggaggcctaggcttttgcaaagatcgatcaagagacaggatgaggatcgtttcgcatgattgaacaagatggattgcacgcaggttctccggccgcttgggtggagaggctattcggctatgactgggcacaacagacaatcggctgctctgatgccgccgtgttccggctgtcagcgcaggggcgcccggttctttttgtcaagaccgacctgtccggtgccctgaatgaactgcaagacgaggcagcgcggctatcgtggctggccacgacgggcgttccttgcgcagctgtgctcgacgttgtcactgaagcgggaagggactggctgctattgggcgaagtgccggggcaggatctcctgtcatctcaccttgctcctgccgagaaagtatccatcatggctgatgcaatgcggcggctgcatacgcttgatccggctacctgcccattcgaccaccaagcgaaacatcgcatcgagcgagcacgtactcggatggaagccggtcttgtcgatcaggatgatctggacgaagagcatcaggggctcgcgccagccgaactgttcgccaggctcaaggcgagcatgcccgacggcgaggatctcgtcgtgacccatggcgatgcctgcttgccgaatatcatggtggaaaatggccgcttttctggattcatcgactgtggccggctgggtgtggcggaccgctatcaggacatagcgttggctacccgtgatattgctgaagagcttggcggcgaatgggctgaccgcttcctcgtgctttacggtatcgccgctcccgattcgcagcgcatcgccttctatcgccttcttgacgagttcttctgactgtcagaccaagtttactcatatatactttagattgatttaaaacttcatttttaatttaaaaggatctaggtgaagatcctttttgataatctcatgaccaaaatcccttaacgtgagttttcgttccactgagcgtcagaccccgtagaaaagatcaaaggatcttcttgagatcctttttttctgcgcgtaatctgctgcttgcaaacaaaaaaaccaccgctaccagcggtggtttgtttgccggatcaagagctaccaactctttttccgaaggtaactggcttcagcagagcgcagataccaaatactgttcttctagtgtagccgtagttaggccaccacttcaagaactctgtagcaccgcctacatacctcgctctgctaatcctgttaccagtggctgctgccagtggcgataagtcgtgtcttaccgggttggactcaagacgatagttaccggataaggcgcagcggtcgggctgaacggggggttcgtgcacacagcccagcttggagcgaacgacctacaccgaactgagatacctacagcgtgagctatgagaaagcgccacgcttcccgaagggagaaaggcggacaggtatccggtaagcggcagggtcggaacaggagagcgcacgagggagcttccagggggaaacgcctggtatctttatagtcctgtcgggtttcgccacctctgacttgagcgtcgatttttgtgatgctcgtcaggggggcggagcctatggaaaaacgccagcaacgcggcctttttacggttcctggccttttgctggccttttgctcacatgt

SEQ ID NO: 128 - DNA, 7389 bp, synthetic construct
  misc_feature 1..7389: note = pAV-RPE65-intron-CYP4V2-T2A-RdCVF
  source 1..7389: mol_type = other DNA
cctgcaggcagctgcgcgctcgctcgctcactgaggccgcccgggcgtcgggcgacctttggtcgcccggcctcagtgagcgagcgagcgcgcagagagggagtggccaactccatcactaggggttcctgcggccggtcgcgtctagtactagtcgcgtaggatcctattgtgcaaataagtgctcactccaaattagtggtatatttattgaagtttaatattgtgtttgtgatacagaagtatttgctttaattctaaataaaaattttatgcttttattgctggtttaagaagatttggattatccttgtactttgaggagaagtttcttatttgaaatattttggaaacaggtcttttaatgtggaaagatagatattaatctcctcttctattactctccaagatccaacaaaagtgattataccccccaaaatatgatggtagtatcttatactaccatcattttataggcatagggctcttagctgcaaataatggaactaactctaataaagcagaacgcaaatattgtaaatattagagagctaacaatctctgggatggctaaaggatggagcttggaggctacccagccagtaacaatattccgggctccactgttgaatggagacactacaactgccttggatgggcagagatattatggatgctaagccccaggtgctaccattaggacttctaccactgtccctaacgggtggagcccatcacatgcctatgccctcactgtaaggaaatgaagctactgttgtatatcttgggaagcacttggattaattgttatacagttttgttgaagaagacccctagggtaagtagccataactgcacactaaatttaaaattgttaatgagtttctcaaaaaaaatgttaaggttgttagctggtatagtatatatcttgcctgttttccaaggacttctttgggcagtaccttgtctgtgctggcaagcaactgagacttaatgaaagagtattggagatatgaatgaattgatgctgtatactctcagagtgccaaacatataccaatggacaagaaggtgaggcagagagcagacaggcattagtgacaagcaaagatatgcagaatttcattctcagcaaatcaaaagtcctcaacctggttggaagaatattggcactgaatggtatcaataaggttgctagagagggttagaggtgcacaatgtgcttccataacattttatacttctccaatcttagcactaatcaaacatggttgaatactttgtttactataactcttacagagttataagatctgtgaagacagggacagggacaatacccatctctgtctggttcataggtggtatgtaatagatatttttaaaaataagtgagttaatgaatgagggtgagaatgaaggcacagaggtattagggggaggtgggccccagagaatggtgccaaggtccagtggggtgactgggatcagctcaggcctgacgctggccactcccacctagctcctttctttctaatctgttctcattctccttgggaaggattgaggtctctggaaaacagccaaacaactgttatgggaacagcaagcccaaataaagccaagcatcagggggatctgagagctgaaagcaacttctgttccccctccctcagctgaaggggtggggaagggctcccaaagccataactccttttaagggatttagaaggcataaaaaggcccctggctgagaacttccttcttcattctgcagttgggtaagtatcaaggttacaagacaggtttaaggagaccaatagaaactgggcttgtcgagacagagaagactcttgcgtttctgataggcacctattggtcttactgacatccactttgcctttctctccacaggaattccgccaccatggcggggctctggctggggctcgtgtggcagaagctgctgctgtggggcgcggcgagtgccctttccctggccggcgccagtctggtcctgagtctgctgcagagggtggcgagctacgcgcggaaatggcagcagatgcggcccatccccacggtggcccgcgcctacccactggtgggccacgcgctgctgatgaagccggacgggcgagaattttttcagcagatcattgagtacacagaggaataccgccacatgccgctgctgaagctctgggtcgggccagtgcccatggtggccctttataatgcagaaaatgtggaggtaattttaactagttcaaagcaaattgacaaatcctctatgtacaagtttttagaaccatggcttggcctaggacttcttacaagtactggaaacaaatggcgctccaggagaaagatgttaacacccactttccattttaccattctggaagatttcttagatatcatgaatgaacaagcaaatatattggttaagaaacttgaaaaacacattaaccaagaagcatttaactgctttttttacatcactctttgtgccttagatatcatctgtgaaacagctatggggaagaatattggtgctcaaagtaatgatgattccgagtatgtccgtgcagtttatagaatgagtgagatgatatttcgaagaataaagatgccctggctttggcttgatctctggtaccttatgtttaaagaaggatgggaacacaaaaagagccttcagatcctacatacttttaccaacagtgtcatcgcggaacgggccaatgaaatgaacgccaatgaagactgtagaggtgatggcaggggctctgccccctccaaaaataaacgcagggcctttcttgacttgcttttaagtgtgactgatgacgaagggaacaggctaagtcatgaagatattcgagaagaagttgacaccttcatgtttgaggggcacgatacaactgcagctgcaataaactggtccttatacctgttgggttctaacccagaagtccagaaaaaagtggatcatgaattggatgacgtgtttgggaagtctgaccgtcccgctacagtagaagacctgaagaaacttcggtatctggaatgtgttattaaggagacccttcgcctttttccttctgttcctttatttgcccgtagtgttagtgaagattgtgaagtggcaggttacagagttctaaaaggcactgaagccgtcatcattccctatgcattgcacagagatccgagatacttccccaaccccgaggagttccagcctgagcggttcttccccgagaatgcacaagggcgccatccatatgcctacgtgcccttctctgctggccccaggaactgtataggtcaaaagtttgctgtgatggaagaaaagaccattctttcgtgcatcctgaggcacttttggatagaatccaaccagaaaagagaagagcttggtctagaaggacagttgattcttcgtccaagtaatggcatctggatcaagttgaagaggagaaatgcagatgaacgcggaagcggagagggcagaggaagtctgctaacatgcggtgacgtcgaggagaatcctggacctatggcctccctgttctctggccgcatcctgatccgcaacaatagcgaccaggacgagctggatacggaggctgaggtcagtcgcaggctggagaaccggctggtgctgctgttctttggtgctggggcttgtccacagtgccaggccttcgtgcccatcctcaaggacttcttcgtgcggctcacagatgagttctatgtactgcgggcggctcagctggccctggtgtacgtgtcccaggactccacggaggagcagcaggacctgttcctcaaggacatgccaaagaaatggcttttcctgccctttgaggatgatctgaggaggtaaacgcgtggtttatccgatccaccggatctagataagatatccgatccaccggatctagataactgatcataatcagccataccacatttgtagaggttttacttgctttaaaaaacctcccacacctccccctgaacctgaaacataaaatgaatgcaattggcggccgcctcgagctgtgccttctagttgccagccatctgttgtttgcccctcccccgtgccttccttgaccctggaaggtgccactcccactgtcctttcctaataaaatgaggaaattgcatcgcattgtctgagtaggtgtcattctattctggggggtggggtggggcaggacagcaagggggaggattgggaagacaatagcaggcatgctggggatgcggtgggctctatggggtaaccacgtgcggacccaacggccgcaggaacccctagtgatggagttggccactccctctctgcgcgctcgctcgctcactgaggccgggcgaccaaaggtcgcccgacgcccgggctttgcccgggcggcctcagtgagcgagcgagcgcgcagctgcctgcaggggcgcctgatgcggtattttctccttacgcatctgtgcggtatttcacaccgcatacgtcaaagcaaccatagtacgcgccctgtagcggcacattaagcgcggcgggtgtggtggttacgcgcagcgtgaccgctacacttgccagcgccttagcgcccgctcctttcgctttcttcccttcctttctcgccacgttcgccggctttccccgtcaagctctaaatcgggggctccctttagggttccgatttagtgctttacggcacctcgaccccaaaaaacttgatttgggtgatggttcacgtagtgggccatcgccctgatagacggtttttcgccctttgacgttggagtccacgttctttaatagtggactcttgttccaaactggaacaacactcaactctatctcgggctattcttttgatttataagggattttgccgatttcggtctattggttaaaaaatgagctgatttaacaaaaatttaacgcgaattttaacaaaatattaacgtttacaattttatggtgcactctcagtacaatctgctctgatgccgcatagttaagccagccccgacacccgccaacacccgctgacgcgccctgacgggcttgtctgctcccggcatccgcttacagacaagctgtgaccgtctccgggagctgcatgtgtcagaggttttcaccgtcatcaccgaaacgcgcgagacgaaagggcctcgtgatacgcctatttttataggttaatgtcatgataataatggtttcttagacgtcaggtggcacttttcggggaaatgtgcgcggaacccctatttgtttatttttctaaatacattcaaatatgtatccgctcatgagacaataaccctgataaatgcttcaataatattgaaaaaggaagagtcctgaggcggaaagaaccagctgtggaatgtgtgtcagttagggtgtggaaagtccccaggctccccagcaggcagaagtatgcaaagcatgcatctcaattagtcagcaaccaggtgtggaaagtccccaggctccccagcaggcagaagtatgcaaagcatgcatctcaattagtcagcaaccatagtcccgcccctaactccgcccatcccgcccctaactccgcccagttccgcccattctccgccccatggctgactaattttttttatttatgcagaggccgaggccgcctcggcctctgagctattccagaagtagtgaggaggcttttttggaggcctaggcttttgcaaagatcgatcaagagacaggatgaggatcgtttcgcatgattgaacaagatggattgcacgcaggttctccggccgcttgggtggagaggctattcggctatgactgggcacaacagacaatcggctgctctgatgccgccgtgttccggctgtcagcgcaggggcgcccggttctttttgtcaagaccgacctgtccggtgccctgaatgaactgcaagacgaggcagcgcggctatcgtggctggccacgacgggcgttccttgcgcagctgtgctcgacgttgtcactgaagcgggaagggactggctgctattgggcgaagtgccggggcaggatctcctgtcatctcaccttgctcctgccgagaaagtatccatcatggctgatgcaatgcggcggctgcatacgcttgatccggctacctgcccattcgaccaccaagcgaaacatcgcatcgagcgagcacgtactcggatggaagccggtcttgtcgatcaggatgatctggacgaagagcatcaggggctcgcgccagccgaactgttcgccaggctcaaggcgagcatgcccgacggcgaggatctcgtcgtgacccatggcgatgcctgcttgccgaatatcatggtggaaaatggccgcttttctggattcatcgactgtggccggctgggtgtggcggaccgctatcaggacatagcgttggctacccgtgatattgctgaagagcttggcggcgaatgggctgaccgcttcctcgtgctttacggtatcgccgctcccgattcgcagcgcatcgccttctatcgccttcttgacgagttcttctgactgtcagaccaagtttactcatatatactttagattgatttaaaacttcatttttaatttaaaaggatctaggtgaagatcctttttgataatctcatgaccaaaatcccttaacgtgagttttcgttccactgagcgtcagaccccgtagaaaagatcaaaggatcttcttgagatcctttttttctgcgcgtaatctgctgcttgcaaacaaaaaaaccaccgctaccagcggtggtttgtttgccggatcaagagctaccaactctttttccgaaggtaactggcttcagcagagcgcagataccaaatactgttcttctagtgtagccgtagttaggccaccacttcaagaactctgtagcaccgcctacatacctcgctctgctaatcctgttaccagtggctgctgccagtggcgataagtcgtgtcttaccgggttggactcaagacgatagttaccggataaggcgcagcggtcgggctgaacggggggttcgtgcacacagcccagcttggagcgaacgacctacaccgaactgagatacctacagcgtgagctatgagaaagcgccacgcttcccgaagggagaaaggcggacaggtatccggtaagcggcagggtcggaacaggagagcgcacgagggagcttccagggggaaacgcctggtatctttatagtcctgtcgggtttcgccacctctgacttgagcgtcgatttttgtgatgctcgtcaggggggcggagcctatggaaaaacgccagcaacgcggcctttttacggttcctggccttttgctggccttttgctcacatgt

SEQ ID NO: 129 - DNA, 7744 bp, synthetic construct
  misc_feature 1..7744: note = pAV-CYP4V2 Pf-SV40 intron-CYP4V2-P2A-RdCVF
  source 1..7744: mol_type = other DNA
cctgcaggcagctgcgcgctcgctcgctcactgaggccgcccgggcgtcgggcgacctttggtcgcccggcctcagtgagcgagcgagcgcgcagagagggagtggccaactccatcactaggggttcctgcggccggtcgcgtctagtactagtcgcgtaggatccacccacctcatcctgcacctgtcactgcgtgggaccctgtgctccaggcaggggcacctcactgccccctgagctcattttacccctcctggctctgcagcatttctgaccatttctgcccaggccgagactcactgctgcccagagcaatctcccttctctccttctggaggggaggggttgtatgttacccgcctggttttatccacagaggttagcagagactgatacagacaaaccctttttctttctaattttagattcaagagcacatgtgcaggtttgttaaatttgcctgacgctgaggtttgagtttctattgatcccctcacctgaatagggaacacagtacccaatacacagtttttcaaccattactccccttccttcctccccctattttagaatccccagtatgtagacaaattgtttacttttatagctgtaattaaccttattatagctcagcctcaaccctttagagaggaggaaactaaagcccatgagacttgcttaaagatactaagtgaacatatttattttttaaagtgttaaagtgattaaacaatgtagacgtgaatgaaataaaaagcgtaagttccccatcttcattcccactccatagagctgatcagtatttttacttgcagacattagtggagccgtagagaaagaaaccttttctccaaaagaaggcattactttacacactccgttctgcaacttgttttgttcacttgctatttcacgtcagcccatgcagatgacttaaaacaaattcaaatggagaaaagccttaggcatgtttttctctgcactaaagaggccctgcaggtggctgtggccaacttatgcagtggcttcgagtgaacgaacgtaattagtaattaagcaaagcgggcatccaggacattcagtttcatcttcctggcactttagtgtttaggaagggcctggcctctcggggagcgacactcctcgcccggccactttgtaagaagcatcgagcgtggaaaaggggctggggtcagcactggggccctctgccgggaagagagactggcggccagcacacgcgtctccccaggctgaaatggggcaccctctcgcggcccttccctcccttcccgggctgggtggcaggtcttggctcttctgcgagtaccccgcggctgcggtctcccggcacccgctgagcagcctcgcccgccttcctctcccacccgcccctgcgtgctctccggggctccggcttcctcggtctggtgcctggtgcgtattttggaaaatacctggctcataaccacctcattgagctcccagtgtcccagtgggccagcggacacacacgggtagctgacttccctaacgtgtccccaaagcctccctggattacagcgcccgctgctccatgtgaccccgcgggagccaggacgcgccccgcctcccggggctgcaagttgcgcagggagcgagcgatgcgcagcagagctgggctccgagccggatgcgccttcctttcctctccagagcaggctgcccgcccgcggaatcccgcacgtagagcaacctcgcagcaccctcagaacagccccgctggggcgcgccgggctgccgcggtgacctttccgacgcccctgaccccgcatccggaggcggccggaagtgtcgccggcctcctcccggcgcagcctccgggcctccagtgcaatcactacgccctggggcccggaaaccgttttccggtctttcgctttcggctggggcgtggaggccgcggtgctgcgtaggccgggccgggcgcaggaacagccccgtggcgccctctctggccgccgcccgggcgggaaacgtcgttccggggaccgggcgaccccgcagcggggagcgcgccaggtccgcgcggggaagtgggcggtgtgcggccggcaccgcctcgcaccacgcccccgcgggcccgcactttcccggagtgcaccccgcggccgccagccggggcggtaagtttagtctttttgtcttttatttcaggtcccggatccggtggtggtgcaaatcaaagaactgctcctcagtggatgttgcctttacttctaggcgaattccgccaccatggcggggctctggctggggctcgtgtggcagaagctgctgctgtggggcgcggcgagtgccctttccctggccggcgccagtctggtcctgagtctgctgcagagggtggcgagctacgcgcggaaatggcagcagatgcggcccatccccacggtggcccgcgcctacccactggtgggccacgcgctgctgatgaagccggacgggcgagaattttttcagcagatcattgagtacacagaggaataccgccacatgccgctgctgaagctctgggtcgggccagtgcccatggtggccctttataatgcagaaaatgtggaggtaattttaactagttcaaagcaaattgacaaatcctctatgtacaagtttttagaaccatggcttggcctaggacttcttacaagtactggaaacaaatggcgctccaggagaaagatgttaacacccactttccattttaccattctggaagatttcttagatatcatgaatgaacaagcaaatatattggttaagaaacttgaaaaacacattaaccaagaagcatttaactgctttttttacatcactctttgtgccttagatatcatctgtgaaacagctatggggaagaatattggtgctcaaagtaatgatgattccgagtatgtccgtgcagtttatagaatgagtgagatgatatttcgaagaataaagatgccctggctttggcttgatctctggtaccttatgtttaaagaaggatgggaacacaaaaagagccttcagatcctacatacttttaccaacagtgtcatcgcggaacgggccaatgaaatgaacgccaatgaagactgtagaggtgatggcaggggctctgccccctccaaaaataaacgcagggcctttcttgacttgcttttaagtgtgactgatgacgaagggaacaggctaagtcatgaagatattcgagaagaagttgacaccttcatgtttgaggggcacgatacaactgcagctgcaataaactggtccttatacctgttgggttctaacccagaagtccagaaaaaagtggatcatgaattggatgacgtgtttgggaagtctgaccgtcccgctacagtagaagacctgaagaaacttcggtatctggaatgtgttattaaggagacccttcgcctttttccttctgttcctttatttgcccgtagtgttagtgaagattgtgaagtggcaggttacagagttctaaaaggcactgaagccgtcatcattccctatgcattgcacagagatccgagatacttccccaaccccgaggagttccagcctgagcggttcttccccgagaatgcacaagggcgccatccatatgcctacgtgcccttctctgctggccccaggaactgtataggtcaaaagtttgctgtgatggaagaaaagaccattctttcgtgcatcctgaggcacttttggatagaatccaaccagaaaagagaagagcttggtctagaaggacagttgattcttcgtccaagtaatggcatctggatcaagttgaagaggagaaatgcagatgaacgcggaagcggagctactaacttcagcctgctgaagcaggctggagacgtggaggagaaccctggacctatggcctccctgttctctggccgcatcctgatccgcaacaatagcgaccaggacgagctggatacggaggctgaggtcagtcgcaggctggagaaccggctggtgctgctgttctttggtgctggggcttgtccacagtgccaggccttcgtgcccatcctcaaggacttcttcgtgcggctcacagatgagttctatgtactgcgggcggctcagctggccctggtgtacgtgtcccaggactccacggaggagcagcaggacctgttcctcaaggacatgccaaagaaatggcttttcctgccctttgaggatgatctgaggaggtaaacgcgtggtttatccgatccaccggatctagataagatatccgatccaccggatctagataactgatcataatcagccataccacatttgtagaggttttacttgctttaaaaaacctcccacacctccccctgaacctgaaacataaaatgaatgcaattggcggccgcctcgagctgtgccttctagttgccagccatctgttgtttgcccctcccccgtgccttccttgaccctggaaggtgccactcccactgtcctttcctaataaaatgaggaaattgcatcgcattgtctgagtaggtgtcattctattctggggggtggggtggggcaggacagcaagggggaggattgggaagacaatagcaggcatgctggggatgcggtgggctctatggggtaaccacgtgcggacccaacggccgcaggaacccctagtgatggagttggccactccctctctgcgcgctcgctcgctcactgaggccgggcgaccaaaggtcgcccgacgcccgggctttgcccgggcggcctcagtgagcgagcgagcgcgcagctgcctgcaggggcgcctgatgcggtattttctccttacgcatctgtgcggtatttcacaccgcatacgtcaaagcaaccatagtacgcgccctgtagcggcacattaagcgcggcgggtgtggtggttacgcgcagcgtgaccgctacacttgccagcgccttagcgcccgctcctttcgctttcttcccttcctttctcgccacgttcgccggctttccccgtcaagctctaaatcgggggctccctttagggttccgatttagtgctttacggcacctcgaccccaaaaaacttgatttgggtgatggttcacgtagtgggccatcgccctgatagacggtttttcgccctttgacgttggagtccacgttctttaatagtggactcttgttccaaactggaacaacactcaactctatctcgggctattcttttgatttataagggattttgccgatttcggtctattggttaaaaaatgagctgatttaacaaaaatttaacgcgaattttaacaaaatattaacgtttacaattttatggtgcactctcagtacaatctgctctgatgccgcatagttaagccagccccgacacccgccaacacccgctgacgcgccctgacgggcttgtctgctcccggcatccgcttacagacaagctgtgaccgtctccgggagctgcatgtgtcagaggttttcaccgtcatcaccgaaacgcgcgagacgaaagggcctcgtgatacgcctatttttataggttaatgtcatgataataatggtttcttagacgtcaggtggcacttttcggggaaatgtgcgcggaacccctatttgtttatttttctaaatacattcaaatatgtatccgctcatgagacaataaccctgataaatgcttcaataatattgaaaaaggaagagtcctgaggcggaaagaaccagctgtggaatgtgtgtcagttagggtgtggaaagtccccaggctccccagcaggcagaagtatgcaaagcatgcatctcaattagtcagcaaccaggtgtggaaagtccccaggctccccagcaggcagaagtatgcaaagcatgcatctcaattagtcagcaaccatagtcccgcccctaactccgcccatcccgcccctaactccgcccagttccgcccattctccgccccatggctgactaattttttttatttatgcagaggccgaggccgcctcggcctctgagctattccagaagtagtgaggaggcttttttggaggcctaggcttttgcaaagatcgatcaagagacaggatgaggatcgtttcgcatgattgaacaagatggattgcacgcaggttctccggccgcttgggtggagaggctattcggctatgactgggcacaacagacaatcggctgctctgatgccgccgtgttccggctgtcagcgcaggggcgcccggttctttttgtcaagaccgacctgtccggtgccctgaatgaactgcaagacgaggcagcgcggctatcgtggctggccacgacgggcgttccttgcgcagctgtgctcgacgttgtcactgaagcgggaagggactggctgctattgggcgaagtgccggggcaggatctcctgtcatctcaccttgctcctgccgagaaagtatccatcatggctgatgcaatgcggcggctgcatacgcttgatccggctacctgcccattcgaccaccaagcgaaacatcgcatcgagcgagcacgtactcggatggaagccggtcttgtcgatcaggatgatctggacgaagagcatcaggggctcgcgccagccgaactgttcgccaggctcaaggcgagcatgcccgacggcgaggatctcgtcgtgacccatggcgatgcctgcttgccgaatatcatggtggaaaatggccgcttttctggattcatcgactgtggccggctgggtgtggcggaccgctatcaggacatagcgttggctacccgtgatattgctgaagagcttggcggcgaatgggctgaccgcttcctcgtgctttacggtatcgccgctcccgattcgcagcgcatcgccttctatcgccttcttgacgagttcttctgactgtcagaccaagtttactcatatatactttagattgatttaaaacttcatttttaatttaaaaggatctaggtgaagatcctttttgataatctcatgaccaaaatcccttaacgtgagttttcgttccactgagcgtcagaccccgtagaaaagatcaaaggatcttcttgagatcctttttttctgcgcgtaatctgctgcttgcaaacaaaaaaaccaccgctaccagcggtggtttgtttgccggatcaagagctaccaactctttttccgaaggtaactggcttcagcagagcgcagataccaaatactgttcttctagtgtagccgtagttaggccaccacttcaagaactctgtagcaccgcctacatacctcgctctgctaatcctgttaccagtggctgctgccagtggcgataagtcgtgtcttaccgggttggactcaagacgatagttaccggataaggcgcagcggtcgggctgaacggggggttcgtgcacacagcccagcttggagcgaacgacctacaccgaactgagatacctacagcgtgagctatgagaaagcgccacgcttcccgaagggagaaaggcggacaggtatccggtaagcggcagggtcggaacaggagagcgcacgagggagcttccagggggaaacgcctggtatctttatagtcctgtcgggtttcgccacctctgacttgagcgtcgatttttgtgatgctcgtcaggggggcggagcctatggaaaaacgccagcaacgcggcctttttacggttcctggccttttgctggccttttgctcacatgt

SEQ ID NO: 130 - DNA, 6844 bp, synthetic construct
  misc_feature 1..6844: note = pAV-CYP4V2 p3-SV40 intron-CYP4V2-P2A-RdCVF
  source 1..6844: mol_type = other DNA
cctgcaggcagctgcgcgctcgctcgctcactgaggccgcccgggcgtcgggcgacctttggtcgcccggcctcagtgagcgagcgagcgcgcagagagggagtggccaactccatcactaggggttcctgcggccggtcgcgtctagtactagtcgcgtaggatccgcatccaggacattcagtttcatcttcctggcactttagtgtttaggaagggcctggcctctcggggagcgacactcctcgcccggccactttgtaagaagcatcgagcgtggaaaaggggctggggtcagcactggggccctctgccgggaagagagactggcggccagcacacgcgtctccccaggctgaaatggggcaccctctcgcggcccttccctcccttcccgggctgggtggcaggtcttggctcttctgcgagtaccccgcggctgcggtctcccggcacccgctgagcagcctcgcccgccttcctctcccacccgcccctgcgtgctctccggggctccggcttcctcggtctggtgcctggtgcgtattttggaaaatacctggctcataaccacctcattgagctcccagtgtcccagtgggccagcggacacacacgggtagctgacttccctaacgtgtccccaaagcctccctggattacagcgcccgctgctccatgtgaccccgcgggagccaggacgcgccccgcctcccggggctgcaagttgcgcagggagcgagcgatgcgcagcagagctgggctccgagccggatgcgccttcctttcctctccagagcaggctgcccgcccgcggaatcccgcacgtagagcaacctcgcagcaccctcagaacagccccgctggggcgcgccgggctgccgcggtgacctttccgacgcccctgaccccgcatccggaggcggccggaagtgtcgccggcctcctcccggcgcagcctccgggcctccagtgcaatcactacgccctggggcccggaaaccgttttccggtctttcgctttcggctggggcgtggaggccgcggtgctgcgtaggccgggccgggcgcaggaacagccccgtggcgccctctctggccgccgcccgggcgggaaacgtcgttccggggaccgggcgaccccgcagcggggagcgcgccaggtccgcgcggggaagtgggcggtgtgcggccggcaccgcctcgcaccacgcccccgcgggcccgcactttcccggagtgcaccccgcggccgccagccggggcggtaagtttagtctttttgtcttttatttcaggtcccggatccggtggtggtgcaaatcaaagaactgctcctcagtggatgttgcctttacttctaggcgaattccgccaccatggcggggctctggctggggctcgtgtggcagaagctgctgctgtggggcgcggcgagtgccctttccctggccggcgccagtctggtcctgagtctgctgcagagggtggcgagctacgcgcggaaatggcagcagatgcggcccatccccacggtggcccgcgcctacccactggtgggccacgcgctgctgatgaagccggacgggcgagaattttttcagcagatcattgagtacacagaggaataccgccacatgccgctgctgaagctctgggtcgggccagtgcccatggtggccctttataatgcagaaaatgtggaggtaattttaactagttcaaagcaaattgacaaatcctctatgtacaagtttttagaaccatggcttggcctaggacttcttacaagtactggaaacaaatggcgctccaggagaaagatgttaacacccactttccattttaccattctggaagatttcttagatatcatgaatgaacaagcaaatatattggttaagaaacttgaaaaacacattaaccaagaagcatttaactgctttttttacatcactctttgtgccttagatatcatctgtgaaacagctatggggaagaatattggtgctcaaagtaatgatgattccgagtatgtccgtgcagtttatagaatgagtgagatgatatttcgaagaataaagatgccctggctttggcttgatctctggtaccttatgtttaaagaaggatgggaacacaaaaagagccttcagatcctacatacttttaccaacagtgtcatcgcggaacgggccaatgaaatgaacgccaatgaagactgtagaggtgatggcaggggctctgccccctccaaaaataaacgcagggcctttcttgacttgcttttaagtgtgactgatgacgaagggaacaggctaagtcatgaagatattcgagaagaagttgacaccttcatgtttgaggggcacgatacaactgcagctgcaataaactggtccttatacctgttgggttctaacccagaagtccagaaaaaagtggatcatgaattggatgacgtgtttgggaagtctgaccgtcccgctacagtagaagacctgaagaaacttcggtatctggaatgtgttattaaggagacccttcgcctttttccttctgttcctttatttgcccgtagtgttagtgaagattgtgaagtggcaggttacagagttctaaaaggcactgaagccgtcatcattccctatgcattgcacagagatccgagatacttccccaaccccgaggagttccagcctgagcggttcttccccgagaatgcacaagggcgccatccatatgcctacgtgcccttctctgctggccccaggaactgtataggtcaaaagtttgctgtgatggaagaaaagaccattctttcgtgcatcctgaggcacttttggatagaatccaaccagaaaagagaagagcttggtctagaaggacagttgattcttcgtccaagtaatggcatctggatcaagttgaagaggagaaatgcagatgaacgcggaagcggagctactaacttcagcctgctgaagcaggctggagacgtggaggagaaccctggacctatggcctccctgttctctggccgcatcctgatccgcaacaatagcgaccaggacgagctggatacggaggctgaggtcagtcgcaggctggagaaccggctggtgctgctgttctttggtgctggggcttgtccacagtgccaggccttcgtgcccatcctcaaggacttcttcgtgcggctcacagatgagttctatgtactgcgggcggctcagctggccctggtgtacgtgtcccaggactccacggaggagcagcaggacctgttcctcaaggacatgccaaagaaatggcttttcctgccctttgaggatgatctgaggaggtaaacgcgtggtttatccgatccaccggatctagataagatatccgatccaccggatctagataactgatcataatcagccataccacatttgtagaggttttacttgctttaaaaaacctcccacacctccccctgaacctgaaacataaaatgaatgcaattggcggccgcctcgagctgtgccttctagttgccagccatctgttgtttgcccctcccccgtgccttccttgaccctggaaggtgccactcccactgtcctttcctaataaaatgaggaaattgcatcgcattgtctgagtaggtgtcattctattctggggggtggggtggggcaggacagcaagggggaggattgggaagacaatagcaggcatgctggggatgcggtgggctctatggggtaaccacgtgcggacccaacggccgcaggaacccctagtgatggagttggccactccctctctgcgcgctcgctcgctcactgaggccgggcgaccaaaggtcgcccgacgcccgggctttgcccgggcggcctcagtgagcgagcgagcgcgcagctgcctgcaggggcgcctgatgcggtattttctccttacgcatctgtgcggtatttcacaccgcatacgtcaaagcaaccatagtacgcgccctgtagcggcacattaagcgcggcgggtgtggtggttacgcgcagcgtgaccgctacacttgccagcgccttagcgcccgctcctttcgctttcttcccttcctttctcgccacgttcgccggctttccccgtcaagctctaaatcgggggctccctttagggttccgatttagtgctttacggcacctcgaccccaaaaaacttgatttgggtgatggttcacgtagtgggccatcgccctgatagacggtttttcgccctttgacgttggagtccacgttctttaatagtggactcttgttccaaactggaacaacactcaactctatctcgggctattcttttgatttataagggattttgccgatttcggtctattggttaaaaaatgagctgatttaacaaaaatttaacgcgaattttaacaaaatattaacgtttacaattttatggtgcactctcagtacaatctgctctgatgccgcatagttaagccagccccgacacccgccaacacccgctgacgcgccctgacgggcttgtctgctcccggcatccgcttacagacaagctgtgaccgtctccgggagctgcatgtgtcagaggttttcaccgtcatcaccgaaacgcgcgagacgaaagggcctcgtgatacgcctatttttataggttaatgtcatgataataatggtttcttagacgtcaggtggcacttttcggggaaatgtgcgcggaacccctatttgtttatttttctaaatacattcaaatatgtatccgctcatgagacaataaccctgataaatgcttcaataatattgaaaaaggaagagtcctgaggcggaaagaaccagctgtggaatgtgtgtcagttagggtgtggaaagtccccaggctccccagcaggcagaagtatgcaaagcatgcatctcaattagtcagcaaccaggtgtggaaagtccccaggctccccagcaggcagaagtatgcaaagcatgcatctcaattagtcagcaaccatagtcccgcccctaactccgcccatcccgcccctaactccgcccagttccgcccattctccgccccatggctgactaattttttttatttatgcagaggccgaggccgcctcggcctctgagctattccagaagtagtgaggaggcttttttggaggcctaggcttttgcaaagatcgatcaagagacaggatgaggatcgtttcgcatgattgaacaagatggattgcacgcaggttctccggccgcttgggtggagaggctattcggctatgactgggcacaacagacaatcggctgctctgatgccgccgtgttccggctgtcagcgcaggggcgcccggttctttttgtcaagaccgacctgtccggtgccctgaatgaactgcaagacgaggcagcgcggctatcgtggctggccacgacgggcgttccttgcgcagctgtgctcgacgttgtcactgaagcgggaagggactggctgctattgggcgaagtgccggggcaggatctcctgtcatctcaccttgctcctgccgagaaagtatccatcatggctgatgcaatgcggcggctgcatacgcttgatccggctacctgcccattcgaccaccaagcgaaacatcgcatcgagcgagcacgtactcggatggaagccggtcttgtcgatcaggatgatctggacgaagagcatcaggggctcgcgccagccgaactgttcgccaggctcaaggcgagcatgcccgacggcgaggatctcgtcgtgacccatggcgatgcctgcttgccgaatatcatggtggaaaatggccgcttttctggattcatcgactgtggccggctgggtgtggcggaccgctatcaggacatagcgttggctacccgtgatattgctgaagagcttggcggcgaatgggctgaccgcttcctcgtgctttacggtatcgccgctcccgattcgcagcgcatcgccttctatcgccttcttgacgagttcttctgactgtcagaccaagtttactcatatatactttagattgatttaaaacttcatttttaatttaaaaggatctaggtgaagatcctttttgataatctcatgaccaaaatcccttaacgtgagttttcgttccactgagcgtcagaccccgtagaaaagatcaaaggatcttcttgagatcctttttttctgcgcgtaatctgctgcttgcaaacaaaaaaaccaccgctaccagcggtggtttgtttgccggatcaagagctaccaactctttttccgaaggtaactggcttcagcagagcgcagataccaaatactgttcttctagtgtagccgtagttaggccaccacttcaagaactctgtagcaccgcctacatacctcgctctgctaatcctgttaccagtggctgctgccagtggcgataagtcgtgtcttaccgggttggactcaagacgatagttaccggataaggcgcagcggtcgggctgaacggggggttcgtgcacacagcccagcttggagcgaacgacctacaccgaactgagatacctacagcgtgagctatgagaaagcgccacgcttcccgaagggagaaaggcggacaggtatccggtaagcggcagggtcggaacaggagagcgcacgagggagcttccagggggaaacgcctggtatctttatagtcctgtcgggtttcgccacctctgacttgagcgtcgatttttgtgatgctcgtcaggggggcggagcctatggaaaaacgccagcaacgcggcctttttacggttcctggccttttgctggccttttgctcacatgt

SEQ ID NO: 131 - DNA, 6278 bp, synthetic construct
  misc_feature 1..6278: note = pAV-p5-intron-CYP4V2-P2A-RdCVF-BGH
  source 1..6278: mol_type = other DNA
cctgcaggcagctgcgcgctcgctcgctcactgaggccgcccgggcgtcgggcgacctttggtcgcccggcctcagtgagcgagcgagcgcgcagagagggagtggccaactccatcactaggggttcctgcggccggtcgcgtctagtactagtcgcgtaggatccgagccggatgcgccttcctttcctctccagagcaggctgcccgcccgcggaatcccgcacgtagagcaacctcgcagcaccctcagaacagccccgctggggcgcgccgggctgccgcggtgacctttccgacgcccctgaccccgcatccggaggcggccggaagtgtcgccggcctcctcccggcgcagcctccgggcctccagtgcaatcactacgccctggggcccggaaaccgttttccggtctttcgctttcggctggggcgtggaggccgcggtgctgcgtaggccgggccgggcgcaggaacagccccgtggcgccctctctggccgccgcccgggcgggaaacgtcgttccggggaccgggcgaccccgcagcggggagcgcgccaggtccgcgcggggaagtgggcggtgtgcggccggcaccgcctcgcaccacgcccccgcgggcccgcactttcccggagtgcaccccgcggccgccagccggggcggtaagtatcaaggttacaagacaggtttaaggagaccaatagaaactgggcttgtcgagacagagaagactcttgcgtttctgataggcacctattggtcttactgacatccactttgcctttctctccacaggaattccgccaccatggcggggctctggctggggctcgtgtggcagaagctgctgctgtggggcgcggcgagtgccctttccctggccggcgccagtctggtcctgagtctgctgcagagggtggcgagctacgcgcggaaatggcagcagatgcggcccatccccacggtggcccgcgcctacccactggtgggccacgcgctgctgatgaagccggacgggcgagaattttttcagcagatcattgagtacacagaggaataccgccacatgccgctgctgaagctctgggtcgggccagtgcccatggtggccctttataatgcagaaaatgtggaggtaattttaactagttcaaagcaaattgacaaatcctctatgtacaagtttttagaaccatggcttggcctaggacttcttacaagtactggaaacaaatggcgctccaggagaaagatgttaacacccactttccattttaccattctggaagatttcttagatatcatgaatgaacaagcaaatatattggttaagaaacttgaaaaacacattaaccaagaagcatttaactgctttttttacatcactctttgtgccttagatatcatctgtgaaacagctatggggaagaatattggtgctcaaagtaatgatgattccgagtatgtccgtgcagtttatagaatgagtgagatgatatttcgaagaataaagatgccctggctttggcttgatctctggtaccttatgtttaaagaaggatgggaacacaaaaagagccttcagatcctacatacttttaccaacagtgtcatcgcggaacgggccaatgaaatgaacgccaatgaagactgtagaggtgatggcaggggctctgccccctccaaaaataaacgcagggcctttcttgacttgcttttaagtgtgactgatgacgaagggaacaggctaagtcatgaagatattcgagaagaagttgacaccttcatgtttgaggggcacgatacaactgcagctgcaataaactggtccttatacctgttgggttctaacccagaagtccagaaaaaagtggatcatgaattggatgacgtgtttgggaagtctgaccgtcccgctacagtagaagacctgaagaaacttcggtatctggaatgtgttattaaggagacccttcgcctttttccttctgttcctttatttgcccgtagtgttagtgaagattgtgaagtggcaggttacagagttctaaaaggcactgaagccgtcatcattccctatgcattgcacagagatccgagatacttccccaaccccgaggagttccagcctgagcggttcttccccgagaatgcacaagggcgccatccatatgcctacgtgcccttctctgctggccccaggaactgtataggtcaaaagtttgctgtgatggaagaaaagaccattctttcgtgcatcctgaggcacttttggatagaatccaaccagaaaagagaagagcttggtctagaaggacagttgattcttcgtccaagtaatggcatctggatcaagttgaagaggagaaatgcagatgaacgcggaagcggagctactaacttcagcctgctgaagcaggctggagacgtggaggagaaccctggacctatggcctccctgttctctggccgcatcctgatccgcaacaatagcgaccaggacgagctggatacggaggctgaggtcagtcgcaggctggagaaccggctggtgctgctgttctttggtgctggggcttgtccacagtgccaggccttcgtgcccatcctcaaggacttcttcgtgcggctcacagatgagttctatgtactgcgggcggctcagctggccctggtgtacgtgtcccaggactccacggaggagcagcaggacctgttcctcaaggacatgccaaagaaatggcttttcctgccctttgaggatgatctgaggaggtaaacgcgtggtttatccgatccaccggatctagataagatatccgatccaccggatctagataactgatcataatcagccataccacatttgtagaggttttacttgctttaaaaaacctcccacacctccccctgaacctgaaacataaaatgaatgcaattggcggccgcctcgagctgtgccttctagttgccagccatctgttgtttgcccctcccccgtgccttccttgaccctggaaggtgccactcccactgtcctttcctaataaaatgaggaaattgcatcgcattgtctgagtaggtgtcattctattctggggggtggggtggggcaggacagcaagggggaggattgggaagacaatagcaggcatgctggggatgcggtgggctctatggggtaaccacgtgcggacccaacggccgcaggaacccctagtgatggagttggccactccctctctgcgcgctcgctcgctcactgaggccgggcgaccaaaggtcgcccgacgcccgggctttgcccgggcggcctcagtgagcgagcgagcgcgcagctgcctgcaggggcgcctgatgcggtattttctccttacgcatctgtgcggtatttcacaccgcatacgtcaaagcaaccatagtacgcgccctgtagcggcacattaagcgcggcgggtgtggtggttacgcgcagcgtgaccgctacacttgccagcgccttagcgcccgctcctttcgctttcttcccttcctttctcgccacgttcgccggctttccccgtcaagctctaaatcgggggctccctttagggttccgatttagtgctttacggcacctcgaccccaaaaaacttgatttgggtgatggttcacgtagtgggccatcgccctgatagacggtttttcgccctttgacgttggagtccacgttctttaatagtggactcttgttccaaactggaacaacactcaactctatctcgggctattcttttgatttataagggattttgccgatttcggtctattggttaaaaaatgagctgatttaacaaaaatttaacgcgaattttaacaaaatattaacgtttacaattttatggtgcactctcagtacaatctgctctgatgccgcatagttaagccagccccgacacccgccaacacccgctgacgcgccctgacgggcttgtctgctcccggcatccgcttacagacaagctgtgaccgtctccgggagctgcatgtgtcagaggttttcaccgtcatcaccgaaacgcgcgagacgaaagggcctcgtgatacgcctatttttataggttaatgtcatgataataatggtttcttagacgtcaggtggcacttttcggggaaatgtgcgcggaacccctatttgtttatttttctaaatacattcaaatatgtatccgctcatgagacaataaccctgataaatgcttcaataatattgaaaaaggaagagtcctgaggcggaaagaaccagctgtggaatgtgtgtcagttagggtgtggaaagtccccaggctccccagcaggcagaagtatgcaaagcatgcatctcaattagtcagcaaccaggtgtggaaagtccccaggctccccagcaggcagaagtatgcaaagcatgcatctcaattagtcagcaaccatagtcccgcccctaactccgcccatcccgcccctaactccgcccagttccgcccattctccgccccatggctgactaattttttttatttatgcagaggccgaggccgcctcggcctctgagctattccagaagtagtgaggaggcttttttggaggcctaggcttttgcaaagatcgatcaagagacaggatgaggatcgtttcgcatgattgaacaagatggattgcacgcaggttctccggccgcttgggtggagaggctattcggctatgactgggcacaacagacaatcggctgctctgatgccgccgtgttccggctgtcagcgcaggggcgcccggttctttttgtcaagaccgacctgtccggtgccctgaatgaactgcaagacgaggcagcgcggctatcgtggctggccacgacgggcgttccttgcgcagctgtgctcgacgttgtcactgaagcgggaagggactggctgctattgggcgaagtgccggggcaggatctcctgtcatctcaccttgctcctgccgagaaagtatccatcatggctgatgcaatgcggcggctgcatacgcttgatccggctacctgcccattcgaccaccaagcgaaacatcgcatcgagcgagcacgtactcggatggaagccggtcttgtcgatcaggatgatctggacgaagagcatcaggggctcgcgccagccgaactgttcgccaggctcaaggcgagcatgcccgacggcgaggatctcgtcgtgacccatggcgatgcctgcttgccgaatatcatggtggaaaatggccgcttttctggattcatcgactgtggccggctgggtgtggcggaccgctatcaggacatagcgttggctacccgtgatattgctgaagagcttggcggcgaatgggctgaccgcttcctcgtgctttacggtatcgccgctcccgattcgcagcgcatcgccttctatcgccttcttgacgagttcttctgactgtcagaccaagtttactcatatatactttagattgatttaaaacttcatttttaatttaaaaggatctaggtgaagatcctttttgataatctcatgaccaaaatcccttaacgtgagttttcgttccactgagcgtcagaccccgtagaaaagatcaaaggatcttcttgagatcctttttttctgcgcgtaatctgctgcttgcaaacaaaaaaaccaccgctaccagcggtggtttgtttgccggatcaagagctaccaactctttttccgaaggtaactggcttcagcagagcgcagataccaaatactgttcttctagtgtagccgtagttaggccaccacttcaagaactctgtagcaccgcctacatacctcgctctgctaatcctgttaccagtggctgctgccagtggcgataagtcgtgtcttaccgggttggactcaagacgatagttaccggataaggcgcagcggtcgggctgaacggggggttcgtgcacacagcccagcttggagcgaacgacctacaccgaactgagatacctacagcgtgagctatgagaaagcgccacgcttcccgaagggagaaaggcggacaggtatccggtaagcggcagggtcggaacaggagagcgcacgagggagcttccagggggaaacgcctggtatctttatagtcctgtcgggtttcgccacctctgacttgagcgtcgatttttgtgatgctcgtcaggggggcggagcctatggaaaaacgccagcaacgcggcctttttacggttcctggccttttgctggccttttgctcacatgt

SEQ ID NO: 132 - DNA, 6277 bp, synthetic construct
  misc_feature 1..6277: note = pAV-p5-CDS intron-CYP4V2-P2A-RdCVF-BGH
  source 1..6277: mol_type = other DNA
cctgcaggcagctgcgcgctcgctcgctcactgaggccgcccgggcgtcgggcgacctttggtcgcccggcctcagtgagcgagcgagcgcgcagagagggagtggccaactccatcactaggggttcctgcggccggtcgcgtctagtactagtcgcgtaggatccgagccggatgcgccttcctttcctctccagagcaggctgcccgcccgcggaatcccgcacgtagagcaacctcgcagcaccctcagaacagccccgctggggcgcgccgggctgccgcggtgacctttccgacgcccctgaccccgcatccggaggcggccggaagtgtcgccggcctcctcccggcgcagcctccgggcctccagtgcaatcactacgccctggggcccggaaaccgttttccggtctttcgctttcggctggggcgtggaggccgcggtgctgcgtaggccgggccgggcgcaggaacagccccgtggcgccctctctggccgccgcccgggcgggaaacgtcgttccggggaccgggcgaccccgcagcggggagcgcgccaggtccgcgcggggaagtgggcggtgtgcggccggcaccgcctcgcaccacgcccccgcgggcccgcactttcccggagtgcaccccgcggccgccagccggggcggaattcgccaccatggcggggctctggctggggctcgtgtggcagaagctgctgctgtggggcgcggcgagtgccctttccctggccggcgccagtctggtcctgagtctgctgcagagggtggcgagctacgcgcggaaatggcagcagatgcggcccatccccacggtggcccgcgcctacccactggtgggccacgcgctgctgatgaagccggacgggcgaggtaagtatcaaggttacaagacaggtttaaggagaccaatagaaactgggcttgtcgagacagagaagactcttgcgtttctgataggcacctattggtcttactgacatccactttgcctttctctccacagaattttttcagcagatcattgagtacacagaggaataccgccacatgccgctgctgaagctctgggtcgggccagtgcccatggtggccctttataatgcagaaaatgtggaggtaattttaactagttcaaagcaaattgacaaatcctctatgtacaagtttttagaaccatggcttggcctaggacttcttacaagtactggaaacaaatggcgctccaggagaaagatgttaacacccactttccattttaccattctggaagatttcttagatatcatgaatgaacaagcaaatatattggttaagaaacttgaaaaacacattaaccaagaagcatttaactgctttttttacatcactctttgtgccttagatatcatctgtgaaacagctatggggaagaatattggtgctcaaagtaatgatgattccgagtatgtccgtgcagtttatagaatgagtgagatgatatttcgaagaataaagatgccctggctttggcttgatctctggtaccttatgtttaaagaaggatgggaacacaaaaagagccttcagatcctacatacttttaccaacagtgtcatcgcggaacgggccaatgaaatgaacgccaatgaagactgtagaggtgatggcaggggctctgccccctccaaaaataaacgcagggcctttcttgacttgcttttaagtgtgactgatgacgaagggaacaggctaagtcatgaagatattcgagaagaagttgacaccttcatgtttgaggggcacgatacaactgcagctgcaataaactggtccttatacctgttgggttctaacccagaagtccagaaaaaagtggatcatgaattggatgacgtgtttgggaagtctgaccgtcccgctacagtagaagacctgaagaaacttcggtatctggaatgtgttattaaggagacccttcgcctttttccttctgttcctttatttgcccgtagtgttagtgaagattgtgaagtggcaggttacagagttctaaaaggcactgaagccgtcatcattccctatgcattgcacagagatccgagatacttccccaaccccgaggagttccagcctgagcggttcttccccgagaatgcacaagggcgccatccatatgcctacgtgcccttctctgctggccccaggaactgtataggtcaaaagtttgctgtgatggaagaaaagaccattctttcgtgcatcctgaggcacttttggatagaatccaaccagaaaagagaagagcttggtctagaaggacagttgattcttcgtccaagtaatggcatctggatcaagttgaagaggagaaatgcagatgaacgcggaagcggagctactaacttcagcctgctgaagcaggctggagacgtggaggagaaccctggacctatggcctccctgttctctggccgcatcctgatccgcaacaatagcgaccaggacgagctggatacggaggctgaggtcagtcgcaggctggagaaccggctggtgctgctgttctttggtgctggggcttgtccacagtgccaggccttcgtgcccatcctcaaggacttcttcgtgcggctcacagatgagttctatgtactgcgggcggctcagctggccctggtgtacgtgtcccaggactccacggaggagcagcaggacctgttcctcaaggacatgccaaagaaatggcttttcctgccctttgaggatgatctgaggaggtgaacgcgtggtttatccgatccaccggatctagataagatatccgatccaccggatctagataactgatcataatcagccataccacatttgtagaggttttacttgctttaaaaaacctcccacacctccccctgaacctgaaacataaaatgaatgcaattggcggccgcctcgagctgtgccttctagttgccagccatctgttgtttgcccctcccccgtgccttccttgaccctggaaggtgccactcccactgtcctttcctaataaaatgaggaaattgcatcgcattgtctgagtaggtgtcattctattctggggggtggggtggggcaggacagcaagggggaggattgggaagacaatagcaggcatgctggggatgcggtgggctctatggggtaaccacgtgcggacccaacggccgcaggaacccctagtgatggagttggccactccctctctgcgcgctcgctcgctcactgaggccgggcgaccaaaggtcgcccgacgcccgggctttgcccgggcggcctcagtgagcgagcgagcgcgcagctgcctgcaggggcgcctgatgcggtattttctccttacgcatctgtgcggtatttcacaccgcatacgtcaaagcaaccatagtacgcgccctgtagcggcacattaagcgcggcgggtgtggtggttacgcgcagcgtgaccgctacacttgccagcgccttagcgcccgctcctttcgctttcttcccttcctttctcgccacgttcgccggctttccccgtcaagctctaaatcgggggctccctttagggttccgatttagtgctttacggcacctcgaccccaaaaaacttgatttgggtgatggttcacgtagtgggccatcgccctgatagacggtttttcgccctttgacgttggagtccacgttctttaatagtggactcttgttccaaactggaacaacactcaactctatctcgggctattcttttgatttataagggattttgccgatttcggtctattggttaaaaaatgagctgatttaacaaaaatttaacgcgaattttaacaaaatattaacgtttacaattttatggtgcactctcagtacaatctgctctgatgccgcatagttaagccagccccgacacccgccaacacccgctgacgcgccctgacgggcttgtctgctcccggcatccgcttacagacaagctgtgaccgtctccgggagctgcatgtgtcagaggttttcaccgtcatcaccgaaacgcgcgagacgaaagggcctcgtgatacgcctatttttataggttaatgtcatgataataatggtttcttagacgtcaggtggcacttttcggggaaatgtgcgcggaacccctatttgtttatttttctaaatacattcaaatatgtatccgctcatgagacaataaccctgataaatgcttcaataatattgaaaaaggaagagtcctgaggcggaaagaaccagctgtggaatgtgtgtcagttagggtgtggaaagtccccaggctccccagcaggcagaagtatgcaaagcatgcatctcaattagtcagcaaccaggtgtggaaagtccccaggctccccagcaggcagaagtatgcaaagcatgcatctcaattagtcagcaaccatagtcccgcccctaactccgcccatcccgcccctaactccgcccagttccgcccattctccgccccatggctgactaattttttttatttatgcagaggccgaggccgcctcggcctctgagctattccagaagtagtgaggaggcttttttggaggcctaggcttttgcaaagatcgatcaagagacaggatgaggatcgtttcgcatgattgaacaagatggattgcacgcaggttctccggccgcttgggtggagaggctattcggctatgactgggcacaacagacaatcggctgctctgatgccgccgtgttccggctgtcagcgcaggggcgcccggttctttttgtcaagaccgacctgtccggtgccctgaatgaactgcaagacgaggcagcgcggctatcgtggctggccacgacgggcgttccttgcgcagctgtgctcgacgttgtcactgaagcgggaagggactggctgctattgggcgaagtgccggggcaggatctcctgtcatctcaccttgctcctgccgagaaagtatccatcatggctgatgcaatgcggcggctgcatacgcttgatccggctacctgcccattcgaccaccaagcgaaacatcgcatcgagcgagcacgtactcggatggaagccggtcttgtcgatcaggatgatctggacgaagagcatcaggggctcgcgccagccgaactgttcgccaggctcaaggcgagcatgcccgacggcgaggatctcgtcgtgacccatggcgatgcctgcttgccgaatatcatggtggaaaatggccgcttttctggattcatcgactgtggccggctgggtgtggcggaccgctatcaggacatagcgttggctacccgtgatattgctgaagagcttggcggcgaatgggctgaccgcttcctcgtgctttacggtatcgccgctcccgattcgcagcgcatcgccttctatcgccttcttgacgagttcttctgactgtcagaccaagtttactcatatatactttagattgatttaaaacttcatttttaatttaaaaggatctaggtgaagatcctttttgataatctcatgaccaaaatcccttaacgtgagttttcgttccactgagcgtcagaccccgtagaaaagatcaaaggatcttcttgagatcctttttttctgcgcgtaatctgctgcttgcaaacaaaaaaaccaccgctaccagcggtggtttgtttgccggatcaagagctaccaactctttttccgaaggtaactggcttcagcagagcgcagataccaaatactgttcttctagtgtagccgtagttaggccaccacttcaagaactctgtagcaccgcctacatacctcgctctgctaatcctgttaccagtggctgctgccagtggcgataagtcgtgtcttaccgggttggactcaagacgatagttaccggataaggcgcagcggtcgggctgaacggggggttcgtgcacacagcccagcttggagcgaacgacctacaccgaactgagatacctacagcgtgagctatgagaaagcgccacgcttcccgaagggagaaaggcggacaggtatccggtaagcggcagggtcggaacaggagagcgcacgagggagcttccagggggaaacgcctggtatctttatagtcctgtcgggtttcgccacctctgacttgagcgtcgatttttgtgatgctcgtcaggggggcggagcctatggaaaaacgccagcaacgcggcctttttacggttcctggccttttgctggccttttgctcacatgt

SEQ ID NO: 133 - DNA, 7313 bp, synthetic construct
  misc_feature 1..7313: note = pAAV-RC5-Amp
  source 1..7313: mol_type = other DNA
atcgttaacgccccgcgccggccgctctagaactagtggatcccccggaagatcagaagttcctattccgaagttcctattctctagaaagtataggaacttctgatctgcgcagccgccatgccggggttttacgagattgtgattaaggtccccagcgaccttgacgagcatctgcccggcatttctgacagctttgtgaactgggtggccgagaaggaatgggagttgccgccagattctgacatggatctgaatctgattgagcaggcacccctgaccgtggccgagaagctgcagcgcgactttctgacggaatggcgccgtgtgagtaaggccccggaggcccttttctttgtgcaatttgagaagggagagagctacttccacatgcacgtgctcgtggaaaccaccggggtgaaatccatggttttgggacgtttcctgagtcagattcgcgaaaaactgattcagagaatttaccgcgggatcgagccgactttgccaaactggttcgcggtcacaaagaccagaaatggcgccggaggcgggaacaaggtggtggatgagtgctacatccccaattacttgctccccaaaacccagcctgagctccagtgggcgtggactaatatggaacagtatttaagcgcctgtttgaatctcacggagcgtaaacggttggtggcgcagcatctgacgcacgtgtcgcagacgcaggagcagaacaaagagaatcagaatcccaattctgatgcgccggtgatcagatcaaaaacttcagccaggtacatggagctggtcgggtggctcgtggacaaggggattacctcggagaagcagtggatccaggaggaccaggcctcatacatctccttcaatgcggcctccaactcgcggtcccaaatcaaggctgccttggacaatgcgggaaagattatgagcctgactaaaaccgcccccgactacctggtgggccagcagcccgtggaggacatttccagcaatcggatttataaaattttggaactaaacgggtacgatccccaatatgcggcttccgtctttctgggatgggccacgaaaaagttcggcaagaggaacaccatctggctgtttgggcctgcaactaccgggaagaccaacatcgcggaggccatagcccacactgtgcccttctacgggtgcgtaaactggaccaatgagaactttcccttcaacgactgtgtcgacaagatggtgatctggtgggaggaggggaagatgaccgccaaggtcgtggagtcggccaaagccattctcggaggaagcaaggtgcgcgtggaccagaaatgcaagtcctcggcccagatagacccgactcccgtgatcgtcacctccaacaccaacatgtgcgccgtgattgacgggaactcaacgaccttcgaacaccagcagccgttgcaagaccggatgttcaaatttgaactcacccgccgtctggatcatgactttgggaaggtcaccaagcaggaagtcaaagactttttccggtgggcaaaggatcacgtggttgaggtggagcatgaattctacgtcaaaaagggtggagccaagaaaagacccgcccccagtgacgcagatataagtgagcccaaacgggtgcgcgagtcagttgcgcagccatcgacgtcagacgcggaagcttcgatcaactacgcagacaggtaccaaaacaaatgttctcgtcacgtgggcatgaatctgatgctgtttccctgcagacaatgcgagagaatgaatcagaattcaaatatctgcttcactcacggacagaaagactgtttagagtgctttcccgtgtcagaatctcaacccgtttctgtcgtcaaaaaggcgtatcagaaactgtgctacattcatcatatcatgggaaaggtgccagacgcttgcactgcctgcgatctggtcaatgtggatttggatgactgcatctttgaacaataaatgatttgtaaataaatttagtagtcatgtcttttgttgatcaccctccagattggttggaagaagttggtgaaggtcttcgcgagtttttgggccttgaagcgggcccaccgaaaccaaaacccaatcagcagcatcaagatcaagcccgtggtcttgtgctgcctggttataactatctcggacccggaaacggtctcgatcgaggagagcctgtcaacagggcagacgaggtcgcgcgagagcacgacatctcgtacaacgagcagcttgaggcgggagacaacccctacctcaagtacaaccacgcggacgccgagtttcaggagaagctcgccgacgacacatccttcgggggaaacctcggaaaggcagtctttcaggccaagaaaagggttctcgaaccttttggcctggttgaagagggtgctaagacggcccctaccggaaagcggatagacgaccactttccaaaaagaaagaaggctcggaccgaagaggactccaagccttccacctcgtcagacgccgaagctggacccagcggatcccagcagctgcaaatcccagcccaaccagcctcaagtttgggagctgatacaatgtctgcgggaggtggcggcccattgggcgacaataaccaaggtgccgatggagtgggcaatgcctcgggagattggcattgcgattccacgtggatgggggacagagtcgtcaccaagtccacccgaacctgggtgctgcccagctacaacaaccaccagtaccgagagatcaaaagcggctccgtcgacggaagcaacgccaacgcctactttggatacagcaccccctgggggtactttgactttaaccgcttccacagccactggagcccccgagactggcaaagactcatcaacaactactggggcttcagaccccggtccctcagagtcaaaatcttcaacattcaagtcaaagaggtcacggtgcaggactccaccaccaccatcgccaacaacctcacctccaccgtccaagtgtttacggacgacgactaccagctgccctacgtcgtcggcaacgggaccgagggatgcctgccggccttccctccgcaggtctttacgctgccgcagtacggttacgcgacgctgaaccgcgacaacacagaaaatcccaccgagaggagcagcttcttctgcctagagtactttcccagcaagatgctgagaacgggcaacaactttgagtttacctacaactttgaggaggtgcccttccactccagcttcgctcccagtcagaacctgttcaagctggccaacccgctggtggaccagtacttgtaccgcttcgtgagcacaaataacactggcggagtccagttcaacaagaacctggccgggagatacgccaacacctacaaaaactggttcccggggcccatgggccgaacccagggctggaacctgggctccggggtcaaccgcgccagtgtcagcgccttcgccacgaccaataggatggagctcgagggcgcgagttaccaggtgcccccgcagccgaacggcatgaccaacaacctccagggcagcaacacctatgccctggagaacactatgatcttcaacagccagccggcgaacccgggcaccaccgccacgtacctcgagggcaacatgctcatcaccagcgagagcgagacgcagccggtgaaccgcgtggcgtacaacgtcggcgggcagatggccaccaacaaccagagctccaccactgcccccgcgaccggcacgtacaacctccaggaaatcgtgcccggcagcgtgtggatggagagggacgtgtacctccaaggacccatctgggccaagatcccagagacgggggcgcactttcacccctctccggccatgggcggattcggactcaaacacccaccgcccatgatgctcatcaagaacacgcctgtgcccggaaatatcaccagcttctcggacgtgcccgtcagcagcttcatcacccagtacagcaccgggcaggtcaccgtggagatggagtgggagctcaagaaggaaaactccaagaggtggaacccagagatccagtacacaaacaactacaacgacccccagtttgtggactttgccccggacagcaccggggaatacagaaccaccagacctatcggaacccgataccttacccgacccctttaacccattcatgtcgcataccctcaataaaccggttaattcgtgtcagttgaactttggtctcatgtcgttattatcttatctggtcaccagatccccgtagataagtagcatggcgggttaatcattaactacagcccgggcgtttaaacagcgggcggaggggtggagtcgtgacgtgaattacgtcatagggttagggaggtcctgtattagaggtcacgtgagtgttttgcgacattttgcgacaccatgtggtctcgctgggggggggggcccgagtgagcacgcagggtctccattttgaagcgggaggtttgaacgagcgctggcgcgctcactggccgtcgttttacaacgtcgtgactgggaaaaccctggcgttacccaacttaatcgccttgcagcacatccccctttcgccagctggcgtaatagcgaagaggcccgcaccgatcgcccttcccaacagttgcgcagcctgaatggcgaatggaaattgtaagcgttaatattttgttaaaattcgcgttaaatttttgttaaatcagctcatttttttaaccaataggccgaaatcggcaaaatcccttataaatcaaaagaatagaccgagatagggttgagtgttgttccagtttggaacaagagtccactattaagaacgtggactccaacgtcaaagggcgaaaaaccgtctatcagggcgatggcccactacgtgaaccatcaccctaatcaagttttttggggtcgaggtgccgtaaagcactaaatcggaaccctaaagggagcccccgatttagagcttgacggggaaagccggcgaacgtggcgagaaaggaagggaagaaagcgaaaggagcgggcgctagggcgctggcaagtgtagcggtcacgctgcgcgtaaccaccacacccgccgcgcttaatgcgccgctacagggcgcgtcaggtggcacttttcggggaaatgtgcgcggaacccctatttgtttatttttctaaatacattcaaatatgtatccgctcatgagacaataaccctgataaatgcttcaataatattgaaaaaggaagagtatgagtattcaacatttccgtgtcgcccttattcccttttttgcggcattttgccttcctgtttttgctcacccagaaacgctggtgaaagtaaaagatgctgaagatcagttgggtgcacgagtgggttacatcgaactggatctcaacagcggtaagatccttgagagttttcgccccgaagaacgttttccaatgatgagcacttttaaagttctgctatgtggcgcggtattatcccgtattgacgccgggcaagagcaactcggtcgccgcatacactattctcagaatgacttggttgagtactcaccagtcacagaaaagcatcttacggatggcatgacagtaagagaattatgcagtgctgccataaccatgagtgataacactgcggccaacttacttctgacaacgatcggaggaccgaaggagctaaccgcttttttgcacaacatgggggatcatgtaactcgccttgatcgttgggaaccggagctgaatgaagccataccaaacgacgagcgtgacaccacgatgcctgtagcaatggcaacaacgttgcgcaaactattaactggcgaactacttactctagcttcccggcaacaattaatagactggatggaggcggataaagttgcaggaccacttctgcgctcggcccttccggctggctggtttattgctgataaatctggagccggtgagcgtgggtctcgcggtatcattgcagcactggggccagatggtaagccctcccgtatcgtagttatctacacgacggggagtcaggcaactatggatgaacgaaatagacagatcgctgagataggtgcctcactgattaagcattggtaactgtcagaccaagtttactcatatatactttagattgatttaaaacttcatttttaatttaaaaggatctaggtgaagatcctttttgataatctcatgaccaaaatcccttaacgtgagttttcgttccactgagcgtcagaccccgtagaaaagatcaaaggatcttcttgagatcctttttttctgcgcgtaatctgctgcttgcaaacaaaaaaaccaccgctaccagcggtggtttgtttgccggatcaagagctaccaactctttttccgaaggtaactggcttcagcagagcgcagataccaaatactgttcttctagtgtagccgtagttaggccaccacttcaagaactctgtagcaccgcctacatacctcgctctgctaatcctgttaccagtggctgctgccagtggcgataagtcgtgtcttaccgggttggactcaagacgatagttaccggataaggcgcagcggtcgggctgaacggggggttcgtgcacacagcccagcttggagcgaacgacctacaccgaactgagatacctacagcgtgagctatgagaaagcgccacgcttcccgaagggagaaaggcggacaggtatccggtaagcggcagggtcggaacaggagagcgcacgagggagcttccagggggaaacgcctggtatctttatagtcctgtcgggtttcgccacctctgacttgagcgtcgatttttgtgatgctcgtcaggggggcggagcctatggaaaaacgccagcaacgcggcctttttacggttcctggccttttgctggccttttgctcacatgttctttcctgcgttatcccctgattctgtggataaccgtattaccgcctttgagtgagctgataccgctcgccgcagccgaacgaccgagcgcagcgagtcagtgagcgaggaagcggaagagcgcccaatacgcaaaccgcctctccccgcgcgttggccgattcattaatgcagctggcacgacaggtttcccgactggaaagcgggcagtgagcgcaacgcaattaatgtgagttagctcactcattaggcaccccaggctttacactttatgcttccggctcgtatgttgtgtggaattgtgagcggataacaatttcacacaggaaacagctatgaccatgattacgccaagcgcgccgat

SEQ ID NO: 134 - DNA, 2257 bp, synthetic construct
  misc_feature 1..2257: note = RC8-cap
  source 1..2257: mol_type = other DNA
ataaatgatttaaatcaggtatggctgccgatggttatcttccagattggctcgaggacaacctctctgagggcattcgcgagtggtgggcgctgaaacctggagccccgaagcccaaagccaaccagcaaaagcaggacgacggccggggtctggtgcttcctggctacaagtacctcggacccttcaacggactcgacaagggggagcccgtcaacgcggcggacgcagcggccctcgagcacgacaaggcctacgaccagcagctgcaggcgggtgacaatccgtacctgcggtataaccacgccgacgccgagtttcaggagcgtctgcaagaagatacgtcttttgggggcaacctcgggcgagcagtcttccaggccaagaagcgggttctcgaacctctcggtctggttgaggaaggcgctaagacggctcctggaaagaagagaccggtagagccatcaccccagcgttctccagactcctctacgggcatcggcaagaaaggccaacagcccgccagaaaaagactcaattttggtcagactggcgactcagagtcagttccagaccctcaacctctcggagaacctccagcagcgccctctggtgtgggacctaatacaatggctgcaggcggtggcgcaccaatggcagacaataacgaaggcgccgacggagtgggtagttcctcgggaaattggcattgcgattccacatggctgggcgacagagtcatcaccaccagcacccgaacctgggccctgcccacctacaacaaccacctctacaagcaaatctccaacgggacatcgggaggagccaccaacgacaacacctacttcggctacagcaccccctgggggtattttgactttaacagattccactgccacttttcaccacgtgactggcagcgactcatcaacaacaactggggattccggcccaagagactcagcttcaagctcttcaacatccaggtcaaggaggtcacgcagaatgaaggcaccaagaccatcgccaataacctcaccagcaccatccaggtgtttacggactcggagtaccagctgccgtacgttctcggctctgcccaccagggctgcctgcctccgttcccggcggacgtgttcatgattccccagtacggctacctaacactcaacaacggtagtcaggccgtgggacgctcctccttctactgcctggaatactttccttcgcagatgctgagaaccggcaacaacttccagtttacttacaccttcgaggacgtgcctttccacagcagctacgcccacagccagagcttggaccggctgatgaatcctctgattgaccagtacctgtactacttgtctcggactcaaacaacaggaggcacggcaaatacgcagactctgggcttcagccaaggtgggcctaatacaatggccaatcaggcaaagaactggctgccaggaccctgttaccgccaacaacgcgtctcaacgacaaccgggcaaaacaacaatagcaactttgcctggactgctgggaccaaataccatctgaatggaagaaattcattggctaatcctggcatcgctatggcaacacacaaagacgacgaggagcgtttttttcccagtaacgggatcctgatttttggcaaacaaaatgctgccagagacaatgcggattacagcgatgtcatgctcaccagcgaggaagaaatcaaaaccactaaccctgtggctacagaggaatacggtatcgtggcagataacttgcagcagcaaaacacggctcctcaaattggaactgtcaacagccagggggccttacccggtatggtctggcagaaccgggacgtgtacctgcagggtcccatctgggccaagattcctcacacggacggcaacttccacccgtctccgctgatgggcggctttggcctgaaacatcctccgcctcagatcctgatcaagaacacgcctgtacctgcggatcctccgaccaccttcaaccagtcaaagctgaactctttcatcacgcaatacagcaccggacaggtcagcgtggaaattgaatgggagctgcagaaggaaaacagcaagcgctggaaccccgagatccagtacacctccaactactacaaatctacaagtgtggactttgctgttaatacagaaggcgtgtactctgaaccccgccccattggcacccgttacctcacccgtaatctgtaattgcttgttaatcaataaac

SEQ ID NO: 135 - DNA, 7663 bp, synthetic construct
  misc_feature 1..7663: note = AAV2/8
  source 1..7663: mol_type = other DNA
atcgttaacgccccgcgccggccgctctagaactagtggatcccccggaagatcagaagttcctattccgaagttcctattctctagaaagtataggaacttctgatctgcgcagccgccatgccggggttttacgagattgtgattaaggtccccagcgaccttgacgagcatctgcccggcatttctgacagctttgtgaactgggtggccgagaaggaatgggagttgccgccagattctgacatggatctgaatctgattgagcaggcacccctgaccgtggccgagaagctgcagcgcgactttctgacggaatggcgccgtgtgagtaaggccccggaggcccttttctttgtgcaatttgagaagggagagagctacttccacatgcacgtgctcgtggaaaccaccggggtgaaatccatggttttgggacgtttcctgagtcagattcgcgaaaaactgattcagagaatttaccgcgggatcgagccgactttgccaaactggttcgcggtcacaaagaccagaaatggcgccggaggcgggaacaaggtggtggatgagtgctacatccccaattacttgctccccaaaacccagcctgagctccagtgggcgtggactaatatggaacagtatttaagcgcctgtttgaatctcacggagcgtaaacggttggtggcgcagcatctgacgcacgtgtcgcagacgcaggagcagaacaaagagaatcagaatcccaattctgatgcgccggtgatcagatcaaaaacttcagccaggtacatggagctggtcgggtggctcgtggacaaggggattacctcggagaagcagtggatccaggaggaccaggcctcatacatctccttcaatgcggcctccaactcgcggtcccaaatcaaggctgccttggacaatgcgggaaagattatgagcctgactaaaaccgcccccgactacctggtgggccagcagcccgtggaggacatttccagcaatcggatttataaaattttggaactaaacgggtacgatccccaatatgcggcttccgtctttctgggatgggccacgaaaaagttcggcaagaggaacaccatctggctgtttgggcctgcaactaccgggaagaccaacatcgcggaggccatagcccacactgtgcccttctacgggtgcgtaaactggaccaatgagaactttcccttcaacgactgtgtcgacaagatggtgatctggtgggaggaggggaagatgaccgccaaggtcgtggagtcggccaaagccattctcggaggaagcaaggtgcgcgtggaccagaaatgcaagtcctcggcccagatagacccgactcccgtgatcgtcacctccaacaccaacatgtgcgccgtgattgacgggaactcaacgaccttcgaacaccagcagccgttgcaagaccggatgttcaaatttgaactcacccgccgtctggatcatgactttgggaaggtcaccaagcaggaagtcaaagactttttccggtgggcaaaggatcacgtggttgaggtggagcatgaattctacgtcaaaaagggtggagccaagaaaagacccgcccccagtgacgcagatataagtgagcccaaacgggtgcgcgagtcagttgcgcagccatcgacgtcagacgcggaagcttcgatcaactacgcagacaggtaccaaaacaaatgttctcgtcacgtgggcatgaatctgatgctgtttccctgcagacaatgcgagagaatgaatcagaattcaaatatctgcttcactcacggacagaaagactgtttagagtgctttcccgtgtcagaatctcaacccgtttctgtcgtcaaaaaggcgtatcagaaactgtgctacattcatcatatcatgggaaaggtgccagacgcttgcactgcctgcgatctggtcaatgtggatttggatgactgcatctttgaacaataaatgatttaaatcaggtatggctgccgatggttatcttccagattggctcgaggacaacctctctgagggcattcgcgagtggtgggcgctgaaacctggagccccgaagcccaaagccaaccagcaaaagcaggacgacggccggggtctggtgcttcctggctacaagtacctcggacccttcaacggactcgacaagggggagcccgtcaacgcggcggacgcagcggccctcgagcacgacaaggcctacgaccagcagctgcaggcgggtgacaatccgtacctgcggtataaccacgccgacgccgagtttcaggagcgtctgcaagaagatacgtcttttgggggcaacctcgggcgagcagtcttccaggccaagaagcgggttctcgaacctctcggtctggttgaggaaggcgctaagacggctcctggaaagaagagaccggtagagccatcaccccagcgttctccagactcctctacgggcatcggcaagaaaggccaacagcccgccagaaaaagactcaattttggtcagactggcgactcagagtcagttccagaccctcaacctctcggagaacctccagcagcgccctctggtgtgggacctaatacaatggctgcaggcggtggcgcaccaatggcagacaataacgaaggcgccgacggagtgggtagttcctcgggaaattggcattgcgattccacatggctgggcgacagagtcatcaccaccagcacccgaacctgggccctgcccacctacaacaaccacctctacaagcaaatctccaacgggacatcgggaggagccaccaacgacaacacctacttcggctacagcaccccctgggggtattttgactttaacagattccactgccacttttcaccacgtgactggcagcgactcatcaacaacaactggggattccggcccaagagactcagcttcaagctcttcaacatccaggtcaaggaggtcacgcagaatgaaggcaccaagaccatcgccaataacctcaccagcaccatccaggtgtttacggactcggagtaccagctgccgtacgttctcggctctgcccaccagggctgcctgcctccgttcccggcggacgtgttcatgattccccagtacggctacctaacactcaacaacggtagtcaggccgtgggacgctcctccttctactgcctggaatactttccttcgcagatgctgagaaccggcaacaacttccagtttacttacaccttcgaggacgtgcctttccacagcagctacgcccacagccagagcttggaccggctgatgaatcctctgattgaccagtacctgtactacttgtctcggactcaaacaacaggaggcacggcaaatacgcagactctgggcttcagccaaggtgggcctaatacaatggccaatcaggcaaagaactggctgccaggaccctgttaccgccaacaacgcgtctcaacgacaaccgggcaaaacaacaatagcaactttgcctggactgctgggaccaaataccatctgaatggaagaaattcattggctaatcctggcatcgctatggcaacacacaaagacgacgaggagcgtttttttcccagtaacgggatcctgatttttggcaaacaaaatgctgccagagacaatgcggattacagcgatgtcatgctcaccagcgaggaagaaatcaaaaccactaaccctgtggctacagaggaatacggtatcgtggcagataacttgcagcagcaaaacacggctcctcaaattggaactgtcaacagccagggggccttacccggtatggtctggcagaaccgggacgtgtacctgcagggtcccatctgggccaagattcctcacacggacggcaacttccacccgtctccgctgatgggcggctttggcctgaaacatcctccgcctcagatcctgatcaagaacacgcctgtacctgcggatcctccgaccaccttcaaccagtcaaagctgaactctttcatcacgcaatacagcaccggacaggtcagcgtggaaattgaatgggagctgcagaaggaaaacagcaagcgctggaaccccgagatccagtacacctccaactactacaaatctacaagtgtggactttgctgttaatacagaaggcgtgtactctgaaccccgccccattggcacccgttacctcacccgtaatctgtaattgcttgttaatcaataaaccgtttaattcgtttcagttgaactttggtctctgcgtatttctttcttatctagtttccatggctacgtagataagtagcatggcgggttaatcattaactacagcccgggcgtttaaacagcgggcggaggggtggagtcgtgacgtgaattacgtcatagggttagggaggtcctgtattagaggtcacgtgagtgttttgcgacattttgcgacaccatgtggtctcgctgggggggggggcccgagtgagcacgcagggtctccattttgaagcgggaggtttgaacgagcgctggcgcgctcactggccgtcgttttacaacgtcgtgactgggaaaaccctggcgttacccaacttaatcgccttgcagcacatccccctttcgccagctggcgtaatagcgaagaggcccgcaccgatcgcccttcccaacagttgcgcagcctgaatggcgaatggaaattgtaagcgttaatattttgttaaaattcgcgttaaatttttgttaaatcagctcatttttttaaccaataggccgaaatcggcaaaatcccttataaatcaaaagaatagaccgagatagggttgagtgttgttccagtttggaacaagagtccactattaagaacgtggactccaacgtcaaagggcgaaaaaccgtctatcagggcgatggcccactacgtgaaccatcaccctaatcaagttttttggggtcgaggtgccgtaaagcactaaatcggaaccctaaagggagcccccgatttagagcttgacggggaaagccggcgaacgtggcgagaaaggaagggaagaaagcgaaaggagcgggcgctagggcgctggcaagtgtagcggtcacgctgcgcgtaaccaccacacccgccgcgcttaatgcgccgctacagggcgcgtcaggtggcacttttcggggaaatgtgcgcggaacccctatttgtttatttttctaaatacattcaaatatgtatccgctcatgagacaataaccctgataaatgcttcaataatattgaaaaaggaagagtcctgaggcggaaagaaccagctgtggaatgtgtgtcagttagggtgtggaaagtccccaggctccccagcaggcagaagtatgcaaagcatgcatctcaattagtcagcaaccaggtgtggaaagtccccaggctccccagcaggcagaagtatgcaaagcatgcatctcaattagtcagcaaccatagtcccgcccctaactccgcccatcccgcccctaactccgcccagttccgcccattctccgccccatggctgactaattttttttatttatgcagaggccgaggccgcctcggcctctgagctattccagaagtagtgaggaggcttttttggaggcctaggcttttgcaaagatcgatcaagagacaggatgaggatcgtttcgcatgattgaacaagatggattgcacgcaggttctccggccgcttgggtggagaggctattcggctatgactgggcacaacagacaatcggctgctctgatgccgccgtgttccggctgtcagcgcaggggcgcccggttctttttgtcaagaccgacctgtccggtgccctgaatgaactgcaagacgaggcagcgcggctatcgtggctggccacgacgggcgttccttgcgcagctgtgctcgacgttgtcactgaagcgggaagggactggctgctattgggcgaagtgccggggcaggatctcctgtcatctcaccttgctcctgccgagaaagtatccatcatggctgatgcaatgcggcggctgcatacgcttgatccggctacctgcccattcgaccaccaagcgaaacatcgcatcgagcgagcacgtactcggatggaagccggtcttgtcgatcaggatgatctggacgaagagcatcaggggctcgcgccagccgaactgttcgccaggctcaaggcgagcatgcccgacggcgaggatctcgtcgtgacccatggcgatgcctgcttgccgaatatcatggtggaaaatggccgcttttctggattcatcgactgtggccggctgggtgtggcggaccgctatcaggacatagcgttggctacccgtgatattgctgaagagcttggcggcgaatgggctgaccgcttcctcgtgctttacggtatcgccgctcccgattcgcagcgcatcgccttctatcgccttcttgacgagttcttctgactgtcagaccaagtttactcatatatactttagattgatttaaaacttcatttttaatttaaaaggatctaggtgaagatcctttttgataatctcatgaccaaaatcccttaacgtgagttttcgttccactgagcgtcagaccccgtagaaaagatcaaaggatcttcttgagatcctttttttctgcgcgtaatctgctgcttgcaaacaaaaaaaccaccgctaccagcggtggtttgtttgccggatcaagagctaccaactctttttccgaaggtaactggcttcagcagagcgcagataccaaatactgttcttctagtgtagccgtagttaggccaccacttcaagaactctgtagcaccgcctacatacctcgctctgctaatcctgttaccagtggctgctgccagtggcgataagtcgtgtcttaccgggttggactcaagacgatagttaccggataaggcgcagcggtcgggctgaacggggggttcgtgcacacagcccagcttggagcgaacgacctacaccgaactgagatacctacagcgtgagctatgagaaagcgccacgcttcccgaagggagaaaggcggacaggtatccggtaagcggcagggtcggaacaggagagcgcacgagggagcttccagggggaaacgcctggtatctttatagtcctgtcgggtttcgccacctctgacttgagcgtcgatttttgtgatgctcgtcaggggggcggagcctatggaaaaacgccagcaacgcggcctttttacggttcctggccttttgctggccttttgctcacatgttctttcctgcgttatcccctgattctgtggataaccgtattaccgcctttgagtgagctgataccgctcgccgcagccgaacgaccgagcgcagcgagtcagtgagcgaggaagcggaagagcgcccaatacgcaaaccgcctctccccgcgcgttggccgattcattaatgcagctggcacgacaggtttcccgactggaaagcgggcagtgagcgcaacgcaattaatgtgagttagctcactcattaggcaccccaggctttacactttatgcttccggctcgtatgttgtgtggaattgtgagcggataacaatttcacacaggaaacagctatgaccatgattacgccaagcgcgccgat

SEQ ID NO: 136 - DNA, 11635 bp, synthetic construct
  misc_feature 1..11635: note = AAV-helper-Amp
  source 1..11635: mol_type = other DNA
ggtacccaactccatgcttaacagtccccaggtacagcccaccctgcgtcgcaaccaggaacagctctacagcttcctggagcgccactcgccctacttccgcagccacagtgcgcagattaggagcgccacttctttttgtcacttgaaaaacatgtaaaaataatgtactaggagacactttcaataaaggcaaatgtttttatttgtacactctcgggtgattatttaccccccacccttgccgtctgcgccgtttaaaaatcaaaggggttctgccgcgcatcgctatgcgccactggcagggacacgttgcgatactggtgtttagtgctccacttaaactcaggcacaaccatccgcggcagctcggtgaagttttcactccacaggctgcgcaccatcaccaacgcgtttagcaggtcgggcgccgatatcttgaagtcgcagttggggcctccgccctgcgcgcgcgagttgcgatacacagggttgcagcactggaacactatcagcgccgggtggtgcacgctggccagcacgctcttgtcggagatcagatccgcgtccaggtcctccgcgttgctcagggcgaacggagtcaactttggtagctgccttcccaaaaagggtgcatgcccaggctttgagttgcactcgcaccgtagtggcatcagaaggtgaccgtgcccggtctgggcgttaggatacagcgcctgcatgaaagccttgatctgcttaaaagccacctgagcctttgcgccttcagagaagaacatgccgcaagacttgccggaaaactgattggccggacaggccgcgtcatgcacgcagcaccttgcgtcggtgttggagatctgcaccacatttcggccccaccggttcttcacgatcttggccttgctagactgctccttcagcgcgcgctgcccgttttcgctcgtcacatccatttcaatcacgtgctccttatttatcataatgctcccgtgtagacacttaagctcgccttcgatctcagcgcagcggtgcagccacaacgcgcagcccgtgggctcgtggtgcttgtaggttacctctgcaaacgactgcaggtacgcctgcaggaatcgccccatcatcgtcacaaaggtcttgttgctggtgaaggtcagctgcaacccgcggtgctcctcgtttagccaggtcttgcatacggccgccagagcttccacttggtcaggcagtagcttgaagtttgcctttagatcgttatccacgtggtacttgtccatcaacgcgcgcgcagcctccatgcccttctcccacgcagacacgatcggcaggctcagcgggtttatcaccgtgctttcactttccgcttcactggactcttccttttcctcttgcgtccgcataccccgcgccactgggtcgtcttcattcagccgccgcaccgtgcgcttacctcccttgccgtgcttgattagcaccggtgggttgctgaaacccaccatttgtagcgccacatcttctctttcttcctcgctgtccacgatcacctctggggatggcgggcgctcgggcttgggagaggggcgcttctttttctttttggacgcaatggccaaatccgccgtcgaggtcgatggccgcgggctgggtgtgcgcggcaccagcgcatcttgtgacgagtcttcttcgtcctcggactcgagacgccgcctcagccgcttttttgggggcgcgcggggaggcggcggcgacggcgacggggacgacacgtcctccatggttggtggacgtcgcgccgcaccgcgtccgcgctcgggggtggtttcgcgctgctcctcttcccgactggccatttccttctcctataggcagaaaaagatcatggagtcagtcgagaaggaggacagcctaaccgccccctttgagttcgccaccaccgcctccaccgatgccgccaacgcgcctaccaccttccccgtcgaggcacccccgcttgaggaggaggaagtgattatcgagcaggacccaggttttgtaagcgaagacgacgaggatcgctcagtaccaacagaggataaaaagcaagaccaggacgacgcagaggcaaacgaggaacaagtcgggcggggggaccaaaggcatggcgactacctagatgtgggagacgacgtgctgttgaagcatctgcagcgccagtgcgccattatctgcgacgcgttgcaagagcgcagcgatgtgcccctcgccatagcggatgtcagccttgcctacgaacgccacctgttctcaccgcgcgtaccccccaaacgccaagaaaacggcacatgcgagcccaacccgcgcctcaacttctaccccgtatttgccgtgccagaggtgcttgccacctatcacatctttttccaaaactgcaagatacccctatcctgccgtgccaaccgcagccgagcggacaagcagctggccttgcggcagggcgctgtcatacctgatatcgcctcgctcgacgaagtgccaaaaatctttgagggtcttggacgcgacgagaaacgcgcggcaaacgctctgcaacaagaaaacagcgaaaatgaaagtcactgtggagtgctggtggaacttgagggtgacaacgcgcgcctagccgtgctgaaacgcagcatcgaggtcacccactttgcctacccggcacttaacctaccccccaaggttatgagcacagtcatgagcgagctgatcgtgcgccgtgcacgacccctggagagggatgcaaacttgcaagaacaaaccgaggagggcctacccgcagttggcgatgagcagctggcgcgctggcttgagacgcgcgagcctgccgacttggaggagcgacgcaagctaatgatggccgcagtgcttgttaccgtggagcttgagtgcatgcagcggttctttgctgacccggagatgcagcgcaagctagaggaaacgttgcactacacctttcgccagggctacgtgcgccaggcctgcaaaatttccaacgtggagctctgcaacctggtctcctaccttggaattttgcacgaaaaccgcctcgggcaaaacgtgcttcattccacgctcaagggcgaggcgcgccgcgactacgtccgcgactgcgtttacttatttctgtgctacacctggcaaacggccatgggcgtgtggcagcaatgcctggaggagcgcaacctaaaggagctgcagaagctgctaaagcaaaacttgaaggacctatggacggccttcaacgagcgctccgtggccgcgcacctggcggacattatcttccccgaacgcctgcttaaaaccctgcaacagggtctgccagacttcaccagtcaaagcatgttgcaaaactttaggaactttatcctagagcgttcaggaattctgcccgccacctgctgtgcgcttcctagcgactttgtgcccattaagtaccgtgaatgccctccgccgctttggggtcactgctaccttctgcagctagccaactaccttgcctaccactccgacatcatggaagacgtgagcggtgacggcctactggagtgtcactgtcgctgcaacctatgcaccccgcaccgctccctggtctgcaattcgcaactgcttagcgaaagtcaaattatcggtacctttgagctgcagggtccctcgcctgacgaaaagtccgcggctccggggttgaaactcactccggggctgtggacgtcggcttaccttcgcaaatttgtacctgaggactaccacgcccacgagattaggttctacgaagaccaatcccgcccgccaaatgcggagcttaccgcctgcgtcattacccagggccacatccttggccaattgcaagccatcaacaaagcccgccaagagtttctgctacgaaagggacggggggtttacctggacccccagtccggcgaggagctcaacccaatccccccgccgccgcagccctatcagcagccgcgggcccttgcttcccaggatggcacccaaaaagaagctgcagctgccgccgccgccacccacggacgaggaggaatactgggacagtcaggcagaggaggttttggacgaggaggaggagatgatggaagactgggacagcctagacgaagcttccgaggccgaagaggtgtcagacgaaacaccgtcaccctcggtcgcattcccctcgccggcgccccagaaattggcaaccgttcccagcatcgctacaacctccgctcctcaggcgccgccggcactgcctgttcgccgacccaaccgtagatgggacaccactggaaccagggccggtaagtctaagcagccgccgccgttagcccaagagcaacaacagcgccaaggctaccgctcgtggcgcgggcacaagaacgccatagttgcttgcttgcaagactgtgggggcaacatctccttcgcccgccgctttcttctctaccatcacggcgtggccttcccccgtaacatcctgcattactaccgtcatctctacagcccctactgcaccggcggcagcggcagcggcagcaacagcagcggtcacacagaagcaaaggcgaccggatagcaagactctgacaaagcccaagaaatccacagcggcggcagcagcaggaggaggagcgctgcgtctggcgcccaacgaacccgtatcgacccgcgagcttagaaataggatttttcccactctgtatgctatatttcaacaaagcaggggccaagaacaagagctgaaaataaaaaacaggtctctgcgctccctcacccgcagctgcctgtatcacaaaagcgaagatcagcttcggcgcacgctggaagacgcggaggctctcttcagcaaatactgcgcgctgactcttaaggactagtttcgcgccctttctcaaatttaagcgcgaaaactacgtcatctccagcggccacacccggcgccagcacctgtcgtcagcgccattatgagcaaggaaattcccacgccctacatgtggagttaccagccacaaatgggacttgcggctggagctgcccaagactactcaacccgaataaactacatgagcgcgggaccccacatgatatcccgggtcaacggaatccgcgcccaccgaaaccgaattctcctcgaacaggcggctattaccaccacacctcgtaataaccttaatccccgtagttggcccgctgccctggtgtaccaggaaagtcccgctcccaccactgtggtacttcccagagacgcccaggccgaagttcagatgactaactcaggggcgcagcttgcgggcggctttcgtcacagggtgcggtcgcccgggcgttttagggcggagtaacttgcatgtattgggaattgtagtttttttaaaatgggaagtgacgtatcgtgggaaaacggaagtgaagatttgaggaagttgtgggttttttggctttcgtttctgggcgtaggttcgcgtgcggttttctgggtgttttttgtggactttaaccgttacgtcattttttagtcctatatatactcgctctgtacttggccctttttacactgtgactgattgagctggtgccgtgtcgagtggtgttttttaataggtttttttactggtaaggctgactgttatggctgccgctgtggaagcgctgtatgttgttctggagcgggagggtgctattttgcctaggcaggagggtttttcaggtgtttatgtgtttttctctcctattaattttgttatacctcctatgggggctgtaatgttgtctctacgcctgcgggtatgtattcccccgggctatttcggtcgctttttagcactgaccgatgttaaccaacctgatgtgtttaccgagtcttacattatgactccggacatgaccgaggaactgtcggtggtgctttttaatcacggtgaccagtttttttacggtcacgccggcatggccgtagtccgtcttatgcttataagggttgtttttcctgttgtaagacaggcttctaatgtttaaatgtttttttttttgttattttattttgtgtttaatgcaggaacccgcagacatgtttgagagaaaaatggtgtctttttctgtggtggttccggaacttacctgcctttatctgcatgagcatgactacgatgtgcttgcttttttgcgcgaggctttgcctgattttttgagcagcaccttgcattttatatcgccgcccatgcaacaagcttacataggggctacgctggttagcatagctccgagtatgcgtgtcataatcagtgtgggttcttttgtcatggttcctggcggggaagtggccgcgctggtccgtgcagacctgcacgattatgttcagctggccctgcgaagggacctacgggatcgcggtatttttgttaatgttccgcttttgaatcttatacaggtctgtgaggaacctgaatttttgcaatcatgattcgctgcttgaggctgaaggtggagggcgctctggagcagatttttacaatggccggacttaatattcgggatttgcttagagacatattgataaggtggcgagatgaaaattatttgggcatggttgaaggtgctggaatgtttatagaggagattcaccctgaagggtttagcctttacgtccacttggacgtgagggcagtttgccttttggaagccattgtgcaacatcttacaaatgccattatctgttctttggctgtagagtttgaccacgccaccggaggggagcgcgttcacttaatagatcttcattttgaggttttggataatcttttggaataaaaaaaaaaaaacatggttcttccagctcttcccgctcctcccgtgtgtgactcgcagaacgaatgtgtaggttggctgggtgtggcttattctgcggtggtggatgttatcagggcagcggcgcatgaaggagtttacatagaacccgaagccagggggcgcctggatgctttgagagagtggatatactacaactactacacagagcgagctaagcgacgagaccggagacgcagatctgtttgtcacgcccgcacctggttttgcttcaggaaatatgactacgtccggcgttccatttggcatgacactacgaccaacacgatctcggttgtctcggcgcactccgtacagtagggatcgcctacctccttttgagacagagacccgcgctaccatactggaggatcatccgctgctgcccgaatgtaacactttgacaatgcacaacgtgagttacgtgcgaggtcttccctgcagtgtgggatttacgctgattcaggaatgggttgttccctgggatatggttctgacgcgggaggagcttgtaatcctgaggaagtgtatgcacgtgtgcctgtgttgtgccaacattgatatcatgacgagcatgatgatccatggttacgagtcctgggctctccactgtcattgttccagtcccggttccctgcagtgcatagccggcgggcaggttttggccagctggtttaggatggtggtggatggcgccatgtttaatcagaggtttatatggtaccgggaggtggtgaattacaacatgccaaaagaggtaatgtttatgtccagcgtgtttatgaggggtcgccacttaatctacctgcgcttgtggtatgatggccacgtgggttctgtggtccccgccatgagctttggatacagcgccttgcactgtgggattttgaacaatattgtggtgctgtgctgcagttactgtgctgatttaagtgagatcagggtgcgctgctgtgcccggaggacaaggcgtctcatgctgcgggcggtgcgaatcatcgctgaggagaccactgccatgttgtattcctgcaggacggagcggcggcggcagcagtttattcgcgcgctgctgcagcaccaccgccctatcctgatgcacgattatgactctacccccatgtaggcgtggacttccccttcgccgcccgttgagcaaccgcaagttggacagcagcctgtggctcagcagctggacagcgacatgaacttaagcgagctgcccggggagtttattaatatcactgatgagcgtttggctcgacaggaaaccgtgtggaatataacacctaagaatatgtctgttacccatgatatgatgctttttaaggccagccggggagaaaggactgtgtactctgtgtgttgggagggaggtggcaggttgaatactagggttctgtgagtttgattaaggtacggtgatcaatataagctatgtggtggtggggctatactactgaatgaaaaatgacttgaaattttctgcaattgaaaaataaacacgttgaaacataacatgcaacaggttcacgattctttattcctgggcaatgtaggagaaggtgtaagagttggtagcaaaagtttcagtggtgtattttccactttcccaggaccatgtaaaagacatagagtaagtgcttacctcgctagtttctgtggattcactagaatcgatgtaggatgttgcccctcctgacgcggtaggagaaggggagggtgccctgcatgtctgccgctgctcttgctcttgccgctgctgaggaggggggcgcatctgccgcagcaccggatgcatctgggaaaagcaaaaaaggggctcgtccctgtttccggaggaatttgcaagcggggtcttgcatgacggggaggcaaacccccgttcgccgcagtccggccggcccgagactcgaaccgggggtcctgcgactcaacccttggaaaataaccctccggctacagggagcgagccacttaatgctttcgctttccagcctaaccgcttacgccgcgcgcggccagtggccaaaaaagctagcgcagcagccgccgcgcctggaaggaagccaaaaggagcgctcccccgttgtctgacgtcgcacacctgggttcgacacgcgggcggtaaccgcatggatcacggcggacggccggatccggggttcgaaccccggtcgtccgccatgatacccttgcgaatttatccaccagaccacggaagagtgcccgcttacaggctctccttttgcacggtctagagcgtcaacgactgcgcacgcctcaccggccagagcgtcccgaccatggagcactttttgccgctgcgcaacatctggaaccgcgtccgcgactttccgcgcgcctccaccaccgccgccggcatcacctggatgtccaggtacatctacggattacgtcgacgtttaaaccatatgatcagctcactcaaaggcggtaatacggttatccacagaatcaggggataacgcaggaaagaacatgtgagcaaaaggccagcaaaaggccaggaaccgtaaaaaggccgcgttgctggcgtttttccataggctccgcccccctgacgagcatcacaaaaatcgacgctcaagtcagaggtggcgaaacccgacaggactataaagataccaggcgtttccccctggaagctccctcgtgcgctctcctgttccgaccctgccgcttaccggatacctgtccgcctttctcccttcgggaagcgtggcgctttctcatagctcacgctgtaggtatctcagttcggtgtaggtcgttcgctccaagctgggctgtgtgcacgaaccccccgttcagcccgaccgctgcgccttatccggtaactatcgtcttgagtccaacccggtaagacacgacttatcgccactggcagcagccactggtaacaggattagcagagcgaggtatgtaggcggtgctacagagttcttgaagtggtggcctaactacggctacactagaagaacagtatttggtatctgcgctctgctgaagccagttaccttcggaaaaagagttggtagctcttgatccggcaaacaaaccaccgctggtagcggtggtttttttgtttgcaagcagcagattacgcgcagaaaaaaaggatctcaagaagatcctttgatcttttctacggggtctgacgctcagtggaacgaaaactcacgttaagggattttggtcatgagattatcaaaaaggatcttcacctagatccttttaaattaaaaatgaagttttaaatcaatctaaagtatatatgagtaaacttggtctgacagttaccaatgcttaatcagtgaggcacctatctcagcgatctgtctatttcgttcatccatagttgcctgactccccgtcgtgtagataactacgatacgggagggcttaccatctggccccagtgctgcaatgataccgcgagacccacgctcaccggctccagatttatcagcaataaaccagccagccggaagggccgagcgcagaagtggtcctgcaactttatccgcctccatccagtctattaattgttgccgggaagctagagtaagtagttcgccagttaatagtttgcgcaacgttgttgccattgctacaggcatcgtggtgtcacgctcgtcgtttggtatggcttcattcagctccggttcccaacgatcaaggcgagttacatgatcccccatgttgtgcaaaaaagcggttagctccttcggtcctccgatcgttgtcagaagtaagttggccgcagtgttatcactcatggttatggcagcactgcataattctcttactgtcatgccatccgtaagatgcttttctgtgactggtgagtactcaaccaagtcattctgagaatagtgtatgcggcgaccgagttgctcttgcccggcgtcaatacgggataataccgcgccacatagcagaactttaaaagtgctcatcattggaaaacgttcttcggggcgaaaactctcaaggatcttaccgctgttgagatccagttcgatgtaacccactcgtgcacccaactgatcttcagcatcttttactttcaccagcgtttctgggtgagcaaaaacaggaaggcaaaatgccgcaaaaaagggaataagggcgacacggaaatgttgaatactcatactcttcctttttcaatattattgaagcatttatcagggttattgtctcatgagcggatacatatttgaatgtatttagaaaaataaacaaataggggttccgcgcacatttccccgaaaagtgccacctaaattgtaagcgttaatattttgttaaaattcgcgttaaatttttgttaaatcagctcattttttaaccaataggccgaaatcggcaaaatcccttataaatcaaaagaatagaccgagatagggttgagtgttgttccagtttggaacaagagtccactattaaagaacgtggactccaacgtcaaagggcgaaaaaccgtctatcagggcgatggcccactacgtgaaccatcaccctaatcaagttttttggggtcgaggtgccgtaaagcactaaatcggaaccctaaagggagcccccgatttagagcttgacggggaaagccggcgaacgtggcgagaaaggaagggaagaaagcgaaaggagcgggcgctagggcgctggcaagtgtagcggtcacgctgcgcgtaaccaccacacccgccgcgcttaatgcgccgctacagggcgcgatggatcc

SEQ ID NO: 137 - DNA, 11962 bp, synthetic construct
  misc_feature 1..11962: note = AAV-helper
  source 1..11962: mol_type = other DNA
ggtacccaactccatgcttaacagtccccaggtacagcccaccctgcgtcgcaaccaggaacagctctacagcttcctggagcgccactcgccctacttccgcagccacagtgcgcagattaggagcgccacttctttttgtcacttgaaaaacatgtaaaaataatgtactaggagacactttcaataaaggcaaatgtttttatttgtacactctcgggtgattatttaccccccacccttgccgtctgcgccgtttaaaaatcaaaggggttctgccgcgcatcgctatgcgccactggcagggacacgttgcgatactggtgtttagtgctccacttaaactcaggcacaaccatccgcggcagctcggtgaagttttcactccacaggctgcgcaccatcaccaacgcgtttagcaggtcgggcgccgatatcttgaagtcgcagttggggcctccgccctgcgcgcgcgagttgcgatacacagggttgcagcactggaacactatcagcgccgggtggtgcacgctggccagcacgctcttgtcggagatcagatccgcgtccaggtcctccgcgttgctcagggcgaacggagtcaactttggtagctgccttcccaaaaagggtgcatgcccaggctttgagttgcactcgcaccgtagtggcatcagaaggtgaccgtgcccggtctgggcgttaggatacagcgcctgcatgaaagccttgatctgcttaaaagccacctgagcctttgcgccttcagagaagaacatgccgcaagacttgccggaaaactgattggccggacaggccgcgtcatgcacgcagcaccttgcgtcggtgttggagatctgcaccacatttcggccccaccggttcttcacgatcttggccttgctagactgctccttcagcgcgcgctgcccgttttcgctcgtcacatccatttcaatcacgtgctccttatttatcataatgctcccgtgtagacacttaagctcgccttcgatctcagcgcagcggtgcagccacaacgcgcagcccgtgggctcgtggtgcttgtaggttacctctgcaaacgactgcaggtacgcctgcaggaatcgccccatcatcgtcacaaaggtcttgttgctggtgaaggtcagctgcaacccgcggtgctcctcgtttagccaggtcttgcatacggccgccagagcttccacttggtcaggcagtagcttgaagtttgcctttagatcgttatccacgtggtacttgtccatcaacgcgcgcgcagcctccatgcccttctcccacgcagacacgatcggcaggctcagcgggtttatcaccgtgctttcactttccgcttcactggactcttccttttcctcttgcgtccgcataccccgcgccactgggtcgtcttcattcagccgccgcaccgtgcgcttacctcccttgccgtgcttgattagcaccggtgggttgctgaaacccaccatttgtagcgccacatcttctctttcttcctcgctgtccacgatcacctctggggatggcgggcgctcgggcttgggagaggggcgcttctttttctttttggacgcaatggccaaatccgccgtcgaggtcgatggccgcgggctgggtgtgcgcggcaccagcgcatcttgtgacgagtcttcttcgtcctcggactcgagacgccgcctcagccgcttttttgggggcgcgcggggaggcggcggcgacggcgacggggacgacacgtcctccatggttggtggacgtcgcgccgcaccgcgtccgcgctcgggggtggtttcgcgctgctcctcttcccgactggccatttccttctcctataggcagaaaaagatcatggagtcagtcgagaaggaggacagcctaaccgccccctttgagttcgccaccaccgcctccaccgatgccgccaacgcgcctaccaccttccccgtcgaggcacccccgcttgaggaggaggaagtgattatcgagcaggacccaggttttgtaagcgaagacgacgaggatcgctcagtaccaacagaggataaaaagcaagaccaggacgacgcagaggcaaacgaggaacaagtcgggcggggggaccaaaggcatggcgactacctagatgtgggagacgacgtgctgttgaagcatctgcagcgccagtgcgccattatctgcgacgcgttgcaagagcgcagcgatgtgcccctcgccatagcggatgtcagccttgcctacgaacgccacctgttctcaccgcgcgtaccccccaaacgccaagaaaacggcacatgcgagcccaacccgcgcctcaacttctaccccgtatttgccgtgccagaggtgcttgccacctatcacatctttttccaaaactgcaagatacccctatcctgccgtgccaaccgcagccgagcggacaagcagctggccttgcggcagggcgctgtcatacctgatatcgcctcgctcgacgaagtgccaaaaatctttgagggtcttggacgcgacgagaaacgcgcggcaaacgctctgcaacaagaaaacagcgaaaatgaaagtcactgtggagtgctggtggaacttgagggtgacaacgcgcgcctagccgtgctgaaacgcagcatcgaggtcacccactttgcctacccggcacttaacctaccccccaaggttatgagcacagtcatgagcgagctgatcgtgcgccgtgcacgacccctggagagggatgcaaacttgcaagaacaaaccgaggagggcctacccgcagttggcgatgagcagctggcgcgctggcttgagacgcgcgagcctgccgacttggaggagcgacgcaagctaatgatggccgcagtgcttgttaccgtggagcttgagtgcatgcagcggttctttgctgacccggagatgcagcgcaagctagaggaaacgttgcactacacctttcgccagggctacgtgcgccaggcctgcaaaatttccaacgtggagctctgcaacctggtctcctaccttggaattttgcacgaaaaccgcctcgggcaaaacgtgcttcattccacgctcaagggcgaggcgcgccgcgactacgtccgcgactgcgtttacttatttctgtgctacacctggcaaacggccatgggcgtgtggcagcaatgcctggaggagcgcaacctaaaggagctgcagaagctgctaaagcaaaacttgaaggacctatggacggccttcaacgagcgctccgtggccgcgcacctggcggacattatcttccccgaacgcctgcttaaaaccctgcaacagggtctgccagacttcaccagtcaaagcatgttgcaaaactttaggaactttatcctagagcgttcaggaattctgcccgccacctgctgtgcgcttcctagcgactttgtgcccattaagtaccgtgaatgccctccgccgctttggggtcactgctaccttctgcagctagccaactaccttgcctaccactccgacatcatggaagacgtgagcggtgacggcctactggagtgtcactgtcgctgcaacctatgcaccccgcaccgctccctggtctgcaattcgcaactgcttagcgaaagtcaaattatcggtacctttgagctgcagggtccctcgcctgacgaaaagtccgcggctccggggttgaaactcactccggggctgtggacgtcggcttaccttcgcaaatttgtacctgaggactaccacgcccacgagattaggttctacgaagaccaatcccgcccgccaaatgcggagcttaccgcctgcgtcattacccagggccacatccttggccaattgcaagccatcaacaaagcccgccaagagtttctgctacgaaagggacggggggtttacctggacccccagtccggcgaggagctcaacccaatccccccgccgccgcagccctatcagcagccgcgggcccttgcttcccaggatggcacccaaaaagaagctgcagctgccgccgccgccacccacggacgaggaggaatactgggacagtcaggcagaggaggttttggacgaggaggaggagatgatggaagactgggacagcctagacgaagcttccgaggccgaagaggtgtcagacgaaacaccgtcaccctcggtcgcattcccctcgccggcgccccagaaattggcaaccgttcccagcatcgctacaacctccgctcctcaggcgccgccggcactgcctgttcgccgacccaaccgtagatgggacaccactggaaccagggccggtaagtctaagcagccgccgccgttagcccaagagcaacaacagcgccaaggctaccgctcgtggcgcgggcacaagaacgccatagttgcttgcttgcaagactgtgggggcaacatctccttcgcccgccgctttcttctctaccatcacggcgtggccttcccccgtaacatcctgcattactaccgtcatctctacagcccctactgcaccggcggcagcggcagcggcagcaacagcagcggtcacacagaagcaaaggcgaccggatagcaagactctgacaaagcccaagaaatccacagcggcggcagcagcaggaggaggagcgctgcgtctggcgcccaacgaacccgtatcgacccgcgagcttagaaataggatttttcccactctgtatgctatatttcaacaaagcaggggccaagaacaagagctgaaaataaaaaacaggtctctgcgctccctcacccgcagctgcctgtatcacaaaagcgaagatcagcttcggcgcacgctggaagacgcggaggctctcttcagcaaatactgcgcgctgactcttaaggactagtttcgcgccctttctcaaatttaagcgcgaaaactacgtcatctccagcggccacacccggcgccagcacctgtcgtcagcgccattatgagcaaggaaattcccacgccctacatgtggagttaccagccacaaatgggacttgcggctggagctgcccaagactactcaacccgaataaactacatgagcgcgggaccccacatgatatcccgggtcaacggaatccgcgcccaccgaaaccgaattctcctcgaacaggcggctattaccaccacacctcgtaataaccttaatccccgtagttggcccgctgccctggtgtaccaggaaagtcccgctcccaccactgtggtacttcccagagacgcccaggccgaagttcagatgactaactcaggggcgcagcttgcgggcggctttcgtcacagggtgcggtcgcccgggcgttttagggcggagtaacttgcatgtattgggaattgtagtttttttaaaatgggaagtgacgtatcgtgggaaaacggaagtgaagatttgaggaagttgtgggttttttggctttcgtttctgggcgtaggttcgcgtgcggttttctgggtgttttttgtggactttaaccgttacgtcattttttagtcctatatatactcgctctgtacttggccctttttacactgtgactgattgagctggtgccgtgtcgagtggtgttttttaataggtttttttactggtaaggctgactgttatggctgccgctgtggaagcgctgtatgttgttctggagcgggagggtgctattttgcctaggcaggagggtttttcaggtgtttatgtgtttttctctcctattaattttgttatacctcctatgggggctgtaatgttgtctctacgcctgcgggtatgtattcccccgggctatttcggtcgctttttagcactgaccgatgttaaccaacctgatgtgtttaccgagtcttacattatgactccggacatgaccgaggaactgtcggtggtgctttttaatcacggtgaccagtttttttacggtcacgccggcatggccgtagtccgtcttatgcttataagggttgtttttcctgttgtaagacaggcttctaatgtttaaatgtttttttttttgttattttattttgtgtttaatgcaggaacccgcagacatgtttgagagaaaaatggtgtctttttctgtggtggttccggaacttacctgcctttatctgcatgagcatgactacgatgtgcttgcttttttgcgcgaggctttgcctgattttttgagcagcaccttgcattttatatcgccgcccatgcaacaagcttacataggggctacgctggttagcatagctccgagtatgcgtgtcataatcagtgtgggttcttttgtcatggttcctggcggggaagtggccgcgctggtccgtgcagacctgcacgattatgttcagctggccctgcgaagggacctacgggatcgcggtatttttgttaatgttccgcttttgaatcttatacaggtctgtgaggaacctgaatttttgcaatcatgattcgctgcttgaggctgaaggtggagggcgctctggagcagatttttacaatggccggacttaatattcgggatttgcttagagacatattgataaggtggcgagatgaaaattatttgggcatggttgaaggtgctggaatgtttatagaggagattcaccctgaagggtttagcctttacgtccacttggacgtgagggcagtttgccttttggaagccattgtgcaacatcttacaaatgccattatctgttctttggctgtagagtttgaccacgccaccggaggggagcgcgttcacttaatagatcttcattttgaggttttggataatcttttggaataaaaaaaaaaaaacatggttcttccagctcttcccgctcctcccgtgtgtgactcgcagaacgaatgtgtaggttggctgggtgtggcttattctgcggtggtggatgttatcagggcagcggcgcatgaaggagtttacatagaacccgaagccagggggcgcctggatgctttgagagagtggatatactacaactactacacagagcgagctaagcgacgagaccggagacgcagatctgtttgtcacgcccgcacctggttttgcttcaggaaatatgactacgtccggcgttccatttggcatgacactacgaccaacacgatctcggttgtctcggcgcactccgtacagtagggatcgcctacctccttttgagacagagacccgcgctaccatactggaggatcatccgctgctgcccgaatgtaacactttgacaatgcacaacgtgagttacgtgcgaggtcttccctgcagtgtgggatttacgctgattcaggaatgggttgttccctgggatatggttctgacgcgggaggagcttgtaatcctgaggaagtgtatgcacgtgtgcctgtgttgtgccaacattgatatcatgacgagcatgatgatccatggttacgagtcctgggctctccactgtcattgttccagtcccggttccctgcagtgcatagccggcgggcaggttttggccagctggtttaggatggtggtggatggcgccatgtttaatcagaggtttatatggtaccgggaggtggtgaattacaacatgccaaaagaggtaatgtttatgtccagcgtgtttatgaggggtcgccacttaatctacctgcgcttgtggtatgatggccacgtgggttctgtggtccccgccatgagctttggatacagcgccttgcactgtgggattttgaacaatattgtggtgctgtgctgcagttactgtgctgatttaagtgagatcagggtgcgctgctgtgcccggaggacaaggcgtctcatgctgcgggcggtgcgaatcatcgctgaggagaccactgccatgttgtattcctgcaggacggagcggcggcggcagcagtttattcgcgcgctgctgcagcaccaccgccctatcctgatgcacgattatgactctacccccatgtaggcgtggacttccccttcgccgcccgttgagcaaccgcaagttggacagcagcctgtggctcagcagctggacagcgacatgaacttaagcgagctgcccggggagtttattaatatcactgatgagcgtttggctcgacaggaaaccgtgtggaatataacacctaagaatatgtctgttacccatgatatgatgctttttaaggccagccggggagaaaggactgtgtactctgtgtgttgggagggaggtggcaggttgaatactagggttctgtgagtttgattaaggtacggtgatcaatataagctatgtggtggtggggctatactactgaatgaaaaatgacttgaaattttctgcaattgaaaaataaacacgttgaaacataacatgcaacaggttcacgattctttattcctgggcaatgtaggagaaggtgtaagagttggtagcaaaagtttcagtggtgtattttccactttcccaggaccatgtaaaagacatagagtaagtgcttacctcgctagtttctgtggattcactagaatcgatgtaggatgttgcccctcctgacgcggtaggagaaggggagggtgccctgcatgtctgccgctgctcttgctcttgccgctgctgaggaggggggcgcatctgccgcagcaccggatgcatctgggaaaagcaaaaaaggggctcgtccctgtttccggaggaatttgcaagcggggtcttgcatgacggggaggcaaacccccgttcgccgcagtccggccggcccgagactcgaaccgggggtcctgcgactcaacccttggaaaataaccctccggctacagggagcgagccacttaatgctttcgctttccagcctaaccgcttacgccgcgcgcggccagtggccaaaaaagctagcgcagcagccgccgcgcctggaaggaagccaaaaggagcgctcccccgttgtctgacgtcgcacacctgggttcgacacgcgggcggtaaccgcatggatcacggcggacggccggatccggggttcgaaccccggtcgtccgccatgatacccttgcgaatttatccaccagaccacggaagagtgcccgcttacaggctctccttttgcacggtctagagcgtcaacgactgcgcacgcctcaccggccagagcgtcccgaccatggagcactttttgccgctgcgcaacatctggaaccgcgtccgcgactttccgcgcgcctccaccaccgccgccggcatcacctggatgtccaggtacatctacggattacgtcgacgtttaaaccatatgatcagctcactcaaaggcggtaatacggttatccacagaatcaggggataacgcaggaaagaacatgtgagcaaaaggccagcaaaaggccaggaaccgtaaaaaggccgcgttgctggcgtttttccataggctccgcccccctgacgagcatcacaaaaatcgacgctcaagtcagaggtggcgaaacccgacaggactataaagataccaggcgtttccccctggaagctccctcgtgcgctctcctgttccgaccctgccgcttaccggatacctgtccgcctttctcccttcgggaagcgtggcgctttctcatagctcacgctgtaggtatctcagttcggtgtaggtcgttcgctccaagctgggctgtgtgcacgaaccccccgttcagcccgaccgctgcgccttatccggtaactatcgtcttgagtccaacccggtaagacacgacttatcgccactggcagcagccactggtaacaggattagcagagcgaggtatgtaggcggtgctacagagttcttgaagtggtggcctaactacggctacactagaagaacagtatttggtatctgcgctctgctgaagccagttaccttcggaaaaagagttggtagctcttgatccggcaaacaaaccaccgctggtagcggtggtttttttgtttgcaagcagcagattacgcgcagaaaaaaaggatctcaagaagatcctttgatcttttctacggggtctgacgctcagtggaacgaaaactcacgttaagggattttggtcatgagattatcaaaaaggatcttcacctagatccttttaaattaaaaatgaagttttaaatcaatctaaagtatatatgagtaaacttggtctgacagtcagaagaactcgtcaagaaggcgatagaaggcgatgcgctgcgaatcgggagcggcgataccgtaaagcacgaggaagcggtcagcccattcgccgccaagctcttcagcaatatcacgggtagccaacgctatgtcctgatagcggtccgccacacccagccggccacagtcgatgaatccagaaaagcggccattttccaccatgatattcggcaagcaggcatcgccatgggtcacgacgagatcctcgccgtcgggcatgctcgccttgagcctggcgaacagttcggctggcgcgagcccctgatgctcttcgtccagatcatcctgatcgacaagaccggcttccatccgagtacgtgctcgctcgatgcgatgtttcgcttggtggtcgaatgggcaggtagccggatcaagcgtatgcagccgccgcattgcatcagccatgatggatactttctcggcaggagcaaggtgagatgacaggagatcctgccccggcacttcgcccaatagcagccagtcccttcccgcttcagtgacaacgtcgagcacagctgcgcaaggaacgcccgtcgtggccagccacgatagccgcgctgcctcgtcttgcagttcattcagggcaccggacaggtcggtcttgacaaaaagaaccgggcgcccctgcgctgacagccggaacacggcggcatcagagcagccgattgtctgttgtgcccagtcatagccgaatagcctctccacccaagcggccggagaacctgcgtgcaatccatcttgttcaatcatgcgaaacgatcctcatcctgtctcttgatcgatctttgcaaaagcctaggcctccaaaaaagcctcctcactacttctggaatagctcagaggccgaggcggcctcggcctctgcataaataaaaaaaattagtcagccatggggcggagaatgggcggaactgggcggagttaggggcgggatgggcggagttaggggcgggactatggttgctgactaattgagatgcatgctttgcatacttctgcctgctggggagcctggggactttccacacctggttgctgactaattgagatgcatgctttgcatacttctgcctgctggggagcctggggactttccacaccctaactgacacacattccacagctggttctttccgcctcaggactcttcctttttcaatattattgaagcatttatcagggttattgtctcatgagcggatacatatttgaatgtatttagaaaaataaacaaataggggttccgcgcacatttccccgaaaagtgccacctaaattgtaagcgttaatattttgttaaaattcgcgttaaatttttgttaaatcagctcattttttaaccaataggccgaaatcggcaaaatcccttataaatcaaaagaatagaccgagatagggttgagtgttgttccagtttggaacaagagtccactattaaagaacgtggactccaacgtcaaagggcgaaaaaccgtctatcagggcgatggcccactacgtgaaccatcaccctaatcaagttttttggggtcgaggtgccgtaaagcactaaatcggaaccctaaagggagcccccgatttagagcttgacggggaaagccggcgaacgtggcgagaaaggaagggaagaaagcgaaaggagcgggcgctagggcgctggcaagtgtagcggtcacgctgcgcgtaaccaccacacccgccgcgcttaatgcgccgctacagggcgcgatggatcc

SEQ ID NO: 138 - DNA, 22 bp, synthetic construct
  misc_feature 1..22: note = human ACTB RT-F
  source 1..22: mol_type = other DNA
caccattggcaatgagcggttc

SEQ ID NO: 139 - DNA, 22 bp, synthetic construct
  misc_feature 1..22: note = human ACTB RT-R
  source 1..22: mol_type = other DNA
aggtctttgcggatgtccacgt

SEQ ID NO: 140 - DNA, 22 bp, synthetic construct
  misc_feature 1..22: note = human TNF-a RT-F
  source 1..22: mol_type = other DNA
ctcttctgcctgctgcactttg

SEQ ID NO: 141 - DNA, 22 bp, synthetic construct
  misc_feature 1..22: note = human TNF-a RT-R
  source 1..22: mol_type = other DNA
atgggctacaggcttgtcactc

SEQ ID NO: 142 - DNA, 23 bp, synthetic construct
  misc_feature 1..23: note = human IFN-gamma RT-F
  source 1..23: mol_type = other DNA
gagtgtggagaccatcaaggaag

SEQ ID NO: 143 - DNA, 24 bp, synthetic construct
  misc_feature 1..24: note = human IFN-gamma RT-R
  source 1..24: mol_type = other DNA
tgctttgcgttggacattcaagtc

SEQ ID NO: 144 - DNA, 22 bp, synthetic construct
  misc_feature 1..22: note = human NLRP3 RT-F
  source 1..22: mol_type = other DNA
ggactgaagcacctgttgtgca

SEQ ID NO: 145 - DNA, 22 bp, synthetic construct
  misc_feature 1..22: note = human NLRP3 RT-R
  source 1..22: mol_type = other DNA
tcctgagtctcccaaggcattc

SEQ ID NO: 146 - DNA, 23 bp, synthetic construct
  misc_feature 1..23: note = mouse ACTB RT-F
  source 1..23: mol_type = other DNA
cattgctgacaggatgcagaagg

SEQ ID NO: 147 - DNA, 22 bp, synthetic construct
  misc_feature 1..22: note = mouse ACTB RT-R
  source 1..22: mol_type = other DNA
tgctggaaggtggacagtgagg

SEQ ID NO: 148 - DNA, 22 bp, synthetic construct
  misc_feature 1..22: note = mouse TNF-a RT-F
  source 1..22: mol_type = other DNA
ggtgcctatgtctcagcctctt

SEQ ID NO: 149 - DNA, 23 bp, synthetic construct
  misc_feature 1..23: note = mouse TNF-a RT-R
  source 1..23: mol_type = other DNA
gccatagaactgatgagagggag

SEQ ID NO: 150 - DNA, 23 bp, synthetic construct
  misc_feature 1..23: note = mouse IFN-gamma RT-F
  source 1..23: mol_type = other DNA
cagcaacagcaaggcgaaaaagg

SEQ ID NO: 151 - DNA, 22 bp, synthetic construct
  misc_feature 1..22: note = mouse IFN-gamma RT-R
  source 1..22: mol_type = other DNA
tttccgcttcctgaggctggat

SEQ ID NO: 152 - DNA, 22 bp, synthetic construct
  misc_feature 1..22: note = mouse NLRP3 RT-F
  source 1..22: mol_type = other DNA
tcacaactcgcccaaggaggaa

SEQ ID NO: 153 - DNA, 22 bp, synthetic construct
  misc_feature 1..22: note = mouse NLRP3 RT-R
  source 1..22: mol_type = other DNA
aagagaccacggcagaagctag

SEQ ID NO: 154 - DNA, 21 bp, synthetic construct
  misc_feature 1..21: note = ITR-F
  source 1..21: mol_type = other DNA
ggaacccctagtgatggagtt

SEQ ID NO: 155 - DNA, 16 bp, synthetic construct
  misc_feature 1..16: note = ITR-R
  source 1..16: mol_type = other DNA
cggcctcagtgagcga